European Patent Application EP 4 768 581 A1, published July 1, 2026. Title: Stable target editing guide RNA with phosphate modification. Applicant: FUKUOKA UNIVERSITY. Application JP. The sequence listing filed with the application follows.

SEQUENCE LISTING (132 sequences)

SEQ ID NO: 1 - RNA, 24 nt, synthetic construct
  source 1..24: mol_type = other RNA
aaagcatgccatcacctcccctgt

SEQ ID NO: 2 - RNA, 25 nt, Homo sapiens
  source 1..25: mol_type = mRNA
acaggggaggtgatagcattgcttt

SEQ ID NO: 3 - DNA, 41 bp, synthetic construct
  source 1..41: mol_type = other DNA
ctaatacgactcactatagggcctcttcgctattacgccag

SEQ ID NO: 4 - DNA, 24 bp, synthetic construct
  source 1..24: mol_type = other DNA
ggaaacagctatgaccatgattac

SEQ ID NO: 5 - DNA, 21 bp, synthetic construct
  source 1..21: mol_type = other DNA
ctaatacgactcactataggg

SEQ ID NO: 6 - DNA, 27 bp, synthetic construct
  source 1..27: mol_type = other DNA
cagcagatgtggatcagcaagcaggag

SEQ ID NO: 7 - DNA, 25 bp, synthetic construct
  source 1..25: mol_type = other DNA
ggaagggggggcacgaaggctcatc

SEQ ID NO: 8 - DNA, 26 bp, synthetic construct
  source 1..26: mol_type = other DNA
ggtgacagcagtcggttggagcgagc

SEQ ID NO: 9 - DNA, 57 bp, synthetic construct
  source 1..57: mol_type = other DNA
aattcgcataaggctgtgctgaccatcgacaagaaagggactgaagctgctggggca

SEQ ID NO: 10 - DNA, 57 bp, synthetic construct
  source 1..57: mol_type = other DNA
agcttgccccagcagcttcagtccctttcttgtcgatggtcagcacagccttatgcg

SEQ ID NO: 11 - DNA, 41 bp, synthetic construct
  source 1..41: mol_type = other DNA
ctaatacgactcactataggtatgacaatgaatacggctac

SEQ ID NO: 12 - DNA, 22 bp, synthetic construct
  source 1..22: mol_type = other DNA
ggtattcaagagagtagggagg

SEQ ID NO: 13 - DNA, 20 bp, synthetic construct
  source 1..20: mol_type = other DNA
tgttcctacccccaatgtgt

SEQ ID NO: 14 - DNA, 20 bp, synthetic construct
  source 1..20: mol_type = other DNA
gcagcgaactttattgatgg

SEQ ID NO: 15 - RNA, 24 nt, synthetic construct
  source 1..24: mol_type = other RNA
  modified_base 1: mod_base = OTHER; note = 2'-O-methyladenosine
  modified_base 2: mod_base = OTHER; note = 2'-O,4'-C-methylene-briged adenosine
  modified_base 3: mod_base = OTHER; note = 2'-O-methyladenosine
  modified_base 4: mod_base = OTHER; note = 2'-O,4'-C-methylene-briged guanosine
  modified_base 5: mod_base = cm
  modified_base 6: mod_base = OTHER; note = 2'-deoxy-2'-fluoroadenosine
  modified_base 7: mod_base = OTHER; note = 2'-deoxy-2'-fluorouridine
  modified_base 8: mod_base = gm
  modified_base 9: mod_base = cm
  modified_base 10: mod_base = OTHER; note = 2'-deoxycytidine
  modified_base 11: mod_base = OTHER; note = 2'-deoxyadenosine
  modified_base 12: mod_base = um
  modified_base 13: mod_base = OTHER; note = 2'-deoxy-2'-fluorocytidine
  modified_base 14: mod_base = OTHER; note = 2'-O-methyladenosine
  modified_base 15: mod_base = OTHER; note = 2'-deoxy-2'-fluorocytidine
  modified_base 16: mod_base = cm
  modified_base 17: mod_base = OTHER; note = 2'-deoxy-2'-fluorouridine
  modified_base 18: mod_base = cm
  modified_base 19: mod_base = OTHER; note = 2'-deoxy-2'-fluorocytidine
  modified_base 20: mod_base = cm
  modified_base 21: mod_base = OTHER; note = 2'-O,4'-C-methylene-briged cytidine
  modified_base 22: mod_base = um
  modified_base 23: mod_base = OTHER; note = 2'-O,4'-C-methylene-briged guanosine
  modified_base 24: mod_base = um
  modified_base 1^2: mod_base = OTHER; note = phosphorotioate bond between nucleosides
  modified_base 2^3: mod_base = OTHER; note = phosphorothioate bond between nucleosides
  modified_base 3^4: mod_base = OTHER; note = phosphorothioate bond between nucleosides
  modified_base 4^5: mod_base = OTHER; note = phosphorothioate bond between nucleosides
  modified_base 5^6: mod_base = OTHER; note = phosphorothioate bond between nucleosides
  modified_base 7^8: mod_base = OTHER; note = phosphorothioate bond between nucleosides
  modified_base 6^7: mod_base = OTHER; note = phosphorothioate bond between nucleosides
  modified_base 8^9: mod_base = OTHER; note = phosphorothioate bond between nucleosides
  modified_base 9^10: mod_base = OTHER; note = phosphorothioate bond between nucleosides
  modified_base 10^11: mod_base = OTHER; note = phosphorothioate bond between nucleosides
  modified_base 11^12: mod_base = OTHER; note = methylphosphonate bond between nucleosides
  modified_base 12^13: mod_base = OTHER; note = phosphorothioate bond between nucleosides
  modified_base 13^14: mod_base = OTHER; note = phosphorothioate bond between nucleosides
  modified_base 14^15: mod_base = OTHER; note = methylphosphonate bond between nucleosides
  modified_base 15^16: mod_base = OTHER; note = phosphorothioate bond between nucleosides
  modified_base 16^17: mod_base = OTHER; note = phosphorothioate bond between nucleosides
  modified_base 17^18: mod_base = OTHER; note = phosphorothioate bond between nucleosides
  modified_base 18^19: mod_base = OTHER; note = phosphorothioate bond between nucleosides
  modified_base 19^20: mod_base = OTHER; note = phosphorothioate bond between nucleosides
  modified_base 20^21: mod_base = OTHER; note = phosphorothioate bond between nucleosides
  modified_base 21^22: mod_base = OTHER; note = phosphorothioate bond between nucleosides
  modified_base 22^23: mod_base = OTHER; note = phosphorothioate bond between nucleosides
  modified_base 23^24: mod_base = OTHER; note = phosphorothioate bond between nucleosides
aaagcatgccatcacctcccctgt

SEQ ID NO: 16 - RNA, 24 nt, synthetic construct
  source 1..24: mol_type = other RNA
  modified_base 1: mod_base = OTHER; note = 2'-O-methyladenosine
  modified_base 2: mod_base = OTHER; note = 2'-O,4'-C-methylene-briged adenosine
  modified_base 3: mod_base = OTHER; note = 2'-O-methyladenosine
  modified_base 4: mod_base = OTHER; note = 2'-O,4'-C-methylene-briged guanosine
  modified_base 5: mod_base = cm
  modified_base 6: mod_base = OTHER; note = 2'-deoxy-2'-fluoroadenosine
  modified_base 7: mod_base = OTHER; note = 2'-deoxy-2'-fluorouridine
  modified_base 8: mod_base = gm
  modified_base 9: mod_base = cm
  modified_base 10: mod_base = OTHER; note = 2'-deoxycytidine
  modified_base 11: mod_base = OTHER; note = 2'-deoxyadenosine
  modified_base 12: mod_base = um
  modified_base 13: mod_base = OTHER; note = 2'-deoxy-2'-fluorocytidine
  modified_base 14: mod_base = OTHER; note = 2'-O-methyladenosine
  modified_base 15: mod_base = OTHER; note = 2'-deoxy-2'-fluorocytidine
  modified_base 16: mod_base = cm
  modified_base 17: mod_base = OTHER; note = 2'-deoxy-2'-fluorouridine
  modified_base 18: mod_base = cm
  modified_base 19: mod_base = OTHER; note = 2'-deoxy-2'-fluorocytidine
  modified_base 20: mod_base = cm
  modified_base 21: mod_base = OTHER; note = 2'-O,4'-C-methylene-briged cytidine
  modified_base 22: mod_base = um
  modified_base 23: mod_base = OTHER; note = 2'-O,4'-C-methylene-briged guanosine
  modified_base 24: mod_base = um
  modified_base 1^2: mod_base = OTHER; note = phosphorotioate bond between nucleosides
  modified_base 2^3: mod_base = OTHER; note = phosphorothioate bond between nucleosides
  modified_base 3^4: mod_base = OTHER; note = phosphorothioate bond between nucleosides
  modified_base 4^5: mod_base = OTHER; note = phosphorothioate bond between nucleosides
  modified_base 5^6: mod_base = OTHER; note = phosphorothioate bond between nucleosides
  modified_base 7^8: mod_base = OTHER; note = phosphorothioate bond between nucleosides
  modified_base 6^7: mod_base = OTHER; note = phosphorothioate bond between nucleosides
  modified_base 8^9: mod_base = OTHER; note = phosphorothioate bond between nucleosides
  modified_base 9^10: mod_base = OTHER; note = phosphorothioate bond between nucleosides
  modified_base 10^11: mod_base = OTHER; note = phosphorothioate bond between nucleosides
  modified_base 11^12: mod_base = OTHER; note = methylphosphonate bond between nucleosides
  modified_base 12^13: mod_base = OTHER; note = phosphorothioate bond between nucleosides
  modified_base 13^14: mod_base = OTHER; note = phosphorothioate bond between nucleosides
  modified_base 14^15: mod_base = OTHER; note = phosphorothioate bond between nucleosides
  modified_base 15^16: mod_base = OTHER; note = phosphorothioate bond between nucleosides
  modified_base 16^17: mod_base = OTHER; note = phosphorothioate bond between nucleosides
  modified_base 17^18: mod_base = OTHER; note = phosphorothioate bond between nucleosides
  modified_base 18^19: mod_base = OTHER; note = phosphorothioate bond between nucleosides
  modified_base 19^20: mod_base = OTHER; note = phosphorothioate bond between nucleosides
  modified_base 20^21: mod_base = OTHER; note = phosphorothioate bond between nucleosides
  modified_base 21^22: mod_base = OTHER; note = phosphorothioate bond between nucleosides
  modified_base 22^23: mod_base = OTHER; note = phosphorothioate bond between nucleosides
  modified_base 23^24: mod_base = OTHER; note = phosphorothioate bond between nucleosides
aaagcatgccatcacctcccctgt

SEQ ID NO: 17 - RNA, 24 nt, synthetic construct
  source 1..24: mol_type = other RNA
  modified_base 1: mod_base = OTHER; note = 2'-O-methyladenosine
  modified_base 2: mod_base = OTHER; note = 2'-O,4'-C-methylene-briged adenosine
  modified_base 3: mod_base = OTHER; note = 2'-O-methyladenosine
  modified_base 4: mod_base = OTHER; note = 2'-O,4'-C-methylene-briged guanosine
  modified_base 5: mod_base = cm
  modified_base 6: mod_base = OTHER; note = 2'-deoxy-2'-fluoroadenosine
  modified_base 7: mod_base = OTHER; note = 2'-deoxy-2'-fluorouridine
  modified_base 8: mod_base = gm
  modified_base 9: mod_base = cm
  modified_base 10: mod_base = OTHER; note = 2'-deoxycytidine
  modified_base 11: mod_base = OTHER; note = 2'-deoxyadenosine
  modified_base 12: mod_base = um
  modified_base 13: mod_base = OTHER; note = 2'-deoxy-2'-fluorocytidine
  modified_base 14: mod_base = OTHER; note = 2'-O-methyladenosine
  modified_base 15: mod_base = OTHER; note = 2'-deoxy-2'-fluorocytidine
  modified_base 16: mod_base = cm
  modified_base 17: mod_base = OTHER; note = 2'-deoxy-2'-fluorouridine
  modified_base 18: mod_base = cm
  modified_base 19: mod_base = OTHER; note = 2'-deoxy-2'-fluorocytidine
  modified_base 20: mod_base = cm
  modified_base 21: mod_base = OTHER; note = 2'-O,4'-C-methylene-briged cytidine
  modified_base 22: mod_base = um
  modified_base 23: mod_base = OTHER; note = 2'-O,4'-C-methylene-briged guanosine
  modified_base 24: mod_base = um
  modified_base 1^2: mod_base = OTHER; note = phosphorotioate bond between nucleosides
  modified_base 2^3: mod_base = OTHER; note = phosphorothioate bond between nucleosides
  modified_base 3^4: mod_base = OTHER; note = phosphorothioate bond between nucleosides
  modified_base 4^5: mod_base = OTHER; note = phosphorothioate bond between nucleosides
  modified_base 5^6: mod_base = OTHER; note = phosphorothioate bond between nucleosides
  modified_base 7^8: mod_base = OTHER; note = phosphorothioate bond between nucleosides
  modified_base 6^7: mod_base = OTHER; note = phosphorothioate bond between nucleosides
  modified_base 8^9: mod_base = OTHER; note = phosphorothioate bond between nucleosides
  modified_base 9^10: mod_base = OTHER; note = phosphorothioate bond between nucleosides
  modified_base 10^11: mod_base = OTHER; note = phosphorothioate bond between nucleosides
  modified_base 11^12: mod_base = OTHER; note = phosphorothioate bond between nucleosides
  modified_base 12^13: mod_base = OTHER; note = methylphosphonate bond between nucleosides
  modified_base 13^14: mod_base = OTHER; note = phosphorothioate bond between nucleosides
  modified_base 14^15: mod_base = OTHER; note = methylphosphonate bond between nucleosides
  modified_base 15^16: mod_base = OTHER; note = phosphorothioate bond between nucleosides
  modified_base 16^17: mod_base = OTHER; note = phosphorothioate bond between nucleosides
  modified_base 17^18: mod_base = OTHER; note = phosphorothioate bond between nucleosides
  modified_base 18^19: mod_base = OTHER; note = phosphorothioate bond between nucleosides
  modified_base 19^20: mod_base = OTHER; note = phosphorothioate bond between nucleosides
  modified_base 20^21: mod_base = OTHER; note = phosphorothioate bond between nucleosides
  modified_base 21^22: mod_base = OTHER; note = phosphorothioate bond between nucleosides
  modified_base 22^23: mod_base = OTHER; note = phosphorothioate bond between nucleosides
  modified_base 23^24: mod_base = OTHER; note = phosphorothioate bond between nucleosides
aaagcatgccatcacctcccctgt

SEQ ID NO: 18 - RNA, 24 nt, synthetic construct
  source 1..24: mol_type = other RNA
  modified_base 1: mod_base = OTHER; note = 2'-O-methyladenosine
  modified_base 2: mod_base = OTHER; note = 2'-O,4'-C-methylene-briged adenosine
  modified_base 3: mod_base = OTHER; note = 2'-O-methyladenosine
  modified_base 4: mod_base = OTHER; note = 2'-O,4'-C-methylene-briged guanosine
  modified_base 5: mod_base = cm
  modified_base 6: mod_base = OTHER; note = 2'-deoxy-2'-fluoroadenosine
  modified_base 7: mod_base = OTHER; note = 2'-deoxy-2'-fluorouridine
  modified_base 8: mod_base = gm
  modified_base 9: mod_base = cm
  modified_base 10: mod_base = OTHER; note = 2'-deoxycytidine
  modified_base 11: mod_base = OTHER; note = 2'-deoxyadenosine
  modified_base 12: mod_base = um
  modified_base 13: mod_base = OTHER; note = 2'-deoxy-2'-fluorocytidine
  modified_base 14: mod_base = OTHER; note = 2'-O-methyladenosine
  modified_base 15: mod_base = OTHER; note = 2'-deoxy-2'-fluorocytidine
  modified_base 16: mod_base = cm
  modified_base 17: mod_base = OTHER; note = 2'-deoxy-2'-fluorouridine
  modified_base 18: mod_base = cm
  modified_base 19: mod_base = OTHER; note = 2'-deoxy-2'-fluorocytidine
  modified_base 20: mod_base = cm
  modified_base 21: mod_base = OTHER; note = 2'-O,4'-C-methylene-briged cytidine
  modified_base 22: mod_base = um
  modified_base 23: mod_base = OTHER; note = 2'-O,4'-C-methylene-briged guanosine
  modified_base 24: mod_base = um
  modified_base 1^2: mod_base = OTHER; note = phosphorotioate bond between nucleosides
  modified_base 2^3: mod_base = OTHER; note = phosphorothioate bond between nucleosides
  modified_base 3^4: mod_base = OTHER; note = phosphorothioate bond between nucleosides
  modified_base 4^5: mod_base = OTHER; note = phosphorothioate bond between nucleosides
  modified_base 5^6: mod_base = OTHER; note = phosphorothioate bond between nucleosides
  modified_base 7^8: mod_base = OTHER; note = phosphorothioate bond between nucleosides
  modified_base 6^7: mod_base = OTHER; note = phosphorothioate bond between nucleosides
  modified_base 8^9: mod_base = OTHER; note = phosphorothioate bond between nucleosides
  modified_base 9^10: mod_base = OTHER; note = phosphorothioate bond between nucleosides
  modified_base 10^11: mod_base = OTHER; note = phosphorothioate bond between nucleosides
  modified_base 11^12: mod_base = OTHER; note = phosphorothioate bond between nucleosides
  modified_base 12^13: mod_base = OTHER; note = methylphosphonate bond between nucleosides
  modified_base 13^14: mod_base = OTHER; note = phosphorothioate bond between nucleosides
  modified_base 14^15: mod_base = OTHER; note = methylphosphonate bond between nucleosides
  modified_base 15^16: mod_base = OTHER; note = phosphorothioate bond between nucleosides
  modified_base 16^17: mod_base = OTHER; note = phosphorothioate bond between nucleosides
  modified_base 17^18: mod_base = OTHER; note = phosphorothioate bond between nucleosides
  modified_base 18^19: mod_base = OTHER; note = phosphorothioate bond between nucleosides
  modified_base 19^20: mod_base = OTHER; note = phosphorothioate bond between nucleosides
  modified_base 20^21: mod_base = OTHER; note = phosphorothioate bond between nucleosides
  modified_base 21^22: mod_base = OTHER; note = phosphorothioate bond between nucleosides
  modified_base 22^23: mod_base = OTHER; note = phosphorothioate bond between nucleosides
  modified_base 23^24: mod_base = OTHER; note = phosphorothioate bond between nucleosides
aaagcatgccatcacctcccctgt

SEQ ID NO: 19 - RNA, 24 nt, synthetic construct
  source 1..24: mol_type = other RNA
  modified_base 1: mod_base = OTHER; note = 2'-O-methyladenosine
  modified_base 2: mod_base = OTHER; note = 2'-O,4'-C-methylene-briged adenosine
  modified_base 3: mod_base = OTHER; note = 2'-O-methyladenosine
  modified_base 4: mod_base = OTHER; note = 2'-O,4'-C-methylene-briged guanosine
  modified_base 5: mod_base = cm
  modified_base 6: mod_base = OTHER; note = 2'-deoxy-2'-fluoroadenosine
  modified_base 7: mod_base = OTHER; note = 2'-deoxy-2'-fluorouridine
  modified_base 8: mod_base = gm
  modified_base 9: mod_base = cm
  modified_base 10: mod_base = OTHER; note = 2'-deoxycytidine
  modified_base 11: mod_base = OTHER; note = 2'-deoxyadenosine
  modified_base 12: mod_base = um
  modified_base 13: mod_base = OTHER; note = 2'-deoxy-2'-fluorocytidine
  modified_base 14: mod_base = OTHER; note = 2'-O-methyladenosine
  modified_base 15: mod_base = OTHER; note = 2'-deoxy-2'-fluorocytidine
  modified_base 16: mod_base = cm
  modified_base 17: mod_base = OTHER; note = 2'-deoxy-2'-fluorouridine
  modified_base 18: mod_base = cm
  modified_base 19: mod_base = OTHER; note = 2'-deoxy-2'-fluorocytidine
  modified_base 20: mod_base = cm
  modified_base 21: mod_base = OTHER; note = 2'-O,4'-C-methylene-briged cytidine
  modified_base 22: mod_base = um
  modified_base 23: mod_base = OTHER; note = 2'-O,4'-C-methylene-briged guanosine
  modified_base 24: mod_base = um
  modified_base 1^2: mod_base = OTHER; note = methylphosphonate bond between nucleosides
  modified_base 2^3: mod_base = OTHER; note = phosphorothioate bond between nucleosides
  modified_base 3^4: mod_base = OTHER; note = phosphorothioate bond between nucleosides
  modified_base 4^5: mod_base = OTHER; note = phosphorothioate bond between nucleosides
  modified_base 5^6: mod_base = OTHER; note = phosphorothioate bond between nucleosides
  modified_base 7^8: mod_base = OTHER; note = phosphorothioate bond between nucleosides
  modified_base 6^7: mod_base = OTHER; note = phosphorothioate bond between nucleosides
  modified_base 8^9: mod_base = OTHER; note = phosphorothioate bond between nucleosides
  modified_base 9^10: mod_base = OTHER; note = phosphorothioate bond between nucleosides
  modified_base 10^11: mod_base = OTHER; note = phosphorothioate bond between nucleosides
  modified_base 11^12: mod_base = OTHER; note = phosphorothioate bond between nucleosides
  modified_base 12^13: mod_base = OTHER; note = phosphorothioate bond between nucleosides
  modified_base 13^14: mod_base = OTHER; note = phosphorothioate bond between nucleosides
  modified_base 14^15: mod_base = OTHER; note = phosphorothioate bond between nucleosides
  modified_base 15^16: mod_base = OTHER; note = phosphorothioate bond between nucleosides
  modified_base 16^17: mod_base = OTHER; note = phosphorothioate bond between nucleosides
  modified_base 17^18: mod_base = OTHER; note = phosphorothioate bond between nucleosides
  modified_base 18^19: mod_base = OTHER; note = phosphorothioate bond between nucleosides
  modified_base 19^20: mod_base = OTHER; note = phosphorothioate bond between nucleosides
  modified_base 20^21: mod_base = OTHER; note = phosphorothioate bond between nucleosides
  modified_base 21^22: mod_base = OTHER; note = phosphorothioate bond between nucleosides
  modified_base 22^23: mod_base = OTHER; note = phosphorothioate bond between nucleosides
  modified_base 23^24: mod_base = OTHER; note = phosphorothioate bond between nucleosides
aaagcatgccatcacctcccctgt

SEQ ID NO: 20 - RNA, 24 nt, synthetic construct
  source 1..24: mol_type = other RNA
  modified_base 1: mod_base = OTHER; note = 2'-O-methyladenosine
  modified_base 2: mod_base = OTHER; note = 2'-O,4'-C-methylene-briged adenosine
  modified_base 3: mod_base = OTHER; note = 2'-O-methyladenosine
  modified_base 4: mod_base = OTHER; note = 2'-O,4'-C-methylene-briged guanosine
  modified_base 5: mod_base = cm
  modified_base 6: mod_base = OTHER; note = 2'-deoxy-2'-fluoroadenosine
  modified_base 7: mod_base = OTHER; note = 2'-deoxy-2'-fluorouridine
  modified_base 8: mod_base = gm
  modified_base 9: mod_base = cm
  modified_base 10: mod_base = OTHER; note = 2'-deoxycytidine
  modified_base 11: mod_base = OTHER; note = 2'-deoxyadenosine
  modified_base 12: mod_base = um
  modified_base 13: mod_base = OTHER; note = 2'-deoxy-2'-fluorocytidine
  modified_base 14: mod_base = OTHER; note = 2'-O-methyladenosine
  modified_base 15: mod_base = OTHER; note = 2'-deoxy-2'-fluorocytidine
  modified_base 16: mod_base = cm
  modified_base 17: mod_base = OTHER; note = 2'-deoxy-2'-fluorouridine
  modified_base 18: mod_base = cm
  modified_base 19: mod_base = OTHER; note = 2'-deoxy-2'-fluorocytidine
  modified_base 20: mod_base = cm
  modified_base 21: mod_base = OTHER; note = 2'-O,4'-C-methylene-briged cytidine
  modified_base 22: mod_base = um
  modified_base 23: mod_base = OTHER; note = 2'-O,4'-C-methylene-briged guanosine
  modified_base 24: mod_base = um
  modified_base 1^2: mod_base = OTHER; note = phosphorotioate bond between nucleosides
  modified_base 2^3: mod_base = OTHER; note = phosphorothioate bond between nucleosides
  modified_base 3^4: mod_base = OTHER; note = methylphosphonate bond between nucleosides
  modified_base 4^5: mod_base = OTHER; note = phosphorothioate bond between nucleosides
  modified_base 5^6: mod_base = OTHER; note = phosphorothioate bond between nucleosides
  modified_base 7^8: mod_base = OTHER; note = phosphorothioate bond between nucleosides
  modified_base 6^7: mod_base = OTHER; note = phosphorothioate bond between nucleosides
  modified_base 8^9: mod_base = OTHER; note = phosphorothioate bond between nucleosides
  modified_base 9^10: mod_base = OTHER; note = phosphorothioate bond between nucleosides
  modified_base 10^11: mod_base = OTHER; note = phosphorothioate bond between nucleosides
  modified_base 11^12: mod_base = OTHER; note = phosphorothioate bond between nucleosides
  modified_base 12^13: mod_base = OTHER; note = phosphorothioate bond between nucleosides
  modified_base 13^14: mod_base = OTHER; note = phosphorothioate bond between nucleosides
  modified_base 14^15: mod_base = OTHER; note = phosphorothioate bond between nucleosides
  modified_base 15^16: mod_base = OTHER; note = phosphorothioate bond between nucleosides
  modified_base 16^17: mod_base = OTHER; note = phosphorothioate bond between nucleosides
  modified_base 17^18: mod_base = OTHER; note = phosphorothioate bond between nucleosides
  modified_base 18^19: mod_base = OTHER; note = phosphorothioate bond between nucleosides
  modified_base 19^20: mod_base = OTHER; note = phosphorothioate bond between nucleosides
  modified_base 20^21: mod_base = OTHER; note = phosphorothioate bond between nucleosides
  modified_base 21^22: mod_base = OTHER; note = phosphorothioate bond between nucleosides
  modified_base 22^23: mod_base = OTHER; note = phosphorothioate bond between nucleosides
  modified_base 23^24: mod_base = OTHER; note = phosphorothioate bond between nucleosides
aaagcatgccatcacctcccctgt

SEQ ID NO: 21 - RNA, 24 nt, synthetic construct
  source 1..24: mol_type = other RNA
  modified_base 1: mod_base = OTHER; note = 2'-O-methyladenosine
  modified_base 2: mod_base = OTHER; note = 2'-O,4'-C-methylene-briged adenosine
  modified_base 3: mod_base = OTHER; note = 2'-O-methyladenosine
  modified_base 4: mod_base = OTHER; note = 2'-O,4'-C-methylene-briged guanosine
  modified_base 5: mod_base = cm
  modified_base 6: mod_base = OTHER; note = 2'-deoxy-2'-fluoroadenosine
  modified_base 7: mod_base = OTHER; note = 2'-deoxy-2'-fluorouridine
  modified_base 8: mod_base = gm
  modified_base 9: mod_base = cm
  modified_base 10: mod_base = OTHER; note = 2'-deoxycytidine
  modified_base 11: mod_base = OTHER; note = 2'-deoxyadenosine
  modified_base 12: mod_base = um
  modified_base 13: mod_base = OTHER; note = 2'-deoxy-2'-fluorocytidine
  modified_base 14: mod_base = OTHER; note = 2'-O-methyladenosine
  modified_base 15: mod_base = OTHER; note = 2'-deoxy-2'-fluorocytidine
  modified_base 16: mod_base = cm
  modified_base 17: mod_base = OTHER; note = 2'-deoxy-2'-fluorouridine
  modified_base 18: mod_base = cm
  modified_base 19: mod_base = OTHER; note = 2'-deoxy-2'-fluorocytidine
  modified_base 20: mod_base = cm
  modified_base 21: mod_base = OTHER; note = 2'-O,4'-C-methylene-briged cytidine
  modified_base 22: mod_base = um
  modified_base 23: mod_base = OTHER; note = 2'-O,4'-C-methylene-briged guanosine
  modified_base 24: mod_base = um
  modified_base 1^2: mod_base = OTHER; note = phosphorotioate bond between nucleosides
  modified_base 2^3: mod_base = OTHER; note = phosphorothioate bond between nucleosides
  modified_base 3^4: mod_base = OTHER; note = phosphorothioate bond between nucleosides
  modified_base 4^5: mod_base = OTHER; note = phosphorothioate bond between nucleosides
  modified_base 5^6: mod_base = OTHER; note = methylphosphonate bond between nucleosides
  modified_base 7^8: mod_base = OTHER; note = phosphorothioate bond between nucleosides
  modified_base 6^7: mod_base = OTHER; note = phosphorothioate bond between nucleosides
  modified_base 8^9: mod_base = OTHER; note = phosphorothioate bond between nucleosides
  modified_base 9^10: mod_base = OTHER; note = phosphorothioate bond between nucleosides
  modified_base 10^11: mod_base = OTHER; note = phosphorothioate bond between nucleosides
  modified_base 11^12: mod_base = OTHER; note = phosphorothioate bond between nucleosides
  modified_base 12^13: mod_base = OTHER; note = phosphorothioate bond between nucleosides
  modified_base 13^14: mod_base = OTHER; note = phosphorothioate bond between nucleosides
  modified_base 14^15: mod_base = OTHER; note = phosphorothioate bond between nucleosides
  modified_base 15^16: mod_base = OTHER; note = phosphorothioate bond between nucleosides
  modified_base 16^17: mod_base = OTHER; note = phosphorothioate bond between nucleosides
  modified_base 17^18: mod_base = OTHER; note = phosphorothioate bond between nucleosides
  modified_base 18^19: mod_base = OTHER; note = phosphorothioate bond between nucleosides
  modified_base 19^20: mod_base = OTHER; note = phosphorothioate bond between nucleosides
  modified_base 20^21: mod_base = OTHER; note = phosphorothioate bond between nucleosides
  modified_base 21^22: mod_base = OTHER; note = phosphorothioate bond between nucleosides
  modified_base 22^23: mod_base = OTHER; note = phosphorothioate bond between nucleosides
  modified_base 23^24: mod_base = OTHER; note = phosphorothioate bond between nucleosides
aaagcatgccatcacctcccctgt

SEQ ID NO: 22 - RNA, 24 nt, synthetic construct
  source 1..24: mol_type = other RNA
  modified_base 1: mod_base = OTHER; note = 2'-O-methyladenosine
  modified_base 2: mod_base = OTHER; note = 2'-O,4'-C-methylene-briged adenosine
  modified_base 3: mod_base = OTHER; note = 2'-O-methyladenosine
  modified_base 4: mod_base = OTHER; note = 2'-O,4'-C-methylene-briged guanosine
  modified_base 5: mod_base = cm
  modified_base 6: mod_base = OTHER; note = 2'-deoxy-2'-fluoroadenosine
  modified_base 7: mod_base = OTHER; note = 2'-deoxy-2'-fluorouridine
  modified_base 8: mod_base = gm
  modified_base 9: mod_base = cm
  modified_base 10: mod_base = OTHER; note = 2'-deoxycytidine
  modified_base 11: mod_base = OTHER; note = 2'-deoxyadenosine
  modified_base 12: mod_base = um
  modified_base 13: mod_base = OTHER; note = 2'-deoxy-2'-fluorocytidine
  modified_base 14: mod_base = OTHER; note = 2'-O-methyladenosine
  modified_base 15: mod_base = OTHER; note = 2'-deoxy-2'-fluorocytidine
  modified_base 16: mod_base = cm
  modified_base 17: mod_base = OTHER; note = 2'-deoxy-2'-fluorouridine
  modified_base 18: mod_base = cm
  modified_base 19: mod_base = OTHER; note = 2'-deoxy-2'-fluorocytidine
  modified_base 20: mod_base = cm
  modified_base 21: mod_base = OTHER; note = 2'-O,4'-C-methylene-briged cytidine
  modified_base 22: mod_base = um
  modified_base 23: mod_base = OTHER; note = 2'-O,4'-C-methylene-briged guanosine
  modified_base 24: mod_base = um
  modified_base 1^2: mod_base = OTHER; note = phosphorotioate bond between nucleosides
  modified_base 2^3: mod_base = OTHER; note = phosphorothioate bond between nucleosides
  modified_base 3^4: mod_base = OTHER; note = phosphorothioate bond between nucleosides
  modified_base 4^5: mod_base = OTHER; note = phosphorothioate bond between nucleosides
  modified_base 7^8: mod_base = OTHER; note = phosphorothioate bond between nucleosides
  modified_base 6^7: mod_base = OTHER; note = phosphorothioate bond between nucleosides
  modified_base 8^9: mod_base = OTHER; note = phosphorothioate bond between nucleosides
  modified_base 9^10: mod_base = OTHER; note = methylphosphonate bond between nucleosides
  modified_base 10^11: mod_base = OTHER; note = phosphorothioate bond between nucleosides
  modified_base 11^12: mod_base = OTHER; note = phosphorothioate bond between nucleosides
  modified_base 12^13: mod_base = OTHER; note = phosphorothioate bond between nucleosides
  modified_base 13^14: mod_base = OTHER; note = phosphorothioate bond between nucleosides
  modified_base 14^15: mod_base = OTHER; note = phosphorothioate bond between nucleosides
  modified_base 15^16: mod_base = OTHER; note = phosphorothioate bond between nucleosides
  modified_base 16^17: mod_base = OTHER; note = phosphorothioate bond between nucleosides
  modified_base 17^18: mod_base = OTHER; note = phosphorothioate bond between nucleosides
  modified_base 18^19: mod_base = OTHER; note = phosphorothioate bond between nucleosides
  modified_base 19^20: mod_base = OTHER; note = phosphorothioate bond between nucleosides
  modified_base 20^21: mod_base = OTHER; note = phosphorothioate bond between nucleosides
  modified_base 21^22: mod_base = OTHER; note = phosphorothioate bond between nucleosides
  modified_base 22^23: mod_base = OTHER; note = phosphorothioate bond between nucleosides
  modified_base 23^24: mod_base = OTHER; note = phosphorothioate bond between nucleosides
aaagcatgccatcacctcccctgt

SEQ ID NO: 23 - RNA, 24 nt, synthetic construct
  source 1..24: mol_type = other RNA
  modified_base 1: mod_base = OTHER; note = 2'-O-methyladenosine
  modified_base 2: mod_base = OTHER; note = 2'-O,4'-C-methylene-briged adenosine
  modified_base 3: mod_base = OTHER; note = 2'-O-methyladenosine
  modified_base 4: mod_base = OTHER; note = 2'-O,4'-C-methylene-briged guanosine
  modified_base 5: mod_base = cm
  modified_base 6: mod_base = OTHER; note = 2'-deoxy-2'-fluoroadenosine
  modified_base 7: mod_base = OTHER; note = 2'-deoxy-2'-fluorouridine
  modified_base 8: mod_base = gm
  modified_base 9: mod_base = cm
  modified_base 10: mod_base = OTHER; note = 2'-deoxycytidine
  modified_base 11: mod_base = OTHER; note = 2'-deoxyadenosine
  modified_base 12: mod_base = um
  modified_base 13: mod_base = OTHER; note = 2'-deoxy-2'-fluorocytidine
  modified_base 14: mod_base = OTHER; note = 2'-O-methyladenosine
  modified_base 15: mod_base = OTHER; note = 2'-deoxy-2'-fluorocytidine
  modified_base 16: mod_base = cm
  modified_base 17: mod_base = OTHER; note = 2'-deoxy-2'-fluorouridine
  modified_base 18: mod_base = cm
  modified_base 19: mod_base = OTHER; note = 2'-deoxy-2'-fluorocytidine
  modified_base 20: mod_base = cm
  modified_base 21: mod_base = OTHER; note = 2'-O,4'-C-methylene-briged cytidine
  modified_base 22: mod_base = um
  modified_base 23: mod_base = OTHER; note = 2'-O,4'-C-methylene-briged guanosine
  modified_base 24: mod_base = um
  modified_base 1^2: mod_base = OTHER; note = phosphorotioate bond between nucleosides
  modified_base 2^3: mod_base = OTHER; note = phosphorothioate bond between nucleosides
  modified_base 3^4: mod_base = OTHER; note = phosphorothioate bond between nucleosides
  modified_base 4^5: mod_base = OTHER; note = phosphorothioate bond between nucleosides
  modified_base 5^6: mod_base = OTHER; note = phosphorothioate bond between nucleosides
  modified_base 7^8: mod_base = OTHER; note = phosphorothioate bond between nucleosides
  modified_base 6^7: mod_base = OTHER; note = phosphorothioate bond between nucleosides
  modified_base 8^9: mod_base = OTHER; note = phosphorothioate bond between nucleosides
  modified_base 9^10: mod_base = OTHER; note = phosphorothioate bond between nucleosides
  modified_base 10^11: mod_base = OTHER; note = phosphorothioate bond between nucleosides
  modified_base 11^12: mod_base = OTHER; note = phosphorothioate bond between nucleosides
  modified_base 12^13: mod_base = OTHER; note = phosphorothioate bond between nucleosides
  modified_base 13^14: mod_base = OTHER; note = phosphorothioate bond between nucleosides
  modified_base 14^15: mod_base = OTHER; note = phosphorothioate bond between nucleosides
  modified_base 15^16: mod_base = OTHER; note = phosphorothioate bond between nucleosides
  modified_base 16^17: mod_base = OTHER; note = methylphosphonate bond between nucleosides
  modified_base 17^18: mod_base = OTHER; note = phosphorothioate bond between nucleosides
  modified_base 18^19: mod_base = OTHER; note = phosphorothioate bond between nucleosides
  modified_base 19^20: mod_base = OTHER; note = phosphorothioate bond between nucleosides
  modified_base 20^21: mod_base = OTHER; note = phosphorothioate bond between nucleosides
  modified_base 21^22: mod_base = OTHER; note = phosphorothioate bond between nucleosides
  modified_base 22^23: mod_base = OTHER; note = phosphorothioate bond between nucleosides
  modified_base 23^24: mod_base = OTHER; note = phosphorothioate bond between nucleosides
aaagcatgccatcacctcccctgt

SEQ ID NO: 24 - RNA, 24 nt, synthetic construct
  source 1..24: mol_type = other RNA
  modified_base 1: mod_base = OTHER; note = 2'-O-methyladenosine
  modified_base 2: mod_base = OTHER; note = 2'-O,4'-C-methylene-briged adenosine
  modified_base 3: mod_base = OTHER; note = 2'-O-methyladenosine
  modified_base 4: mod_base = OTHER; note = 2'-O,4'-C-methylene-briged guanosine
  modified_base 5: mod_base = cm
  modified_base 6: mod_base = OTHER; note = 2'-deoxy-2'-fluoroadenosine
  modified_base 7: mod_base = OTHER; note = 2'-deoxy-2'-fluorouridine
  modified_base 8: mod_base = gm
  modified_base 9: mod_base = cm
  modified_base 10: mod_base = OTHER; note = 2'-deoxycytidine
  modified_base 11: mod_base = OTHER; note = 2'-deoxyadenosine
  modified_base 12: mod_base = um
  modified_base 13: mod_base = OTHER; note = 2'-deoxy-2'-fluorocytidine
  modified_base 14: mod_base = OTHER; note = 2'-O-methyladenosine
  modified_base 15: mod_base = OTHER; note = 2'-deoxy-2'-fluorocytidine
  modified_base 16: mod_base = cm
  modified_base 17: mod_base = OTHER; note = 2'-deoxy-2'-fluorouridine
  modified_base 18: mod_base = cm
  modified_base 19: mod_base = OTHER; note = 2'-deoxy-2'-fluorocytidine
  modified_base 20: mod_base = cm
  modified_base 21: mod_base = OTHER; note = 2'-O,4'-C-methylene-briged cytidine
  modified_base 22: mod_base = um
  modified_base 23: mod_base = OTHER; note = 2'-O,4'-C-methylene-briged guanosine
  modified_base 24: mod_base = um
  modified_base 1^2: mod_base = OTHER; note = phosphorotioate bond between nucleosides
  modified_base 2^3: mod_base = OTHER; note = phosphorothioate bond between nucleosides
  modified_base 3^4: mod_base = OTHER; note = phosphorothioate bond between nucleosides
  modified_base 4^5: mod_base = OTHER; note = phosphorothioate bond between nucleosides
  modified_base 5^6: mod_base = OTHER; note = phosphorothioate bond between nucleosides
  modified_base 7^8: mod_base = OTHER; note = phosphorothioate bond between nucleosides
  modified_base 6^7: mod_base = OTHER; note = phosphorothioate bond between nucleosides
  modified_base 8^9: mod_base = OTHER; note = phosphorothioate bond between nucleosides
  modified_base 9^10: mod_base = OTHER; note = phosphorothioate bond between nucleosides
  modified_base 10^11: mod_base = OTHER; note = phosphorothioate bond between nucleosides
  modified_base 11^12: mod_base = OTHER; note = phosphorothioate bond between nucleosides
  modified_base 12^13: mod_base = OTHER; note = phosphorothioate bond between nucleosides
  modified_base 13^14: mod_base = OTHER; note = phosphorothioate bond between nucleosides
  modified_base 14^15: mod_base = OTHER; note = phosphorothioate bond between nucleosides
  modified_base 15^16: mod_base = OTHER; note = phosphorothioate bond between nucleosides
  modified_base 16^17: mod_base = OTHER; note = phosphorothioate bond between nucleosides
  modified_base 17^18: mod_base = OTHER; note = phosphorothioate bond between nucleosides
  modified_base 18^19: mod_base = OTHER; note = methylphosphonate bond between nucleosides
  modified_base 19^20: mod_base = OTHER; note = phosphorothioate bond between nucleosides
  modified_base 20^21: mod_base = OTHER; note = phosphorothioate bond between nucleosides
  modified_base 21^22: mod_base = OTHER; note = phosphorothioate bond between nucleosides
  modified_base 22^23: mod_base = OTHER; note = phosphorothioate bond between nucleosides
  modified_base 23^24: mod_base = OTHER; note = phosphorothioate bond between nucleosides
aaagcatgccatcacctcccctgt

SEQ ID NO: 25 - RNA, 24 nt, synthetic construct
  source 1..24: mol_type = other RNA
  modified_base 1: mod_base = OTHER; note = 2'-O-methyladenosine
  modified_base 2: mod_base = OTHER; note = 2'-O,4'-C-methylene-briged adenosine
  modified_base 3: mod_base = OTHER; note = 2'-O-methyladenosine
  modified_base 4: mod_base = OTHER; note = 2'-O,4'-C-methylene-briged guanosine
  modified_base 5: mod_base = cm
  modified_base 6: mod_base = OTHER; note = 2'-deoxy-2'-fluoroadenosine
  modified_base 7: mod_base = OTHER; note = 2'-deoxy-2'-fluorouridine
  modified_base 8: mod_base = gm
  modified_base 9: mod_base = cm
  modified_base 10: mod_base = OTHER; note = 2'-deoxycytidine
  modified_base 11: mod_base = OTHER; note = 2'-deoxyadenosine
  modified_base 12: mod_base = um
  modified_base 13: mod_base = OTHER; note = 2'-deoxy-2'-fluorocytidine
  modified_base 14: mod_base = OTHER; note = 2'-O-methyladenosine
  modified_base 15: mod_base = OTHER; note = 2'-deoxy-2'-fluorocytidine
  modified_base 16: mod_base = cm
  modified_base 17: mod_base = OTHER; note = 2'-deoxy-2'-fluorouridine
  modified_base 18: mod_base = cm
  modified_base 19: mod_base = OTHER; note = 2'-deoxy-2'-fluorocytidine
  modified_base 20: mod_base = cm
  modified_base 21: mod_base = OTHER; note = 2'-O,4'-C-methylene-briged cytidine
  modified_base 22: mod_base = um
  modified_base 23: mod_base = OTHER; note = 2'-O,4'-C-methylene-briged guanosine
  modified_base 24: mod_base = um
  modified_base 1^2: mod_base = OTHER; note = phosphorotioate bond between nucleosides
  modified_base 2^3: mod_base = OTHER; note = phosphorothioate bond between nucleosides
  modified_base 3^4: mod_base = OTHER; note = phosphorothioate bond between nucleosides
  modified_base 4^5: mod_base = OTHER; note = phosphorothioate bond between nucleosides
  modified_base 5^6: mod_base = OTHER; note = phosphorothioate bond between nucleosides
  modified_base 7^8: mod_base = OTHER; note = phosphorothioate bond between nucleosides
  modified_base 6^7: mod_base = OTHER; note = phosphorothioate bond between nucleosides
  modified_base 8^9: mod_base = OTHER; note = phosphorothioate bond between nucleosides
  modified_base 9^10: mod_base = OTHER; note = phosphorothioate bond between nucleosides
  modified_base 10^11: mod_base = OTHER; note = phosphorothioate bond between nucleosides
  modified_base 11^12: mod_base = OTHER; note = phosphorothioate bond between nucleosides
  modified_base 12^13: mod_base = OTHER; note = phosphorothioate bond between nucleosides
  modified_base 13^14: mod_base = OTHER; note = phosphorothioate bond between nucleosides
  modified_base 14^15: mod_base = OTHER; note = phosphorothioate bond between nucleosides
  modified_base 15^16: mod_base = OTHER; note = phosphorothioate bond between nucleosides
  modified_base 16^17: mod_base = OTHER; note = phosphorothioate bond between nucleosides
  modified_base 17^18: mod_base = OTHER; note = phosphorothioate bond between nucleosides
  modified_base 18^19: mod_base = OTHER; note = phosphorothioate bond between nucleosides
  modified_base 19^20: mod_base = OTHER; note = phosphorothioate bond between nucleosides
  modified_base 20^21: mod_base = OTHER; note = methylphosphonate bond between nucleosides
  modified_base 21^22: mod_base = OTHER; note = phosphorothioate bond between nucleosides
  modified_base 22^23: mod_base = OTHER; note = phosphorothioate bond between nucleosides
  modified_base 23^24: mod_base = OTHER; note = phosphorothioate bond between nucleosides
aaagcatgccatcacctcccctgt

SEQ ID NO: 26 - RNA, 24 nt, synthetic construct
  source 1..24: mol_type = other RNA
  modified_base 1: mod_base = OTHER; note = 2'-O-methyladenosine
  modified_base 2: mod_base = OTHER; note = 2'-O,4'-C-methylene-briged adenosine
  modified_base 3: mod_base = OTHER; note = 2'-O-methyladenosine
  modified_base 4: mod_base = OTHER; note = 2'-O,4'-C-methylene-briged guanosine
  modified_base 5: mod_base = cm
  modified_base 6: mod_base = OTHER; note = 2'-deoxy-2'-fluoroadenosine
  modified_base 7: mod_base = OTHER; note = 2'-deoxy-2'-fluorouridine
  modified_base 8: mod_base = gm
  modified_base 9: mod_base = cm
  modified_base 10: mod_base = OTHER; note = 2'-deoxycytidine
  modified_base 11: mod_base = OTHER; note = 2'-deoxyadenosine
  modified_base 12: mod_base = um
  modified_base 13: mod_base = OTHER; note = 2'-deoxy-2'-fluorocytidine
  modified_base 14: mod_base = OTHER; note = 2'-O-methyladenosine
  modified_base 15: mod_base = OTHER; note = 2'-deoxy-2'-fluorocytidine
  modified_base 16: mod_base = cm
  modified_base 17: mod_base = OTHER; note = 2'-deoxy-2'-fluorouridine
  modified_base 18: mod_base = cm
  modified_base 19: mod_base = OTHER; note = 2'-deoxy-2'-fluorocytidine
  modified_base 20: mod_base = cm
  modified_base 21: mod_base = OTHER; note = 2'-O,4'-C-methylene-briged cytidine
  modified_base 22: mod_base = um
  modified_base 23: mod_base = OTHER; note = 2'-O,4'-C-methylene-briged guanosine
  modified_base 24: mod_base = um
  modified_base 1^2: mod_base = OTHER; note = phosphorotioate bond between nucleosides
  modified_base 2^3: mod_base = OTHER; note = phosphorothioate bond between nucleosides
  modified_base 3^4: mod_base = OTHER; note = phosphorothioate bond between nucleosides
  modified_base 4^5: mod_base = OTHER; note = phosphorothioate bond between nucleosides
  modified_base 5^6: mod_base = OTHER; note = phosphorothioate bond between nucleosides
  modified_base 7^8: mod_base = OTHER; note = phosphorothioate bond between nucleosides
  modified_base 6^7: mod_base = OTHER; note = phosphorothioate bond between nucleosides
  modified_base 8^9: mod_base = OTHER; note = phosphorothioate bond between nucleosides
  modified_base 9^10: mod_base = OTHER; note = phosphorothioate bond between nucleosides
  modified_base 10^11: mod_base = OTHER; note = phosphorothioate bond between nucleosides
  modified_base 11^12: mod_base = OTHER; note = phosphorothioate bond between nucleosides
  modified_base 12^13: mod_base = OTHER; note = phosphorothioate bond between nucleosides
  modified_base 13^14: mod_base = OTHER; note = phosphorothioate bond between nucleosides
  modified_base 14^15: mod_base = OTHER; note = phosphorothioate bond between nucleosides
  modified_base 15^16: mod_base = OTHER; note = phosphorothioate bond between nucleosides
  modified_base 16^17: mod_base = OTHER; note = phosphorothioate bond between nucleosides
  modified_base 17^18: mod_base = OTHER; note = phosphorothioate bond between nucleosides
  modified_base 18^19: mod_base = OTHER; note = phosphorothioate bond between nucleosides
  modified_base 19^20: mod_base = OTHER; note = phosphorothioate bond between nucleosides
  modified_base 20^21: mod_base = OTHER; note = phosphorothioate bond between nucleosides
  modified_base 21^22: mod_base = OTHER; note = phosphorothioate bond between nucleosides
  modified_base 22^23: mod_base = OTHER; note = methylphosphonate bond between nucleosides
  modified_base 23^24: mod_base = OTHER; note = phosphorothioate bond between nucleosides
aaagcatgccatcacctcccctgt

SEQ ID NO: 27 - RNA, 24 nt, synthetic construct
  source 1..24: mol_type = other RNA
  modified_base 1: mod_base = OTHER; note = 2'-O-methyladenosine
  modified_base 2: mod_base = OTHER; note = 2'-O,4'-C-methylene-briged adenosine
  modified_base 3: mod_base = OTHER; note = 2'-O-methyladenosine
  modified_base 4: mod_base = OTHER; note = 2'-O,4'-C-methylene-briged guanosine
  modified_base 5: mod_base = cm
  modified_base 6: mod_base = OTHER; note = 2'-deoxy-2'-fluoroadenosine
  modified_base 7: mod_base = OTHER; note = 2'-deoxy-2'-fluorouridine
  modified_base 8: mod_base = gm
  modified_base 9: mod_base = cm
  modified_base 10: mod_base = OTHER; note = 2'-deoxycytidine
  modified_base 11: mod_base = OTHER; note = 2'-deoxyadenosine
  modified_base 12: mod_base = um
  modified_base 13: mod_base = OTHER; note = 2'-deoxy-2'-fluorocytidine
  modified_base 14: mod_base = OTHER; note = 2'-O-methyladenosine
  modified_base 15: mod_base = OTHER; note = 2'-deoxy-2'-fluorocytidine
  modified_base 16: mod_base = cm
  modified_base 17: mod_base = OTHER; note = 2'-deoxy-2'-fluorouridine
  modified_base 18: mod_base = cm
  modified_base 19: mod_base = OTHER; note = 2'-deoxy-2'-fluorocytidine
  modified_base 20: mod_base = cm
  modified_base 21: mod_base = OTHER; note = 2'-O,4'-C-methylene-briged cytidine
  modified_base 22: mod_base = um
  modified_base 23: mod_base = OTHER; note = 2'-O,4'-C-methylene-briged guanosine
  modified_base 24: mod_base = um
  modified_base 1^2: mod_base = OTHER; note = phosphorotioate bond between nucleosides
  modified_base 2^3: mod_base = OTHER; note = phosphorothioate bond between nucleosides
  modified_base 3^4: mod_base = OTHER; note = phosphorothioate bond between nucleosides
  modified_base 4^5: mod_base = OTHER; note = phosphorothioate bond between nucleosides
  modified_base 5^6: mod_base = OTHER; note = phosphorothioate bond between nucleosides
  modified_base 7^8: mod_base = OTHER; note = phosphorothioate bond between nucleosides
  modified_base 6^7: mod_base = OTHER; note = phosphorothioate bond between nucleosides
  modified_base 8^9: mod_base = OTHER; note = phosphorothioate bond between nucleosides
  modified_base 9^10: mod_base = OTHER; note = phosphorothioate bond between nucleosides
  modified_base 10^11: mod_base = OTHER; note = phosphorothioate bond between nucleosides
  modified_base 11^12: mod_base = OTHER; note = ethylphosphate bond between nucleosides
  modified_base 12^13: mod_base = OTHER; note = phosphorothioate bond between nucleosides
  modified_base 13^14: mod_base = OTHER; note = phosphorothioate bond between nucleosides
  modified_base 14^15: mod_base = OTHER; note = ethylphosphate bond between nucleosides
  modified_base 15^16: mod_base = OTHER; note = phosphorothioate bond between nucleosides
  modified_base 16^17: mod_base = OTHER; note = phosphorothioate bond between nucleosides
  modified_base 17^18: mod_base = OTHER; note = phosphorothioate bond between nucleosides
  modified_base 18^19: mod_base = OTHER; note = phosphorothioate bond between nucleosides
  modified_base 19^20: mod_base = OTHER; note = phosphorothioate bond between nucleosides
  modified_base 20^21: mod_base = OTHER; note = phosphorothioate bond between nucleosides
  modified_base 21^22: mod_base = OTHER; note = phosphorothioate bond between nucleosides
  modified_base 22^23: mod_base = OTHER; note = phosphorothioate bond between nucleosides
  modified_base 23^24: mod_base = OTHER; note = phosphorothioate bond between nucleosides
aaagcatgccatcacctcccctgt

SEQ ID NO: 28 - RNA, 24 nt, synthetic construct
  source 1..24: mol_type = other RNA
  modified_base 1: mod_base = OTHER; note = 2'-O-methyladenosine
  modified_base 2: mod_base = OTHER; note = 2'-O,4'-C-methylene-briged adenosine
  modified_base 3: mod_base = OTHER; note = 2'-O-methyladenosine
  modified_base 4: mod_base = OTHER; note = 2'-O,4'-C-methylene-briged guanosine
  modified_base 5: mod_base = cm
  modified_base 6: mod_base = OTHER; note = 2'-deoxy-2'-fluoroadenosine
  modified_base 7: mod_base = OTHER; note = 2'-deoxy-2'-fluorouridine
  modified_base 8: mod_base = gm
  modified_base 9: mod_base = cm
  modified_base 10: mod_base = OTHER; note = 2'-deoxycytidine
  modified_base 11: mod_base = OTHER; note = 2'-deoxyadenosine
  modified_base 12: mod_base = um
  modified_base 13: mod_base = OTHER; note = 2'-deoxy-2'-fluorocytidine
  modified_base 14: mod_base = OTHER; note = 2'-O-methyladenosine
  modified_base 15: mod_base = OTHER; note = 2'-deoxy-2'-fluorocytidine
  modified_base 16: mod_base = cm
  modified_base 17: mod_base = OTHER; note = 2'-deoxy-2'-fluorouridine
  modified_base 18: mod_base = cm
  modified_base 19: mod_base = OTHER; note = 2'-deoxy-2'-fluorocytidine
  modified_base 20: mod_base = cm
  modified_base 21: mod_base = OTHER; note = 2'-O,4'-C-methylene-briged cytidine
  modified_base 22: mod_base = um
  modified_base 23: mod_base = OTHER; note = 2'-O,4'-C-methylene-briged guanosine
  modified_base 24: mod_base = um
  modified_base 1^2: mod_base = OTHER; note = phosphorotioate bond between nucleosides
  modified_base 2^3: mod_base = OTHER; note = phosphorothioate bond between nucleosides
  modified_base 3^4: mod_base = OTHER; note = phosphorothioate bond between nucleosides
  modified_base 4^5: mod_base = OTHER; note = phosphorothioate bond between nucleosides
  modified_base 5^6: mod_base = OTHER; note = phosphorothioate bond between nucleosides
  modified_base 7^8: mod_base = OTHER; note = phosphorothioate bond between nucleosides
  modified_base 6^7: mod_base = OTHER; note = phosphorothioate bond between nucleosides
  modified_base 8^9: mod_base = OTHER; note = phosphorothioate bond between nucleosides
  modified_base 9^10: mod_base = OTHER; note = phosphorothioate bond between nucleosides
  modified_base 10^11: mod_base = OTHER; note = phosphorothioate bond between nucleosides
  modified_base 11^12: mod_base = OTHER; note = ethylphosphate bond between nucleosides
  modified_base 12^13: mod_base = OTHER; note = phosphorothioate bond between nucleosides
  modified_base 13^14: mod_base = OTHER; note = phosphorothioate bond between nucleosides
  modified_base 14^15: mod_base = OTHER; note = phosphorothioate bond between nucleosides
  modified_base 15^16: mod_base = OTHER; note = phosphorothioate bond between nucleosides
  modified_base 16^17: mod_base = OTHER; note = phosphorothioate bond between nucleosides
  modified_base 17^18: mod_base = OTHER; note = phosphorothioate bond between nucleosides
  modified_base 18^19: mod_base = OTHER; note = phosphorothioate bond between nucleosides
  modified_base 19^20: mod_base = OTHER; note = phosphorothioate bond between nucleosides
  modified_base 20^21: mod_base = OTHER; note = phosphorothioate bond between nucleosides
  modified_base 21^22: mod_base = OTHER; note = phosphorothioate bond between nucleosides
  modified_base 22^23: mod_base = OTHER; note = phosphorothioate bond between nucleosides
  modified_base 23^24: mod_base = OTHER; note = phosphorothioate bond between nucleosides
aaagcatgccatcacctcccctgt

SEQ ID NO: 29 - RNA, 24 nt, synthetic construct
  source 1..24: mol_type = other RNA
  modified_base 1: mod_base = OTHER; note = 2'-O-methyladenosine
  modified_base 2: mod_base = OTHER; note = 2'-O,4'-C-methylene-briged adenosine
  modified_base 3: mod_base = OTHER; note = 2'-O-methyladenosine
  modified_base 4: mod_base = OTHER; note = 2'-O,4'-C-methylene-briged guanosine
  modified_base 5: mod_base = cm
  modified_base 6: mod_base = OTHER; note = 2'-deoxy-2'-fluoroadenosine
  modified_base 7: mod_base = OTHER; note = 2'-deoxy-2'-fluorouridine
  modified_base 8: mod_base = gm
  modified_base 9: mod_base = cm
  modified_base 10: mod_base = OTHER; note = 2'-deoxycytidine
  modified_base 11: mod_base = OTHER; note = 2'-deoxyadenosine
  modified_base 12: mod_base = um
  modified_base 13: mod_base = OTHER; note = 2'-deoxy-2'-fluorocytidine
  modified_base 14: mod_base = OTHER; note = 2'-O-methyladenosine
  modified_base 15: mod_base = OTHER; note = 2'-deoxy-2'-fluorocytidine
  modified_base 16: mod_base = cm
  modified_base 17: mod_base = OTHER; note = 2'-deoxy-2'-fluorouridine
  modified_base 18: mod_base = cm
  modified_base 19: mod_base = OTHER; note = 2'-deoxy-2'-fluorocytidine
  modified_base 20: mod_base = cm
  modified_base 21: mod_base = OTHER; note = 2'-O,4'-C-methylene-briged cytidine
  modified_base 22: mod_base = um
  modified_base 23: mod_base = OTHER; note = 2'-O,4'-C-methylene-briged guanosine
  modified_base 24: mod_base = um
  modified_base 1^2: mod_base = OTHER; note = phosphorotioate bond between nucleosides
  modified_base 2^3: mod_base = OTHER; note = phosphorothioate bond between nucleosides
  modified_base 3^4: mod_base = OTHER; note = phosphorothioate bond between nucleosides
  modified_base 4^5: mod_base = OTHER; note = phosphorothioate bond between nucleosides
  modified_base 5^6: mod_base = OTHER; note = phosphorothioate bond between nucleosides
  modified_base 7^8: mod_base = OTHER; note = phosphorothioate bond between nucleosides
  modified_base 6^7: mod_base = OTHER; note = phosphorothioate bond between nucleosides
  modified_base 8^9: mod_base = OTHER; note = phosphorothioate bond between nucleosides
  modified_base 9^10: mod_base = OTHER; note = phosphorothioate bond between nucleosides
  modified_base 10^11: mod_base = OTHER; note = phosphorothioate bond between nucleosides
  modified_base 11^12: mod_base = OTHER; note = phosphorothioate bond between nucleosides
  modified_base 12^13: mod_base = OTHER; note = phosphorothioate bond between nucleosides
  modified_base 13^14: mod_base = OTHER; note = phosphorothioate bond between nucleosides
  modified_base 14^15: mod_base = OTHER; note = ethylphosphate bond between nucleosides
  modified_base 15^16: mod_base = OTHER; note = phosphorothioate bond between nucleosides
  modified_base 16^17: mod_base = OTHER; note = phosphorothioate bond between nucleosides
  modified_base 17^18: mod_base = OTHER; note = phosphorothioate bond between nucleosides
  modified_base 18^19: mod_base = OTHER; note = phosphorothioate bond between nucleosides
  modified_base 19^20: mod_base = OTHER; note = phosphorothioate bond between nucleosides
  modified_base 20^21: mod_base = OTHER; note = phosphorothioate bond between nucleosides
  modified_base 21^22: mod_base = OTHER; note = phosphorothioate bond between nucleosides
  modified_base 22^23: mod_base = OTHER; note = phosphorothioate bond between nucleosides
  modified_base 23^24: mod_base = OTHER; note = phosphorothioate bond between nucleosides
aaagcatgccatcacctcccctgt

SEQ ID NO: 30 - RNA, 24 nt, synthetic construct
  source 1..24: mol_type = other RNA
  modified_base 1: mod_base = OTHER; note = 2'-O-methyladenosine
  modified_base 2: mod_base = OTHER; note = 2'-O,4'-C-methylene-briged adenosine
  modified_base 3: mod_base = OTHER; note = 2'-O-methyladenosine
  modified_base 4: mod_base = OTHER; note = 2'-O,4'-C-methylene-briged guanosine
  modified_base 5: mod_base = cm
  modified_base 6: mod_base = OTHER; note = 2'-deoxy-2'-fluoroadenosine
  modified_base 7: mod_base = OTHER; note = 2'-deoxy-2'-fluorouridine
  modified_base 8: mod_base = gm
  modified_base 9: mod_base = cm
  modified_base 10: mod_base = OTHER; note = 2'-deoxycytidine
  modified_base 11: mod_base = OTHER; note = 2'-deoxyadenosine
  modified_base 12: mod_base = um
  modified_base 13: mod_base = OTHER; note = 2'-deoxy-2'-fluorocytidine
  modified_base 14: mod_base = OTHER; note = 2'-O-methyladenosine
  modified_base 15: mod_base = OTHER; note = 2'-deoxy-2'-fluorocytidine
  modified_base 16: mod_base = cm
  modified_base 17: mod_base = OTHER; note = 2'-deoxy-2'-fluorouridine
  modified_base 18: mod_base = cm
  modified_base 19: mod_base = OTHER; note = 2'-deoxy-2'-fluorocytidine
  modified_base 20: mod_base = cm
  modified_base 21: mod_base = OTHER; note = 2'-O,4'-C-methylene-briged cytidine
  modified_base 22: mod_base = um
  modified_base 23: mod_base = OTHER; note = 2'-O,4'-C-methylene-briged guanosine
  modified_base 24: mod_base = um
  modified_base 1^2: mod_base = OTHER; note = phosphorotioate bond between nucleosides
  modified_base 2^3: mod_base = OTHER; note = phosphorothioate bond between nucleosides
  modified_base 3^4: mod_base = OTHER; note = phosphorothioate bond between nucleosides
  modified_base 4^5: mod_base = OTHER; note = phosphorothioate bond between nucleosides
  modified_base 5^6: mod_base = OTHER; note = phosphorothioate bond between nucleosides
  modified_base 7^8: mod_base = OTHER; note = phosphorothioate bond between nucleosides
  modified_base 6^7: mod_base = OTHER; note = phosphorothioate bond between nucleosides
  modified_base 8^9: mod_base = OTHER; note = phosphorothioate bond between nucleosides
  modified_base 9^10: mod_base = OTHER; note = phosphorothioate bond between nucleosides
  modified_base 10^11: mod_base = OTHER; note = phosphorothioate bond between nucleosides
  modified_base 11^12: mod_base = OTHER; note = isopropylphosphate bond between nucleosides
  modified_base 12^13: mod_base = OTHER; note = phosphorothioate bond between nucleosides
  modified_base 13^14: mod_base = OTHER; note = phosphorothioate bond between nucleosides
  modified_base 14^15: mod_base = OTHER; note = phosphorohioate bond between nucleosides
  modified_base 15^16: mod_base = OTHER; note = phosphorothioate bond between nucleosides
  modified_base 16^17: mod_base = OTHER; note = phosphorothioate bond between nucleosides
  modified_base 17^18: mod_base = OTHER; note = phosphorothioate bond between nucleosides
  modified_base 18^19: mod_base = OTHER; note = phosphorothioate bond between nucleosides
  modified_base 19^20: mod_base = OTHER; note = phosphorothioate bond between nucleosides
  modified_base 20^21: mod_base = OTHER; note = phosphorothioate bond between nucleosides
  modified_base 21^22: mod_base = OTHER; note = phosphorothioate bond between nucleosides
  modified_base 22^23: mod_base = OTHER; note = phosphorothioate bond between nucleosides
  modified_base 23^24: mod_base = OTHER; note = phosphorothioate bond between nucleosides
aaagcatgccatcacctcccctgt

SEQ ID NO: 31 - RNA, 24 nt, synthetic construct
  source 1..24: mol_type = other RNA
  modified_base 1: mod_base = OTHER; note = 2'-O-methyladenosine
  modified_base 2: mod_base = OTHER; note = 2'-O,4'-C-methylene-briged adenosine
  modified_base 3: mod_base = OTHER; note = 2'-O-methyladenosine
  modified_base 4: mod_base = OTHER; note = 2'-O,4'-C-methylene-briged guanosine
  modified_base 5: mod_base = cm
  modified_base 6: mod_base = OTHER; note = 2'-deoxy-2'-fluoroadenosine
  modified_base 7: mod_base = OTHER; note = 2'-deoxy-2'-fluorouridine
  modified_base 8: mod_base = gm
  modified_base 9: mod_base = cm
  modified_base 10: mod_base = OTHER; note = 2'-deoxycytidine
  modified_base 11: mod_base = OTHER; note = 2'-deoxyadenosine
  modified_base 12: mod_base = um
  modified_base 13: mod_base = OTHER; note = 2'-deoxy-2'-fluorocytidine
  modified_base 14: mod_base = OTHER; note = 2'-O-methyladenosine
  modified_base 15: mod_base = OTHER; note = 2'-deoxy-2'-fluorocytidine
  modified_base 16: mod_base = cm
  modified_base 17: mod_base = OTHER; note = 2'-deoxy-2'-fluorouridine
  modified_base 18: mod_base = cm
  modified_base 19: mod_base = OTHER; note = 2'-deoxy-2'-fluorocytidine
  modified_base 20: mod_base = cm
  modified_base 21: mod_base = OTHER; note = 2'-O,4'-C-methylene-briged cytidine
  modified_base 22: mod_base = um
  modified_base 23: mod_base = OTHER; note = 2'-O,4'-C-methylene-briged guanosine
  modified_base 24: mod_base = um
  modified_base 1^2: mod_base = OTHER; note = phosphorotioate bond between nucleosides
  modified_base 2^3: mod_base = OTHER; note = phosphorothioate bond between nucleosides
  modified_base 3^4: mod_base = OTHER; note = phosphorothioate bond between nucleosides
  modified_base 4^5: mod_base = OTHER; note = phosphorothioate bond between nucleosides
  modified_base 5^6: mod_base = OTHER; note = phosphorothioate bond between nucleosides
  modified_base 7^8: mod_base = OTHER; note = phosphorothioate bond between nucleosides
  modified_base 6^7: mod_base = OTHER; note = phosphorothioate bond between nucleosides
  modified_base 8^9: mod_base = OTHER; note = phosphorothioate bond between nucleosides
  modified_base 9^10: mod_base = OTHER; note = phosphorothioate bond between nucleosides
  modified_base 10^11: mod_base = OTHER; note = phosphorothioate bond between nucleosides
  modified_base 11^12: mod_base = OTHER; note = methylthiophosphonate bond between nucleosides
  modified_base 12^13: mod_base = OTHER; note = phosphorothioate bond between nucleosides
  modified_base 13^14: mod_base = OTHER; note = phosphorothioate bond between nucleosides
  modified_base 14^15: mod_base = OTHER; note = methylthiophosphonate bond between nucleosides
  modified_base 15^16: mod_base = OTHER; note = phosphorothioate bond between nucleosides
  modified_base 16^17: mod_base = OTHER; note = phosphorothioate bond between nucleosides
  modified_base 17^18: mod_base = OTHER; note = phosphorothioate bond between nucleosides
  modified_base 18^19: mod_base = OTHER; note = phosphorothioate bond between nucleosides
  modified_base 19^20: mod_base = OTHER; note = phosphorothioate bond between nucleosides
  modified_base 20^21: mod_base = OTHER; note = phosphorothioate bond between nucleosides
  modified_base 21^22: mod_base = OTHER; note = phosphorothioate bond between nucleosides
  modified_base 22^23: mod_base = OTHER; note = phosphorothioate bond between nucleosides
  modified_base 23^24: mod_base = OTHER; note = phosphorothioate bond between nucleosides
aaagcatgccatcacctcccctgt

SEQ ID NO: 32 - RNA, 24 nt, synthetic construct
  source 1..24: mol_type = other RNA
  modified_base 1: mod_base = OTHER; note = 2'-O-methyladenosine
  modified_base 2: mod_base = OTHER; note = 2'-O,4'-C-methylene-briged adenosine
  modified_base 3: mod_base = OTHER; note = 2'-O-methyladenosine
  modified_base 4: mod_base = OTHER; note = 2'-O,4'-C-methylene-briged guanosine
  modified_base 5: mod_base = cm
  modified_base 6: mod_base = OTHER; note = 2'-deoxy-2'-fluoroadenosine
  modified_base 7: mod_base = OTHER; note = 2'-deoxy-2'-fluorouridine
  modified_base 8: mod_base = gm
  modified_base 9: mod_base = cm
  modified_base 10: mod_base = OTHER; note = 2'-deoxycytidine
  modified_base 11: mod_base = OTHER; note = 2'-deoxyadenosine
  modified_base 12: mod_base = um
  modified_base 13: mod_base = OTHER; note = 2'-deoxy-2'-fluorocytidine
  modified_base 14: mod_base = OTHER; note = 2'-O-methyladenosine
  modified_base 15: mod_base = OTHER; note = 2'-deoxy-2'-fluorocytidine
  modified_base 16: mod_base = cm
  modified_base 17: mod_base = OTHER; note = 2'-deoxy-2'-fluorouridine
  modified_base 18: mod_base = cm
  modified_base 19: mod_base = OTHER; note = 2'-deoxy-2'-fluorocytidine
  modified_base 20: mod_base = cm
  modified_base 21: mod_base = OTHER; note = 2'-O,4'-C-methylene-briged cytidine
  modified_base 22: mod_base = um
  modified_base 23: mod_base = OTHER; note = 2'-O,4'-C-methylene-briged guanosine
  modified_base 24: mod_base = um
  modified_base 1^2: mod_base = OTHER; note = phosphorotioate bond between nucleosides
  modified_base 2^3: mod_base = OTHER; note = phosphorothioate bond between nucleosides
  modified_base 3^4: mod_base = OTHER; note = phosphorothioate bond between nucleosides
  modified_base 4^5: mod_base = OTHER; note = phosphorothioate bond between nucleosides
  modified_base 5^6: mod_base = OTHER; note = phosphorothioate bond between nucleosides
  modified_base 7^8: mod_base = OTHER; note = phosphorothioate bond between nucleosides
  modified_base 6^7: mod_base = OTHER; note = phosphorothioate bond between nucleosides
  modified_base 8^9: mod_base = OTHER; note = phosphorothioate bond between nucleosides
  modified_base 9^10: mod_base = OTHER; note = phosphorothioate bond between nucleosides
  modified_base 10^11: mod_base = OTHER; note = phosphorothioate bond between nucleosides
  modified_base 11^12: mod_base = OTHER; note = methylthiophosphonate bond between nucleosides
  modified_base 12^13: mod_base = OTHER; note = phosphorothioate bond between nucleosides
  modified_base 13^14: mod_base = OTHER; note = phosphorothioate bond between nucleosides
  modified_base 14^15: mod_base = OTHER; note = phosphorothioate bond between nucleosides
  modified_base 15^16: mod_base = OTHER; note = phosphorothioate bond between nucleosides
  modified_base 16^17: mod_base = OTHER; note = phosphorothioate bond between nucleosides
  modified_base 17^18: mod_base = OTHER; note = phosphorothioate bond between nucleosides
  modified_base 18^19: mod_base = OTHER; note = phosphorothioate bond between nucleosides
  modified_base 19^20: mod_base = OTHER; note = phosphorothioate bond between nucleosides
  modified_base 20^21: mod_base = OTHER; note = phosphorothioate bond between nucleosides
  modified_base 21^22: mod_base = OTHER; note = phosphorothioate bond between nucleosides
  modified_base 22^23: mod_base = OTHER; note = phosphorothioate bond between nucleosides
  modified_base 23^24: mod_base = OTHER; note = phosphorothioate bond between nucleosides
aaagcatgccatcacctcccctgt

SEQ ID NO: 33 - RNA, 24 nt, synthetic construct
  source 1..24: mol_type = other RNA
  modified_base 1: mod_base = OTHER; note = 2'-O-methyladenosine
  modified_base 2: mod_base = OTHER; note = 2'-O,4'-C-methylene-briged adenosine
  modified_base 3: mod_base = OTHER; note = 2'-O-methyladenosine
  modified_base 4: mod_base = OTHER; note = 2'-O,4'-C-methylene-briged guanosine
  modified_base 5: mod_base = cm
  modified_base 6: mod_base = OTHER; note = 2'-deoxy-2'-fluoroadenosine
  modified_base 7: mod_base = OTHER; note = 2'-deoxy-2'-fluorouridine
  modified_base 8: mod_base = gm
  modified_base 9: mod_base = cm
  modified_base 10: mod_base = OTHER; note = 2'-deoxycytidine
  modified_base 11: mod_base = OTHER; note = 2'-deoxyadenosine
  modified_base 12: mod_base = um
  modified_base 13: mod_base = OTHER; note = 2'-deoxy-2'-fluorocytidine
  modified_base 14: mod_base = OTHER; note = 2'-O-methyladenosine
  modified_base 15: mod_base = OTHER; note = 2'-deoxy-2'-fluorocytidine
  modified_base 16: mod_base = cm
  modified_base 17: mod_base = OTHER; note = 2'-deoxy-2'-fluorouridine
  modified_base 18: mod_base = cm
  modified_base 19: mod_base = OTHER; note = 2'-deoxy-2'-fluorocytidine
  modified_base 20: mod_base = cm
  modified_base 21: mod_base = OTHER; note = 2'-O,4'-C-methylene-briged cytidine
  modified_base 22: mod_base = um
  modified_base 23: mod_base = OTHER; note = 2'-O,4'-C-methylene-briged guanosine
  modified_base 24: mod_base = um
  modified_base 1^2: mod_base = OTHER; note = phosphorotioate bond between nucleosides
  modified_base 2^3: mod_base = OTHER; note = phosphorothioate bond between nucleosides
  modified_base 3^4: mod_base = OTHER; note = phosphorothioate bond between nucleosides
  modified_base 4^5: mod_base = OTHER; note = phosphorothioate bond between nucleosides
  modified_base 5^6: mod_base = OTHER; note = phosphorothioate bond between nucleosides
  modified_base 7^8: mod_base = OTHER; note = phosphorothioate bond between nucleosides
  modified_base 6^7: mod_base = OTHER; note = phosphorothioate bond between nucleosides
  modified_base 8^9: mod_base = OTHER; note = phosphorothioate bond between nucleosides
  modified_base 9^10: mod_base = OTHER; note = phosphorothioate bond between nucleosides
  modified_base 10^11: mod_base = OTHER; note = phosphorothioate bond between nucleosides
  modified_base 11^12: mod_base = OTHER; note = phosphorothioate bond between nucleosides
  modified_base 12^13: mod_base = OTHER; note = phosphorothioate bond between nucleosides
  modified_base 13^14: mod_base = OTHER; note = phosphorothioate bond between nucleosides
  modified_base 14^15: mod_base = OTHER; note = methylthiophosphonate bond between nucleosides
  modified_base 15^16: mod_base = OTHER; note = phosphorothioate bond between nucleosides
  modified_base 16^17: mod_base = OTHER; note = phosphorothioate bond between nucleosides
  modified_base 17^18: mod_base = OTHER; note = phosphorothioate bond between nucleosides
  modified_base 18^19: mod_base = OTHER; note = phosphorothioate bond between nucleosides
  modified_base 19^20: mod_base = OTHER; note = phosphorothioate bond between nucleosides
  modified_base 20^21: mod_base = OTHER; note = phosphorothioate bond between nucleosides
  modified_base 21^22: mod_base = OTHER; note = phosphorothioate bond between nucleosides
  modified_base 22^23: mod_base = OTHER; note = phosphorothioate bond between nucleosides
  modified_base 23^24: mod_base = OTHER; note = phosphorothioate bond between nucleosides
aaagcatgccatcacctcccctgt

SEQ ID NO: 34 - RNA, 24 nt, synthetic construct
  source 1..24: mol_type = other RNA
  modified_base 1: mod_base = OTHER; note = 2'-O-methyladenosine
  modified_base 2: mod_base = OTHER; note = 2'-O,4'-C-methylene-briged adenosine
  modified_base 3: mod_base = OTHER; note = 2'-O-methyladenosine
  modified_base 4: mod_base = OTHER; note = 2'-O,4'-C-methylene-briged guanosine
  modified_base 5: mod_base = cm
  modified_base 6: mod_base = OTHER; note = 2'-deoxy-2'-fluoroadenosine
  modified_base 7: mod_base = OTHER; note = 2'-deoxy-2'-fluorouridine
  modified_base 8: mod_base = gm
  modified_base 9: mod_base = cm
  modified_base 10: mod_base = OTHER; note = 2'-deoxycytidine
  modified_base 11: mod_base = OTHER; note = 2'-deoxyadenosine
  modified_base 12: mod_base = um
  modified_base 13: mod_base = OTHER; note = 2'-deoxy-2'-fluorocytidine
  modified_base 14: mod_base = OTHER; note = 2'-O-methyladenosine
  modified_base 15: mod_base = OTHER; note = 2'-deoxy-2'-fluorocytidine
  modified_base 16: mod_base = cm
  modified_base 17: mod_base = OTHER; note = 2'-deoxy-2'-fluorouridine
  modified_base 18: mod_base = cm
  modified_base 19: mod_base = OTHER; note = 2'-deoxy-2'-fluorocytidine
  modified_base 20: mod_base = cm
  modified_base 21: mod_base = OTHER; note = 2'-O,4'-C-methylene-briged cytidine
  modified_base 22: mod_base = um
  modified_base 23: mod_base = OTHER; note = 2'-O,4'-C-methylene-briged guanosine
  modified_base 24: mod_base = um
  modified_base 1^2: mod_base = OTHER; note = phosphorotioate bond between nucleosides
  modified_base 2^3: mod_base = OTHER; note = phosphorothioate bond between nucleosides
  modified_base 3^4: mod_base = OTHER; note = phosphorothioate bond between nucleosides
  modified_base 4^5: mod_base = OTHER; note = phosphorothioate bond between nucleosides
  modified_base 5^6: mod_base = OTHER; note = phosphorothioate bond between nucleosides
  modified_base 7^8: mod_base = OTHER; note = phosphorothioate bond between nucleosides
  modified_base 6^7: mod_base = OTHER; note = phosphorothioate bond between nucleosides
  modified_base 8^9: mod_base = OTHER; note = methylphosphonate bond between nucleosides
  modified_base 9^10: mod_base = OTHER; note = phosphorothioate bond between nucleosides
  modified_base 10^11: mod_base = OTHER; note = phosphorothioate bond between nucleosides
  modified_base 11^12: mod_base = OTHER; note = phosphorothioate bond between nucleosides
  modified_base 12^13: mod_base = OTHER; note = phosphorothioate bond between nucleosides
  modified_base 13^14: mod_base = OTHER; note = phosphorothioate bond between nucleosides
  modified_base 14^15: mod_base = OTHER; note = phosphorothioate bond between nucleosides
  modified_base 15^16: mod_base = OTHER; note = phosphorothioate bond between nucleosides
  modified_base 16^17: mod_base = OTHER; note = phosphorothioate bond between nucleosides
  modified_base 17^18: mod_base = OTHER; note = phosphorothioate bond between nucleosides
  modified_base 18^19: mod_base = OTHER; note = phosphorothioate bond between nucleosides
  modified_base 19^20: mod_base = OTHER; note = phosphorothioate bond between nucleosides
  modified_base 20^21: mod_base = OTHER; note = phosphorothioate bond between nucleosides
  modified_base 21^22: mod_base = OTHER; note = phosphorothioate bond between nucleosides
  modified_base 22^23: mod_base = OTHER; note = phosphorothioate bond between nucleosides
  modified_base 23^24: mod_base = OTHER; note = phosphorothioate bond between nucleosides
aaagcatgccatcacctcccctgt

SEQ ID NO: 35 - RNA, 24 nt, synthetic construct
  source 1..24: mol_type = other RNA
  modified_base 1: mod_base = OTHER; note = 2'-O-methyladenosine
  modified_base 2: mod_base = OTHER; note = 2'-O,4'-C-methylene-briged adenosine
  modified_base 3: mod_base = OTHER; note = 2'-O-methyladenosine
  modified_base 4: mod_base = OTHER; note = 2'-O,4'-C-methylene-briged guanosine
  modified_base 5: mod_base = cm
  modified_base 6: mod_base = OTHER; note = 2'-deoxy-2'-fluoroadenosine
  modified_base 7: mod_base = OTHER; note = 2'-deoxy-2'-fluorouridine
  modified_base 8: mod_base = gm
  modified_base 9: mod_base = cm
  modified_base 10: mod_base = OTHER; note = 2'-deoxycytidine
  modified_base 11: mod_base = OTHER; note = 2'-deoxyadenosine
  modified_base 12: mod_base = um
  modified_base 13: mod_base = OTHER; note = 2'-deoxy-2'-fluorocytidine
  modified_base 14: mod_base = OTHER; note = 2'-O-methyladenosine
  modified_base 15: mod_base = OTHER; note = 2'-deoxy-2'-fluorocytidine
  modified_base 16: mod_base = cm
  modified_base 17: mod_base = OTHER; note = 2'-deoxy-2'-fluorouridine
  modified_base 18: mod_base = cm
  modified_base 19: mod_base = OTHER; note = 2'-deoxy-2'-fluorocytidine
  modified_base 20: mod_base = cm
  modified_base 21: mod_base = OTHER; note = 2'-O,4'-C-methylene-briged cytidine
  modified_base 22: mod_base = um
  modified_base 23: mod_base = OTHER; note = 2'-O,4'-C-methylene-briged guanosine
  modified_base 24: mod_base = um
  modified_base 1^2: mod_base = OTHER; note = phosphorotioate bond between nucleosides
  modified_base 2^3: mod_base = OTHER; note = phosphorothioate bond between nucleosides
  modified_base 3^4: mod_base = OTHER; note = phosphorothioate bond between nucleosides
  modified_base 4^5: mod_base = OTHER; note = phosphorothioate bond between nucleosides
  modified_base 5^6: mod_base = OTHER; note = phosphorothioate bond between nucleosides
  modified_base 7^8: mod_base = OTHER; note = phosphorothioate bond between nucleosides
  modified_base 6^7: mod_base = OTHER; note = phosphorothioate bond between nucleosides
  modified_base 8^9: mod_base = OTHER; note = phosphorothioate bond between nucleosides
  modified_base 9^10: mod_base = OTHER; note = phosphorothioate bond between nucleosides
  modified_base 10^11: mod_base = OTHER; note = phosphorothioate bond between nucleosides
  modified_base 11^12: mod_base = OTHER; note = ethylphosphonate bond between nucleosides
  modified_base 12^13: mod_base = OTHER; note = phosphorothioate bond between nucleosides
  modified_base 13^14: mod_base = OTHER; note = phosphorothioate bond between nucleosides
  modified_base 14^15: mod_base = OTHER; note = phosphorothioate bond between nucleosides
  modified_base 15^16: mod_base = OTHER; note = phosphorothioate bond between nucleosides
  modified_base 16^17: mod_base = OTHER; note = phosphorothioate bond between nucleosides
  modified_base 17^18: mod_base = OTHER; note = phosphorothioate bond between nucleosides
  modified_base 18^19: mod_base = OTHER; note = phosphorothioate bond between nucleosides
  modified_base 19^20: mod_base = OTHER; note = phosphorothioate bond between nucleosides
  modified_base 20^21: mod_base = OTHER; note = phosphorothioate bond between nucleosides
  modified_base 21^22: mod_base = OTHER; note = phosphorothioate bond between nucleosides
  modified_base 22^23: mod_base = OTHER; note = phosphorothioate bond between nucleosides
  modified_base 23^24: mod_base = OTHER; note = phosphorothioate bond between nucleosides
aaagcatgccatcacctcccctgt

SEQ ID NO: 36 - RNA, 24 nt, synthetic construct
  source 1..24: mol_type = other RNA
  modified_base 1: mod_base = OTHER; note = 2'-O-methyladenosine
  modified_base 2: mod_base = OTHER; note = 2'-O,4'-C-methylene-briged adenosine
  modified_base 3: mod_base = OTHER; note = 2'-O-methyladenosine
  modified_base 4: mod_base = OTHER; note = 2'-O,4'-C-methylene-briged guanosine
  modified_base 5: mod_base = cm
  modified_base 6: mod_base = OTHER; note = 2'-deoxy-2'-fluoroadenosine
  modified_base 7: mod_base = OTHER; note = 2'-deoxy-2'-fluorouridine
  modified_base 8: mod_base = gm
  modified_base 9: mod_base = cm
  modified_base 10: mod_base = OTHER; note = 2'-deoxycytidine
  modified_base 11: mod_base = OTHER; note = 2'-deoxyadenosine
  modified_base 12: mod_base = um
  modified_base 13: mod_base = OTHER; note = 2'-deoxy-2'-fluorocytidine
  modified_base 14: mod_base = OTHER; note = 2'-O-methyladenosine
  modified_base 15: mod_base = OTHER; note = 2'-deoxy-2'-fluorocytidine
  modified_base 16: mod_base = cm
  modified_base 17: mod_base = OTHER; note = 2'-deoxy-2'-fluorouridine
  modified_base 18: mod_base = cm
  modified_base 19: mod_base = OTHER; note = 2'-deoxy-2'-fluorocytidine
  modified_base 20: mod_base = cm
  modified_base 21: mod_base = OTHER; note = 2'-O,4'-C-methylene-briged cytidine
  modified_base 22: mod_base = um
  modified_base 23: mod_base = OTHER; note = 2'-O,4'-C-methylene-briged guanosine
  modified_base 24: mod_base = um
  modified_base 1^2: mod_base = OTHER; note = phosphorotioate bond between nucleosides
  modified_base 2^3: mod_base = OTHER; note = phosphorothioate bond between nucleosides
  modified_base 3^4: mod_base = OTHER; note = phosphorothioate bond between nucleosides
  modified_base 4^5: mod_base = OTHER; note = phosphorothioate bond between nucleosides
  modified_base 5^6: mod_base = OTHER; note = phosphorothioate bond between nucleosides
  modified_base 7^8: mod_base = OTHER; note = phosphorothioate bond between nucleosides
  modified_base 6^7: mod_base = OTHER; note = phosphorothioate bond between nucleosides
  modified_base 8^9: mod_base = OTHER; note = phosphorothioate bond between nucleosides
  modified_base 9^10: mod_base = OTHER; note = phosphorothioate bond between nucleosides
  modified_base 10^11: mod_base = OTHER; note = phosphorothioate bond between nucleosides
  modified_base 11^12: mod_base = OTHER; note = propylphosphonate bond between nucleosides
  modified_base 12^13: mod_base = OTHER; note = phosphorothioate bond between nucleosides
  modified_base 13^14: mod_base = OTHER; note = phosphorothioate bond between nucleosides
  modified_base 14^15: mod_base = OTHER; note = methylphosphonate bond between nucleosides
  modified_base 15^16: mod_base = OTHER; note = phosphorothioate bond between nucleosides
  modified_base 16^17: mod_base = OTHER; note = phosphorothioate bond between nucleosides
  modified_base 17^18: mod_base = OTHER; note = phosphorothioate bond between nucleosides
  modified_base 18^19: mod_base = OTHER; note = phosphorothioate bond between nucleosides
  modified_base 19^20: mod_base = OTHER; note = phosphorothioate bond between nucleosides
  modified_base 20^21: mod_base = OTHER; note = phosphorothioate bond between nucleosides
  modified_base 21^22: mod_base = OTHER; note = phosphorothioate bond between nucleosides
  modified_base 22^23: mod_base = OTHER; note = phosphorothioate bond between nucleosides
  modified_base 23^24: mod_base = OTHER; note = phosphorothioate bond between nucleosides
aaagcatgccatcacctcccctgt

SEQ ID NO: 37 - RNA, 24 nt, synthetic construct
  source 1..24: mol_type = other RNA
  modified_base 1: mod_base = OTHER; note = 2'-O-methyladenosine
  modified_base 2: mod_base = OTHER; note = 2'-O,4'-C-methylene-briged adenosine
  modified_base 3: mod_base = OTHER; note = 2'-O-methyladenosine
  modified_base 4: mod_base = OTHER; note = 2'-O,4'-C-methylene-briged guanosine
  modified_base 5: mod_base = cm
  modified_base 6: mod_base = OTHER; note = 2'-deoxy-2'-fluoroadenosine
  modified_base 7: mod_base = OTHER; note = 2'-deoxy-2'-fluorouridine
  modified_base 8: mod_base = gm
  modified_base 9: mod_base = cm
  modified_base 10: mod_base = OTHER; note = 2'-deoxycytidine
  modified_base 11: mod_base = OTHER; note = 2'-deoxyadenosine
  modified_base 12: mod_base = um
  modified_base 13: mod_base = OTHER; note = 2'-deoxy-2'-fluorocytidine
  modified_base 14: mod_base = OTHER; note = 2'-O-methyladenosine
  modified_base 15: mod_base = OTHER; note = 2'-deoxy-2'-fluorocytidine
  modified_base 16: mod_base = cm
  modified_base 17: mod_base = OTHER; note = 2'-deoxy-2'-fluorouridine
  modified_base 18: mod_base = cm
  modified_base 19: mod_base = OTHER; note = 2'-deoxy-2'-fluorocytidine
  modified_base 20: mod_base = cm
  modified_base 21: mod_base = OTHER; note = 2'-O,4'-C-methylene-briged cytidine
  modified_base 22: mod_base = um
  modified_base 23: mod_base = OTHER; note = 2'-O,4'-C-methylene-briged guanosine
  modified_base 24: mod_base = um
  modified_base 1^2: mod_base = OTHER; note = phosphorotioate bond between nucleosides
  modified_base 2^3: mod_base = OTHER; note = phosphorothioate bond between nucleosides
  modified_base 3^4: mod_base = OTHER; note = phosphorothioate bond between nucleosides
  modified_base 4^5: mod_base = OTHER; note = phosphorothioate bond between nucleosides
  modified_base 5^6: mod_base = OTHER; note = phosphorothioate bond between nucleosides
  modified_base 7^8: mod_base = OTHER; note = phosphorothioate bond between nucleosides
  modified_base 6^7: mod_base = OTHER; note = phosphorothioate bond between nucleosides
  modified_base 8^9: mod_base = OTHER; note = phosphorothioate bond between nucleosides
  modified_base 9^10: mod_base = OTHER; note = phosphorothioate bond between nucleosides
  modified_base 10^11: mod_base = OTHER; note = phosphorothioate bond between nucleosides
  modified_base 11^12: mod_base = OTHER; note = isopropylphosphonate bond between nucleosides
  modified_base 12^13: mod_base = OTHER; note = phosphorothioate bond between nucleosides
  modified_base 13^14: mod_base = OTHER; note = phosphorothioate bond between nucleosides
  modified_base 14^15: mod_base = OTHER; note = phosphorothioate bond between nucleosides
  modified_base 15^16: mod_base = OTHER; note = phosphorothioate bond between nucleosides
  modified_base 16^17: mod_base = OTHER; note = phosphorothioate bond between nucleosides
  modified_base 17^18: mod_base = OTHER; note = phosphorothioate bond between nucleosides
  modified_base 18^19: mod_base = OTHER; note = phosphorothioate bond between nucleosides
  modified_base 19^20: mod_base = OTHER; note = phosphorothioate bond between nucleosides
  modified_base 20^21: mod_base = OTHER; note = phosphorothioate bond between nucleosides
  modified_base 21^22: mod_base = OTHER; note = phosphorothioate bond between nucleosides
  modified_base 22^23: mod_base = OTHER; note = phosphorothioate bond between nucleosides
  modified_base 23^24: mod_base = OTHER; note = phosphorothioate bond between nucleosides
aaagcatgccatcacctcccctgt

SEQ ID NO: 38 - RNA, 24 nt, synthetic construct
  source 1..24: mol_type = other RNA
  modified_base 1: mod_base = OTHER; note = 2'-O-methyladenosine
  modified_base 2: mod_base = OTHER; note = 2'-O,4'-C-methylene-briged adenosine
  modified_base 3: mod_base = OTHER; note = 2'-O-methyladenosine
  modified_base 4: mod_base = OTHER; note = 2'-O,4'-C-methylene-briged guanosine
  modified_base 5: mod_base = cm
  modified_base 6: mod_base = OTHER; note = 2'-deoxy-2'-fluoroadenosine
  modified_base 7: mod_base = OTHER; note = 2'-deoxy-2'-fluorouridine
  modified_base 8: mod_base = gm
  modified_base 9: mod_base = cm
  modified_base 10: mod_base = OTHER; note = 2'-deoxycytidine
  modified_base 11: mod_base = OTHER; note = 2'-deoxyadenosine
  modified_base 12: mod_base = um
  modified_base 13: mod_base = OTHER; note = 2'-deoxy-2'-fluorocytidine
  modified_base 14: mod_base = OTHER; note = 2'-O-methyladenosine
  modified_base 15: mod_base = OTHER; note = 2'-deoxy-2'-fluorocytidine
  modified_base 16: mod_base = cm
  modified_base 17: mod_base = OTHER; note = 2'-deoxy-2'-fluorouridine
  modified_base 18: mod_base = cm
  modified_base 19: mod_base = OTHER; note = 2'-deoxy-2'-fluorocytidine
  modified_base 20: mod_base = cm
  modified_base 21: mod_base = OTHER; note = 2'-O,4'-C-methylene-briged cytidine
  modified_base 22: mod_base = um
  modified_base 23: mod_base = OTHER; note = 2'-O,4'-C-methylene-briged guanosine
  modified_base 24: mod_base = um
  modified_base 1^2: mod_base = OTHER; note = phosphorotioate bond between nucleosides
  modified_base 2^3: mod_base = OTHER; note = phosphorothioate bond between nucleosides
  modified_base 3^4: mod_base = OTHER; note = phosphorothioate bond between nucleosides
  modified_base 4^5: mod_base = OTHER; note = phosphorothioate bond between nucleosides
  modified_base 5^6: mod_base = OTHER; note = phosphorothioate bond between nucleosides
  modified_base 7^8: mod_base = OTHER; note = phosphorothioate bond between nucleosides
  modified_base 6^7: mod_base = OTHER; note = phosphorothioate bond between nucleosides
  modified_base 8^9: mod_base = OTHER; note = phosphorothioate bond between nucleosides
  modified_base 9^10: mod_base = OTHER; note = phosphorothioate bond between nucleosides
  modified_base 10^11: mod_base = OTHER; note = phosphorothioate bond between nucleosides
  modified_base 12^13: mod_base = OTHER; note = phosphorothioate bond between nucleosides
  modified_base 13^14: mod_base = OTHER; note = phosphorothioate bond between nucleosides
  modified_base 15^16: mod_base = OTHER; note = phosphorothioate bond between nucleosides
  modified_base 16^17: mod_base = OTHER; note = phosphorothioate bond between nucleosides
  modified_base 17^18: mod_base = OTHER; note = phosphorothioate bond between nucleosides
  modified_base 18^19: mod_base = OTHER; note = phosphorothioate bond between nucleosides
  modified_base 19^20: mod_base = OTHER; note = phosphorothioate bond between nucleosides
  modified_base 20^21: mod_base = OTHER; note = phosphorothioate bond between nucleosides
  modified_base 21^22: mod_base = OTHER; note = phosphorothioate bond between nucleosides
  modified_base 22^23: mod_base = OTHER; note = phosphorothioate bond between nucleosides
  modified_base 23^24: mod_base = OTHER; note = phosphorothioate bond between nucleosides
aaagcatgccatcacctcccctgt

SEQ ID NO: 39 - RNA, 24 nt, synthetic construct
  source 1..24: mol_type = other RNA
  modified_base 1: mod_base = OTHER; note = 2'-O-methyladenosine
  modified_base 2: mod_base = OTHER; note = 2'-O,4'-C-methylene-briged adenosine
  modified_base 3: mod_base = OTHER; note = 2'-O-methyladenosine
  modified_base 4: mod_base = OTHER; note = 2'-O,4'-C-methylene-briged guanosine
  modified_base 5: mod_base = cm
  modified_base 6: mod_base = OTHER; note = 2'-deoxy-2'-fluoroadenosine
  modified_base 7: mod_base = OTHER; note = 2'-deoxy-2'-fluorouridine
  modified_base 8: mod_base = gm
  modified_base 9: mod_base = cm
  modified_base 10: mod_base = OTHER; note = 2'-deoxycytidine
  modified_base 11: mod_base = OTHER; note = 2'-deoxyadenosine
  modified_base 12: mod_base = um
  modified_base 13: mod_base = OTHER; note = 2'-deoxy-2'-fluorocytidine
  modified_base 14: mod_base = OTHER; note = 2'-O-methyladenosine
  modified_base 15: mod_base = OTHER; note = 2'-deoxy-2'-fluorocytidine
  modified_base 16: mod_base = cm
  modified_base 17: mod_base = OTHER; note = 2'-deoxy-2'-fluorouridine
  modified_base 18: mod_base = cm
  modified_base 19: mod_base = OTHER; note = 2'-deoxy-2'-fluorocytidine
  modified_base 20: mod_base = cm
  modified_base 21: mod_base = OTHER; note = 2'-O,4'-C-methylene-briged cytidine
  modified_base 22: mod_base = um
  modified_base 23: mod_base = OTHER; note = 2'-O,4'-C-methylene-briged guanosine
  modified_base 24: mod_base = um
  modified_base 1^2: mod_base = OTHER; note = phosphorotioate bond between nucleosides
  modified_base 2^3: mod_base = OTHER; note = phosphorothioate bond between nucleosides
  modified_base 3^4: mod_base = OTHER; note = phosphorothioate bond between nucleosides
  modified_base 4^5: mod_base = OTHER; note = phosphorothioate bond between nucleosides
  modified_base 5^6: mod_base = OTHER; note = phosphorothioate bond between nucleosides
  modified_base 7^8: mod_base = OTHER; note = phosphorothioate bond between nucleosides
  modified_base 6^7: mod_base = OTHER; note = phosphorothioate bond between nucleosides
  modified_base 8^9: mod_base = OTHER; note = phosphorothioate bond between nucleosides
  modified_base 9^10: mod_base = OTHER; note = phosphorothioate bond between nucleosides
  modified_base 10^11: mod_base = OTHER; note = phosphorothioate bond between nucleosides
  modified_base 11^12: mod_base = OTHER; note = methylphosphonate bond between nucleosides
  modified_base 12^13: mod_base = OTHER; note = phosphorothioate bond between nucleosides
  modified_base 13^14: mod_base = OTHER; note = phosphorothioate bond between nucleosides
  modified_base 15^16: mod_base = OTHER; note = phosphorothioate bond between nucleosides
  modified_base 16^17: mod_base = OTHER; note = phosphorothioate bond between nucleosides
  modified_base 17^18: mod_base = OTHER; note = phosphorothioate bond between nucleosides
  modified_base 18^19: mod_base = OTHER; note = phosphorothioate bond between nucleosides
  modified_base 19^20: mod_base = OTHER; note = phosphorothioate bond between nucleosides
  modified_base 20^21: mod_base = OTHER; note = phosphorothioate bond between nucleosides
  modified_base 21^22: mod_base = OTHER; note = phosphorothioate bond between nucleosides
  modified_base 22^23: mod_base = OTHER; note = phosphorothioate bond between nucleosides
  modified_base 23^24: mod_base = OTHER; note = phosphorothioate bond between nucleosides
  modified_base 14^15: mod_base = OTHER; note = phosphorothioate bond between nucleosides
aaagcatgccatcacctcccctgt

SEQ ID NO: 40 - RNA, 24 nt, synthetic construct
  source 1..24: mol_type = other RNA
  modified_base 1: mod_base = OTHER; note = 2'-O-methyladenosine
  modified_base 2: mod_base = OTHER; note = 2'-O,4'-C-methylene-briged adenosine
  modified_base 3: mod_base = OTHER; note = 2'-O-methyladenosine
  modified_base 4: mod_base = OTHER; note = 2'-O,4'-C-methylene-briged guanosine
  modified_base 5: mod_base = cm
  modified_base 6: mod_base = OTHER; note = 2'-deoxy-2'-fluoroadenosine
  modified_base 7: mod_base = OTHER; note = 2'-deoxy-2'-fluorouridine
  modified_base 8: mod_base = gm
  modified_base 9: mod_base = cm
  modified_base 10: mod_base = OTHER; note = 2'-deoxycytidine
  modified_base 11: mod_base = OTHER; note = 2'-deoxyadenosine
  modified_base 12: mod_base = um
  modified_base 13: mod_base = OTHER; note = 2'-deoxy-2'-fluorocytidine
  modified_base 14: mod_base = OTHER; note = 2'-O-methyladenosine
  modified_base 15: mod_base = OTHER; note = 2'-deoxy-2'-fluorocytidine
  modified_base 16: mod_base = cm
  modified_base 17: mod_base = OTHER; note = 2'-deoxy-2'-fluorouridine
  modified_base 18: mod_base = cm
  modified_base 19: mod_base = OTHER; note = 2'-deoxy-2'-fluorocytidine
  modified_base 20: mod_base = cm
  modified_base 21: mod_base = OTHER; note = 2'-O,4'-C-methylene-briged cytidine
  modified_base 22: mod_base = um
  modified_base 23: mod_base = OTHER; note = 2'-O,4'-C-methylene-briged guanosine
  modified_base 24: mod_base = um
  modified_base 1^2: mod_base = OTHER; note = phosphorotioate bond between nucleosides
  modified_base 2^3: mod_base = OTHER; note = phosphorothioate bond between nucleosides
  modified_base 3^4: mod_base = OTHER; note = phosphorothioate bond between nucleosides
  modified_base 4^5: mod_base = OTHER; note = phosphorothioate bond between nucleosides
  modified_base 5^6: mod_base = OTHER; note = phosphorothioate bond between nucleosides
  modified_base 7^8: mod_base = OTHER; note = phosphorothioate bond between nucleosides
  modified_base 6^7: mod_base = OTHER; note = phosphorothioate bond between nucleosides
  modified_base 8^9: mod_base = OTHER; note = phosphorothioate bond between nucleosides
  modified_base 9^10: mod_base = OTHER; note = phosphorothioate bond between nucleosides
  modified_base 10^11: mod_base = OTHER; note = phosphorothioate bond between nucleosides
  modified_base 11^12: mod_base = OTHER; note = phosphorothioate bond between nucleosides
  modified_base 12^13: mod_base = OTHER; note = phosphorothioate bond between nucleosides
  modified_base 13^14: mod_base = OTHER; note = phosphorothioate bond between nucleosides
  modified_base 15^16: mod_base = OTHER; note = phosphorothioate bond between nucleosides
  modified_base 16^17: mod_base = OTHER; note = phosphorothioate bond between nucleosides
  modified_base 17^18: mod_base = OTHER; note = phosphorothioate bond between nucleosides
  modified_base 18^19: mod_base = OTHER; note = phosphorothioate bond between nucleosides
  modified_base 19^20: mod_base = OTHER; note = phosphorothioate bond between nucleosides
  modified_base 20^21: mod_base = OTHER; note = phosphorothioate bond between nucleosides
  modified_base 21^22: mod_base = OTHER; note = phosphorothioate bond between nucleosides
  modified_base 22^23: mod_base = OTHER; note = phosphorothioate bond between nucleosides
  modified_base 23^24: mod_base = OTHER; note = phosphorothioate bond between nucleosides
aaagcatgccatcacctcccctgt

SEQ ID NO: 41 - RNA, 24 nt, synthetic construct
  source 1..24: mol_type = other RNA
  modified_base 1: mod_base = OTHER; note = 2'-O-methyladenosine
  modified_base 2: mod_base = OTHER; note = 2'-O,4'-C-methylene-briged adenosine
  modified_base 3: mod_base = OTHER; note = 2'-O-methyladenosine
  modified_base 4: mod_base = OTHER; note = 2'-O,4'-C-methylene-briged guanosine
  modified_base 5: mod_base = cm
  modified_base 6: mod_base = OTHER; note = 2'-deoxy-2'-fluoroadenosine
  modified_base 7: mod_base = OTHER; note = 2'-deoxy-2'-fluorouridine
  modified_base 8: mod_base = gm
  modified_base 9: mod_base = cm
  modified_base 10: mod_base = OTHER; note = 2'-deoxycytidine
  modified_base 11: mod_base = OTHER; note = 2'-deoxyadenosine
  modified_base 12: mod_base = um
  modified_base 13: mod_base = OTHER; note = 2'-deoxy-2'-fluorocytidine
  modified_base 14: mod_base = OTHER; note = 2'-O-methyladenosine
  modified_base 15: mod_base = OTHER; note = 2'-deoxy-2'-fluorocytidine
  modified_base 16: mod_base = cm
  modified_base 17: mod_base = OTHER; note = 2'-deoxy-2'-fluorouridine
  modified_base 18: mod_base = cm
  modified_base 19: mod_base = OTHER; note = 2'-deoxy-2'-fluorocytidine
  modified_base 20: mod_base = cm
  modified_base 21: mod_base = OTHER; note = 2'-O,4'-C-methylene-briged cytidine
  modified_base 22: mod_base = um
  modified_base 23: mod_base = OTHER; note = 2'-O,4'-C-methylene-briged guanosine
  modified_base 24: mod_base = um
  modified_base 1^2: mod_base = OTHER; note = phosphorotioate bond between nucleosides
  modified_base 2^3: mod_base = OTHER; note = phosphorothioate bond between nucleosides
  modified_base 3^4: mod_base = OTHER; note = phosphorothioate bond between nucleosides
  modified_base 4^5: mod_base = OTHER; note = phosphorothioate bond between nucleosides
  modified_base 5^6: mod_base = OTHER; note = phosphorothioate bond between nucleosides
  modified_base 7^8: mod_base = OTHER; note = phosphorothioate bond between nucleosides
  modified_base 6^7: mod_base = OTHER; note = ethylphosphate bond between nucleosides
  modified_base 8^9: mod_base = OTHER; note = phosphorothioate bond between nucleosides
  modified_base 9^10: mod_base = OTHER; note = phosphorothioate bond between nucleosides
  modified_base 10^11: mod_base = OTHER; note = phosphorothioate bond between nucleosides
  modified_base 11^12: mod_base = OTHER; note = phosphorothioate bond between nucleosides
  modified_base 12^13: mod_base = OTHER; note = phosphorothioate bond between nucleosides
  modified_base 13^14: mod_base = OTHER; note = phosphorothioate bond between nucleosides
  modified_base 14^15: mod_base = OTHER; note = phosphorothioate bond between nucleosides
  modified_base 15^16: mod_base = OTHER; note = phosphorothioate bond between nucleosides
  modified_base 16^17: mod_base = OTHER; note = phosphorothioate bond between nucleosides
  modified_base 17^18: mod_base = OTHER; note = phosphorothioate bond between nucleosides
  modified_base 18^19: mod_base = OTHER; note = phosphorothioate bond between nucleosides
  modified_base 19^20: mod_base = OTHER; note = phosphorothioate bond between nucleosides
  modified_base 20^21: mod_base = OTHER; note = phosphorothioate bond between nucleosides
  modified_base 21^22: mod_base = OTHER; note = phosphorothioate bond between nucleosides
  modified_base 22^23: mod_base = OTHER; note = phosphorothioate bond between nucleosides
  modified_base 23^24: mod_base = OTHER; note = phosphorothioate bond between nucleosides
aaagcatgccatcacctcccctgt

SEQ ID NO: 42 - RNA, 24 nt, synthetic construct
  source 1..24: mol_type = other RNA
  modified_base 1: mod_base = OTHER; note = 2'-O-methyladenosine
  modified_base 2: mod_base = OTHER; note = 2'-O,4'-C-methylene-briged adenosine
  modified_base 3: mod_base = OTHER; note = 2'-O-methyladenosine
  modified_base 4: mod_base = OTHER; note = 2'-O,4'-C-methylene-briged guanosine
  modified_base 5: mod_base = cm
  modified_base 6: mod_base = OTHER; note = 2'-deoxy-2'-fluoroadenosine
  modified_base 7: mod_base = OTHER; note = 2'-deoxy-2'-fluorouridine
  modified_base 8: mod_base = gm
  modified_base 9: mod_base = cm
  modified_base 10: mod_base = OTHER; note = 2'-deoxycytidine
  modified_base 11: mod_base = OTHER; note = 2'-deoxyadenosine
  modified_base 12: mod_base = um
  modified_base 13: mod_base = OTHER; note = 2'-deoxy-2'-fluorocytidine
  modified_base 14: mod_base = OTHER; note = 2'-O-methyladenosine
  modified_base 15: mod_base = OTHER; note = 2'-deoxy-2'-fluorocytidine
  modified_base 16: mod_base = cm
  modified_base 17: mod_base = OTHER; note = 2'-deoxy-2'-fluorouridine
  modified_base 18: mod_base = cm
  modified_base 19: mod_base = OTHER; note = 2'-deoxy-2'-fluorocytidine
  modified_base 20: mod_base = cm
  modified_base 21: mod_base = OTHER; note = 2'-O,4'-C-methylene-briged cytidine
  modified_base 22: mod_base = um
  modified_base 23: mod_base = OTHER; note = 2'-O,4'-C-methylene-briged guanosine
  modified_base 24: mod_base = um
  modified_base 1^2: mod_base = OTHER; note = phosphorotioate bond between nucleosides
  modified_base 2^3: mod_base = OTHER; note = phosphorothioate bond between nucleosides
  modified_base 3^4: mod_base = OTHER; note = phosphorothioate bond between nucleosides
  modified_base 4^5: mod_base = OTHER; note = phosphorothioate bond between nucleosides
  modified_base 5^6: mod_base = OTHER; note = phosphorothioate bond between nucleosides
  modified_base 7^8: mod_base = OTHER; note = ethylphosphate bond between nucleosides
  modified_base 6^7: mod_base = OTHER; note = phosphorothioate bond between nucleosides
  modified_base 8^9: mod_base = OTHER; note = phosphorothioate bond between nucleosides
  modified_base 9^10: mod_base = OTHER; note = phosphorothioate bond between nucleosides
  modified_base 10^11: mod_base = OTHER; note = phosphorothioate bond between nucleosides
  modified_base 11^12: mod_base = OTHER; note = phosphorothioate bond between nucleosides
  modified_base 12^13: mod_base = OTHER; note = phosphorothioate bond between nucleosides
  modified_base 13^14: mod_base = OTHER; note = phosphorothioate bond between nucleosides
  modified_base 14^15: mod_base = OTHER; note = phosphorothioate bond between nucleosides
  modified_base 15^16: mod_base = OTHER; note = phosphorothioate bond between nucleosides
  modified_base 16^17: mod_base = OTHER; note = phosphorothioate bond between nucleosides
  modified_base 17^18: mod_base = OTHER; note = phosphorothioate bond between nucleosides
  modified_base 18^19: mod_base = OTHER; note = phosphorothioate bond between nucleosides
  modified_base 19^20: mod_base = OTHER; note = phosphorothioate bond between nucleosides
  modified_base 20^21: mod_base = OTHER; note = phosphorothioate bond between nucleosides
  modified_base 21^22: mod_base = OTHER; note = phosphorothioate bond between nucleosides
  modified_base 22^23: mod_base = OTHER; note = phosphorothioate bond between nucleosides
  modified_base 23^24: mod_base = OTHER; note = phosphorothioate bond between nucleosides
aaagcatgccatcacctcccctgt

SEQ ID NO: 43 - RNA, 24 nt, synthetic construct
  source 1..24: mol_type = other RNA
  modified_base 1: mod_base = OTHER; note = 2'-O-methyladenosine
  modified_base 2: mod_base = OTHER; note = 2'-O,4'-C-methylene-briged adenosine
  modified_base 3: mod_base = OTHER; note = 2'-O-methyladenosine
  modified_base 4: mod_base = OTHER; note = 2'-O,4'-C-methylene-briged guanosine
  modified_base 5: mod_base = cm
  modified_base 6: mod_base = OTHER; note = 2'-deoxy-2'-fluoroadenosine
  modified_base 7: mod_base = OTHER; note = 2'-deoxy-2'-fluorouridine
  modified_base 8: mod_base = gm
  modified_base 9: mod_base = cm
  modified_base 10: mod_base = OTHER; note = 2'-deoxycytidine
  modified_base 11: mod_base = OTHER; note = 2'-deoxyadenosine
  modified_base 12: mod_base = um
  modified_base 13: mod_base = OTHER; note = 2'-deoxy-2'-fluorocytidine
  modified_base 14: mod_base = OTHER; note = 2'-O-methyladenosine
  modified_base 15: mod_base = OTHER; note = 2'-deoxy-2'-fluorocytidine
  modified_base 16: mod_base = cm
  modified_base 17: mod_base = OTHER; note = 2'-deoxy-2'-fluorouridine
  modified_base 18: mod_base = cm
  modified_base 19: mod_base = OTHER; note = 2'-deoxy-2'-fluorocytidine
  modified_base 20: mod_base = cm
  modified_base 21: mod_base = OTHER; note = 2'-O,4'-C-methylene-briged cytidine
  modified_base 22: mod_base = um
  modified_base 23: mod_base = OTHER; note = 2'-O,4'-C-methylene-briged guanosine
  modified_base 24: mod_base = um
  modified_base 1^2: mod_base = OTHER; note = phosphorotioate bond between nucleosides
  modified_base 2^3: mod_base = OTHER; note = phosphorothioate bond between nucleosides
  modified_base 3^4: mod_base = OTHER; note = phosphorothioate bond between nucleosides
  modified_base 4^5: mod_base = OTHER; note = phosphorothioate bond between nucleosides
  modified_base 5^6: mod_base = OTHER; note = phosphorothioate bond between nucleosides
  modified_base 7^8: mod_base = OTHER; note = phosphorothioate bond between nucleosides
  modified_base 6^7: mod_base = OTHER; note = phosphorothioate bond between nucleosides
  modified_base 8^9: mod_base = OTHER; note = phosphorothioate bond between nucleosides
  modified_base 9^10: mod_base = OTHER; note = phosphorothioate bond between nucleosides
  modified_base 10^11: mod_base = OTHER; note = phosphorothioate bond between nucleosides
  modified_base 11^12: mod_base = OTHER; note = phosphorothioate bond between nucleosides
  modified_base 12^13: mod_base = OTHER; note = phosphorothioate bond between nucleosides
  modified_base 13^14: mod_base = OTHER; note = ethylphosphate bond between nucleosides
  modified_base 14^15: mod_base = OTHER; note = phosphorothioate bond between nucleosides
  modified_base 15^16: mod_base = OTHER; note = phosphorothioate bond between nucleosides
  modified_base 16^17: mod_base = OTHER; note = phosphorothioate bond between nucleosides
  modified_base 17^18: mod_base = OTHER; note = phosphorothioate bond between nucleosides
  modified_base 18^19: mod_base = OTHER; note = phosphorothioate bond between nucleosides
  modified_base 19^20: mod_base = OTHER; note = phosphorothioate bond between nucleosides
  modified_base 20^21: mod_base = OTHER; note = phosphorothioate bond between nucleosides
  modified_base 21^22: mod_base = OTHER; note = phosphorothioate bond between nucleosides
  modified_base 22^23: mod_base = OTHER; note = phosphorothioate bond between nucleosides
  modified_base 23^24: mod_base = OTHER; note = phosphorothioate bond between nucleosides
aaagcatgccatcacctcccctgt

SEQ ID NO: 44 - RNA, 24 nt, synthetic construct
  source 1..24: mol_type = other RNA
  modified_base 1: mod_base = OTHER; note = 2'-O-methyladenosine
  modified_base 2: mod_base = OTHER; note = 2'-O,4'-C-methylene-briged adenosine
  modified_base 3: mod_base = OTHER; note = 2'-O-methyladenosine
  modified_base 4: mod_base = OTHER; note = 2'-O,4'-C-methylene-briged guanosine
  modified_base 5: mod_base = cm
  modified_base 6: mod_base = OTHER; note = 2'-deoxy-2'-fluoroadenosine
  modified_base 7: mod_base = OTHER; note = 2'-deoxy-2'-fluorouridine
  modified_base 8: mod_base = gm
  modified_base 9: mod_base = cm
  modified_base 10: mod_base = OTHER; note = 2'-deoxycytidine
  modified_base 11: mod_base = OTHER; note = 2'-deoxyadenosine
  modified_base 12: mod_base = um
  modified_base 13: mod_base = OTHER; note = 2'-deoxy-2'-fluorocytidine
  modified_base 14: mod_base = OTHER; note = 2'-O-methyladenosine
  modified_base 15: mod_base = OTHER; note = 2'-deoxy-2'-fluorocytidine
  modified_base 16: mod_base = cm
  modified_base 17: mod_base = OTHER; note = 2'-deoxy-2'-fluorouridine
  modified_base 18: mod_base = cm
  modified_base 19: mod_base = OTHER; note = 2'-deoxy-2'-fluorocytidine
  modified_base 20: mod_base = cm
  modified_base 21: mod_base = OTHER; note = 2'-O,4'-C-methylene-briged cytidine
  modified_base 22: mod_base = um
  modified_base 23: mod_base = OTHER; note = 2'-O,4'-C-methylene-briged guanosine
  modified_base 24: mod_base = um
  modified_base 1^2: mod_base = OTHER; note = phosphorotioate bond between nucleosides
  modified_base 2^3: mod_base = OTHER; note = phosphorothioate bond between nucleosides
  modified_base 3^4: mod_base = OTHER; note = phosphorothioate bond between nucleosides
  modified_base 4^5: mod_base = OTHER; note = phosphorothioate bond between nucleosides
  modified_base 5^6: mod_base = OTHER; note = phosphorothioate bond between nucleosides
  modified_base 7^8: mod_base = OTHER; note = phosphorothioate bond between nucleosides
  modified_base 6^7: mod_base = OTHER; note = phosphorothioate bond between nucleosides
  modified_base 8^9: mod_base = OTHER; note = phosphorothioate bond between nucleosides
  modified_base 9^10: mod_base = OTHER; note = phosphorothioate bond between nucleosides
  modified_base 10^11: mod_base = OTHER; note = phosphorothioate bond between nucleosides
  modified_base 11^12: mod_base = OTHER; note = phosphorothioate bond between nucleosides
  modified_base 12^13: mod_base = OTHER; note = phosphorothioate bond between nucleosides
  modified_base 13^14: mod_base = OTHER; note = phosphorothioate bond between nucleosides
  modified_base 14^15: mod_base = OTHER; note = phosphorothioate bond between nucleosides
  modified_base 15^16: mod_base = OTHER; note = ethylphosphate bond between nucleosides
  modified_base 16^17: mod_base = OTHER; note = phosphorothioate bond between nucleosides
  modified_base 17^18: mod_base = OTHER; note = phosphorothioate bond between nucleosides
  modified_base 18^19: mod_base = OTHER; note = phosphorothioate bond between nucleosides
  modified_base 19^20: mod_base = OTHER; note = phosphorothioate bond between nucleosides
  modified_base 20^21: mod_base = OTHER; note = phosphorothioate bond between nucleosides
  modified_base 21^22: mod_base = OTHER; note = phosphorothioate bond between nucleosides
  modified_base 22^23: mod_base = OTHER; note = phosphorothioate bond between nucleosides
  modified_base 23^24: mod_base = OTHER; note = phosphorothioate bond between nucleosides
aaagcatgccatcacctcccctgt

SEQ ID NO: 45 - RNA, 24 nt, synthetic construct
  source 1..24: mol_type = other RNA
  modified_base 1: mod_base = OTHER; note = 2'-O-methyladenosine
  modified_base 2: mod_base = OTHER; note = 2'-O,4'-C-methylene-briged adenosine
  modified_base 3: mod_base = OTHER; note = 2'-O-methyladenosine
  modified_base 4: mod_base = OTHER; note = 2'-O,4'-C-methylene-briged guanosine
  modified_base 5: mod_base = cm
  modified_base 6: mod_base = OTHER; note = 2'-deoxy-2'-fluoroadenosine
  modified_base 7: mod_base = OTHER; note = 2'-deoxy-2'-fluorouridine
  modified_base 8: mod_base = gm
  modified_base 9: mod_base = cm
  modified_base 10: mod_base = OTHER; note = 2'-deoxycytidine
  modified_base 11: mod_base = OTHER; note = 2'-deoxyadenosine
  modified_base 12: mod_base = um
  modified_base 13: mod_base = OTHER; note = 2'-deoxy-2'-fluorocytidine
  modified_base 14: mod_base = OTHER; note = 2'-O-methyladenosine
  modified_base 15: mod_base = OTHER; note = 2'-deoxy-2'-fluorocytidine
  modified_base 16: mod_base = cm
  modified_base 17: mod_base = OTHER; note = 2'-deoxy-2'-fluorouridine
  modified_base 18: mod_base = cm
  modified_base 19: mod_base = OTHER; note = 2'-deoxy-2'-fluorocytidine
  modified_base 20: mod_base = cm
  modified_base 21: mod_base = OTHER; note = 2'-O,4'-C-methylene-briged cytidine
  modified_base 22: mod_base = um
  modified_base 23: mod_base = OTHER; note = 2'-O,4'-C-methylene-briged guanosine
  modified_base 24: mod_base = um
  modified_base 1^2: mod_base = OTHER; note = phosphorotioate bond between nucleosides
  modified_base 2^3: mod_base = OTHER; note = phosphorothioate bond between nucleosides
  modified_base 3^4: mod_base = OTHER; note = phosphorothioate bond between nucleosides
  modified_base 4^5: mod_base = OTHER; note = phosphorothioate bond between nucleosides
  modified_base 5^6: mod_base = OTHER; note = phosphorothioate bond between nucleosides
  modified_base 7^8: mod_base = OTHER; note = phosphorothioate bond between nucleosides
  modified_base 6^7: mod_base = OTHER; note = phosphorothioate bond between nucleosides
  modified_base 8^9: mod_base = OTHER; note = phosphorothioate bond between nucleosides
  modified_base 9^10: mod_base = OTHER; note = phosphorothioate bond between nucleosides
  modified_base 10^11: mod_base = OTHER; note = phosphorothioate bond between nucleosides
  modified_base 11^12: mod_base = OTHER; note = phosphorothioate bond between nucleosides
  modified_base 12^13: mod_base = OTHER; note = phosphorothioate bond between nucleosides
  modified_base 13^14: mod_base = OTHER; note = phosphorothioate bond between nucleosides
  modified_base 14^15: mod_base = OTHER; note = phosphorothioate bond between nucleosides
  modified_base 15^16: mod_base = OTHER; note = phosphorothioate bond between nucleosides
  modified_base 16^17: mod_base = OTHER; note = phosphorothioate bond between nucleosides
  modified_base 17^18: mod_base = OTHER; note = ethylphosphate bond between nucleosides
  modified_base 18^19: mod_base = OTHER; note = phosphorothioate bond between nucleosides
  modified_base 19^20: mod_base = OTHER; note = phosphorothioate bond between nucleosides
  modified_base 20^21: mod_base = OTHER; note = phosphorothioate bond between nucleosides
  modified_base 21^22: mod_base = OTHER; note = phosphorothioate bond between nucleosides
  modified_base 22^23: mod_base = OTHER; note = phosphorothioate bond between nucleosides
  modified_base 23^24: mod_base = OTHER; note = phosphorothioate bond between nucleosides
aaagcatgccatcacctcccctgt

SEQ ID NO: 46 - RNA, 24 nt, synthetic construct
  source 1..24: mol_type = other RNA
  modified_base 1: mod_base = OTHER; note = 2'-O-methyladenosine
  modified_base 2: mod_base = OTHER; note = 2'-O,4'-C-methylene-briged adenosine
  modified_base 3: mod_base = OTHER; note = 2'-O-methyladenosine
  modified_base 4: mod_base = OTHER; note = 2'-O,4'-C-methylene-briged guanosine
  modified_base 5: mod_base = cm
  modified_base 6: mod_base = OTHER; note = 2'-deoxy-2'-fluoroadenosine
  modified_base 7: mod_base = OTHER; note = 2'-deoxy-2'-fluorouridine
  modified_base 8: mod_base = gm
  modified_base 9: mod_base = cm
  modified_base 10: mod_base = OTHER; note = 2'-deoxycytidine
  modified_base 11: mod_base = OTHER; note = 2'-deoxyadenosine
  modified_base 12: mod_base = um
  modified_base 13: mod_base = OTHER; note = 2'-deoxy-2'-fluorocytidine
  modified_base 14: mod_base = OTHER; note = 2'-O-methyladenosine
  modified_base 15: mod_base = OTHER; note = 2'-deoxy-2'-fluorocytidine
  modified_base 16: mod_base = cm
  modified_base 17: mod_base = OTHER; note = 2'-deoxy-2'-fluorouridine
  modified_base 18: mod_base = cm
  modified_base 19: mod_base = OTHER; note = 2'-deoxy-2'-fluorocytidine
  modified_base 20: mod_base = cm
  modified_base 21: mod_base = OTHER; note = 2'-O,4'-C-methylene-briged cytidine
  modified_base 22: mod_base = um
  modified_base 23: mod_base = OTHER; note = 2'-O,4'-C-methylene-briged guanosine
  modified_base 24: mod_base = um
  modified_base 1^2: mod_base = OTHER; note = phosphorotioate bond between nucleosides
  modified_base 2^3: mod_base = OTHER; note = phosphorothioate bond between nucleosides
  modified_base 3^4: mod_base = OTHER; note = phosphorothioate bond between nucleosides
  modified_base 4^5: mod_base = OTHER; note = phosphorothioate bond between nucleosides
  modified_base 5^6: mod_base = OTHER; note = phosphorothioate bond between nucleosides
  modified_base 7^8: mod_base = OTHER; note = phosphorothioate bond between nucleosides
  modified_base 6^7: mod_base = OTHER; note = phosphorothioate bond between nucleosides
  modified_base 8^9: mod_base = OTHER; note = phosphorothioate bond between nucleosides
  modified_base 9^10: mod_base = OTHER; note = phosphorothioate bond between nucleosides
  modified_base 10^11: mod_base = OTHER; note = phosphorothioate bond between nucleosides
  modified_base 11^12: mod_base = OTHER; note = phosphorothioate bond between nucleosides
  modified_base 12^13: mod_base = OTHER; note = phosphorothioate bond between nucleosides
  modified_base 13^14: mod_base = OTHER; note = phosphorothioate bond between nucleosides
  modified_base 14^15: mod_base = OTHER; note = phosphorothioate bond between nucleosides
  modified_base 15^16: mod_base = OTHER; note = phosphorothioate bond between nucleosides
  modified_base 16^17: mod_base = OTHER; note = phosphorothioate bond between nucleosides
  modified_base 17^18: mod_base = OTHER; note = phosphorothioate bond between nucleosides
  modified_base 18^19: mod_base = OTHER; note = phosphorothioate bond between nucleosides
  modified_base 19^20: mod_base = OTHER; note = ethylphosphate bond between nucleosides
  modified_base 20^21: mod_base = OTHER; note = phosphorothioate bond between nucleosides
  modified_base 21^22: mod_base = OTHER; note = phosphorothioate bond between nucleosides
  modified_base 22^23: mod_base = OTHER; note = phosphorothioate bond between nucleosides
  modified_base 23^24: mod_base = OTHER; note = phosphorothioate bond between nucleosides
aaagcatgccatcacctcccctgt

SEQ ID NO: 47 - RNA, 24 nt, synthetic construct
  source 1..24: mol_type = other RNA
  modified_base 1: mod_base = OTHER; note = 2'-O-methyladenosine
  modified_base 2: mod_base = OTHER; note = 2'-O,4'-C-methylene-briged adenosine
  modified_base 3: mod_base = OTHER; note = 2'-O-methyladenosine
  modified_base 4: mod_base = OTHER; note = 2'-O,4'-C-methylene-briged guanosine
  modified_base 5: mod_base = cm
  modified_base 6: mod_base = OTHER; note = 2'-deoxy-2'-fluoroadenosine
  modified_base 7: mod_base = OTHER; note = 2'-deoxy-2'-fluorouridine
  modified_base 8: mod_base = gm
  modified_base 9: mod_base = cm
  modified_base 10: mod_base = OTHER; note = 2'-deoxycytidine
  modified_base 11: mod_base = OTHER; note = 2'-deoxyadenosine
  modified_base 12: mod_base = um
  modified_base 13: mod_base = OTHER; note = 2'-deoxy-2'-fluorocytidine
  modified_base 14: mod_base = OTHER; note = 2'-O-methyladenosine
  modified_base 15: mod_base = OTHER; note = 2'-deoxy-2'-fluorocytidine
  modified_base 16: mod_base = cm
  modified_base 17: mod_base = OTHER; note = 2'-deoxy-2'-fluorouridine
  modified_base 18: mod_base = cm
  modified_base 19: mod_base = OTHER; note = 2'-deoxy-2'-fluorocytidine
  modified_base 20: mod_base = cm
  modified_base 21: mod_base = cm
  modified_base 22: mod_base = um
  modified_base 23: mod_base = OTHER; note = 2'-O,4'-C-methylene-briged guanosine
  modified_base 24: mod_base = um
  modified_base 1^2: mod_base = OTHER; note = phosphorotioate bond between nucleosides
  modified_base 2^3: mod_base = OTHER; note = phosphorothioate bond between nucleosides
  modified_base 3^4: mod_base = OTHER; note = phosphorothioate bond between nucleosides
  modified_base 4^5: mod_base = OTHER; note = phosphorothioate bond between nucleosides
  modified_base 5^6: mod_base = OTHER; note = phosphorothioate bond between nucleosides
  modified_base 7^8: mod_base = OTHER; note = phosphorothioate bond between nucleosides
  modified_base 6^7: mod_base = OTHER; note = phosphorothioate bond between nucleosides
  modified_base 8^9: mod_base = OTHER; note = phosphorothioate bond between nucleosides
  modified_base 9^10: mod_base = OTHER; note = phosphorothioate bond between nucleosides
  modified_base 10^11: mod_base = OTHER; note = phosphorothioate bond between nucleosides
  modified_base 11^12: mod_base = OTHER; note = methylphosphonate bond between nucleosides
  modified_base 12^13: mod_base = OTHER; note = phosphorothioate bond between nucleosides
  modified_base 13^14: mod_base = OTHER; note = phosphorothioate bond between nucleosides
  modified_base 14^15: mod_base = OTHER; note = methylphosphonate bond between nucleosides
  modified_base 15^16: mod_base = OTHER; note = phosphorothioate bond between nucleosides
  modified_base 16^17: mod_base = OTHER; note = phosphorothioate bond between nucleosides
  modified_base 17^18: mod_base = OTHER; note = phosphorothioate bond between nucleosides
  modified_base 18^19: mod_base = OTHER; note = phosphorothioate bond between nucleosides
  modified_base 19^20: mod_base = OTHER; note = phosphorothioate bond between nucleosides
  modified_base 20^21: mod_base = OTHER; note = phosphorothioate bond between nucleosides
  modified_base 21^22: mod_base = OTHER; note = phosphorothioate bond between nucleosides
  modified_base 22^23: mod_base = OTHER; note = phosphorothioate bond between nucleosides
  modified_base 23^24: mod_base = OTHER; note = phosphorothioate bond between nucleosides
aaagcatgccatcacctcccctgt

SEQ ID NO: 48 - RNA, 24 nt, synthetic construct
  source 1..24: mol_type = other RNA
  modified_base 1: mod_base = OTHER; note = 2'-O-methyladenosine
  modified_base 2: mod_base = OTHER; note = 2'-O,4'-C-methylene-briged adenosine
  modified_base 3: mod_base = OTHER; note = 2'-O-methyladenosine
  modified_base 4: mod_base = gm
  modified_base 5: mod_base = cm
  modified_base 6: mod_base = OTHER; note = 2'-deoxy-2'-fluoroadenosine
  modified_base 7: mod_base = OTHER; note = 2'-deoxy-2'-fluorouridine
  modified_base 8: mod_base = gm
  modified_base 9: mod_base = cm
  modified_base 10: mod_base = OTHER; note = 2'-deoxycytidine
  modified_base 11: mod_base = OTHER; note = 2'-deoxyadenosine
  modified_base 12: mod_base = um
  modified_base 13: mod_base = OTHER; note = 2'-deoxy-2'-fluorocytidine
  modified_base 14: mod_base = OTHER; note = 2'-O-methyladenosine
  modified_base 15: mod_base = OTHER; note = 2'-deoxy-2'-fluorocytidine
  modified_base 16: mod_base = cm
  modified_base 17: mod_base = OTHER; note = 2'-deoxy-2'-fluorouridine
  modified_base 18: mod_base = cm
  modified_base 19: mod_base = OTHER; note = 2'-deoxy-2'-fluorocytidine
  modified_base 20: mod_base = cm
  modified_base 21: mod_base = OTHER; note = 2'-O,4'-C-methylene-briged cytidine
  modified_base 22: mod_base = um
  modified_base 23: mod_base = OTHER; note = 2'-O,4'-C-methylene-briged guanosine
  modified_base 24: mod_base = um
  modified_base 1^2: mod_base = OTHER; note = phosphorotioate bond between nucleosides
  modified_base 2^3: mod_base = OTHER; note = phosphorothioate bond between nucleosides
  modified_base 3^4: mod_base = OTHER; note = phosphorothioate bond between nucleosides
  modified_base 4^5: mod_base = OTHER; note = phosphorothioate bond between nucleosides
  modified_base 5^6: mod_base = OTHER; note = phosphorothioate bond between nucleosides
  modified_base 7^8: mod_base = OTHER; note = phosphorothioate bond between nucleosides
  modified_base 6^7: mod_base = OTHER; note = phosphorothioate bond between nucleosides
  modified_base 8^9: mod_base = OTHER; note = phosphorothioate bond between nucleosides
  modified_base 9^10: mod_base = OTHER; note = phosphorothioate bond between nucleosides
  modified_base 10^11: mod_base = OTHER; note = phosphorothioate bond between nucleosides
  modified_base 11^12: mod_base = OTHER; note = methylphosphonate bond between nucleosides
  modified_base 12^13: mod_base = OTHER; note = phosphorothioate bond between nucleosides
  modified_base 13^14: mod_base = OTHER; note = phosphorothioate bond between nucleosides
  modified_base 14^15: mod_base = OTHER; note = methylphosphonate bond between nucleosides
  modified_base 15^16: mod_base = OTHER; note = phosphorothioate bond between nucleosides
  modified_base 16^17: mod_base = OTHER; note = phosphorothioate bond between nucleosides
  modified_base 17^18: mod_base = OTHER; note = phosphorothioate bond between nucleosides
  modified_base 18^19: mod_base = OTHER; note = phosphorothioate bond between nucleosides
  modified_base 19^20: mod_base = OTHER; note = phosphorothioate bond between nucleosides
  modified_base 20^21: mod_base = OTHER; note = phosphorothioate bond between nucleosides
  modified_base 21^22: mod_base = OTHER; note = phosphorothioate bond between nucleosides
  modified_base 22^23: mod_base = OTHER; note = phosphorothioate bond between nucleosides
  modified_base 23^24: mod_base = OTHER; note = phosphorothioate bond between nucleosides
aaagcatgccatcacctcccctgt

SEQ ID NO: 49 - RNA, 24 nt, synthetic construct
  source 1..24: mol_type = other RNA
  modified_base 1: mod_base = OTHER; note = 2'-O-methyladenosine
  modified_base 2: mod_base = OTHER; note = 2'-O,4'-C-methylene-briged adenosine
  modified_base 3: mod_base = OTHER; note = 2'-O-methyladenosine
  modified_base 4: mod_base = gm
  modified_base 5: mod_base = cm
  modified_base 6: mod_base = OTHER; note = 2'-deoxy-2'-fluoroadenosine
  modified_base 7: mod_base = OTHER; note = 2'-deoxy-2'-fluorouridine
  modified_base 8: mod_base = gm
  modified_base 9: mod_base = cm
  modified_base 10: mod_base = OTHER; note = 2'-deoxycytidine
  modified_base 11: mod_base = OTHER; note = 2'-deoxyadenosine
  modified_base 12: mod_base = um
  modified_base 13: mod_base = OTHER; note = 2'-deoxy-2'-fluorocytidine
  modified_base 14: mod_base = OTHER; note = 2'-O-methyladenosine
  modified_base 15: mod_base = OTHER; note = 2'-deoxy-2'-fluorocytidine
  modified_base 16: mod_base = cm
  modified_base 17: mod_base = OTHER; note = 2'-deoxy-2'-fluorouridine
  modified_base 18: mod_base = cm
  modified_base 19: mod_base = OTHER; note = 2'-deoxy-2'-fluorocytidine
  modified_base 20: mod_base = cm
  modified_base 21: mod_base = cm
  modified_base 22: mod_base = um
  modified_base 23: mod_base = OTHER; note = 2'-O,4'-C-methylene-briged guanosine
  modified_base 24: mod_base = um
  modified_base 1^2: mod_base = OTHER; note = phosphorotioate bond between nucleosides
  modified_base 2^3: mod_base = OTHER; note = phosphorothioate bond between nucleosides
  modified_base 3^4: mod_base = OTHER; note = phosphorothioate bond between nucleosides
  modified_base 4^5: mod_base = OTHER; note = phosphorothioate bond between nucleosides
  modified_base 5^6: mod_base = OTHER; note = phosphorothioate bond between nucleosides
  modified_base 7^8: mod_base = OTHER; note = phosphorothioate bond between nucleosides
  modified_base 6^7: mod_base = OTHER; note = phosphorothioate bond between nucleosides
  modified_base 8^9: mod_base = OTHER; note = phosphorothioate bond between nucleosides
  modified_base 9^10: mod_base = OTHER; note = phosphorothioate bond between nucleosides
  modified_base 10^11: mod_base = OTHER; note = phosphorothioate bond between nucleosides
  modified_base 11^12: mod_base = OTHER; note = methylphosphonate bond between nucleosides
  modified_base 12^13: mod_base = OTHER; note = phosphorothioate bond between nucleosides
  modified_base 13^14: mod_base = OTHER; note = phosphorothioate bond between nucleosides
  modified_base 14^15: mod_base = OTHER; note = methylphosphonate bond between nucleosides
  modified_base 15^16: mod_base = OTHER; note = phosphorothioate bond between nucleosides
  modified_base 16^17: mod_base = OTHER; note = phosphorothioate bond between nucleosides
  modified_base 17^18: mod_base = OTHER; note = phosphorothioate bond between nucleosides
  modified_base 18^19: mod_base = OTHER; note = phosphorothioate bond between nucleosides
  modified_base 19^20: mod_base = OTHER; note = phosphorothioate bond between nucleosides
  modified_base 20^21: mod_base = OTHER; note = phosphorothioate bond between nucleosides
  modified_base 21^22: mod_base = OTHER; note = phosphorothioate bond between nucleosides
  modified_base 22^23: mod_base = OTHER; note = phosphorothioate bond between nucleosides
  modified_base 23^24: mod_base = OTHER; note = phosphorothioate bond between nucleosides
aaagcatgccatcacctcccctgt

SEQ ID NO: 50 - RNA, 24 nt, synthetic construct
  source 1..24: mol_type = other RNA
  modified_base 1: mod_base = OTHER; note = 2'-O,4'-C-methylene-briged adenosine
  modified_base 2: mod_base = OTHER; note = 2'-O-methyladenosine
  modified_base 3: mod_base = OTHER; note = 2'-O-methyladenosine
  modified_base 4: mod_base = OTHER; note = 2'-O,4'-C-methylene-briged guanosine
  modified_base 5: mod_base = cm
  modified_base 6: mod_base = OTHER; note = 2'-deoxy-2'-fluoroadenosine
  modified_base 7: mod_base = OTHER; note = 2'-deoxy-2'-fluorouridine
  modified_base 8: mod_base = gm
  modified_base 9: mod_base = cm
  modified_base 10: mod_base = OTHER; note = 2'-deoxycytidine
  modified_base 11: mod_base = OTHER; note = 2'-deoxyadenosine
  modified_base 12: mod_base = um
  modified_base 13: mod_base = OTHER; note = 2'-deoxy-2'-fluorocytidine
  modified_base 14: mod_base = OTHER; note = 2'-O-methyladenosine
  modified_base 15: mod_base = OTHER; note = 2'-deoxy-2'-fluorocytidine
  modified_base 16: mod_base = cm
  modified_base 17: mod_base = OTHER; note = 2'-deoxy-2'-fluorouridine
  modified_base 18: mod_base = cm
  modified_base 19: mod_base = OTHER; note = 2'-deoxy-2'-fluorocytidine
  modified_base 20: mod_base = cm
  modified_base 21: mod_base = cm
  modified_base 22: mod_base = um
  modified_base 23: mod_base = OTHER; note = 2'-O,4'-C-methylene-briged guanosine
  modified_base 24: mod_base = um
  modified_base 1^2: mod_base = OTHER; note = phosphorotioate bond between nucleosides
  modified_base 2^3: mod_base = OTHER; note = phosphorothioate bond between nucleosides
  modified_base 3^4: mod_base = OTHER; note = phosphorothioate bond between nucleosides
  modified_base 4^5: mod_base = OTHER; note = phosphorothioate bond between nucleosides
  modified_base 5^6: mod_base = OTHER; note = phosphorothioate bond between nucleosides
  modified_base 7^8: mod_base = OTHER; note = phosphorothioate bond between nucleosides
  modified_base 6^7: mod_base = OTHER; note = phosphorothioate bond between nucleosides
  modified_base 8^9: mod_base = OTHER; note = phosphorothioate bond between nucleosides
  modified_base 9^10: mod_base = OTHER; note = phosphorothioate bond between nucleosides
  modified_base 10^11: mod_base = OTHER; note = phosphorothioate bond between nucleosides
  modified_base 11^12: mod_base = OTHER; note = methylphosphonate bond between nucleosides
  modified_base 12^13: mod_base = OTHER; note = phosphorothioate bond between nucleosides
  modified_base 13^14: mod_base = OTHER; note = phosphorothioate bond between nucleosides
  modified_base 14^15: mod_base = OTHER; note = methylphosphonate bond between nucleosides
  modified_base 15^16: mod_base = OTHER; note = phosphorothioate bond between nucleosides
  modified_base 16^17: mod_base = OTHER; note = phosphorothioate bond between nucleosides
  modified_base 17^18: mod_base = OTHER; note = phosphorothioate bond between nucleosides
  modified_base 18^19: mod_base = OTHER; note = phosphorothioate bond between nucleosides
  modified_base 19^20: mod_base = OTHER; note = phosphorothioate bond between nucleosides
  modified_base 20^21: mod_base = OTHER; note = phosphorothioate bond between nucleosides
  modified_base 21^22: mod_base = OTHER; note = phosphorothioate bond between nucleosides
  modified_base 22^23: mod_base = OTHER; note = phosphorothioate bond between nucleosides
  modified_base 23^24: mod_base = OTHER; note = phosphorothioate bond between nucleosides
aaagcatgccatcacctcccctgt

SEQ ID NO: 51 - RNA, 24 nt, synthetic construct
  source 1..24: mol_type = other RNA
  modified_base 1: mod_base = OTHER; note = 2'-O-methyladenosine
  modified_base 2: mod_base = OTHER; note = 2'-O-methyladenosine
  modified_base 3: mod_base = OTHER; note = 2'-O-methyladenosine
  modified_base 4: mod_base = OTHER; note = 2'-O,4'-C-methylene-briged guanosine
  modified_base 5: mod_base = cm
  modified_base 6: mod_base = OTHER; note = 2'-deoxy-2'-fluoroadenosine
  modified_base 7: mod_base = OTHER; note = 2'-deoxy-2'-fluorouridine
  modified_base 8: mod_base = gm
  modified_base 9: mod_base = cm
  modified_base 10: mod_base = OTHER; note = 2'-deoxycytidine
  modified_base 11: mod_base = OTHER; note = 2'-deoxyadenosine
  modified_base 12: mod_base = um
  modified_base 13: mod_base = OTHER; note = 2'-deoxy-2'-fluorocytidine
  modified_base 14: mod_base = OTHER; note = 2'-O-methyladenosine
  modified_base 15: mod_base = OTHER; note = 2'-deoxy-2'-fluorocytidine
  modified_base 16: mod_base = cm
  modified_base 17: mod_base = OTHER; note = 2'-deoxy-2'-fluorouridine
  modified_base 18: mod_base = cm
  modified_base 19: mod_base = OTHER; note = 2'-deoxy-2'-fluorocytidine
  modified_base 20: mod_base = cm
  modified_base 21: mod_base = cm
  modified_base 22: mod_base = um
  modified_base 23: mod_base = gm
  modified_base 24: mod_base = um
  modified_base 1^2: mod_base = OTHER; note = phosphorotioate bond between nucleosides
  modified_base 2^3: mod_base = OTHER; note = phosphorothioate bond between nucleosides
  modified_base 3^4: mod_base = OTHER; note = phosphorothioate bond between nucleosides
  modified_base 4^5: mod_base = OTHER; note = phosphorothioate bond between nucleosides
  modified_base 5^6: mod_base = OTHER; note = phosphorothioate bond between nucleosides
  modified_base 7^8: mod_base = OTHER; note = phosphorothioate bond between nucleosides
  modified_base 6^7: mod_base = OTHER; note = phosphorothioate bond between nucleosides
  modified_base 8^9: mod_base = OTHER; note = phosphorothioate bond between nucleosides
  modified_base 10^11: mod_base = OTHER; note = phosphorothioate bond between nucleosides
  modified_base 11^12: mod_base = OTHER; note = methylphosphonate bond between nucleosides
  modified_base 12^13: mod_base = OTHER; note = phosphorothioate bond between nucleosides
  modified_base 13^14: mod_base = OTHER; note = phosphorothioate bond between nucleosides
  modified_base 14^15: mod_base = OTHER; note = methylphosphonate bond between nucleosides
  modified_base 15^16: mod_base = OTHER; note = phosphorothioate bond between nucleosides
  modified_base 16^17: mod_base = OTHER; note = phosphorothioate bond between nucleosides
  modified_base 17^18: mod_base = OTHER; note = phosphorothioate bond between nucleosides
  modified_base 18^19: mod_base = OTHER; note = phosphorothioate bond between nucleosides
  modified_base 19^20: mod_base = OTHER; note = phosphorothioate bond between nucleosides
  modified_base 20^21: mod_base = OTHER; note = phosphorothioate bond between nucleosides
  modified_base 21^22: mod_base = OTHER; note = phosphorothioate bond between nucleosides
  modified_base 22^23: mod_base = OTHER; note = phosphorothioate bond between nucleosides
  modified_base 23^24: mod_base = OTHER; note = phosphorothioate bond between nucleosides
aaagcatgccatcacctcccctgt

SEQ ID NO: 52 - RNA, 24 nt, synthetic construct
  source 1..24: mol_type = other RNA
  modified_base 1: mod_base = OTHER; note = 2'-O-methyladenosine
  modified_base 2: mod_base = OTHER; note = 2'-O,4'-C-methylene-briged adenosine
  modified_base 3: mod_base = OTHER; note = 2'-O-methyladenosine
  modified_base 4: mod_base = OTHER; note = 2'-O,4'-C-methylene-briged guanosine
  modified_base 5: mod_base = cm
  modified_base 6: mod_base = OTHER; note = 2'-deoxy-2'-fluoroadenosine
  modified_base 7: mod_base = OTHER; note = 2'-deoxy-2'-fluorouridine
  modified_base 8: mod_base = gm
  modified_base 9: mod_base = cm
  modified_base 10: mod_base = OTHER; note = 2'-deoxycytidine
  modified_base 11: mod_base = OTHER; note = 2'-deoxyadenosine
  modified_base 12: mod_base = um
  modified_base 13: mod_base = OTHER; note = 2'-deoxy-2'-fluorocytidine
  modified_base 14: mod_base = OTHER; note = 2'-O-methyladenosine
  modified_base 15: mod_base = OTHER; note = 2'-deoxy-2'-fluorocytidine
  modified_base 16: mod_base = cm
  modified_base 17: mod_base = OTHER; note = 2'-deoxy-2'-fluorouridine
  modified_base 18: mod_base = cm
  modified_base 19: mod_base = OTHER; note = 2'-deoxy-2'-fluorocytidine
  modified_base 20: mod_base = cm
  modified_base 21: mod_base = OTHER; note = 2'-O,4'-C-methylene-briged cytidine
  modified_base 22: mod_base = um
  modified_base 23: mod_base = OTHER; note = 2'-O,4'-C-methylene-briged guanosine
  modified_base 24: mod_base = um
  modified_base 1^2: mod_base = OTHER; note = phosphorotioate bond between nucleosides
  modified_base 2^3: mod_base = OTHER; note = phosphorothioate bond between nucleosides
  modified_base 3^4: mod_base = OTHER; note = phosphorothioate bond between nucleosides
  modified_base 4^5: mod_base = OTHER; note = phosphorothioate bond between nucleosides
  modified_base 5^6: mod_base = OTHER; note = ethylphosphate bond between nucleosides
  modified_base 7^8: mod_base = OTHER; note = phosphorothioate bond between nucleosides
  modified_base 6^7: mod_base = OTHER; note = phosphorothioate bond between nucleosides
  modified_base 8^9: mod_base = OTHER; note = phosphorothioate bond between nucleosides
  modified_base 9^10: mod_base = OTHER; note = phosphorothioate bond between nucleosides
  modified_base 10^11: mod_base = OTHER; note = phosphorothioate bond between nucleosides
  modified_base 11^12: mod_base = OTHER; note = ethylphosphate bond between nucleosides
  modified_base 12^13: mod_base = OTHER; note = phosphorothioate bond between nucleosides
  modified_base 13^14: mod_base = OTHER; note = phosphorothioate bond between nucleosides
  modified_base 14^15: mod_base = OTHER; note = ethylphosphate bond between nucleosides
  modified_base 15^16: mod_base = OTHER; note = phosphorothioate bond between nucleosides
  modified_base 16^17: mod_base = OTHER; note = phosphorothioate bond between nucleosides
  modified_base 17^18: mod_base = OTHER; note = phosphorothioate bond between nucleosides
  modified_base 18^19: mod_base = OTHER; note = phosphorothioate bond between nucleosides
  modified_base 19^20: mod_base = OTHER; note = phosphorothioate bond between nucleosides
  modified_base 20^21: mod_base = OTHER; note = phosphorothioate bond between nucleosides
  modified_base 21^22: mod_base = OTHER; note = phosphorothioate bond between nucleosides
  modified_base 22^23: mod_base = OTHER; note = phosphorothioate bond between nucleosides
  modified_base 23^24: mod_base = OTHER; note = phosphorothioate bond between nucleosides
aaagcatgccatcacctcccctgt

SEQ ID NO: 53 - RNA, 24 nt, synthetic construct
  source 1..24: mol_type = other RNA
  modified_base 1: mod_base = OTHER; note = 2'-O-methyladenosine
  modified_base 2: mod_base = OTHER; note = 2'-O,4'-C-methylene-briged adenosine
  modified_base 3: mod_base = OTHER; note = 2'-O-methyladenosine
  modified_base 4: mod_base = OTHER; note = 2'-O,4'-C-methylene-briged guanosine
  modified_base 5: mod_base = cm
  modified_base 6: mod_base = OTHER; note = 2'-deoxy-2'-fluoroadenosine
  modified_base 7: mod_base = OTHER; note = 2'-deoxy-2'-fluorouridine
  modified_base 8: mod_base = gm
  modified_base 9: mod_base = cm
  modified_base 10: mod_base = OTHER; note = 2'-deoxycytidine
  modified_base 11: mod_base = OTHER; note = 2'-deoxyadenosine
  modified_base 12: mod_base = um
  modified_base 13: mod_base = OTHER; note = 2'-deoxy-2'-fluorocytidine
  modified_base 14: mod_base = OTHER; note = 2'-O-methyladenosine
  modified_base 15: mod_base = OTHER; note = 2'-deoxy-2'-fluorocytidine
  modified_base 16: mod_base = cm
  modified_base 17: mod_base = OTHER; note = 2'-deoxy-2'-fluorouridine
  modified_base 18: mod_base = cm
  modified_base 19: mod_base = OTHER; note = 2'-deoxy-2'-fluorocytidine
  modified_base 20: mod_base = cm
  modified_base 21: mod_base = OTHER; note = 2'-O,4'-C-methylene-briged cytidine
  modified_base 22: mod_base = um
  modified_base 23: mod_base = OTHER; note = 2'-O,4'-C-methylene-briged guanosine
  modified_base 24: mod_base = um
  modified_base 1^2: mod_base = OTHER; note = phosphorotioate bond between nucleosides
  modified_base 2^3: mod_base = OTHER; note = phosphorothioate bond between nucleosides
  modified_base 3^4: mod_base = OTHER; note = phosphorothioate bond between nucleosides
  modified_base 4^5: mod_base = OTHER; note = phosphorothioate bond between nucleosides
  modified_base 5^6: mod_base = OTHER; note = phosphorothioate bond between nucleosides
  modified_base 7^8: mod_base = OTHER; note = phosphorothioate bond between nucleosides
  modified_base 6^7: mod_base = OTHER; note = phosphorothioate bond between nucleosides
  modified_base 8^9: mod_base = OTHER; note = phosphorothioate bond between nucleosides
  modified_base 9^10: mod_base = OTHER; note = phosphorothioate bond between nucleosides
  modified_base 10^11: mod_base = OTHER; note = phosphorothioate bond between nucleosides
  modified_base 11^12: mod_base = OTHER; note = ethylphosphate bond between nucleosides
  modified_base 12^13: mod_base = OTHER; note = phosphorothioate bond between nucleosides
  modified_base 13^14: mod_base = OTHER; note = phosphorothioate bond between nucleosides
  modified_base 14^15: mod_base = OTHER; note = ethylphosphate bond between nucleosides
  modified_base 15^16: mod_base = OTHER; note = phosphorothioate bond between nucleosides
  modified_base 16^17: mod_base = OTHER; note = phosphorothioate bond between nucleosides
  modified_base 17^18: mod_base = OTHER; note = phosphorothioate bond between nucleosides
  modified_base 18^19: mod_base = OTHER; note = ethylphosphate bond between nucleosides
  modified_base 19^20: mod_base = OTHER; note = phosphorothioate bond between nucleosides
  modified_base 20^21: mod_base = OTHER; note = phosphorothioate bond between nucleosides
  modified_base 21^22: mod_base = OTHER; note = phosphorothioate bond between nucleosides
  modified_base 22^23: mod_base = OTHER; note = phosphorothioate bond between nucleosides
  modified_base 23^24: mod_base = OTHER; note = phosphorothioate bond between nucleosides
aaagcatgccatcacctcccctgt

SEQ ID NO: 54 - RNA, 24 nt, synthetic construct
  source 1..24: mol_type = other RNA
  modified_base 1: mod_base = OTHER; note = 2'-O-methyladenosine
  modified_base 2: mod_base = OTHER; note = 2'-O,4'-C-methylene-briged adenosine
  modified_base 3: mod_base = OTHER; note = 2'-O-methyladenosine
  modified_base 4: mod_base = OTHER; note = 2'-O,4'-C-methylene-briged guanosine
  modified_base 5: mod_base = cm
  modified_base 6: mod_base = OTHER; note = 2'-deoxy-2'-fluoroadenosine
  modified_base 7: mod_base = OTHER; note = 2'-deoxy-2'-fluorouridine
  modified_base 8: mod_base = gm
  modified_base 9: mod_base = cm
  modified_base 10: mod_base = OTHER; note = 2'-deoxycytidine
  modified_base 11: mod_base = OTHER; note = 2'-deoxyadenosine
  modified_base 12: mod_base = um
  modified_base 13: mod_base = OTHER; note = 2'-deoxy-2'-fluorocytidine
  modified_base 14: mod_base = OTHER; note = 2'-O-methyladenosine
  modified_base 15: mod_base = OTHER; note = 2'-deoxy-2'-fluorocytidine
  modified_base 16: mod_base = cm
  modified_base 17: mod_base = OTHER; note = 2'-deoxy-2'-fluorouridine
  modified_base 18: mod_base = cm
  modified_base 19: mod_base = OTHER; note = 2'-deoxy-2'-fluorocytidine
  modified_base 20: mod_base = cm
  modified_base 21: mod_base = OTHER; note = 2'-O,4'-C-methylene-briged cytidine
  modified_base 22: mod_base = um
  modified_base 23: mod_base = OTHER; note = 2'-O,4'-C-methylene-briged guanosine
  modified_base 24: mod_base = um
  modified_base 1^2: mod_base = OTHER; note = phosphorotioate bond between nucleosides
  modified_base 2^3: mod_base = OTHER; note = phosphorothioate bond between nucleosides
  modified_base 3^4: mod_base = OTHER; note = phosphorothioate bond between nucleosides
  modified_base 4^5: mod_base = OTHER; note = phosphorothioate bond between nucleosides
  modified_base 5^6: mod_base = OTHER; note = phosphorothioate bond between nucleosides
  modified_base 7^8: mod_base = OTHER; note = phosphorothioate bond between nucleosides
  modified_base 6^7: mod_base = OTHER; note = phosphorothioate bond between nucleosides
  modified_base 8^9: mod_base = OTHER; note = phosphorothioate bond between nucleosides
  modified_base 9^10: mod_base = OTHER; note = phosphorothioate bond between nucleosides
  modified_base 10^11: mod_base = OTHER; note = phosphorothioate bond between nucleosides
  modified_base 11^12: mod_base = OTHER; note = ethylphosphate bond between nucleosides
  modified_base 12^13: mod_base = OTHER; note = phosphorothioate bond between nucleosides
  modified_base 13^14: mod_base = OTHER; note = phosphorothioate bond between nucleosides
  modified_base 14^15: mod_base = OTHER; note = ethylphosphate bond between nucleosides
  modified_base 15^16: mod_base = OTHER; note = phosphorothioate bond between nucleosides
  modified_base 16^17: mod_base = OTHER; note = phosphorothioate bond between nucleosides
  modified_base 17^18: mod_base = OTHER; note = phosphorothioate bond between nucleosides
  modified_base 18^19: mod_base = OTHER; note = phosphorothioate bond between nucleosides
  modified_base 19^20: mod_base = OTHER; note = phosphorothioate bond between nucleosides
  modified_base 20^21: mod_base = OTHER; note = ethylphosphate bond between nucleosides
  modified_base 21^22: mod_base = OTHER; note = phosphorothioate bond between nucleosides
  modified_base 22^23: mod_base = OTHER; note = phosphorothioate bond between nucleosides
  modified_base 23^24: mod_base = OTHER; note = phosphorothioate bond between nucleosides
aaagcatgccatcacctcccctgt

SEQ ID NO: 55 - RNA, 24 nt, synthetic construct
  source 1..24: mol_type = other RNA
  modified_base 1: mod_base = OTHER; note = 2'-O-methyladenosine
  modified_base 2: mod_base = OTHER; note = 2'-O,4'-C-methylene-briged adenosine
  modified_base 3: mod_base = OTHER; note = 2'-O-methyladenosine
  modified_base 4: mod_base = OTHER; note = 2'-O,4'-C-methylene-briged guanosine
  modified_base 5: mod_base = cm
  modified_base 6: mod_base = OTHER; note = 2'-deoxy-2'-fluoroadenosine
  modified_base 7: mod_base = OTHER; note = 2'-deoxy-2'-fluorouridine
  modified_base 8: mod_base = gm
  modified_base 9: mod_base = cm
  modified_base 10: mod_base = OTHER; note = 2'-deoxycytidine
  modified_base 11: mod_base = OTHER; note = 2'-deoxyadenosine
  modified_base 12: mod_base = um
  modified_base 13: mod_base = OTHER; note = 2'-deoxy-2'-fluorocytidine
  modified_base 14: mod_base = OTHER; note = 2'-O-methyladenosine
  modified_base 15: mod_base = OTHER; note = 2'-deoxy-2'-fluorocytidine
  modified_base 16: mod_base = cm
  modified_base 17: mod_base = OTHER; note = 2'-deoxy-2'-fluorouridine
  modified_base 18: mod_base = cm
  modified_base 19: mod_base = OTHER; note = 2'-deoxy-2'-fluorocytidine
  modified_base 20: mod_base = cm
  modified_base 21: mod_base = OTHER; note = 2'-O,4'-C-methylene-briged cytidine
  modified_base 22: mod_base = um
  modified_base 23: mod_base = OTHER; note = 2'-O,4'-C-methylene-briged guanosine
  modified_base 24: mod_base = um
  modified_base 1^2: mod_base = OTHER; note = phosphorotioate bond between nucleosides
  modified_base 2^3: mod_base = OTHER; note = phosphorothioate bond between nucleosides
  modified_base 3^4: mod_base = OTHER; note = phosphorothioate bond between nucleosides
  modified_base 4^5: mod_base = OTHER; note = phosphorothioate bond between nucleosides
  modified_base 5^6: mod_base = OTHER; note = phosphorothioate bond between nucleosides
  modified_base 7^8: mod_base = OTHER; note = phosphorothioate bond between nucleosides
  modified_base 6^7: mod_base = OTHER; note = phosphorothioate bond between nucleosides
  modified_base 8^9: mod_base = OTHER; note = phosphorothioate bond between nucleosides
  modified_base 9^10: mod_base = OTHER; note = phosphorothioate bond between nucleosides
  modified_base 10^11: mod_base = OTHER; note = phosphorothioate bond between nucleosides
  modified_base 11^12: mod_base = OTHER; note = ethylphosphate bond between nucleosides
  modified_base 13^14: mod_base = OTHER; note = phosphorothioate bond between nucleosides
  modified_base 14^15: mod_base = OTHER; note = ethylphosphate bond between nucleosides
  modified_base 15^16: mod_base = OTHER; note = phosphorothioate bond between nucleosides
  modified_base 16^17: mod_base = OTHER; note = phosphorothioate bond between nucleosides
  modified_base 17^18: mod_base = OTHER; note = phosphorothioate bond between nucleosides
  modified_base 18^19: mod_base = OTHER; note = phosphorothioate bond between nucleosides
  modified_base 19^20: mod_base = OTHER; note = phosphorothioate bond between nucleosides
  modified_base 20^21: mod_base = OTHER; note = phosphorothioate bond between nucleosides
  modified_base 21^22: mod_base = OTHER; note = phosphorothioate bond between nucleosides
  modified_base 22^23: mod_base = OTHER; note = phosphorothioate bond between nucleosides
  modified_base 23^24: mod_base = OTHER; note = phosphorothioate bond between nucleosides
aaagcatgccatcacctcccctgt

SEQ ID NO: 56 - RNA, 24 nt, synthetic construct
  source 1..24: mol_type = other RNA
  modified_base 1: mod_base = OTHER; note = 2'-O-methyladenosine
  modified_base 2: mod_base = OTHER; note = 2'-O,4'-C-methylene-briged adenosine
  modified_base 3: mod_base = OTHER; note = 2'-O-methyladenosine
  modified_base 4: mod_base = OTHER; note = 2'-O,4'-C-methylene-briged guanosine
  modified_base 5: mod_base = cm
  modified_base 6: mod_base = OTHER; note = 2'-deoxy-2'-fluoroadenosine
  modified_base 7: mod_base = OTHER; note = 2'-deoxy-2'-fluorouridine
  modified_base 8: mod_base = gm
  modified_base 9: mod_base = cm
  modified_base 10: mod_base = OTHER; note = 2'-deoxycytidine
  modified_base 11: mod_base = OTHER; note = 2'-deoxyadenosine
  modified_base 12: mod_base = um
  modified_base 13: mod_base = OTHER; note = 2'-deoxy-2'-fluorocytidine
  modified_base 14: mod_base = OTHER; note = 2'-O-methyladenosine
  modified_base 15: mod_base = OTHER; note = 2'-deoxy-2'-fluorocytidine
  modified_base 16: mod_base = cm
  modified_base 17: mod_base = OTHER; note = 2'-deoxy-2'-fluorouridine
  modified_base 18: mod_base = cm
  modified_base 19: mod_base = OTHER; note = 2'-deoxy-2'-fluorocytidine
  modified_base 20: mod_base = cm
  modified_base 21: mod_base = OTHER; note = 2'-O,4'-C-methylene-briged cytidine
  modified_base 22: mod_base = um
  modified_base 23: mod_base = OTHER; note = 2'-O,4'-C-methylene-briged guanosine
  modified_base 24: mod_base = um
  modified_base 1^2: mod_base = OTHER; note = phosphorotioate bond between nucleosides
  modified_base 2^3: mod_base = OTHER; note = phosphorothioate bond between nucleosides
  modified_base 3^4: mod_base = OTHER; note = phosphorothioate bond between nucleosides
  modified_base 4^5: mod_base = OTHER; note = phosphorothioate bond between nucleosides
  modified_base 5^6: mod_base = OTHER; note = phosphorothioate bond between nucleosides
  modified_base 6^7: mod_base = OTHER; note = phosphorothioate bond between nucleosides
  modified_base 8^9: mod_base = OTHER; note = phosphorothioate bond between nucleosides
  modified_base 9^10: mod_base = OTHER; note = phosphorothioate bond between nucleosides
  modified_base 10^11: mod_base = OTHER; note = phosphorothioate bond between nucleosides
  modified_base 11^12: mod_base = OTHER; note = ethylphosphate bond between nucleosides
  modified_base 13^14: mod_base = OTHER; note = phosphorothioate bond between nucleosides
  modified_base 14^15: mod_base = OTHER; note = ethylphosphate bond between nucleosides
  modified_base 15^16: mod_base = OTHER; note = phosphorothioate bond between nucleosides
  modified_base 16^17: mod_base = OTHER; note = phosphorothioate bond between nucleosides
  modified_base 17^18: mod_base = OTHER; note = phosphorothioate bond between nucleosides
  modified_base 18^19: mod_base = OTHER; note = phosphorothioate bond between nucleosides
  modified_base 19^20: mod_base = OTHER; note = phosphorothioate bond between nucleosides
  modified_base 20^21: mod_base = OTHER; note = phosphorothioate bond between nucleosides
  modified_base 21^22: mod_base = OTHER; note = phosphorothioate bond between nucleosides
  modified_base 22^23: mod_base = OTHER; note = phosphorothioate bond between nucleosides
  modified_base 23^24: mod_base = OTHER; note = phosphorothioate bond between nucleosides
aaagcatgccatcacctcccctgt

SEQ ID NO: 57 - RNA, 24 nt, synthetic construct
  source 1..24: mol_type = other RNA
  modified_base 1: mod_base = OTHER; note = 2'-O-methyladenosine
  modified_base 2: mod_base = OTHER; note = 2'-O,4'-C-methylene-briged adenosine
  modified_base 3: mod_base = OTHER; note = 2'-O-methyladenosine
  modified_base 4: mod_base = OTHER; note = 2'-O,4'-C-methylene-briged guanosine
  modified_base 5: mod_base = cm
  modified_base 6: mod_base = OTHER; note = 2'-deoxy-2'-fluoroadenosine
  modified_base 7: mod_base = OTHER; note = 2'-deoxy-2'-fluorouridine
  modified_base 8: mod_base = gm
  modified_base 9: mod_base = cm
  modified_base 10: mod_base = OTHER; note = 2'-deoxycytidine
  modified_base 11: mod_base = OTHER; note = 2'-deoxyadenosine
  modified_base 12: mod_base = um
  modified_base 13: mod_base = OTHER; note = 2'-deoxy-2'-fluorocytidine
  modified_base 14: mod_base = OTHER; note = 2'-O-methyladenosine
  modified_base 15: mod_base = OTHER; note = 2'-deoxy-2'-fluorocytidine
  modified_base 16: mod_base = cm
  modified_base 17: mod_base = OTHER; note = 2'-deoxy-2'-fluorouridine
  modified_base 18: mod_base = cm
  modified_base 19: mod_base = OTHER; note = 2'-deoxy-2'-fluorocytidine
  modified_base 20: mod_base = cm
  modified_base 21: mod_base = OTHER; note = 2'-O,4'-C-methylene-briged cytidine
  modified_base 22: mod_base = um
  modified_base 23: mod_base = OTHER; note = 2'-O,4'-C-methylene-briged guanosine
  modified_base 24: mod_base = um
  modified_base 1^2: mod_base = OTHER; note = phosphorotioate bond between nucleosides
  modified_base 3^4: mod_base = OTHER; note = phosphorothioate bond between nucleosides
  modified_base 5^6: mod_base = OTHER; note = phosphorothioate bond between nucleosides
  modified_base 7^8: mod_base = OTHER; note = phosphorothioate bond between nucleosides
  modified_base 6^7: mod_base = OTHER; note = phosphorothioate bond between nucleosides
  modified_base 8^9: mod_base = OTHER; note = phosphorothioate bond between nucleosides
  modified_base 9^10: mod_base = OTHER; note = phosphorothioate bond between nucleosides
  modified_base 10^11: mod_base = OTHER; note = phosphorothioate bond between nucleosides
  modified_base 11^12: mod_base = OTHER; note = ethylphosphate bond between nucleosides
  modified_base 13^14: mod_base = OTHER; note = phosphorothioate bond between nucleosides
  modified_base 14^15: mod_base = OTHER; note = ethylphosphate bond between nucleosides
  modified_base 15^16: mod_base = OTHER; note = phosphorothioate bond between nucleosides
  modified_base 16^17: mod_base = OTHER; note = phosphorothioate bond between nucleosides
  modified_base 17^18: mod_base = OTHER; note = phosphorothioate bond between nucleosides
  modified_base 18^19: mod_base = OTHER; note = phosphorothioate bond between nucleosides
  modified_base 19^20: mod_base = OTHER; note = phosphorothioate bond between nucleosides
  modified_base 20^21: mod_base = OTHER; note = phosphorothioate bond between nucleosides
  modified_base 22^23: mod_base = OTHER; note = phosphorothioate bond between nucleosides
aaagcatgccatcacctcccctgt

SEQ ID NO: 58 - RNA, 24 nt, synthetic construct
  source 1..24: mol_type = other RNA
  modified_base 1: mod_base = OTHER; note = 2'-O-methyladenosine
  modified_base 2: mod_base = OTHER; note = 2'-O,4'-C-methylene-briged adenosine
  modified_base 3: mod_base = OTHER; note = 2'-O-methyladenosine
  modified_base 4: mod_base = OTHER; note = 2'-O,4'-C-methylene-briged guanosine
  modified_base 5: mod_base = cm
  modified_base 6: mod_base = OTHER; note = 2'-deoxy-2'-fluoroadenosine
  modified_base 7: mod_base = OTHER; note = 2'-deoxy-2'-fluorouridine
  modified_base 8: mod_base = gm
  modified_base 9: mod_base = cm
  modified_base 10: mod_base = OTHER; note = 2'-deoxycytidine
  modified_base 11: mod_base = OTHER; note = 2'-deoxyadenosine
  modified_base 12: mod_base = um
  modified_base 13: mod_base = OTHER; note = 2'-deoxy-2'-fluorocytidine
  modified_base 14: mod_base = OTHER; note = 2'-O-methyladenosine
  modified_base 15: mod_base = OTHER; note = 2'-deoxy-2'-fluorocytidine
  modified_base 16: mod_base = cm
  modified_base 17: mod_base = OTHER; note = 2'-deoxy-2'-fluorouridine
  modified_base 18: mod_base = cm
  modified_base 19: mod_base = OTHER; note = 2'-deoxy-2'-fluorocytidine
  modified_base 20: mod_base = cm
  modified_base 21: mod_base = OTHER; note = 2'-O,4'-C-methylene-briged cytidine
  modified_base 22: mod_base = um
  modified_base 23: mod_base = OTHER; note = 2'-O,4'-C-methylene-briged guanosine
  modified_base 24: mod_base = um
  modified_base 1^2: mod_base = OTHER; note = phosphorotioate bond between nucleosides
  modified_base 2^3: mod_base = OTHER; note = phosphorothioate bond between nucleosides
  modified_base 4^5: mod_base = OTHER; note = phosphorothioate bond between nucleosides
  modified_base 7^8: mod_base = OTHER; note = phosphorothioate bond between nucleosides
  modified_base 6^7: mod_base = OTHER; note = phosphorothioate bond between nucleosides
  modified_base 8^9: mod_base = OTHER; note = phosphorothioate bond between nucleosides
  modified_base 9^10: mod_base = OTHER; note = phosphorothioate bond between nucleosides
  modified_base 10^11: mod_base = OTHER; note = phosphorothioate bond between nucleosides
  modified_base 11^12: mod_base = OTHER; note = ethylphosphate bond between nucleosides
  modified_base 13^14: mod_base = OTHER; note = phosphorothioate bond between nucleosides
  modified_base 14^15: mod_base = OTHER; note = ethylphosphate bond between nucleosides
  modified_base 15^16: mod_base = OTHER; note = phosphorothioate bond between nucleosides
  modified_base 16^17: mod_base = OTHER; note = phosphorothioate bond between nucleosides
  modified_base 17^18: mod_base = OTHER; note = phosphorothioate bond between nucleosides
  modified_base 18^19: mod_base = OTHER; note = phosphorothioate bond between nucleosides
  modified_base 19^20: mod_base = OTHER; note = phosphorothioate bond between nucleosides
  modified_base 21^22: mod_base = OTHER; note = phosphorothioate bond between nucleosides
  modified_base 23^24: mod_base = OTHER; note = phosphorothioate bond between nucleosides
aaagcatgccatcacctcccctgt

SEQ ID NO: 59 - RNA, 24 nt, synthetic construct
  source 1..24: mol_type = other RNA
  modified_base 1: mod_base = OTHER; note = 2'-O-methyladenosine
  modified_base 2: mod_base = OTHER; note = 2'-O,4'-C-methylene-briged adenosine
  modified_base 3: mod_base = OTHER; note = 2'-O-methyladenosine
  modified_base 4: mod_base = OTHER; note = 2'-O,4'-C-methylene-briged guanosine
  modified_base 5: mod_base = cm
  modified_base 6: mod_base = OTHER; note = 2'-deoxy-2'-fluoroadenosine
  modified_base 7: mod_base = OTHER; note = 2'-deoxy-2'-fluorouridine
  modified_base 8: mod_base = gm
  modified_base 9: mod_base = cm
  modified_base 10: mod_base = OTHER; note = 2'-deoxycytidine
  modified_base 11: mod_base = OTHER; note = 2'-deoxyadenosine
  modified_base 12: mod_base = um
  modified_base 13: mod_base = OTHER; note = 2'-deoxy-2'-fluorocytidine
  modified_base 14: mod_base = OTHER; note = 2'-O-methyladenosine
  modified_base 15: mod_base = OTHER; note = 2'-deoxy-2'-fluorocytidine
  modified_base 16: mod_base = cm
  modified_base 17: mod_base = OTHER; note = 2'-deoxy-2'-fluorouridine
  modified_base 18: mod_base = cm
  modified_base 19: mod_base = OTHER; note = 2'-deoxy-2'-fluorocytidine
  modified_base 20: mod_base = cm
  modified_base 21: mod_base = OTHER; note = 2'-O,4'-C-methylene-briged cytidine
  modified_base 22: mod_base = um
  modified_base 23: mod_base = OTHER; note = 2'-O,4'-C-methylene-briged guanosine
  modified_base 24: mod_base = um
  modified_base 1^2: mod_base = OTHER; note = phosphorotioate bond between nucleosides
  modified_base 2^3: mod_base = OTHER; note = phosphorothioate bond between nucleosides
  modified_base 3^4: mod_base = OTHER; note = phosphorothioate bond between nucleosides
  modified_base 4^5: mod_base = OTHER; note = phosphorothioate bond between nucleosides
  modified_base 5^6: mod_base = OTHER; note = phosphorothioate bond between nucleosides
  modified_base 7^8: mod_base = OTHER; note = phosphorothioate bond between nucleosides
  modified_base 6^7: mod_base = OTHER; note = phosphorothioate bond between nucleosides
  modified_base 8^9: mod_base = OTHER; note = phosphorothioate bond between nucleosides
  modified_base 9^10: mod_base = OTHER; note = phosphorothioate bond between nucleosides
  modified_base 10^11: mod_base = OTHER; note = phosphorothioate bond between nucleosides
  modified_base 11^12: mod_base = OTHER; note = ethylphosphate bond between nucleosides
  modified_base 14^15: mod_base = OTHER; note = ethylphosphate bond between nucleosides
  modified_base 16^17: mod_base = OTHER; note = phosphorothioate bond between nucleosides
  modified_base 17^18: mod_base = OTHER; note = phosphorothioate bond between nucleosides
  modified_base 18^19: mod_base = OTHER; note = phosphorothioate bond between nucleosides
  modified_base 19^20: mod_base = OTHER; note = phosphorothioate bond between nucleosides
  modified_base 20^21: mod_base = OTHER; note = phosphorothioate bond between nucleosides
  modified_base 21^22: mod_base = OTHER; note = phosphorothioate bond between nucleosides
  modified_base 22^23: mod_base = OTHER; note = phosphorothioate bond between nucleosides
  modified_base 23^24: mod_base = OTHER; note = phosphorothioate bond between nucleosides
aaagcatgccatcacctcccctgt

SEQ ID NO: 60 - RNA, 24 nt, synthetic construct
  source 1..24: mol_type = other RNA
  modified_base 1: mod_base = OTHER; note = 2'-O-methyladenosine
  modified_base 2: mod_base = OTHER; note = 2'-O,4'-C-methylene-briged adenosine
  modified_base 3: mod_base = OTHER; note = 2'-O-methyladenosine
  modified_base 4: mod_base = OTHER; note = 2'-O,4'-C-methylene-briged guanosine
  modified_base 5: mod_base = cm
  modified_base 6: mod_base = OTHER; note = 2'-deoxy-2'-fluoroadenosine
  modified_base 7: mod_base = OTHER; note = 2'-deoxy-2'-fluorouridine
  modified_base 8: mod_base = gm
  modified_base 9: mod_base = cm
  modified_base 10: mod_base = OTHER; note = 2'-deoxycytidine
  modified_base 11: mod_base = OTHER; note = 2'-deoxyadenosine
  modified_base 12: mod_base = um
  modified_base 13: mod_base = OTHER; note = 2'-deoxy-2'-fluorocytidine
  modified_base 14: mod_base = OTHER; note = 2'-O-methyladenosine
  modified_base 15: mod_base = OTHER; note = 2'-deoxy-2'-fluorocytidine
  modified_base 16: mod_base = cm
  modified_base 17: mod_base = OTHER; note = 2'-deoxy-2'-fluorouridine
  modified_base 18: mod_base = cm
  modified_base 19: mod_base = OTHER; note = 2'-deoxy-2'-fluorocytidine
  modified_base 20: mod_base = cm
  modified_base 21: mod_base = OTHER; note = 2'-O,4'-C-methylene-briged cytidine
  modified_base 22: mod_base = um
  modified_base 23: mod_base = OTHER; note = 2'-O,4'-C-methylene-briged guanosine
  modified_base 24: mod_base = um
  modified_base 1^2: mod_base = OTHER; note = phosphorotioate bond between nucleosides
  modified_base 2^3: mod_base = OTHER; note = phosphorothioate bond between nucleosides
  modified_base 3^4: mod_base = OTHER; note = phosphorothioate bond between nucleosides
  modified_base 4^5: mod_base = OTHER; note = phosphorothioate bond between nucleosides
  modified_base 5^6: mod_base = OTHER; note = phosphorothioate bond between nucleosides
  modified_base 6^7: mod_base = OTHER; note = phosphorothioate bond between nucleosides
  modified_base 11^12: mod_base = OTHER; note = ethylphosphate bond between nucleosides
  modified_base 14^15: mod_base = OTHER; note = ethylphosphate bond between nucleosides
  modified_base 16^17: mod_base = OTHER; note = phosphorothioate bond between nucleosides
  modified_base 17^18: mod_base = OTHER; note = phosphorothioate bond between nucleosides
  modified_base 18^19: mod_base = OTHER; note = phosphorothioate bond between nucleosides
  modified_base 19^20: mod_base = OTHER; note = phosphorothioate bond between nucleosides
  modified_base 20^21: mod_base = OTHER; note = phosphorothioate bond between nucleosides
  modified_base 21^22: mod_base = OTHER; note = phosphorothioate bond between nucleosides
  modified_base 22^23: mod_base = OTHER; note = phosphorothioate bond between nucleosides
  modified_base 23^24: mod_base = OTHER; note = phosphorothioate bond between nucleosides
aaagcatgccatcacctcccctgt

SEQ ID NO: 61 - RNA, 24 nt, synthetic construct
  source 1..24: mol_type = other RNA
  modified_base 1: mod_base = OTHER; note = 2'-O-methyladenosine
  modified_base 2: mod_base = OTHER; note = 2'-O,4'-C-methylene-briged adenosine
  modified_base 3: mod_base = OTHER; note = 2'-O-methyladenosine
  modified_base 4: mod_base = OTHER; note = 2'-O,4'-C-methylene-briged guanosine
  modified_base 5: mod_base = cm
  modified_base 6: mod_base = OTHER; note = 2'-deoxy-2'-fluoroadenosine
  modified_base 7: mod_base = OTHER; note = 2'-deoxy-2'-fluorouridine
  modified_base 8: mod_base = gm
  modified_base 9: mod_base = cm
  modified_base 10: mod_base = OTHER; note = 2'-deoxycytidine
  modified_base 11: mod_base = OTHER; note = 2'-deoxyadenosine
  modified_base 12: mod_base = um
  modified_base 13: mod_base = OTHER; note = 2'-deoxy-2'-fluorocytidine
  modified_base 14: mod_base = OTHER; note = 2'-O-methyladenosine
  modified_base 15: mod_base = OTHER; note = 2'-deoxy-2'-fluorocytidine
  modified_base 16: mod_base = cm
  modified_base 17: mod_base = OTHER; note = 2'-deoxy-2'-fluorouridine
  modified_base 18: mod_base = cm
  modified_base 19: mod_base = OTHER; note = 2'-deoxy-2'-fluorocytidine
  modified_base 20: mod_base = cm
  modified_base 21: mod_base = OTHER; note = 2'-O,4'-C-methylene-briged cytidine
  modified_base 22: mod_base = um
  modified_base 23: mod_base = OTHER; note = 2'-O,4'-C-methylene-briged guanosine
  modified_base 24: mod_base = um
  modified_base 1^2: mod_base = OTHER; note = phosphorotioate bond between nucleosides
  modified_base 2^3: mod_base = OTHER; note = phosphorothioate bond between nucleosides
  modified_base 3^4: mod_base = OTHER; note = phosphorothioate bond between nucleosides
  modified_base 4^5: mod_base = OTHER; note = phosphorothioate bond between nucleosides
  modified_base 5^6: mod_base = OTHER; note = phosphorothioate bond between nucleosides
  modified_base 6^7: mod_base = OTHER; note = phosphorothioate bond between nucleosides
  modified_base 11^12: mod_base = OTHER; note = ethylphosphate bond between nucleosides
  modified_base 14^15: mod_base = OTHER; note = ethylphosphate bond between nucleosides
  modified_base 20^21: mod_base = OTHER; note = phosphorothioate bond between nucleosides
  modified_base 21^22: mod_base = OTHER; note = phosphorothioate bond between nucleosides
  modified_base 22^23: mod_base = OTHER; note = phosphorothioate bond between nucleosides
  modified_base 23^24: mod_base = OTHER; note = phosphorothioate bond between nucleosides
aaagcatgccatcacctcccctgt

SEQ ID NO: 62 - RNA, 24 nt, synthetic construct
  source 1..24: mol_type = other RNA
  modified_base 1: mod_base = OTHER; note = 2'-O-methyladenosine
  modified_base 2: mod_base = OTHER; note = 2'-O,4'-C-methylene-briged adenosine
  modified_base 3: mod_base = OTHER; note = 2'-O-methyladenosine
  modified_base 4: mod_base = OTHER; note = 2'-O,4'-C-methylene-briged guanosine
  modified_base 5: mod_base = cm
  modified_base 6: mod_base = OTHER; note = 2'-deoxy-2'-fluoroadenosine
  modified_base 7: mod_base = OTHER; note = 2'-deoxy-2'-fluorouridine
  modified_base 8: mod_base = gm
  modified_base 9: mod_base = cm
  modified_base 10: mod_base = OTHER; note = 2'-deoxycytidine
  modified_base 11: mod_base = OTHER; note = 2'-deoxyadenosine
  modified_base 12: mod_base = um
  modified_base 13: mod_base = OTHER; note = 2'-deoxy-2'-fluorocytidine
  modified_base 14: mod_base = OTHER; note = 2'-O-methyladenosine
  modified_base 15: mod_base = OTHER; note = 2'-deoxy-2'-fluorocytidine
  modified_base 16: mod_base = cm
  modified_base 17: mod_base = OTHER; note = 2'-deoxy-2'-fluorouridine
  modified_base 18: mod_base = cm
  modified_base 19: mod_base = OTHER; note = 2'-deoxy-2'-fluorocytidine
  modified_base 20: mod_base = cm
  modified_base 21: mod_base = OTHER; note = 2'-O,4'-C-methylene-briged cytidine
  modified_base 22: mod_base = um
  modified_base 23: mod_base = OTHER; note = 2'-O,4'-C-methylene-briged guanosine
  modified_base 24: mod_base = um
  modified_base 11^12: mod_base = OTHER; note = ethylphosphate bond between nucleosides
  modified_base 14^15: mod_base = OTHER; note = ethylphosphate bond between nucleosides
aaagcatgccatcacctcccctgt

SEQ ID NO: 63 - RNA, 24 nt, synthetic construct
  source 1..24: mol_type = other RNA
  modified_base 1: mod_base = OTHER; note = 2'-O-methyladenosine
  modified_base 2: mod_base = OTHER; note = 2'-O,4'-C-methylene-briged adenosine
  modified_base 3: mod_base = OTHER; note = 2'-O-methyladenosine
  modified_base 4: mod_base = OTHER; note = 2'-O,4'-C-methylene-briged guanosine
  modified_base 5: mod_base = cm
  modified_base 6: mod_base = OTHER; note = 2'-deoxy-2'-fluoroadenosine
  modified_base 7: mod_base = OTHER; note = 2'-deoxy-2'-fluorouridine
  modified_base 8: mod_base = gm
  modified_base 9: mod_base = cm
  modified_base 10: mod_base = OTHER; note = 2'-deoxycytidine
  modified_base 11: mod_base = OTHER; note = 2'-deoxyadenosine
  modified_base 12: mod_base = um
  modified_base 13: mod_base = OTHER; note = 2'-deoxy-2'-fluorocytidine
  modified_base 14: mod_base = OTHER; note = 2'-O-methyladenosine
  modified_base 15: mod_base = OTHER; note = 2'-deoxy-2'-fluorocytidine
  modified_base 16: mod_base = cm
  modified_base 17: mod_base = OTHER; note = 2'-deoxy-2'-fluorouridine
  modified_base 18: mod_base = cm
  modified_base 19: mod_base = OTHER; note = 2'-deoxy-2'-fluorocytidine
  modified_base 20: mod_base = cm
  modified_base 21: mod_base = OTHER; note = 2'-O,4'-C-methylene-briged cytidine
  modified_base 22: mod_base = um
  modified_base 23: mod_base = OTHER; note = 2'-O,4'-C-methylene-briged guanosine
  modified_base 24: mod_base = um
  modified_base 1^2: mod_base = OTHER; note = phosphorotioate bond between nucleosides
  modified_base 2^3: mod_base = OTHER; note = phosphorothioate bond between nucleosides
  modified_base 3^4: mod_base = OTHER; note = phosphorothioate bond between nucleosides
  modified_base 4^5: mod_base = OTHER; note = phosphorothioate bond between nucleosides
  modified_base 5^6: mod_base = OTHER; note = phosphorothioate bond between nucleosides
  modified_base 7^8: mod_base = OTHER; note = phosphorothioate bond between nucleosides
  modified_base 6^7: mod_base = OTHER; note = phosphorothioate bond between nucleosides
  modified_base 8^9: mod_base = OTHER; note = phosphorothioate bond between nucleosides
  modified_base 9^10: mod_base = OTHER; note = phosphorothioate bond between nucleosides
  modified_base 10^11: mod_base = OTHER; note = phosphorothioate bond between nucleosides
  modified_base 11^12: mod_base = OTHER; note = phosphorothioate bond between nucleosides
  modified_base 12^13: mod_base = OTHER; note = phosphorothioate bond between nucleosides
  modified_base 13^14: mod_base = OTHER; note = phosphorothioate bond between nucleosides
  modified_base 14^15: mod_base = OTHER; note = ethylphosphonate bond between nucleosides
  modified_base 15^16: mod_base = OTHER; note = phosphorothioate bond between nucleosides
  modified_base 16^17: mod_base = OTHER; note = phosphorothioate bond between nucleosides
  modified_base 17^18: mod_base = OTHER; note = phosphorothioate bond between nucleosides
  modified_base 18^19: mod_base = OTHER; note = phosphorothioate bond between nucleosides
  modified_base 19^20: mod_base = OTHER; note = phosphorothioate bond between nucleosides
  modified_base 20^21: mod_base = OTHER; note = phosphorothioate bond between nucleosides
  modified_base 21^22: mod_base = OTHER; note = phosphorothioate bond between nucleosides
  modified_base 22^23: mod_base = OTHER; note = phosphorothioate bond between nucleosides
  modified_base 23^24: mod_base = OTHER; note = phosphorothioate bond between nucleosides
aaagcatgccatcacctcccctgt

SEQ ID NO: 64 - RNA, 24 nt, synthetic construct
  source 1..24: mol_type = other RNA
  modified_base 1: mod_base = OTHER; note = 2'-O-methyladenosine
  modified_base 2: mod_base = OTHER; note = 2'-O,4'-C-methylene-briged adenosine
  modified_base 3: mod_base = OTHER; note = 2'-O-methyladenosine
  modified_base 4: mod_base = OTHER; note = 2'-O,4'-C-methylene-briged guanosine
  modified_base 5: mod_base = cm
  modified_base 6: mod_base = OTHER; note = 2'-deoxy-2'-fluoroadenosine
  modified_base 7: mod_base = OTHER; note = 2'-deoxy-2'-fluorouridine
  modified_base 8: mod_base = gm
  modified_base 9: mod_base = cm
  modified_base 10: mod_base = OTHER; note = 2'-deoxycytidine
  modified_base 11: mod_base = OTHER; note = 2'-deoxyadenosine
  modified_base 12: mod_base = um
  modified_base 13: mod_base = OTHER; note = 2'-deoxy-2'-fluorocytidine
  modified_base 14: mod_base = OTHER; note = 2'-O-methyladenosine
  modified_base 15: mod_base = OTHER; note = 2'-deoxy-2'-fluorocytidine
  modified_base 16: mod_base = cm
  modified_base 17: mod_base = OTHER; note = 2'-deoxy-2'-fluorouridine
  modified_base 18: mod_base = cm
  modified_base 19: mod_base = OTHER; note = 2'-deoxy-2'-fluorocytidine
  modified_base 20: mod_base = cm
  modified_base 21: mod_base = OTHER; note = 2'-O,4'-C-methylene-briged cytidine
  modified_base 22: mod_base = um
  modified_base 23: mod_base = OTHER; note = 2'-O,4'-C-methylene-briged guanosine
  modified_base 24: mod_base = um
  modified_base 1^2: mod_base = OTHER; note = phosphorotioate bond between nucleosides
  modified_base 2^3: mod_base = OTHER; note = phosphorothioate bond between nucleosides
  modified_base 3^4: mod_base = OTHER; note = phosphorothioate bond between nucleosides
  modified_base 4^5: mod_base = OTHER; note = phosphorothioate bond between nucleosides
  modified_base 5^6: mod_base = OTHER; note = phosphorothioate bond between nucleosides
  modified_base 7^8: mod_base = OTHER; note = phosphorothioate bond between nucleosides
  modified_base 6^7: mod_base = OTHER; note = phosphorothioate bond between nucleosides
  modified_base 8^9: mod_base = OTHER; note = phosphorothioate bond between nucleosides
  modified_base 9^10: mod_base = OTHER; note = phosphorothioate bond between nucleosides
  modified_base 10^11: mod_base = OTHER; note = phosphorothioate bond between nucleosides
  modified_base 11^12: mod_base = OTHER; note = phosphorothioate bond between nucleosides
  modified_base 12^13: mod_base = OTHER; note = phosphorothioate bond between nucleosides
  modified_base 13^14: mod_base = OTHER; note = phosphorothioate bond between nucleosides
  modified_base 14^15: mod_base = OTHER; note = propylphosphonate bond between nucleosides
  modified_base 15^16: mod_base = OTHER; note = phosphorothioate bond between nucleosides
  modified_base 16^17: mod_base = OTHER; note = phosphorothioate bond between nucleosides
  modified_base 17^18: mod_base = OTHER; note = phosphorothioate bond between nucleosides
  modified_base 18^19: mod_base = OTHER; note = phosphorothioate bond between nucleosides
  modified_base 19^20: mod_base = OTHER; note = phosphorothioate bond between nucleosides
  modified_base 20^21: mod_base = OTHER; note = phosphorothioate bond between nucleosides
  modified_base 21^22: mod_base = OTHER; note = phosphorothioate bond between nucleosides
  modified_base 22^23: mod_base = OTHER; note = phosphorothioate bond between nucleosides
  modified_base 23^24: mod_base = OTHER; note = phosphorothioate bond between nucleosides
aaagcatgccatcacctcccctgt

SEQ ID NO: 65 - RNA, 24 nt, synthetic construct
  source 1..24: mol_type = other RNA
  modified_base 1: mod_base = OTHER; note = 2'-O-methyladenosine
  modified_base 2: mod_base = OTHER; note = 2'-O,4'-C-methylene-briged adenosine
  modified_base 3: mod_base = OTHER; note = 2'-O-methyladenosine
  modified_base 4: mod_base = OTHER; note = 2'-O,4'-C-methylene-briged guanosine
  modified_base 5: mod_base = cm
  modified_base 6: mod_base = OTHER; note = 2'-deoxy-2'-fluoroadenosine
  modified_base 7: mod_base = OTHER; note = 2'-deoxy-2'-fluorouridine
  modified_base 8: mod_base = gm
  modified_base 9: mod_base = cm
  modified_base 10: mod_base = OTHER; note = 2'-deoxycytidine
  modified_base 11: mod_base = OTHER; note = 2'-deoxyadenosine
  modified_base 12: mod_base = um
  modified_base 13: mod_base = OTHER; note = 2'-deoxy-2'-fluorocytidine
  modified_base 14: mod_base = OTHER; note = 2'-O-methyladenosine
  modified_base 15: mod_base = OTHER; note = 2'-deoxy-2'-fluorocytidine
  modified_base 16: mod_base = cm
  modified_base 17: mod_base = OTHER; note = 2'-deoxy-2'-fluorouridine
  modified_base 18: mod_base = cm
  modified_base 19: mod_base = OTHER; note = 2'-deoxy-2'-fluorocytidine
  modified_base 20: mod_base = cm
  modified_base 21: mod_base = OTHER; note = 2'-O,4'-C-methylene-briged cytidine
  modified_base 22: mod_base = um
  modified_base 23: mod_base = OTHER; note = 2'-O,4'-C-methylene-briged guanosine
  modified_base 24: mod_base = um
  modified_base 1^2: mod_base = OTHER; note = phosphorotioate bond between nucleosides
  modified_base 2^3: mod_base = OTHER; note = phosphorothioate bond between nucleosides
  modified_base 3^4: mod_base = OTHER; note = phosphorothioate bond between nucleosides
  modified_base 4^5: mod_base = OTHER; note = phosphorothioate bond between nucleosides
  modified_base 5^6: mod_base = OTHER; note = phosphorothioate bond between nucleosides
  modified_base 7^8: mod_base = OTHER; note = phosphorothioate bond between nucleosides
  modified_base 6^7: mod_base = OTHER; note = phosphorothioate bond between nucleosides
  modified_base 8^9: mod_base = OTHER; note = phosphorothioate bond between nucleosides
  modified_base 9^10: mod_base = OTHER; note = phosphorothioate bond between nucleosides
  modified_base 10^11: mod_base = OTHER; note = phosphorothioate bond between nucleosides
  modified_base 11^12: mod_base = OTHER; note = phosphorothioate bond between nucleosides
  modified_base 12^13: mod_base = OTHER; note = phosphorothioate bond between nucleosides
  modified_base 13^14: mod_base = OTHER; note = phosphorothioate bond between nucleosides
  modified_base 14^15: mod_base = OTHER; note = isopropylphosphonate bond between nucleosides
  modified_base 15^16: mod_base = OTHER; note = phosphorothioate bond between nucleosides
  modified_base 16^17: mod_base = OTHER; note = phosphorothioate bond between nucleosides
  modified_base 17^18: mod_base = OTHER; note = phosphorothioate bond between nucleosides
  modified_base 18^19: mod_base = OTHER; note = phosphorothioate bond between nucleosides
  modified_base 19^20: mod_base = OTHER; note = phosphorothioate bond between nucleosides
  modified_base 20^21: mod_base = OTHER; note = phosphorothioate bond between nucleosides
  modified_base 21^22: mod_base = OTHER; note = phosphorothioate bond between nucleosides
  modified_base 22^23: mod_base = OTHER; note = phosphorothioate bond between nucleosides
  modified_base 23^24: mod_base = OTHER; note = phosphorothioate bond between nucleosides
aaagcatgccatcacctcccctgt

SEQ ID NO: 66 - RNA, 24 nt, synthetic construct
  source 1..24: mol_type = other RNA
  modified_base 1: mod_base = OTHER; note = 2'-O-methyladenosine
  modified_base 2: mod_base = OTHER; note = 2'-O,4'-C-methylene-briged adenosine
  modified_base 3: mod_base = OTHER; note = 2'-O-methyladenosine
  modified_base 4: mod_base = OTHER; note = 2'-O,4'-C-methylene-briged guanosine
  modified_base 5: mod_base = cm
  modified_base 6: mod_base = OTHER; note = 2'-deoxy-2'-fluoroadenosine
  modified_base 7: mod_base = OTHER; note = 2'-deoxy-2'-fluorouridine
  modified_base 8: mod_base = gm
  modified_base 9: mod_base = cm
  modified_base 10: mod_base = OTHER; note = 2'-deoxycytidine
  modified_base 11: mod_base = OTHER; note = 2'-deoxyadenosine
  modified_base 12: mod_base = um
  modified_base 13: mod_base = OTHER; note = 2'-deoxy-2'-fluorocytidine
  modified_base 14: mod_base = OTHER; note = 2'-O-methyladenosine
  modified_base 15: mod_base = OTHER; note = 2'-deoxy-2'-fluorocytidine
  modified_base 16: mod_base = cm
  modified_base 17: mod_base = OTHER; note = 2'-deoxy-2'-fluorouridine
  modified_base 18: mod_base = cm
  modified_base 19: mod_base = OTHER; note = 2'-deoxy-2'-fluorocytidine
  modified_base 20: mod_base = cm
  modified_base 21: mod_base = OTHER; note = 2'-O,4'-C-methylene-briged cytidine
  modified_base 22: mod_base = um
  modified_base 23: mod_base = OTHER; note = 2'-O,4'-C-methylene-briged guanosine
  modified_base 24: mod_base = um
  modified_base 1^2: mod_base = OTHER; note = phosphorotioate bond between nucleosides
  modified_base 2^3: mod_base = OTHER; note = phosphorothioate bond between nucleosides
  modified_base 3^4: mod_base = OTHER; note = phosphorothioate bond between nucleosides
  modified_base 4^5: mod_base = OTHER; note = phosphorothioate bond between nucleosides
  modified_base 5^6: mod_base = OTHER; note = phosphorothioate bond between nucleosides
  modified_base 7^8: mod_base = OTHER; note = phosphorothioate bond between nucleosides
  modified_base 6^7: mod_base = OTHER; note = phosphorothioate bond between nucleosides
  modified_base 8^9: mod_base = OTHER; note = phosphorothioate bond between nucleosides
  modified_base 9^10: mod_base = OTHER; note = phosphorothioate bond between nucleosides
  modified_base 10^11: mod_base = OTHER; note = phosphorothioate bond between nucleosides
  modified_base 11^12: mod_base = OTHER; note = phosphorothioate bond between nucleosides
  modified_base 12^13: mod_base = OTHER; note = phosphorothioate bond between nucleosides
  modified_base 13^14: mod_base = OTHER; note = phosphorothioate bond between nucleosides
  modified_base 14^15: mod_base = OTHER; note = butylphosphonate bond between nucleosides
  modified_base 15^16: mod_base = OTHER; note = phosphorothioate bond between nucleosides
  modified_base 16^17: mod_base = OTHER; note = phosphorothioate bond between nucleosides
  modified_base 17^18: mod_base = OTHER; note = phosphorothioate bond between nucleosides
  modified_base 18^19: mod_base = OTHER; note = phosphorothioate bond between nucleosides
  modified_base 19^20: mod_base = OTHER; note = phosphorothioate bond between nucleosides
  modified_base 20^21: mod_base = OTHER; note = phosphorothioate bond between nucleosides
  modified_base 21^22: mod_base = OTHER; note = phosphorothioate bond between nucleosides
  modified_base 22^23: mod_base = OTHER; note = phosphorothioate bond between nucleosides
  modified_base 23^24: mod_base = OTHER; note = phosphorothioate bond between nucleosides
aaagcatgccatcacctcccctgt

SEQ ID NO: 67 - RNA, 24 nt, synthetic construct
  source 1..24: mol_type = other RNA
  modified_base 1: mod_base = OTHER; note = 2'-O-methyladenosine
  modified_base 2: mod_base = OTHER; note = 2'-O,4'-C-methylene-briged adenosine
  modified_base 3: mod_base = OTHER; note = 2'-O-methyladenosine
  modified_base 4: mod_base = OTHER; note = 2'-O,4'-C-methylene-briged guanosine
  modified_base 5: mod_base = cm
  modified_base 6: mod_base = OTHER; note = 2'-deoxy-2'-fluoroadenosine
  modified_base 7: mod_base = OTHER; note = 2'-deoxy-2'-fluorouridine
  modified_base 8: mod_base = gm
  modified_base 9: mod_base = cm
  modified_base 10: mod_base = OTHER; note = 2'-deoxycytidine
  modified_base 11: mod_base = OTHER; note = 2'-deoxyadenosine
  modified_base 12: mod_base = um
  modified_base 13: mod_base = OTHER; note = 2'-deoxy-2'-fluorocytidine
  modified_base 14: mod_base = OTHER; note = 2'-O-methyladenosine
  modified_base 15: mod_base = OTHER; note = 2'-deoxy-2'-fluorocytidine
  modified_base 16: mod_base = cm
  modified_base 17: mod_base = OTHER; note = 2'-deoxy-2'-fluorouridine
  modified_base 18: mod_base = cm
  modified_base 19: mod_base = OTHER; note = 2'-deoxy-2'-fluorocytidine
  modified_base 20: mod_base = cm
  modified_base 21: mod_base = OTHER; note = 2'-O,4'-C-methylene-briged cytidine
  modified_base 22: mod_base = um
  modified_base 23: mod_base = OTHER; note = 2'-O,4'-C-methylene-briged guanosine
  modified_base 24: mod_base = um
  modified_base 1^2: mod_base = OTHER; note = phosphorotioate bond between nucleosides
  modified_base 2^3: mod_base = OTHER; note = phosphorothioate bond between nucleosides
  modified_base 3^4: mod_base = OTHER; note = phosphorothioate bond between nucleosides
  modified_base 4^5: mod_base = OTHER; note = phosphorothioate bond between nucleosides
  modified_base 5^6: mod_base = OTHER; note = phosphorothioate bond between nucleosides
  modified_base 7^8: mod_base = OTHER; note = phosphorothioate bond between nucleosides
  modified_base 6^7: mod_base = OTHER; note = phosphorothioate bond between nucleosides
  modified_base 8^9: mod_base = OTHER; note = phosphorothioate bond between nucleosides
  modified_base 9^10: mod_base = OTHER; note = phosphorothioate bond between nucleosides
  modified_base 10^11: mod_base = OTHER; note = phosphorothioate bond between nucleosides
  modified_base 11^12: mod_base = OTHER; note = phosphorothioate bond between nucleosides
  modified_base 12^13: mod_base = OTHER; note = phosphorothioate bond between nucleosides
  modified_base 13^14: mod_base = OTHER; note = phosphorothioate bond between nucleosides
  modified_base 14^15: mod_base = OTHER; note = methoxypropylphosphonate bond between nucleosides
  modified_base 15^16: mod_base = OTHER; note = phosphorothioate bond between nucleosides
  modified_base 16^17: mod_base = OTHER; note = phosphorothioate bond between nucleosides
  modified_base 17^18: mod_base = OTHER; note = phosphorothioate bond between nucleosides
  modified_base 18^19: mod_base = OTHER; note = phosphorothioate bond between nucleosides
  modified_base 19^20: mod_base = OTHER; note = phosphorothioate bond between nucleosides
  modified_base 20^21: mod_base = OTHER; note = phosphorothioate bond between nucleosides
  modified_base 21^22: mod_base = OTHER; note = phosphorothioate bond between nucleosides
  modified_base 22^23: mod_base = OTHER; note = phosphorothioate bond between nucleosides
  modified_base 23^24: mod_base = OTHER; note = phosphorothioate bond between nucleosides
aaagcatgccatcacctcccctgt

SEQ ID NO: 68 - RNA, 24 nt, synthetic construct
  source 1..24: mol_type = other RNA
  modified_base 1: mod_base = OTHER; note = 2'-O-methyladenosine
  modified_base 2: mod_base = OTHER; note = 2'-O,4'-C-methylene-briged adenosine
  modified_base 3: mod_base = OTHER; note = 2'-O-methyladenosine
  modified_base 4: mod_base = OTHER; note = 2'-O,4'-C-methylene-briged guanosine
  modified_base 5: mod_base = cm
  modified_base 6: mod_base = OTHER; note = 2'-deoxy-2'-fluoroadenosine
  modified_base 7: mod_base = OTHER; note = 2'-deoxy-2'-fluorouridine
  modified_base 8: mod_base = gm
  modified_base 9: mod_base = cm
  modified_base 10: mod_base = OTHER; note = 2'-deoxycytidine
  modified_base 11: mod_base = OTHER; note = 2'-deoxyadenosine
  modified_base 12: mod_base = um
  modified_base 13: mod_base = OTHER; note = 2'-deoxy-2'-fluorocytidine
  modified_base 14: mod_base = OTHER; note = 2'-O-methyladenosine
  modified_base 15: mod_base = OTHER; note = 2'-deoxy-2'-fluorocytidine
  modified_base 16: mod_base = cm
  modified_base 17: mod_base = OTHER; note = 2'-deoxy-2'-fluorouridine
  modified_base 18: mod_base = cm
  modified_base 19: mod_base = OTHER; note = 2'-deoxy-2'-fluorocytidine
  modified_base 20: mod_base = cm
  modified_base 21: mod_base = OTHER; note = 2'-O,4'-C-methylene-briged cytidine
  modified_base 22: mod_base = um
  modified_base 23: mod_base = OTHER; note = 2'-O,4'-C-methylene-briged guanosine
  modified_base 24: mod_base = um
  modified_base 1^2: mod_base = OTHER; note = phosphorotioate bond between nucleosides
  modified_base 2^3: mod_base = OTHER; note = phosphorothioate bond between nucleosides
  modified_base 3^4: mod_base = OTHER; note = phosphorothioate bond between nucleosides
  modified_base 4^5: mod_base = OTHER; note = phosphorothioate bond between nucleosides
  modified_base 5^6: mod_base = OTHER; note = phosphorothioate bond between nucleosides
  modified_base 7^8: mod_base = OTHER; note = phosphorothioate bond between nucleosides
  modified_base 6^7: mod_base = OTHER; note = phosphorothioate bond between nucleosides
  modified_base 8^9: mod_base = OTHER; note = phosphorothioate bond between nucleosides
  modified_base 9^10: mod_base = OTHER; note = phosphorothioate bond between nucleosides
  modified_base 10^11: mod_base = OTHER; note = phosphorothioate bond between nucleosides
  modified_base 11^12: mod_base = OTHER; note = butylphosphonate bond between nucleosides
  modified_base 12^13: mod_base = OTHER; note = phosphorothioate bond between nucleosides
  modified_base 13^14: mod_base = OTHER; note = phosphorothioate bond between nucleosides
  modified_base 14^15: mod_base = OTHER; note = phosphorohioate bond between nucleosides
  modified_base 15^16: mod_base = OTHER; note = phosphorothioate bond between nucleosides
  modified_base 16^17: mod_base = OTHER; note = phosphorothioate bond between nucleosides
  modified_base 17^18: mod_base = OTHER; note = phosphorothioate bond between nucleosides
  modified_base 18^19: mod_base = OTHER; note = phosphorothioate bond between nucleosides
  modified_base 19^20: mod_base = OTHER; note = phosphorothioate bond between nucleosides
  modified_base 20^21: mod_base = OTHER; note = phosphorothioate bond between nucleosides
  modified_base 21^22: mod_base = OTHER; note = phosphorothioate bond between nucleosides
  modified_base 22^23: mod_base = OTHER; note = phosphorothioate bond between nucleosides
  modified_base 23^24: mod_base = OTHER; note = phosphorothioate bond between nucleosides
aaagcatgccatcacctcccctgt

SEQ ID NO: 69 - RNA, 24 nt, synthetic construct
  source 1..24: mol_type = other RNA
  modified_base 1: mod_base = OTHER; note = 2'-O-methyladenosine
  modified_base 2: mod_base = OTHER; note = 2'-O,4'-C-methylene-briged adenosine
  modified_base 3: mod_base = OTHER; note = 2'-O-methyladenosine
  modified_base 4: mod_base = OTHER; note = 2'-O,4'-C-methylene-briged guanosine
  modified_base 5: mod_base = cm
  modified_base 6: mod_base = OTHER; note = 2'-deoxy-2'-fluoroadenosine
  modified_base 7: mod_base = OTHER; note = 2'-deoxy-2'-fluorouridine
  modified_base 8: mod_base = gm
  modified_base 9: mod_base = cm
  modified_base 10: mod_base = OTHER; note = 2'-deoxycytidine
  modified_base 11: mod_base = OTHER; note = 2'-deoxyadenosine
  modified_base 12: mod_base = um
  modified_base 13: mod_base = OTHER; note = 2'-deoxy-2'-fluorocytidine
  modified_base 14: mod_base = OTHER; note = 2'-O-methyladenosine
  modified_base 15: mod_base = OTHER; note = 2'-deoxy-2'-fluorocytidine
  modified_base 16: mod_base = cm
  modified_base 17: mod_base = OTHER; note = 2'-deoxy-2'-fluorouridine
  modified_base 18: mod_base = cm
  modified_base 19: mod_base = OTHER; note = 2'-deoxy-2'-fluorocytidine
  modified_base 20: mod_base = cm
  modified_base 21: mod_base = OTHER; note = 2'-O,4'-C-methylene-briged cytidine
  modified_base 22: mod_base = um
  modified_base 23: mod_base = OTHER; note = 2'-O,4'-C-methylene-briged guanosine
  modified_base 24: mod_base = um
  modified_base 1^2: mod_base = OTHER; note = phosphorotioate bond between nucleosides
  modified_base 2^3: mod_base = OTHER; note = phosphorothioate bond between nucleosides
  modified_base 3^4: mod_base = OTHER; note = phosphorothioate bond between nucleosides
  modified_base 4^5: mod_base = OTHER; note = phosphorothioate bond between nucleosides
  modified_base 5^6: mod_base = OTHER; note = phosphorothioate bond between nucleosides
  modified_base 7^8: mod_base = OTHER; note = phosphorothioate bond between nucleosides
  modified_base 6^7: mod_base = OTHER; note = phosphorothioate bond between nucleosides
  modified_base 8^9: mod_base = OTHER; note = phosphorothioate bond between nucleosides
  modified_base 9^10: mod_base = OTHER; note = phosphorothioate bond between nucleosides
  modified_base 10^11: mod_base = OTHER; note = phosphorothioate bond between nucleosides
  modified_base 11^12: mod_base = OTHER; note = methoxypropylphosphonate bond between nucleosides
  modified_base 12^13: mod_base = OTHER; note = phosphorothioate bond between nucleosides
  modified_base 13^14: mod_base = OTHER; note = phosphorothioate bond between nucleosides
  modified_base 14^15: mod_base = OTHER; note = phosphorothioate bond between nucleosides
  modified_base 15^16: mod_base = OTHER; note = phosphorothioate bond between nucleosides
  modified_base 16^17: mod_base = OTHER; note = phosphorothioate bond between nucleosides
  modified_base 17^18: mod_base = OTHER; note = phosphorothioate bond between nucleosides
  modified_base 18^19: mod_base = OTHER; note = phosphorothioate bond between nucleosides
  modified_base 19^20: mod_base = OTHER; note = phosphorothioate bond between nucleosides
  modified_base 20^21: mod_base = OTHER; note = phosphorothioate bond between nucleosides
  modified_base 21^22: mod_base = OTHER; note = phosphorothioate bond between nucleosides
  modified_base 22^23: mod_base = OTHER; note = phosphorothioate bond between nucleosides
  modified_base 23^24: mod_base = OTHER; note = phosphorothioate bond between nucleosides
aaagcatgccatcacctcccctgt

SEQ ID NO: 70 - RNA, 24 nt, synthetic construct
  source 1..24: mol_type = other RNA
  modified_base 1: mod_base = OTHER; note = 2'-O-methyladenosine
  modified_base 2: mod_base = OTHER; note = 2'-O,4'-C-methylene-briged adenosine
  modified_base 3: mod_base = OTHER; note = 2'-O-methyladenosine
  modified_base 4: mod_base = OTHER; note = 2'-O,4'-C-methylene-briged guanosine
  modified_base 5: mod_base = cm
  modified_base 6: mod_base = OTHER; note = 2'-deoxy-2'-fluoroadenosine
  modified_base 7: mod_base = OTHER; note = 2'-deoxy-2'-fluorouridine
  modified_base 8: mod_base = gm
  modified_base 9: mod_base = cm
  modified_base 10: mod_base = OTHER; note = 2'-deoxycytidine
  modified_base 11: mod_base = OTHER; note = 2'-deoxyadenosine
  modified_base 12: mod_base = um
  modified_base 13: mod_base = OTHER; note = 2'-deoxy-2'-fluorocytidine
  modified_base 14: mod_base = OTHER; note = 2'-O-methyladenosine
  modified_base 15: mod_base = OTHER; note = 2'-deoxy-2'-fluorocytidine
  modified_base 16: mod_base = cm
  modified_base 17: mod_base = OTHER; note = 2'-deoxy-2'-fluorouridine
  modified_base 18: mod_base = cm
  modified_base 19: mod_base = OTHER; note = 2'-deoxy-2'-fluorocytidine
  modified_base 20: mod_base = cm
  modified_base 21: mod_base = OTHER; note = 2'-O,4'-C-methylene-briged cytidine
  modified_base 22: mod_base = um
  modified_base 23: mod_base = OTHER; note = 2'-O,4'-C-methylene-briged guanosine
  modified_base 24: mod_base = um
  modified_base 1^2: mod_base = OTHER; note = phosphorotioate bond between nucleosides
  modified_base 2^3: mod_base = OTHER; note = phosphorothioate bond between nucleosides
  modified_base 3^4: mod_base = OTHER; note = phosphorothioate bond between nucleosides
  modified_base 4^5: mod_base = OTHER; note = phosphorothioate bond between nucleosides
  modified_base 5^6: mod_base = OTHER; note = phosphorothioate bond between nucleosides
  modified_base 7^8: mod_base = OTHER; note = phosphorothioate bond between nucleosides
  modified_base 6^7: mod_base = OTHER; note = phosphorothioate bond between nucleosides
  modified_base 8^9: mod_base = OTHER; note = phosphorothioate bond between nucleosides
  modified_base 10^11: mod_base = OTHER; note = phosphorothioate bond between nucleosides
  modified_base 11^12: mod_base = OTHER; note = ethylphosphate bond between nucleosides
  modified_base 12^13: mod_base = OTHER; note = phosphorothioate bond between nucleosides
  modified_base 13^14: mod_base = OTHER; note = phosphorothioate bond between nucleosides
  modified_base 14^15: mod_base = OTHER; note = ethylphosphate bond between nucleosides
  modified_base 15^16: mod_base = OTHER; note = phosphorothioate bond between nucleosides
  modified_base 16^17: mod_base = OTHER; note = phosphorothioate bond between nucleosides
  modified_base 17^18: mod_base = OTHER; note = phosphorothioate bond between nucleosides
  modified_base 18^19: mod_base = OTHER; note = phosphorothioate bond between nucleosides
  modified_base 19^20: mod_base = OTHER; note = phosphorothioate bond between nucleosides
  modified_base 20^21: mod_base = OTHER; note = phosphorothioate bond between nucleosides
  modified_base 21^22: mod_base = OTHER; note = phosphorothioate bond between nucleosides
  modified_base 22^23: mod_base = OTHER; note = phosphorothioate bond between nucleosides
  modified_base 23^24: mod_base = OTHER; note = phosphorothioate bond between nucleosides
aaagcatgccatcacctcccctgt

SEQ ID NO: 71 - RNA, 24 nt, synthetic construct
  source 1..24: mol_type = other RNA
  modified_base 1: mod_base = OTHER; note = 2'-O-methyladenosine
  modified_base 2: mod_base = OTHER; note = 2'-O,4'-C-methylene-briged adenosine
  modified_base 3: mod_base = OTHER; note = 2'-O-methyladenosine
  modified_base 4: mod_base = OTHER; note = 2'-O,4'-C-methylene-briged guanosine
  modified_base 5: mod_base = cm
  modified_base 6: mod_base = OTHER; note = 2'-deoxy-2'-fluoroadenosine
  modified_base 7: mod_base = OTHER; note = 2'-deoxy-2'-fluorouridine
  modified_base 8: mod_base = gm
  modified_base 9: mod_base = cm
  modified_base 10: mod_base = OTHER; note = 2'-deoxycytidine
  modified_base 11: mod_base = OTHER; note = 2'-deoxyadenosine
  modified_base 12: mod_base = um
  modified_base 13: mod_base = OTHER; note = 2'-deoxy-2'-fluorocytidine
  modified_base 14: mod_base = OTHER; note = 2'-O-methyladenosine
  modified_base 15: mod_base = OTHER; note = 2'-deoxy-2'-fluorocytidine
  modified_base 16: mod_base = cm
  modified_base 17: mod_base = OTHER; note = 2'-deoxy-2'-fluorouridine
  modified_base 18: mod_base = cm
  modified_base 19: mod_base = OTHER; note = 2'-deoxy-2'-fluorocytidine
  modified_base 20: mod_base = cm
  modified_base 21: mod_base = OTHER; note = 2'-O,4'-C-methylene-briged cytidine
  modified_base 22: mod_base = um
  modified_base 23: mod_base = OTHER; note = 2'-O,4'-C-methylene-briged guanosine
  modified_base 24: mod_base = um
  modified_base 1^2: mod_base = OTHER; note = phosphorotioate bond between nucleosides
  modified_base 2^3: mod_base = OTHER; note = phosphorothioate bond between nucleosides
  modified_base 3^4: mod_base = OTHER; note = phosphorothioate bond between nucleosides
  modified_base 4^5: mod_base = OTHER; note = phosphorothioate bond between nucleosides
  modified_base 5^6: mod_base = OTHER; note = phosphorothioate bond between nucleosides
  modified_base 7^8: mod_base = OTHER; note = phosphorothioate bond between nucleosides
  modified_base 6^7: mod_base = OTHER; note = phosphorothioate bond between nucleosides
  modified_base 9^10: mod_base = OTHER; note = phosphorothioate bond between nucleosides
  modified_base 10^11: mod_base = OTHER; note = phosphorothioate bond between nucleosides
  modified_base 11^12: mod_base = OTHER; note = ethylphosphate bond between nucleosides
  modified_base 12^13: mod_base = OTHER; note = phosphorothioate bond between nucleosides
  modified_base 13^14: mod_base = OTHER; note = phosphorothioate bond between nucleosides
  modified_base 14^15: mod_base = OTHER; note = ethylphosphate bond between nucleosides
  modified_base 15^16: mod_base = OTHER; note = phosphorothioate bond between nucleosides
  modified_base 16^17: mod_base = OTHER; note = phosphorothioate bond between nucleosides
  modified_base 17^18: mod_base = OTHER; note = phosphorothioate bond between nucleosides
  modified_base 18^19: mod_base = OTHER; note = phosphorothioate bond between nucleosides
  modified_base 19^20: mod_base = OTHER; note = phosphorothioate bond between nucleosides
  modified_base 20^21: mod_base = OTHER; note = phosphorothioate bond between nucleosides
  modified_base 21^22: mod_base = OTHER; note = phosphorothioate bond between nucleosides
  modified_base 22^23: mod_base = OTHER; note = phosphorothioate bond between nucleosides
  modified_base 23^24: mod_base = OTHER; note = phosphorothioate bond between nucleosides
aaagcatgccatcacctcccctgt

SEQ ID NO: 72 - RNA, 24 nt, synthetic construct
  source 1..24: mol_type = other RNA
  modified_base 1: mod_base = OTHER; note = 2'-O-methyladenosine
  modified_base 2: mod_base = OTHER; note = 2'-O,4'-C-methylene-briged adenosine
  modified_base 3: mod_base = OTHER; note = 2'-O-methyladenosine
  modified_base 4: mod_base = OTHER; note = 2'-O,4'-C-methylene-briged guanosine
  modified_base 5: mod_base = cm
  modified_base 6: mod_base = OTHER; note = 2'-deoxy-2'-fluoroadenosine
  modified_base 7: mod_base = OTHER; note = 2'-deoxy-2'-fluorouridine
  modified_base 8: mod_base = gm
  modified_base 9: mod_base = cm
  modified_base 10: mod_base = OTHER; note = 2'-deoxycytidine
  modified_base 11: mod_base = OTHER; note = 2'-deoxyadenosine
  modified_base 12: mod_base = um
  modified_base 13: mod_base = OTHER; note = 2'-deoxy-2'-fluorocytidine
  modified_base 14: mod_base = OTHER; note = 2'-O-methyladenosine
  modified_base 15: mod_base = OTHER; note = 2'-deoxy-2'-fluorocytidine
  modified_base 16: mod_base = cm
  modified_base 17: mod_base = OTHER; note = 2'-deoxy-2'-fluorouridine
  modified_base 18: mod_base = cm
  modified_base 19: mod_base = OTHER; note = 2'-deoxy-2'-fluorocytidine
  modified_base 20: mod_base = cm
  modified_base 21: mod_base = OTHER; note = 2'-O,4'-C-methylene-briged cytidine
  modified_base 22: mod_base = um
  modified_base 23: mod_base = OTHER; note = 2'-O,4'-C-methylene-briged guanosine
  modified_base 24: mod_base = um
  modified_base 1^2: mod_base = OTHER; note = phosphorotioate bond between nucleosides
  modified_base 2^3: mod_base = OTHER; note = phosphorothioate bond between nucleosides
  modified_base 3^4: mod_base = OTHER; note = phosphorothioate bond between nucleosides
  modified_base 5^6: mod_base = OTHER; note = phosphorothioate bond between nucleosides
  modified_base 7^8: mod_base = OTHER; note = phosphorothioate bond between nucleosides
  modified_base 6^7: mod_base = OTHER; note = phosphorothioate bond between nucleosides
  modified_base 8^9: mod_base = OTHER; note = phosphorothioate bond between nucleosides
  modified_base 9^10: mod_base = OTHER; note = phosphorothioate bond between nucleosides
  modified_base 10^11: mod_base = OTHER; note = phosphorothioate bond between nucleosides
  modified_base 11^12: mod_base = OTHER; note = ethylphosphate bond between nucleosides
  modified_base 13^14: mod_base = OTHER; note = phosphorothioate bond between nucleosides
  modified_base 14^15: mod_base = OTHER; note = ethylphosphate bond between nucleosides
  modified_base 15^16: mod_base = OTHER; note = phosphorothioate bond between nucleosides
  modified_base 16^17: mod_base = OTHER; note = phosphorothioate bond between nucleosides
  modified_base 17^18: mod_base = OTHER; note = phosphorothioate bond between nucleosides
  modified_base 18^19: mod_base = OTHER; note = phosphorothioate bond between nucleosides
  modified_base 19^20: mod_base = OTHER; note = phosphorothioate bond between nucleosides
  modified_base 20^21: mod_base = OTHER; note = phosphorothioate bond between nucleosides
  modified_base 22^23: mod_base = OTHER; note = phosphorothioate bond between nucleosides
  modified_base 23^24: mod_base = OTHER; note = phosphorothioate bond between nucleosides
aaagcatgccatcacctcccctgt

SEQ ID NO: 73 - RNA, 24 nt, synthetic construct
  source 1..24: mol_type = other RNA
  modified_base 1: mod_base = OTHER; note = 2'-O-methyladenosine
  modified_base 2: mod_base = OTHER; note = 2'-O,4'-C-methylene-briged adenosine
  modified_base 3: mod_base = OTHER; note = 2'-O-methyladenosine
  modified_base 4: mod_base = OTHER; note = 2'-O,4'-C-methylene-briged guanosine
  modified_base 5: mod_base = cm
  modified_base 6: mod_base = OTHER; note = 2'-deoxy-2'-fluoroadenosine
  modified_base 7: mod_base = OTHER; note = 2'-deoxy-2'-fluorouridine
  modified_base 8: mod_base = gm
  modified_base 9: mod_base = cm
  modified_base 10: mod_base = OTHER; note = 2'-deoxycytidine
  modified_base 11: mod_base = OTHER; note = 2'-deoxyadenosine
  modified_base 12: mod_base = um
  modified_base 13: mod_base = OTHER; note = 2'-deoxy-2'-fluorocytidine
  modified_base 14: mod_base = OTHER; note = 2'-O-methyladenosine
  modified_base 15: mod_base = OTHER; note = 2'-deoxy-2'-fluorocytidine
  modified_base 16: mod_base = cm
  modified_base 17: mod_base = OTHER; note = 2'-deoxy-2'-fluorouridine
  modified_base 18: mod_base = cm
  modified_base 19: mod_base = OTHER; note = 2'-deoxy-2'-fluorocytidine
  modified_base 20: mod_base = cm
  modified_base 21: mod_base = OTHER; note = 2'-O,4'-C-methylene-briged cytidine
  modified_base 22: mod_base = um
  modified_base 23: mod_base = OTHER; note = 2'-O,4'-C-methylene-briged guanosine
  modified_base 24: mod_base = um
  modified_base 1^2: mod_base = OTHER; note = phosphorotioate bond between nucleosides
  modified_base 2^3: mod_base = OTHER; note = phosphorothioate bond between nucleosides
  modified_base 3^4: mod_base = OTHER; note = phosphorothioate bond between nucleosides
  modified_base 5^6: mod_base = OTHER; note = phosphorothioate bond between nucleosides
  modified_base 7^8: mod_base = OTHER; note = phosphorothioate bond between nucleosides
  modified_base 6^7: mod_base = OTHER; note = phosphorothioate bond between nucleosides
  modified_base 8^9: mod_base = OTHER; note = phosphorothioate bond between nucleosides
  modified_base 9^10: mod_base = OTHER; note = phosphorothioate bond between nucleosides
  modified_base 10^11: mod_base = OTHER; note = phosphorothioate bond between nucleosides
  modified_base 11^12: mod_base = OTHER; note = ethylphosphate bond between nucleosides
  modified_base 13^14: mod_base = OTHER; note = phosphorothioate bond between nucleosides
  modified_base 14^15: mod_base = OTHER; note = ethylphosphate bond between nucleosides
  modified_base 15^16: mod_base = OTHER; note = phosphorothioate bond between nucleosides
  modified_base 17^18: mod_base = OTHER; note = phosphorothioate bond between nucleosides
  modified_base 18^19: mod_base = OTHER; note = phosphorothioate bond between nucleosides
  modified_base 19^20: mod_base = OTHER; note = phosphorothioate bond between nucleosides
  modified_base 20^21: mod_base = OTHER; note = phosphorothioate bond between nucleosides
  modified_base 22^23: mod_base = OTHER; note = phosphorothioate bond between nucleosides
  modified_base 23^24: mod_base = OTHER; note = phosphorothioate bond between nucleosides
aaagcatgccatcacctcccctgt

SEQ ID NO: 74 - RNA, 24 nt, synthetic construct
  source 1..24: mol_type = other RNA
  modified_base 1: mod_base = OTHER; note = 2'-O-methyladenosine
  modified_base 2: mod_base = OTHER; note = 2'-O,4'-C-methylene-briged adenosine
  modified_base 3: mod_base = OTHER; note = 2'-O-methyladenosine
  modified_base 4: mod_base = OTHER; note = 2'-O,4'-C-methylene-briged guanosine
  modified_base 5: mod_base = cm
  modified_base 6: mod_base = OTHER; note = 2'-deoxy-2'-fluoroadenosine
  modified_base 7: mod_base = OTHER; note = 2'-deoxy-2'-fluorouridine
  modified_base 8: mod_base = gm
  modified_base 9: mod_base = cm
  modified_base 10: mod_base = OTHER; note = 2'-deoxycytidine
  modified_base 11: mod_base = OTHER; note = 2'-deoxyadenosine
  modified_base 12: mod_base = um
  modified_base 13: mod_base = OTHER; note = 2'-deoxy-2'-fluorocytidine
  modified_base 14: mod_base = OTHER; note = 2'-O-methyladenosine
  modified_base 15: mod_base = OTHER; note = 2'-deoxy-2'-fluorocytidine
  modified_base 16: mod_base = cm
  modified_base 17: mod_base = OTHER; note = 2'-deoxy-2'-fluorouridine
  modified_base 18: mod_base = cm
  modified_base 19: mod_base = OTHER; note = 2'-deoxy-2'-fluorocytidine
  modified_base 20: mod_base = cm
  modified_base 21: mod_base = OTHER; note = 2'-O,4'-C-methylene-briged cytidine
  modified_base 22: mod_base = um
  modified_base 23: mod_base = OTHER; note = 2'-O,4'-C-methylene-briged guanosine
  modified_base 24: mod_base = um
  modified_base 1^2: mod_base = OTHER; note = phosphorotioate bond between nucleosides
  modified_base 2^3: mod_base = OTHER; note = phosphorothioate bond between nucleosides
  modified_base 3^4: mod_base = OTHER; note = phosphorothioate bond between nucleosides
  modified_base 5^6: mod_base = OTHER; note = phosphorothioate bond between nucleosides
  modified_base 7^8: mod_base = OTHER; note = phosphorothioate bond between nucleosides
  modified_base 6^7: mod_base = OTHER; note = phosphorothioate bond between nucleosides
  modified_base 8^9: mod_base = OTHER; note = phosphorothioate bond between nucleosides
  modified_base 9^10: mod_base = OTHER; note = phosphorothioate bond between nucleosides
  modified_base 10^11: mod_base = OTHER; note = phosphorothioate bond between nucleosides
  modified_base 11^12: mod_base = OTHER; note = ethylphosphate bond between nucleosides
  modified_base 13^14: mod_base = OTHER; note = phosphorothioate bond between nucleosides
  modified_base 14^15: mod_base = OTHER; note = ethylphosphate bond between nucleosides
  modified_base 15^16: mod_base = OTHER; note = phosphorothioate bond between nucleosides
  modified_base 16^17: mod_base = OTHER; note = phosphorothioate bond between nucleosides
  modified_base 17^18: mod_base = OTHER; note = phosphorothioate bond between nucleosides
  modified_base 19^20: mod_base = OTHER; note = phosphorothioate bond between nucleosides
  modified_base 20^21: mod_base = OTHER; note = phosphorothioate bond between nucleosides
  modified_base 22^23: mod_base = OTHER; note = phosphorothioate bond between nucleosides
  modified_base 23^24: mod_base = OTHER; note = phosphorothioate bond between nucleosides
aaagcatgccatcacctcccctgt

SEQ ID NO: 75 - RNA, 24 nt, synthetic construct
  source 1..24: mol_type = other RNA
  modified_base 1: mod_base = OTHER; note = 2'-O-methyladenosine
  modified_base 2: mod_base = OTHER; note = 2'-O,4'-C-methylene-briged adenosine
  modified_base 3: mod_base = OTHER; note = 2'-O-methyladenosine
  modified_base 4: mod_base = OTHER; note = 2'-O,4'-C-methylene-briged guanosine
  modified_base 5: mod_base = cm
  modified_base 6: mod_base = OTHER; note = 2'-deoxy-2'-fluoroadenosine
  modified_base 7: mod_base = OTHER; note = 2'-deoxy-2'-fluorouridine
  modified_base 8: mod_base = gm
  modified_base 9: mod_base = cm
  modified_base 10: mod_base = OTHER; note = 2'-deoxycytidine
  modified_base 11: mod_base = OTHER; note = 2'-deoxyadenosine
  modified_base 12: mod_base = um
  modified_base 13: mod_base = OTHER; note = 2'-deoxy-2'-fluorocytidine
  modified_base 14: mod_base = OTHER; note = 2'-O-methyladenosine
  modified_base 15: mod_base = OTHER; note = 2'-deoxy-2'-fluorocytidine
  modified_base 16: mod_base = cm
  modified_base 17: mod_base = OTHER; note = 2'-deoxy-2'-fluorouridine
  modified_base 18: mod_base = cm
  modified_base 19: mod_base = OTHER; note = 2'-deoxy-2'-fluorocytidine
  modified_base 20: mod_base = cm
  modified_base 21: mod_base = OTHER; note = 2'-O,4'-C-methylene-briged cytidine
  modified_base 22: mod_base = um
  modified_base 23: mod_base = OTHER; note = 2'-O,4'-C-methylene-briged guanosine
  modified_base 24: mod_base = um
  modified_base 1^2: mod_base = OTHER; note = phosphorotioate bond between nucleosides
  modified_base 2^3: mod_base = OTHER; note = phosphorothioate bond between nucleosides
  modified_base 3^4: mod_base = OTHER; note = phosphorothioate bond between nucleosides
  modified_base 5^6: mod_base = OTHER; note = phosphorothioate bond between nucleosides
  modified_base 7^8: mod_base = OTHER; note = phosphorothioate bond between nucleosides
  modified_base 6^7: mod_base = OTHER; note = phosphorothioate bond between nucleosides
  modified_base 8^9: mod_base = OTHER; note = phosphorothioate bond between nucleosides
  modified_base 9^10: mod_base = OTHER; note = phosphorothioate bond between nucleosides
  modified_base 10^11: mod_base = OTHER; note = phosphorothioate bond between nucleosides
  modified_base 11^12: mod_base = OTHER; note = ethylphosphate bond between nucleosides
  modified_base 13^14: mod_base = OTHER; note = phosphorothioate bond between nucleosides
  modified_base 14^15: mod_base = OTHER; note = ethylphosphate bond between nucleosides
  modified_base 15^16: mod_base = OTHER; note = phosphorothioate bond between nucleosides
  modified_base 16^17: mod_base = OTHER; note = phosphorothioate bond between nucleosides
  modified_base 17^18: mod_base = OTHER; note = phosphorothioate bond between nucleosides
  modified_base 18^19: mod_base = OTHER; note = phosphorothioate bond between nucleosides
  modified_base 19^20: mod_base = OTHER; note = phosphorothioate bond between nucleosides
  modified_base 22^23: mod_base = OTHER; note = phosphorothioate bond between nucleosides
  modified_base 23^24: mod_base = OTHER; note = phosphorothioate bond between nucleosides
aaagcatgccatcacctcccctgt

SEQ ID NO: 76 - RNA, 24 nt, synthetic construct
  source 1..24: mol_type = other RNA
  modified_base 1: mod_base = OTHER; note = 2'-O-methyladenosine
  modified_base 2: mod_base = OTHER; note = 2'-O,4'-C-methylene-briged adenosine
  modified_base 3: mod_base = OTHER; note = 2'-O-methyladenosine
  modified_base 4: mod_base = OTHER; note = 2'-O,4'-C-methylene-briged guanosine
  modified_base 5: mod_base = cm
  modified_base 6: mod_base = OTHER; note = 2'-deoxy-2'-fluoroadenosine
  modified_base 7: mod_base = OTHER; note = 2'-deoxy-2'-fluorouridine
  modified_base 8: mod_base = gm
  modified_base 9: mod_base = cm
  modified_base 10: mod_base = OTHER; note = 2'-deoxycytidine
  modified_base 11: mod_base = OTHER; note = 2'-deoxyadenosine
  modified_base 12: mod_base = um
  modified_base 13: mod_base = OTHER; note = 2'-deoxy-2'-fluorocytidine
  modified_base 14: mod_base = OTHER; note = 2'-O-methyladenosine
  modified_base 15: mod_base = OTHER; note = 2'-deoxy-2'-fluorocytidine
  modified_base 16: mod_base = cm
  modified_base 17: mod_base = OTHER; note = 2'-deoxy-2'-fluorouridine
  modified_base 18: mod_base = cm
  modified_base 19: mod_base = OTHER; note = 2'-deoxy-2'-fluorocytidine
  modified_base 20: mod_base = cm
  modified_base 21: mod_base = OTHER; note = 2'-O,4'-C-methylene-briged cytidine
  modified_base 22: mod_base = um
  modified_base 23: mod_base = OTHER; note = 2'-O,4'-C-methylene-briged guanosine
  modified_base 24: mod_base = um
  modified_base 1^2: mod_base = OTHER; note = phosphorotioate bond between nucleosides
  modified_base 2^3: mod_base = OTHER; note = phosphorothioate bond between nucleosides
  modified_base 3^4: mod_base = OTHER; note = phosphorothioate bond between nucleosides
  modified_base 7^8: mod_base = OTHER; note = phosphorothioate bond between nucleosides
  modified_base 6^7: mod_base = OTHER; note = phosphorothioate bond between nucleosides
  modified_base 8^9: mod_base = OTHER; note = phosphorothioate bond between nucleosides
  modified_base 9^10: mod_base = OTHER; note = phosphorothioate bond between nucleosides
  modified_base 10^11: mod_base = OTHER; note = phosphorothioate bond between nucleosides
  modified_base 11^12: mod_base = OTHER; note = ethylphosphate bond between nucleosides
  modified_base 13^14: mod_base = OTHER; note = phosphorothioate bond between nucleosides
  modified_base 14^15: mod_base = OTHER; note = ethylphosphate bond between nucleosides
  modified_base 15^16: mod_base = OTHER; note = phosphorothioate bond between nucleosides
  modified_base 16^17: mod_base = OTHER; note = phosphorothioate bond between nucleosides
  modified_base 17^18: mod_base = OTHER; note = phosphorothioate bond between nucleosides
  modified_base 18^19: mod_base = OTHER; note = phosphorothioate bond between nucleosides
  modified_base 19^20: mod_base = OTHER; note = phosphorothioate bond between nucleosides
  modified_base 20^21: mod_base = OTHER; note = phosphorothioate bond between nucleosides
  modified_base 22^23: mod_base = OTHER; note = phosphorothioate bond between nucleosides
  modified_base 23^24: mod_base = OTHER; note = phosphorothioate bond between nucleosides
aaagcatgccatcacctcccctgt

SEQ ID NO: 77 - RNA, 24 nt, synthetic construct
  source 1..24: mol_type = other RNA
  modified_base 1: mod_base = OTHER; note = 2'-O-methyladenosine
  modified_base 2: mod_base = OTHER; note = 2'-O,4'-C-methylene-briged adenosine
  modified_base 3: mod_base = OTHER; note = 2'-O-methyladenosine
  modified_base 4: mod_base = OTHER; note = 2'-O,4'-C-methylene-briged guanosine
  modified_base 5: mod_base = cm
  modified_base 6: mod_base = OTHER; note = 2'-deoxy-2'-fluoroadenosine
  modified_base 7: mod_base = OTHER; note = 2'-deoxy-2'-fluorouridine
  modified_base 8: mod_base = gm
  modified_base 9: mod_base = cm
  modified_base 10: mod_base = OTHER; note = 2'-deoxycytidine
  modified_base 11: mod_base = OTHER; note = 2'-deoxyadenosine
  modified_base 12: mod_base = um
  modified_base 13: mod_base = OTHER; note = 2'-deoxy-2'-fluorocytidine
  modified_base 14: mod_base = OTHER; note = 2'-O-methyladenosine
  modified_base 15: mod_base = OTHER; note = 2'-deoxy-2'-fluorocytidine
  modified_base 16: mod_base = cm
  modified_base 17: mod_base = OTHER; note = 2'-deoxy-2'-fluorouridine
  modified_base 18: mod_base = cm
  modified_base 19: mod_base = OTHER; note = 2'-deoxy-2'-fluorocytidine
  modified_base 20: mod_base = cm
  modified_base 21: mod_base = OTHER; note = 2'-O,4'-C-methylene-briged cytidine
  modified_base 22: mod_base = um
  modified_base 23: mod_base = OTHER; note = 2'-O,4'-C-methylene-briged guanosine
  modified_base 24: mod_base = um
  modified_base 1^2: mod_base = OTHER; note = phosphorotioate bond between nucleosides
  modified_base 2^3: mod_base = OTHER; note = phosphorothioate bond between nucleosides
  modified_base 3^4: mod_base = OTHER; note = phosphorothioate bond between nucleosides
  modified_base 7^8: mod_base = OTHER; note = phosphorothioate bond between nucleosides
  modified_base 6^7: mod_base = OTHER; note = phosphorothioate bond between nucleosides
  modified_base 8^9: mod_base = OTHER; note = phosphorothioate bond between nucleosides
  modified_base 9^10: mod_base = OTHER; note = phosphorothioate bond between nucleosides
  modified_base 10^11: mod_base = OTHER; note = phosphorothioate bond between nucleosides
  modified_base 11^12: mod_base = OTHER; note = ethylphosphate bond between nucleosides
  modified_base 13^14: mod_base = OTHER; note = phosphorothioate bond between nucleosides
  modified_base 14^15: mod_base = OTHER; note = ethylphosphate bond between nucleosides
  modified_base 15^16: mod_base = OTHER; note = phosphorothioate bond between nucleosides
  modified_base 16^17: mod_base = OTHER; note = phosphorothioate bond between nucleosides
  modified_base 17^18: mod_base = OTHER; note = phosphorothioate bond between nucleosides
  modified_base 18^19: mod_base = OTHER; note = phosphorothioate bond between nucleosides
  modified_base 19^20: mod_base = OTHER; note = phosphorothioate bond between nucleosides
  modified_base 22^23: mod_base = OTHER; note = phosphorothioate bond between nucleosides
  modified_base 23^24: mod_base = OTHER; note = phosphorothioate bond between nucleosides
aaagcatgccatcacctcccctgt

SEQ ID NO: 78 - RNA, 24 nt, synthetic construct
  source 1..24: mol_type = other RNA
  modified_base 1: mod_base = OTHER; note = 2'-O-methyladenosine
  modified_base 2: mod_base = OTHER; note = 2'-O,4'-C-methylene-briged adenosine
  modified_base 3: mod_base = OTHER; note = 2'-O-methyladenosine
  modified_base 4: mod_base = OTHER; note = 2'-O,4'-C-methylene-briged guanosine
  modified_base 5: mod_base = cm
  modified_base 6: mod_base = OTHER; note = 2'-deoxy-2'-fluoroadenosine
  modified_base 7: mod_base = OTHER; note = 2'-deoxy-2'-fluorouridine
  modified_base 8: mod_base = gm
  modified_base 9: mod_base = cm
  modified_base 10: mod_base = OTHER; note = 2'-deoxycytidine
  modified_base 11: mod_base = OTHER; note = 2'-deoxyadenosine
  modified_base 12: mod_base = um
  modified_base 13: mod_base = OTHER; note = 2'-deoxy-2'-fluorocytidine
  modified_base 14: mod_base = OTHER; note = 2'-O-methyladenosine
  modified_base 15: mod_base = OTHER; note = 2'-deoxy-2'-fluorocytidine
  modified_base 16: mod_base = cm
  modified_base 17: mod_base = OTHER; note = 2'-deoxy-2'-fluorouridine
  modified_base 18: mod_base = cm
  modified_base 19: mod_base = OTHER; note = 2'-deoxy-2'-fluorocytidine
  modified_base 20: mod_base = cm
  modified_base 21: mod_base = OTHER; note = 2'-O,4'-C-methylene-briged cytidine
  modified_base 22: mod_base = um
  modified_base 23: mod_base = OTHER; note = 2'-O,4'-C-methylene-briged guanosine
  modified_base 24: mod_base = um
  modified_base 1^2: mod_base = OTHER; note = phosphorotioate bond between nucleosides
  modified_base 2^3: mod_base = OTHER; note = phosphorothioate bond between nucleosides
  modified_base 3^4: mod_base = OTHER; note = phosphorothioate bond between nucleosides
  modified_base 5^6: mod_base = OTHER; note = phosphorothioate bond between nucleosides
  modified_base 6^7: mod_base = OTHER; note = phosphorothioate bond between nucleosides
  modified_base 8^9: mod_base = OTHER; note = phosphorothioate bond between nucleosides
  modified_base 9^10: mod_base = OTHER; note = phosphorothioate bond between nucleosides
  modified_base 10^11: mod_base = OTHER; note = phosphorothioate bond between nucleosides
  modified_base 11^12: mod_base = OTHER; note = ethylphosphate bond between nucleosides
  modified_base 13^14: mod_base = OTHER; note = phosphorothioate bond between nucleosides
  modified_base 14^15: mod_base = OTHER; note = ethylphosphate bond between nucleosides
  modified_base 15^16: mod_base = OTHER; note = phosphorothioate bond between nucleosides
  modified_base 17^18: mod_base = OTHER; note = phosphorothioate bond between nucleosides
  modified_base 18^19: mod_base = OTHER; note = phosphorothioate bond between nucleosides
  modified_base 19^20: mod_base = OTHER; note = phosphorothioate bond between nucleosides
  modified_base 20^21: mod_base = OTHER; note = phosphorothioate bond between nucleosides
  modified_base 22^23: mod_base = OTHER; note = phosphorothioate bond between nucleosides
  modified_base 23^24: mod_base = OTHER; note = phosphorothioate bond between nucleosides
aaagcatgccatcacctcccctgt

SEQ ID NO: 79 - RNA, 24 nt, synthetic construct
  source 1..24: mol_type = other RNA
  modified_base 1: mod_base = OTHER; note = 2'-O-methyladenosine
  modified_base 2: mod_base = OTHER; note = 2'-O,4'-C-methylene-briged adenosine
  modified_base 3: mod_base = OTHER; note = 2'-O-methyladenosine
  modified_base 4: mod_base = OTHER; note = 2'-O,4'-C-methylene-briged guanosine
  modified_base 5: mod_base = cm
  modified_base 6: mod_base = OTHER; note = 2'-deoxy-2'-fluoroadenosine
  modified_base 7: mod_base = OTHER; note = 2'-deoxy-2'-fluorouridine
  modified_base 8: mod_base = gm
  modified_base 9: mod_base = cm
  modified_base 10: mod_base = OTHER; note = 2'-deoxycytidine
  modified_base 11: mod_base = OTHER; note = 2'-deoxyadenosine
  modified_base 12: mod_base = um
  modified_base 13: mod_base = OTHER; note = 2'-deoxy-2'-fluorocytidine
  modified_base 14: mod_base = OTHER; note = 2'-O-methyladenosine
  modified_base 15: mod_base = OTHER; note = 2'-deoxy-2'-fluorocytidine
  modified_base 16: mod_base = cm
  modified_base 17: mod_base = OTHER; note = 2'-deoxy-2'-fluorouridine
  modified_base 18: mod_base = cm
  modified_base 19: mod_base = OTHER; note = 2'-deoxy-2'-fluorocytidine
  modified_base 20: mod_base = cm
  modified_base 21: mod_base = OTHER; note = 2'-O,4'-C-methylene-briged cytidine
  modified_base 22: mod_base = um
  modified_base 23: mod_base = OTHER; note = 2'-O,4'-C-methylene-briged guanosine
  modified_base 24: mod_base = um
  modified_base 1^2: mod_base = OTHER; note = phosphorotioate bond between nucleosides
  modified_base 2^3: mod_base = OTHER; note = phosphorothioate bond between nucleosides
  modified_base 3^4: mod_base = OTHER; note = phosphorothioate bond between nucleosides
  modified_base 5^6: mod_base = OTHER; note = phosphorothioate bond between nucleosides
  modified_base 6^7: mod_base = OTHER; note = phosphorothioate bond between nucleosides
  modified_base 8^9: mod_base = OTHER; note = phosphorothioate bond between nucleosides
  modified_base 9^10: mod_base = OTHER; note = phosphorothioate bond between nucleosides
  modified_base 10^11: mod_base = OTHER; note = phosphorothioate bond between nucleosides
  modified_base 11^12: mod_base = OTHER; note = ethylphosphate bond between nucleosides
  modified_base 13^14: mod_base = OTHER; note = phosphorothioate bond between nucleosides
  modified_base 14^15: mod_base = OTHER; note = ethylphosphate bond between nucleosides
  modified_base 15^16: mod_base = OTHER; note = phosphorothioate bond between nucleosides
  modified_base 16^17: mod_base = OTHER; note = phosphorothioate bond between nucleosides
  modified_base 17^18: mod_base = OTHER; note = phosphorothioate bond between nucleosides
  modified_base 19^20: mod_base = OTHER; note = phosphorothioate bond between nucleosides
  modified_base 20^21: mod_base = OTHER; note = phosphorothioate bond between nucleosides
  modified_base 22^23: mod_base = OTHER; note = phosphorothioate bond between nucleosides
  modified_base 23^24: mod_base = OTHER; note = phosphorothioate bond between nucleosides
aaagcatgccatcacctcccctgt

SEQ ID NO: 80 - RNA, 24 nt, synthetic construct
  source 1..24: mol_type = other RNA
  modified_base 1: mod_base = OTHER; note = 2'-O-methyladenosine
  modified_base 2: mod_base = OTHER; note = 2'-O,4'-C-methylene-briged adenosine
  modified_base 3: mod_base = OTHER; note = 2'-O-methyladenosine
  modified_base 4: mod_base = OTHER; note = 2'-O,4'-C-methylene-briged guanosine
  modified_base 5: mod_base = cm
  modified_base 6: mod_base = OTHER; note = 2'-deoxy-2'-fluoroadenosine
  modified_base 7: mod_base = OTHER; note = 2'-deoxy-2'-fluorouridine
  modified_base 8: mod_base = gm
  modified_base 9: mod_base = cm
  modified_base 10: mod_base = OTHER; note = 2'-deoxycytidine
  modified_base 11: mod_base = OTHER; note = 2'-deoxyadenosine
  modified_base 12: mod_base = um
  modified_base 13: mod_base = OTHER; note = 2'-deoxy-2'-fluorocytidine
  modified_base 14: mod_base = OTHER; note = 2'-O-methyladenosine
  modified_base 15: mod_base = OTHER; note = 2'-deoxy-2'-fluorocytidine
  modified_base 16: mod_base = cm
  modified_base 17: mod_base = OTHER; note = 2'-deoxy-2'-fluorouridine
  modified_base 18: mod_base = cm
  modified_base 19: mod_base = OTHER; note = 2'-deoxy-2'-fluorocytidine
  modified_base 20: mod_base = cm
  modified_base 21: mod_base = OTHER; note = 2'-O,4'-C-methylene-briged cytidine
  modified_base 22: mod_base = um
  modified_base 23: mod_base = OTHER; note = 2'-O,4'-C-methylene-briged guanosine
  modified_base 24: mod_base = um
  modified_base 1^2: mod_base = OTHER; note = phosphorotioate bond between nucleosides
  modified_base 2^3: mod_base = OTHER; note = phosphorothioate bond between nucleosides
  modified_base 3^4: mod_base = OTHER; note = phosphorothioate bond between nucleosides
  modified_base 5^6: mod_base = OTHER; note = phosphorothioate bond between nucleosides
  modified_base 6^7: mod_base = OTHER; note = phosphorothioate bond between nucleosides
  modified_base 8^9: mod_base = OTHER; note = phosphorothioate bond between nucleosides
  modified_base 9^10: mod_base = OTHER; note = phosphorothioate bond between nucleosides
  modified_base 10^11: mod_base = OTHER; note = phosphorothioate bond between nucleosides
  modified_base 11^12: mod_base = OTHER; note = ethylphosphate bond between nucleosides
  modified_base 13^14: mod_base = OTHER; note = phosphorothioate bond between nucleosides
  modified_base 14^15: mod_base = OTHER; note = ethylphosphate bond between nucleosides
  modified_base 15^16: mod_base = OTHER; note = phosphorothioate bond between nucleosides
  modified_base 16^17: mod_base = OTHER; note = phosphorothioate bond between nucleosides
  modified_base 17^18: mod_base = OTHER; note = phosphorothioate bond between nucleosides
  modified_base 18^19: mod_base = OTHER; note = phosphorothioate bond between nucleosides
  modified_base 19^20: mod_base = OTHER; note = phosphorothioate bond between nucleosides
  modified_base 22^23: mod_base = OTHER; note = phosphorothioate bond between nucleosides
  modified_base 23^24: mod_base = OTHER; note = phosphorothioate bond between nucleosides
aaagcatgccatcacctcccctgt

SEQ ID NO: 81 - RNA, 24 nt, synthetic construct
  source 1..24: mol_type = other RNA
  modified_base 1: mod_base = OTHER; note = 2'-O-methyladenosine
  modified_base 2: mod_base = OTHER; note = 2'-O,4'-C-methylene-briged adenosine
  modified_base 3: mod_base = OTHER; note = 2'-O-methyladenosine
  modified_base 4: mod_base = OTHER; note = 2'-O,4'-C-methylene-briged guanosine
  modified_base 5: mod_base = cm
  modified_base 6: mod_base = OTHER; note = 2'-deoxy-2'-fluoroadenosine
  modified_base 7: mod_base = OTHER; note = 2'-deoxy-2'-fluorouridine
  modified_base 8: mod_base = gm
  modified_base 9: mod_base = cm
  modified_base 10: mod_base = OTHER; note = 2'-deoxycytidine
  modified_base 11: mod_base = OTHER; note = 2'-deoxyadenosine
  modified_base 12: mod_base = um
  modified_base 13: mod_base = OTHER; note = 2'-deoxy-2'-fluorocytidine
  modified_base 14: mod_base = OTHER; note = 2'-O-methyladenosine
  modified_base 15: mod_base = OTHER; note = 2'-deoxy-2'-fluorocytidine
  modified_base 16: mod_base = cm
  modified_base 17: mod_base = OTHER; note = 2'-deoxy-2'-fluorouridine
  modified_base 18: mod_base = cm
  modified_base 19: mod_base = OTHER; note = 2'-deoxy-2'-fluorocytidine
  modified_base 20: mod_base = cm
  modified_base 21: mod_base = OTHER; note = 2'-O,4'-C-methylene-briged cytidine
  modified_base 22: mod_base = um
  modified_base 23: mod_base = OTHER; note = 2'-O,4'-C-methylene-briged guanosine
  modified_base 24: mod_base = um
  modified_base 1^2: mod_base = OTHER; note = phosphorotioate bond between nucleosides
  modified_base 2^3: mod_base = OTHER; note = phosphorothioate bond between nucleosides
  modified_base 3^4: mod_base = OTHER; note = phosphorothioate bond between nucleosides
  modified_base 6^7: mod_base = OTHER; note = phosphorothioate bond between nucleosides
  modified_base 8^9: mod_base = OTHER; note = phosphorothioate bond between nucleosides
  modified_base 9^10: mod_base = OTHER; note = phosphorothioate bond between nucleosides
  modified_base 10^11: mod_base = OTHER; note = phosphorothioate bond between nucleosides
  modified_base 11^12: mod_base = OTHER; note = ethylphosphate bond between nucleosides
  modified_base 13^14: mod_base = OTHER; note = phosphorothioate bond between nucleosides
  modified_base 14^15: mod_base = OTHER; note = ethylphosphate bond between nucleosides
  modified_base 15^16: mod_base = OTHER; note = phosphorothioate bond between nucleosides
  modified_base 16^17: mod_base = OTHER; note = phosphorothioate bond between nucleosides
  modified_base 17^18: mod_base = OTHER; note = phosphorothioate bond between nucleosides
  modified_base 18^19: mod_base = OTHER; note = phosphorothioate bond between nucleosides
  modified_base 19^20: mod_base = OTHER; note = phosphorothioate bond between nucleosides
  modified_base 20^21: mod_base = OTHER; note = phosphorothioate bond between nucleosides
  modified_base 22^23: mod_base = OTHER; note = phosphorothioate bond between nucleosides
  modified_base 23^24: mod_base = OTHER; note = phosphorothioate bond between nucleosides
aaagcatgccatcacctcccctgt

SEQ ID NO: 82 - RNA, 24 nt, synthetic construct
  source 1..24: mol_type = other RNA
  modified_base 1: mod_base = OTHER; note = 2'-O-methyladenosine
  modified_base 2: mod_base = OTHER; note = 2'-O,4'-C-methylene-briged adenosine
  modified_base 3: mod_base = OTHER; note = 2'-O-methyladenosine
  modified_base 4: mod_base = OTHER; note = 2'-O,4'-C-methylene-briged guanosine
  modified_base 5: mod_base = cm
  modified_base 6: mod_base = OTHER; note = 2'-deoxy-2'-fluoroadenosine
  modified_base 7: mod_base = OTHER; note = 2'-deoxy-2'-fluorouridine
  modified_base 8: mod_base = gm
  modified_base 9: mod_base = cm
  modified_base 10: mod_base = OTHER; note = 2'-deoxycytidine
  modified_base 11: mod_base = OTHER; note = 2'-deoxyadenosine
  modified_base 12: mod_base = um
  modified_base 13: mod_base = OTHER; note = 2'-deoxy-2'-fluorocytidine
  modified_base 14: mod_base = OTHER; note = 2'-O-methyladenosine
  modified_base 15: mod_base = OTHER; note = 2'-deoxy-2'-fluorocytidine
  modified_base 16: mod_base = cm
  modified_base 17: mod_base = OTHER; note = 2'-deoxy-2'-fluorouridine
  modified_base 18: mod_base = cm
  modified_base 19: mod_base = OTHER; note = 2'-deoxy-2'-fluorocytidine
  modified_base 20: mod_base = cm
  modified_base 21: mod_base = OTHER; note = 2'-O,4'-C-methylene-briged cytidine
  modified_base 22: mod_base = um
  modified_base 23: mod_base = OTHER; note = 2'-O,4'-C-methylene-briged guanosine
  modified_base 24: mod_base = um
  modified_base 1^2: mod_base = OTHER; note = phosphorotioate bond between nucleosides
  modified_base 2^3: mod_base = OTHER; note = phosphorothioate bond between nucleosides
  modified_base 3^4: mod_base = OTHER; note = phosphorothioate bond between nucleosides
  modified_base 6^7: mod_base = OTHER; note = phosphorothioate bond between nucleosides
  modified_base 8^9: mod_base = OTHER; note = phosphorothioate bond between nucleosides
  modified_base 9^10: mod_base = OTHER; note = phosphorothioate bond between nucleosides
  modified_base 10^11: mod_base = OTHER; note = phosphorothioate bond between nucleosides
  modified_base 11^12: mod_base = OTHER; note = ethylphosphate bond between nucleosides
  modified_base 13^14: mod_base = OTHER; note = phosphorothioate bond between nucleosides
  modified_base 14^15: mod_base = OTHER; note = ethylphosphate bond between nucleosides
  modified_base 15^16: mod_base = OTHER; note = phosphorothioate bond between nucleosides
  modified_base 16^17: mod_base = OTHER; note = phosphorothioate bond between nucleosides
  modified_base 17^18: mod_base = OTHER; note = phosphorothioate bond between nucleosides
  modified_base 18^19: mod_base = OTHER; note = phosphorothioate bond between nucleosides
  modified_base 19^20: mod_base = OTHER; note = phosphorothioate bond between nucleosides
  modified_base 22^23: mod_base = OTHER; note = phosphorothioate bond between nucleosides
  modified_base 23^24: mod_base = OTHER; note = phosphorothioate bond between nucleosides
aaagcatgccatcacctcccctgt

SEQ ID NO: 83 - RNA, 24 nt, synthetic construct
  source 1..24: mol_type = other RNA
  modified_base 1: mod_base = OTHER; note = 2'-O-methyladenosine
  modified_base 2: mod_base = OTHER; note = 2'-O,4'-C-methylene-briged adenosine
  modified_base 3: mod_base = OTHER; note = 2'-O-methyladenosine
  modified_base 4: mod_base = OTHER; note = 2'-O,4'-C-methylene-briged guanosine
  modified_base 5: mod_base = cm
  modified_base 6: mod_base = OTHER; note = 2'-deoxy-2'-fluoroadenosine
  modified_base 7: mod_base = OTHER; note = 2'-deoxy-2'-fluorouridine
  modified_base 8: mod_base = gm
  modified_base 9: mod_base = cm
  modified_base 10: mod_base = OTHER; note = 2'-deoxycytidine
  modified_base 11: mod_base = OTHER; note = 2'-deoxyadenosine
  modified_base 12: mod_base = um
  modified_base 13: mod_base = OTHER; note = 2'-deoxy-2'-fluorocytidine
  modified_base 14: mod_base = OTHER; note = 2'-O-methyladenosine
  modified_base 15: mod_base = OTHER; note = 2'-deoxy-2'-fluorocytidine
  modified_base 16: mod_base = cm
  modified_base 17: mod_base = OTHER; note = 2'-deoxy-2'-fluorouridine
  modified_base 18: mod_base = cm
  modified_base 19: mod_base = OTHER; note = 2'-deoxy-2'-fluorocytidine
  modified_base 20: mod_base = cm
  modified_base 21: mod_base = OTHER; note = 2'-O,4'-C-methylene-briged cytidine
  modified_base 22: mod_base = um
  modified_base 23: mod_base = OTHER; note = 2'-O,4'-C-methylene-briged guanosine
  modified_base 24: mod_base = um
  modified_base 1^2: mod_base = OTHER; note = phosphorotioate bond between nucleosides
  modified_base 2^3: mod_base = OTHER; note = phosphorothioate bond between nucleosides
  modified_base 3^4: mod_base = OTHER; note = phosphorothioate bond between nucleosides
  modified_base 4^5: mod_base = OTHER; note = phosphorothioate bond between nucleosides
  modified_base 5^6: mod_base = OTHER; note = phosphorothioate bond between nucleosides
  modified_base 7^8: mod_base = OTHER; note = phosphorothioate bond between nucleosides
  modified_base 6^7: mod_base = OTHER; note = phosphorothioate bond between nucleosides
  modified_base 8^9: mod_base = OTHER; note = phosphorothioate bond between nucleosides
  modified_base 9^10: mod_base = OTHER; note = phosphorothioate bond between nucleosides
  modified_base 10^11: mod_base = OTHER; note = phosphorothioate bond between nucleosides
  modified_base 11^12: mod_base = OTHER; note = phosphorothioate bond between nucleosides
  modified_base 12^13: mod_base = OTHER; note = phosphorothioate bond between nucleosides
  modified_base 13^14: mod_base = OTHER; note = phosphorothioate bond between nucleosides
  modified_base 14^15: mod_base = OTHER; note = propylphosphate bond between nucleosides
  modified_base 15^16: mod_base = OTHER; note = phosphorothioate bond between nucleosides
  modified_base 16^17: mod_base = OTHER; note = phosphorothioate bond between nucleosides
  modified_base 17^18: mod_base = OTHER; note = phosphorothioate bond between nucleosides
  modified_base 18^19: mod_base = OTHER; note = phosphorothioate bond between nucleosides
  modified_base 19^20: mod_base = OTHER; note = phosphorothioate bond between nucleosides
  modified_base 20^21: mod_base = OTHER; note = phosphorothioate bond between nucleosides
  modified_base 21^22: mod_base = OTHER; note = phosphorothioate bond between nucleosides
  modified_base 22^23: mod_base = OTHER; note = phosphorothioate bond between nucleosides
  modified_base 23^24: mod_base = OTHER; note = phosphorothioate bond between nucleosides
aaagcatgccatcacctcccctgt

SEQ ID NO: 84 - RNA, 24 nt, synthetic construct
  source 1..24: mol_type = other RNA
  modified_base 1: mod_base = OTHER; note = 2'-O-methyladenosine
  modified_base 2: mod_base = OTHER; note = 2'-O,4'-C-methylene-briged adenosine
  modified_base 3: mod_base = OTHER; note = 2'-O-methyladenosine
  modified_base 4: mod_base = OTHER; note = 2'-O,4'-C-methylene-briged guanosine
  modified_base 5: mod_base = cm
  modified_base 6: mod_base = OTHER; note = 2'-deoxy-2'-fluoroadenosine
  modified_base 7: mod_base = OTHER; note = 2'-deoxy-2'-fluorouridine
  modified_base 8: mod_base = gm
  modified_base 9: mod_base = cm
  modified_base 10: mod_base = OTHER; note = 2'-deoxycytidine
  modified_base 11: mod_base = OTHER; note = 2'-deoxyadenosine
  modified_base 12: mod_base = um
  modified_base 13: mod_base = OTHER; note = 2'-deoxy-2'-fluorocytidine
  modified_base 14: mod_base = OTHER; note = 2'-O-methyladenosine
  modified_base 15: mod_base = OTHER; note = 2'-deoxy-2'-fluorocytidine
  modified_base 16: mod_base = cm
  modified_base 17: mod_base = OTHER; note = 2'-deoxy-2'-fluorouridine
  modified_base 18: mod_base = cm
  modified_base 19: mod_base = OTHER; note = 2'-deoxy-2'-fluorocytidine
  modified_base 20: mod_base = cm
  modified_base 21: mod_base = OTHER; note = 2'-O,4'-C-methylene-briged cytidine
  modified_base 22: mod_base = um
  modified_base 23: mod_base = OTHER; note = 2'-O,4'-C-methylene-briged guanosine
  modified_base 24: mod_base = um
  modified_base 1^2: mod_base = OTHER; note = phosphorotioate bond between nucleosides
  modified_base 2^3: mod_base = OTHER; note = phosphorothioate bond between nucleosides
  modified_base 3^4: mod_base = OTHER; note = phosphorothioate bond between nucleosides
  modified_base 4^5: mod_base = OTHER; note = phosphorothioate bond between nucleosides
  modified_base 5^6: mod_base = OTHER; note = phosphorothioate bond between nucleosides
  modified_base 7^8: mod_base = OTHER; note = phosphorothioate bond between nucleosides
  modified_base 6^7: mod_base = OTHER; note = phosphorothioate bond between nucleosides
  modified_base 8^9: mod_base = OTHER; note = phosphorothioate bond between nucleosides
  modified_base 9^10: mod_base = OTHER; note = phosphorothioate bond between nucleosides
  modified_base 10^11: mod_base = OTHER; note = phosphorothioate bond between nucleosides
  modified_base 11^12: mod_base = OTHER; note = phosphorothioate bond between nucleosides
  modified_base 12^13: mod_base = OTHER; note = phosphorothioate bond between nucleosides
  modified_base 13^14: mod_base = OTHER; note = phosphorothioate bond between nucleosides
  modified_base 14^15: mod_base = OTHER; note = butylphosphate bond between nucleosides
  modified_base 15^16: mod_base = OTHER; note = phosphorothioate bond between nucleosides
  modified_base 16^17: mod_base = OTHER; note = phosphorothioate bond between nucleosides
  modified_base 17^18: mod_base = OTHER; note = phosphorothioate bond between nucleosides
  modified_base 18^19: mod_base = OTHER; note = phosphorothioate bond between nucleosides
  modified_base 19^20: mod_base = OTHER; note = phosphorothioate bond between nucleosides
  modified_base 20^21: mod_base = OTHER; note = phosphorothioate bond between nucleosides
  modified_base 21^22: mod_base = OTHER; note = phosphorothioate bond between nucleosides
  modified_base 22^23: mod_base = OTHER; note = phosphorothioate bond between nucleosides
  modified_base 23^24: mod_base = OTHER; note = phosphorothioate bond between nucleosides
aaagcatgccatcacctcccctgt

SEQ ID NO: 85 - RNA, 24 nt, synthetic construct
  source 1..24: mol_type = other RNA
  modified_base 1: mod_base = OTHER; note = 2'-O-methyladenosine
  modified_base 2: mod_base = OTHER; note = 2'-O,4'-C-methylene-briged adenosine
  modified_base 3: mod_base = OTHER; note = 2'-O-methyladenosine
  modified_base 4: mod_base = OTHER; note = 2'-O,4'-C-methylene-briged guanosine
  modified_base 5: mod_base = cm
  modified_base 6: mod_base = OTHER; note = 2'-deoxy-2'-fluoroadenosine
  modified_base 7: mod_base = OTHER; note = 2'-deoxy-2'-fluorouridine
  modified_base 8: mod_base = gm
  modified_base 9: mod_base = cm
  modified_base 10: mod_base = OTHER; note = 2'-deoxycytidine
  modified_base 11: mod_base = OTHER; note = 2'-deoxyadenosine
  modified_base 12: mod_base = um
  modified_base 13: mod_base = OTHER; note = 2'-deoxy-2'-fluorocytidine
  modified_base 14: mod_base = OTHER; note = 2'-O-methyladenosine
  modified_base 15: mod_base = OTHER; note = 2'-deoxy-2'-fluorocytidine
  modified_base 16: mod_base = cm
  modified_base 17: mod_base = OTHER; note = 2'-deoxy-2'-fluorouridine
  modified_base 18: mod_base = cm
  modified_base 19: mod_base = OTHER; note = 2'-deoxy-2'-fluorocytidine
  modified_base 20: mod_base = cm
  modified_base 21: mod_base = OTHER; note = 2'-O,4'-C-methylene-briged cytidine
  modified_base 22: mod_base = um
  modified_base 23: mod_base = OTHER; note = 2'-O,4'-C-methylene-briged guanosine
  modified_base 24: mod_base = um
  modified_base 1^2: mod_base = OTHER; note = phosphorotioate bond between nucleosides
  modified_base 2^3: mod_base = OTHER; note = phosphorothioate bond between nucleosides
  modified_base 3^4: mod_base = OTHER; note = phosphorothioate bond between nucleosides
  modified_base 4^5: mod_base = OTHER; note = phosphorothioate bond between nucleosides
  modified_base 5^6: mod_base = OTHER; note = phosphorothioate bond between nucleosides
  modified_base 7^8: mod_base = OTHER; note = phosphorothioate bond between nucleosides
  modified_base 6^7: mod_base = OTHER; note = phosphorothioate bond between nucleosides
  modified_base 8^9: mod_base = OTHER; note = phosphorothioate bond between nucleosides
  modified_base 9^10: mod_base = OTHER; note = phosphorothioate bond between nucleosides
  modified_base 10^11: mod_base = OTHER; note = phosphorothioate bond between nucleosides
  modified_base 11^12: mod_base = OTHER; note = phosphorohioate bond between nucleosides
  modified_base 12^13: mod_base = OTHER; note = phosphorothioate bond between nucleosides
  modified_base 13^14: mod_base = OTHER; note = phosphorothioate bond between nucleosides
  modified_base 14^15: mod_base = OTHER; note = methoxyethylphosphate bond between nucleosides
  modified_base 15^16: mod_base = OTHER; note = phosphorothioate bond between nucleosides
  modified_base 16^17: mod_base = OTHER; note = phosphorothioate bond between nucleosides
  modified_base 17^18: mod_base = OTHER; note = phosphorothioate bond between nucleosides
  modified_base 18^19: mod_base = OTHER; note = phosphorothioate bond between nucleosides
  modified_base 19^20: mod_base = OTHER; note = phosphorothioate bond between nucleosides
  modified_base 20^21: mod_base = OTHER; note = phosphorothioate bond between nucleosides
  modified_base 21^22: mod_base = OTHER; note = phosphorothioate bond between nucleosides
  modified_base 22^23: mod_base = OTHER; note = phosphorothioate bond between nucleosides
  modified_base 23^24: mod_base = OTHER; note = phosphorothioate bond between nucleosides
aaagcatgccatcacctcccctgt

SEQ ID NO: 86 - RNA, 24 nt, synthetic construct
  source 1..24: mol_type = other RNA
  modified_base 1: mod_base = OTHER; note = 2'-O-methyladenosine
  modified_base 2: mod_base = OTHER; note = 2'-O,4'-C-methylene-briged adenosine
  modified_base 3: mod_base = OTHER; note = 2'-O-methyladenosine
  modified_base 4: mod_base = OTHER; note = 2'-O,4'-C-methylene-briged guanosine
  modified_base 5: mod_base = cm
  modified_base 6: mod_base = OTHER; note = 2'-deoxy-2'-fluoroadenosine
  modified_base 7: mod_base = OTHER; note = 2'-deoxy-2'-fluorouridine
  modified_base 8: mod_base = gm
  modified_base 9: mod_base = cm
  modified_base 10: mod_base = OTHER; note = 2'-deoxycytidine
  modified_base 11: mod_base = OTHER; note = 2'-deoxyadenosine
  modified_base 12: mod_base = um
  modified_base 13: mod_base = OTHER; note = 2'-deoxy-2'-fluorocytidine
  modified_base 14: mod_base = OTHER; note = 2'-O-methyladenosine
  modified_base 15: mod_base = OTHER; note = 2'-deoxy-2'-fluorocytidine
  modified_base 16: mod_base = cm
  modified_base 17: mod_base = OTHER; note = 2'-deoxy-2'-fluorouridine
  modified_base 18: mod_base = cm
  modified_base 19: mod_base = OTHER; note = 2'-deoxy-2'-fluorocytidine
  modified_base 20: mod_base = cm
  modified_base 21: mod_base = OTHER; note = 2'-O,4'-C-methylene-briged cytidine
  modified_base 22: mod_base = um
  modified_base 23: mod_base = OTHER; note = 2'-O,4'-C-methylene-briged guanosine
  modified_base 24: mod_base = um
  modified_base 1^2: mod_base = OTHER; note = phosphorotioate bond between nucleosides
  modified_base 2^3: mod_base = OTHER; note = phosphorothioate bond between nucleosides
  modified_base 3^4: mod_base = OTHER; note = phosphorothioate bond between nucleosides
  modified_base 4^5: mod_base = OTHER; note = phosphorothioate bond between nucleosides
  modified_base 5^6: mod_base = OTHER; note = phosphorothioate bond between nucleosides
  modified_base 7^8: mod_base = OTHER; note = phosphorothioate bond between nucleosides
  modified_base 6^7: mod_base = OTHER; note = phosphorothioate bond between nucleosides
  modified_base 8^9: mod_base = OTHER; note = phosphorothioate bond between nucleosides
  modified_base 9^10: mod_base = OTHER; note = phosphorothioate bond between nucleosides
  modified_base 10^11: mod_base = OTHER; note = phosphorothioate bond between nucleosides
  modified_base 11^12: mod_base = OTHER; note = phosphorothioate bond between nucleosides
  modified_base 12^13: mod_base = OTHER; note = phosphorothioate bond between nucleosides
  modified_base 13^14: mod_base = OTHER; note = phosphorothioate bond between nucleosides
  modified_base 14^15: mod_base = OTHER; note = cyclopropylphosphate bond between nucleosides
  modified_base 15^16: mod_base = OTHER; note = phosphorothioate bond between nucleosides
  modified_base 16^17: mod_base = OTHER; note = phosphorothioate bond between nucleosides
  modified_base 17^18: mod_base = OTHER; note = phosphorothioate bond between nucleosides
  modified_base 18^19: mod_base = OTHER; note = phosphorothioate bond between nucleosides
  modified_base 19^20: mod_base = OTHER; note = phosphorothioate bond between nucleosides
  modified_base 20^21: mod_base = OTHER; note = phosphorothioate bond between nucleosides
  modified_base 21^22: mod_base = OTHER; note = phosphorothioate bond between nucleosides
  modified_base 22^23: mod_base = OTHER; note = phosphorothioate bond between nucleosides
  modified_base 23^24: mod_base = OTHER; note = phosphorothioate bond between nucleosides
aaagcatgccatcacctcccctgt

SEQ ID NO: 87 - RNA, 24 nt, synthetic construct
  source 1..24: mol_type = other RNA
  modified_base 1: mod_base = OTHER; note = 2'-O-methyladenosine
  modified_base 2: mod_base = OTHER; note = 2'-O,4'-C-methylene-briged adenosine
  modified_base 3: mod_base = OTHER; note = 2'-O-methyladenosine
  modified_base 4: mod_base = OTHER; note = 2'-O,4'-C-methylene-briged guanosine
  modified_base 5: mod_base = cm
  modified_base 6: mod_base = OTHER; note = 2'-deoxy-2'-fluoroadenosine
  modified_base 7: mod_base = OTHER; note = 2'-deoxy-2'-fluorouridine
  modified_base 8: mod_base = gm
  modified_base 9: mod_base = cm
  modified_base 10: mod_base = OTHER; note = 2'-deoxycytidine
  modified_base 11: mod_base = OTHER; note = 2'-deoxyadenosine
  modified_base 12: mod_base = um
  modified_base 13: mod_base = OTHER; note = 2'-deoxy-2'-fluorocytidine
  modified_base 14: mod_base = OTHER; note = 2'-O-methyladenosine
  modified_base 15: mod_base = OTHER; note = 2'-deoxy-2'-fluorocytidine
  modified_base 16: mod_base = cm
  modified_base 17: mod_base = OTHER; note = 2'-deoxy-2'-fluorouridine
  modified_base 18: mod_base = cm
  modified_base 19: mod_base = OTHER; note = 2'-deoxy-2'-fluorocytidine
  modified_base 20: mod_base = cm
  modified_base 21: mod_base = OTHER; note = 2'-O,4'-C-methylene-briged cytidine
  modified_base 22: mod_base = um
  modified_base 23: mod_base = OTHER; note = 2'-O,4'-C-methylene-briged guanosine
  modified_base 24: mod_base = um
  modified_base 1^2: mod_base = OTHER; note = phosphorotioate bond between nucleosides
  modified_base 2^3: mod_base = OTHER; note = phosphorothioate bond between nucleosides
  modified_base 3^4: mod_base = OTHER; note = phosphorothioate bond between nucleosides
  modified_base 4^5: mod_base = OTHER; note = phosphorothioate bond between nucleosides
  modified_base 5^6: mod_base = OTHER; note = phosphorothioate bond between nucleosides
  modified_base 7^8: mod_base = OTHER; note = phosphorothioate bond between nucleosides
  modified_base 6^7: mod_base = OTHER; note = phosphorothioate bond between nucleosides
  modified_base 8^9: mod_base = OTHER; note = phosphorothioate bond between nucleosides
  modified_base 9^10: mod_base = OTHER; note = phosphorothioate bond between nucleosides
  modified_base 10^11: mod_base = OTHER; note = phosphorothioate bond between nucleosides
  modified_base 11^12: mod_base = OTHER; note = phosphorothioate bond between nucleosides
  modified_base 12^13: mod_base = OTHER; note = phosphorothioate bond between nucleosides
  modified_base 13^14: mod_base = OTHER; note = phosphorothioate bond between nucleosides
  modified_base 14^15: mod_base = OTHER; note = cyclobutylphosphate bond between nucleosides
  modified_base 15^16: mod_base = OTHER; note = phosphorothioate bond between nucleosides
  modified_base 16^17: mod_base = OTHER; note = phosphorothioate bond between nucleosides
  modified_base 17^18: mod_base = OTHER; note = phosphorothioate bond between nucleosides
  modified_base 18^19: mod_base = OTHER; note = phosphorothioate bond between nucleosides
  modified_base 19^20: mod_base = OTHER; note = phosphorothioate bond between nucleosides
  modified_base 20^21: mod_base = OTHER; note = phosphorothioate bond between nucleosides
  modified_base 21^22: mod_base = OTHER; note = phosphorothioate bond between nucleosides
  modified_base 22^23: mod_base = OTHER; note = phosphorothioate bond between nucleosides
  modified_base 23^24: mod_base = OTHER; note = phosphorothioate bond between nucleosides
aaagcatgccatcacctcccctgt

SEQ ID NO: 88 - RNA, 24 nt, synthetic construct
  source 1..24: mol_type = other RNA
  modified_base 1: mod_base = OTHER; note = 2'-O-methyladenosine
  modified_base 2: mod_base = OTHER; note = 2'-O,4'-C-methylene-briged adenosine
  modified_base 3: mod_base = OTHER; note = 2'-O-methyladenosine
  modified_base 4: mod_base = OTHER; note = 2'-O,4'-C-methylene-briged guanosine
  modified_base 5: mod_base = cm
  modified_base 6: mod_base = OTHER; note = 2'-deoxy-2'-fluoroadenosine
  modified_base 7: mod_base = OTHER; note = 2'-deoxy-2'-fluorouridine
  modified_base 8: mod_base = gm
  modified_base 9: mod_base = cm
  modified_base 10: mod_base = OTHER; note = 2'-deoxycytidine
  modified_base 11: mod_base = OTHER; note = 2'-deoxyadenosine
  modified_base 12: mod_base = um
  modified_base 13: mod_base = OTHER; note = 2'-deoxy-2'-fluorocytidine
  modified_base 14: mod_base = OTHER; note = 2'-O-methyladenosine
  modified_base 15: mod_base = OTHER; note = 2'-deoxy-2'-fluorocytidine
  modified_base 16: mod_base = cm
  modified_base 17: mod_base = OTHER; note = 2'-deoxy-2'-fluorouridine
  modified_base 18: mod_base = cm
  modified_base 19: mod_base = OTHER; note = 2'-deoxy-2'-fluorocytidine
  modified_base 20: mod_base = cm
  modified_base 21: mod_base = OTHER; note = 2'-O,4'-C-methylene-briged cytidine
  modified_base 22: mod_base = um
  modified_base 23: mod_base = OTHER; note = 2'-O,4'-C-methylene-briged guanosine
  modified_base 24: mod_base = um
  modified_base 1^2: mod_base = OTHER; note = phosphorotioate bond between nucleosides
  modified_base 2^3: mod_base = OTHER; note = phosphorothioate bond between nucleosides
  modified_base 3^4: mod_base = OTHER; note = phosphorothioate bond between nucleosides
  modified_base 4^5: mod_base = OTHER; note = phosphorothioate bond between nucleosides
  modified_base 5^6: mod_base = OTHER; note = phosphorothioate bond between nucleosides
  modified_base 7^8: mod_base = OTHER; note = phosphorothioate bond between nucleosides
  modified_base 6^7: mod_base = OTHER; note = phosphorothioate bond between nucleosides
  modified_base 8^9: mod_base = OTHER; note = phosphorothioate bond between nucleosides
  modified_base 9^10: mod_base = OTHER; note = phosphorothioate bond between nucleosides
  modified_base 10^11: mod_base = OTHER; note = phosphorothioate bond between nucleosides
  modified_base 11^12: mod_base = OTHER; note = propylphosphate bond between nucleosides
  modified_base 12^13: mod_base = OTHER; note = phosphorothioate bond between nucleosides
  modified_base 13^14: mod_base = OTHER; note = phosphorothioate bond between nucleosides
  modified_base 14^15: mod_base = OTHER; note = phosphorothioate bond between nucleosides
  modified_base 15^16: mod_base = OTHER; note = phosphorothioate bond between nucleosides
  modified_base 16^17: mod_base = OTHER; note = phosphorothioate bond between nucleosides
  modified_base 17^18: mod_base = OTHER; note = phosphorothioate bond between nucleosides
  modified_base 18^19: mod_base = OTHER; note = phosphorothioate bond between nucleosides
  modified_base 19^20: mod_base = OTHER; note = phosphorothioate bond between nucleosides
  modified_base 20^21: mod_base = OTHER; note = phosphorothioate bond between nucleosides
  modified_base 21^22: mod_base = OTHER; note = phosphorothioate bond between nucleosides
  modified_base 22^23: mod_base = OTHER; note = phosphorothioate bond between nucleosides
  modified_base 23^24: mod_base = OTHER; note = phosphorothioate bond between nucleosides
aaagcatgccatcacctcccctgt

SEQ ID NO: 89 - RNA, 24 nt, synthetic construct
  source 1..24: mol_type = other RNA
  modified_base 1: mod_base = OTHER; note = 2'-O-methyladenosine
  modified_base 2: mod_base = OTHER; note = 2'-O,4'-C-methylene-briged adenosine
  modified_base 3: mod_base = OTHER; note = 2'-O-methyladenosine
  modified_base 4: mod_base = OTHER; note = 2'-O,4'-C-methylene-briged guanosine
  modified_base 5: mod_base = cm
  modified_base 6: mod_base = OTHER; note = 2'-deoxy-2'-fluoroadenosine
  modified_base 7: mod_base = OTHER; note = 2'-deoxy-2'-fluorouridine
  modified_base 8: mod_base = gm
  modified_base 9: mod_base = cm
  modified_base 10: mod_base = OTHER; note = 2'-deoxycytidine
  modified_base 11: mod_base = OTHER; note = 2'-deoxyadenosine
  modified_base 12: mod_base = um
  modified_base 13: mod_base = OTHER; note = 2'-deoxy-2'-fluorocytidine
  modified_base 14: mod_base = OTHER; note = 2'-O-methyladenosine
  modified_base 15: mod_base = OTHER; note = 2'-deoxy-2'-fluorocytidine
  modified_base 16: mod_base = cm
  modified_base 17: mod_base = OTHER; note = 2'-deoxy-2'-fluorouridine
  modified_base 18: mod_base = cm
  modified_base 19: mod_base = OTHER; note = 2'-deoxy-2'-fluorocytidine
  modified_base 20: mod_base = cm
  modified_base 21: mod_base = OTHER; note = 2'-O,4'-C-methylene-briged cytidine
  modified_base 22: mod_base = um
  modified_base 23: mod_base = OTHER; note = 2'-O,4'-C-methylene-briged guanosine
  modified_base 24: mod_base = um
  modified_base 1^2: mod_base = OTHER; note = phosphorotioate bond between nucleosides
  modified_base 2^3: mod_base = OTHER; note = phosphorothioate bond between nucleosides
  modified_base 3^4: mod_base = OTHER; note = phosphorothioate bond between nucleosides
  modified_base 4^5: mod_base = OTHER; note = phosphorothioate bond between nucleosides
  modified_base 5^6: mod_base = OTHER; note = phosphorothioate bond between nucleosides
  modified_base 7^8: mod_base = OTHER; note = phosphorothioate bond between nucleosides
  modified_base 6^7: mod_base = OTHER; note = phosphorothioate bond between nucleosides
  modified_base 8^9: mod_base = OTHER; note = phosphorothioate bond between nucleosides
  modified_base 9^10: mod_base = OTHER; note = phosphorothioate bond between nucleosides
  modified_base 10^11: mod_base = OTHER; note = phosphorothioate bond between nucleosides
  modified_base 11^12: mod_base = OTHER; note = butylphosphate bond between nucleosides
  modified_base 12^13: mod_base = OTHER; note = phosphorothioate bond between nucleosides
  modified_base 13^14: mod_base = OTHER; note = phosphorothioate bond between nucleosides
  modified_base 14^15: mod_base = OTHER; note = phosphorothioate bond between nucleosides
  modified_base 15^16: mod_base = OTHER; note = phosphorothioate bond between nucleosides
  modified_base 16^17: mod_base = OTHER; note = phosphorothioate bond between nucleosides
  modified_base 17^18: mod_base = OTHER; note = phosphorothioate bond between nucleosides
  modified_base 18^19: mod_base = OTHER; note = phosphorothioate bond between nucleosides
  modified_base 19^20: mod_base = OTHER; note = phosphorothioate bond between nucleosides
  modified_base 20^21: mod_base = OTHER; note = phosphorothioate bond between nucleosides
  modified_base 21^22: mod_base = OTHER; note = phosphorothioate bond between nucleosides
  modified_base 22^23: mod_base = OTHER; note = phosphorothioate bond between nucleosides
  modified_base 23^24: mod_base = OTHER; note = phosphorothioate bond between nucleosides
aaagcatgccatcacctcccctgt

SEQ ID NO: 90 - RNA, 24 nt, synthetic construct
  source 1..24: mol_type = other RNA
  modified_base 1: mod_base = OTHER; note = 2'-O-methyladenosine
  modified_base 2: mod_base = OTHER; note = 2'-O,4'-C-methylene-briged adenosine
  modified_base 3: mod_base = OTHER; note = 2'-O-methyladenosine
  modified_base 4: mod_base = OTHER; note = 2'-O,4'-C-methylene-briged guanosine
  modified_base 5: mod_base = cm
  modified_base 6: mod_base = OTHER; note = 2'-deoxy-2'-fluoroadenosine
  modified_base 7: mod_base = OTHER; note = 2'-deoxy-2'-fluorouridine
  modified_base 8: mod_base = gm
  modified_base 9: mod_base = cm
  modified_base 10: mod_base = OTHER; note = 2'-deoxycytidine
  modified_base 11: mod_base = OTHER; note = 2'-deoxyadenosine
  modified_base 12: mod_base = um
  modified_base 13: mod_base = OTHER; note = 2'-deoxy-2'-fluorocytidine
  modified_base 14: mod_base = OTHER; note = 2'-O-methyladenosine
  modified_base 15: mod_base = OTHER; note = 2'-deoxy-2'-fluorocytidine
  modified_base 16: mod_base = cm
  modified_base 17: mod_base = OTHER; note = 2'-deoxy-2'-fluorouridine
  modified_base 18: mod_base = cm
  modified_base 19: mod_base = OTHER; note = 2'-deoxy-2'-fluorocytidine
  modified_base 20: mod_base = cm
  modified_base 21: mod_base = OTHER; note = 2'-O,4'-C-methylene-briged cytidine
  modified_base 22: mod_base = um
  modified_base 23: mod_base = OTHER; note = 2'-O,4'-C-methylene-briged guanosine
  modified_base 24: mod_base = um
  modified_base 1^2: mod_base = OTHER; note = phosphorotioate bond between nucleosides
  modified_base 2^3: mod_base = OTHER; note = phosphorothioate bond between nucleosides
  modified_base 3^4: mod_base = OTHER; note = phosphorothioate bond between nucleosides
  modified_base 4^5: mod_base = OTHER; note = phosphorothioate bond between nucleosides
  modified_base 5^6: mod_base = OTHER; note = phosphorothioate bond between nucleosides
  modified_base 7^8: mod_base = OTHER; note = phosphorothioate bond between nucleosides
  modified_base 6^7: mod_base = OTHER; note = phosphorothioate bond between nucleosides
  modified_base 8^9: mod_base = OTHER; note = phosphorothioate bond between nucleosides
  modified_base 9^10: mod_base = OTHER; note = phosphorothioate bond between nucleosides
  modified_base 10^11: mod_base = OTHER; note = phosphorothioate bond between nucleosides
  modified_base 11^12: mod_base = OTHER; note = methoxylethylphosphate bond between nucleosides
  modified_base 12^13: mod_base = OTHER; note = phosphorothioate bond between nucleosides
  modified_base 13^14: mod_base = OTHER; note = phosphorothioate bond between nucleosides
  modified_base 14^15: mod_base = OTHER; note = phosphorothioate bond between nucleosides
  modified_base 15^16: mod_base = OTHER; note = phosphorothioate bond between nucleosides
  modified_base 16^17: mod_base = OTHER; note = phosphorothioate bond between nucleosides
  modified_base 17^18: mod_base = OTHER; note = phosphorothioate bond between nucleosides
  modified_base 18^19: mod_base = OTHER; note = phosphorothioate bond between nucleosides
  modified_base 19^20: mod_base = OTHER; note = phosphorothioate bond between nucleosides
  modified_base 20^21: mod_base = OTHER; note = phosphorothioate bond between nucleosides
  modified_base 21^22: mod_base = OTHER; note = phosphorothioate bond between nucleosides
  modified_base 22^23: mod_base = OTHER; note = phosphorothioate bond between nucleosides
  modified_base 23^24: mod_base = OTHER; note = phosphorothioate bond between nucleosides
aaagcatgccatcacctcccctgt

SEQ ID NO: 91 - RNA, 24 nt, synthetic construct
  source 1..24: mol_type = other RNA
  modified_base 1: mod_base = OTHER; note = 2'-O-methyladenosine
  modified_base 2: mod_base = OTHER; note = 2'-O,4'-C-methylene-briged adenosine
  modified_base 3: mod_base = OTHER; note = 2'-O-methyladenosine
  modified_base 4: mod_base = OTHER; note = 2'-O,4'-C-methylene-briged guanosine
  modified_base 5: mod_base = cm
  modified_base 6: mod_base = OTHER; note = 2'-deoxy-2'-fluoroadenosine
  modified_base 7: mod_base = OTHER; note = 2'-deoxy-2'-fluorouridine
  modified_base 8: mod_base = gm
  modified_base 9: mod_base = cm
  modified_base 10: mod_base = OTHER; note = 2'-deoxycytidine
  modified_base 11: mod_base = OTHER; note = 2'-deoxyadenosine
  modified_base 12: mod_base = um
  modified_base 13: mod_base = OTHER; note = 2'-deoxy-2'-fluorocytidine
  modified_base 14: mod_base = OTHER; note = 2'-O-methyladenosine
  modified_base 15: mod_base = OTHER; note = 2'-deoxy-2'-fluorocytidine
  modified_base 16: mod_base = cm
  modified_base 17: mod_base = OTHER; note = 2'-deoxy-2'-fluorouridine
  modified_base 18: mod_base = cm
  modified_base 19: mod_base = OTHER; note = 2'-deoxy-2'-fluorocytidine
  modified_base 20: mod_base = cm
  modified_base 21: mod_base = OTHER; note = 2'-O,4'-C-methylene-briged cytidine
  modified_base 22: mod_base = um
  modified_base 23: mod_base = OTHER; note = 2'-O,4'-C-methylene-briged guanosine
  modified_base 24: mod_base = um
  modified_base 1^2: mod_base = OTHER; note = phosphorotioate bond between nucleosides
  modified_base 2^3: mod_base = OTHER; note = phosphorothioate bond between nucleosides
  modified_base 3^4: mod_base = OTHER; note = phosphorothioate bond between nucleosides
  modified_base 4^5: mod_base = OTHER; note = phosphorothioate bond between nucleosides
  modified_base 5^6: mod_base = OTHER; note = phosphorothioate bond between nucleosides
  modified_base 7^8: mod_base = OTHER; note = phosphorothioate bond between nucleosides
  modified_base 6^7: mod_base = OTHER; note = phosphorothioate bond between nucleosides
  modified_base 8^9: mod_base = OTHER; note = phosphorothioate bond between nucleosides
  modified_base 9^10: mod_base = OTHER; note = phosphorothioate bond between nucleosides
  modified_base 10^11: mod_base = OTHER; note = phosphorothioate bond between nucleosides
  modified_base 11^12: mod_base = OTHER; note = cyclopropylphosphate bond between nucleosides
  modified_base 12^13: mod_base = OTHER; note = phosphorothioate bond between nucleosides
  modified_base 13^14: mod_base = OTHER; note = phosphorothioate bond between nucleosides
  modified_base 14^15: mod_base = OTHER; note = phosphorothioate bond between nucleosides
  modified_base 15^16: mod_base = OTHER; note = phosphorothioate bond between nucleosides
  modified_base 16^17: mod_base = OTHER; note = phosphorothioate bond between nucleosides
  modified_base 17^18: mod_base = OTHER; note = phosphorothioate bond between nucleosides
  modified_base 18^19: mod_base = OTHER; note = phosphorothioate bond between nucleosides
  modified_base 19^20: mod_base = OTHER; note = phosphorothioate bond between nucleosides
  modified_base 20^21: mod_base = OTHER; note = phosphorothioate bond between nucleosides
  modified_base 21^22: mod_base = OTHER; note = phosphorothioate bond between nucleosides
  modified_base 22^23: mod_base = OTHER; note = phosphorothioate bond between nucleosides
  modified_base 23^24: mod_base = OTHER; note = phosphorothioate bond between nucleosides
aaagcatgccatcacctcccctgt

SEQ ID NO: 92 - RNA, 24 nt, synthetic construct
  source 1..24: mol_type = other RNA
  modified_base 1: mod_base = OTHER; note = 2'-O-methyladenosine
  modified_base 2: mod_base = OTHER; note = 2'-O,4'-C-methylene-briged adenosine
  modified_base 3: mod_base = OTHER; note = 2'-O-methyladenosine
  modified_base 4: mod_base = OTHER; note = 2'-O,4'-C-methylene-briged guanosine
  modified_base 5: mod_base = cm
  modified_base 6: mod_base = OTHER; note = 2'-deoxy-2'-fluoroadenosine
  modified_base 7: mod_base = OTHER; note = 2'-deoxy-2'-fluorouridine
  modified_base 8: mod_base = gm
  modified_base 9: mod_base = cm
  modified_base 10: mod_base = OTHER; note = 2'-deoxycytidine
  modified_base 11: mod_base = OTHER; note = 2'-deoxyadenosine
  modified_base 12: mod_base = um
  modified_base 13: mod_base = OTHER; note = 2'-deoxy-2'-fluorocytidine
  modified_base 14: mod_base = OTHER; note = 2'-O-methyladenosine
  modified_base 15: mod_base = OTHER; note = 2'-deoxy-2'-fluorocytidine
  modified_base 16: mod_base = cm
  modified_base 17: mod_base = OTHER; note = 2'-deoxy-2'-fluorouridine
  modified_base 18: mod_base = cm
  modified_base 19: mod_base = OTHER; note = 2'-deoxy-2'-fluorocytidine
  modified_base 20: mod_base = cm
  modified_base 21: mod_base = OTHER; note = 2'-O,4'-C-methylene-briged cytidine
  modified_base 22: mod_base = um
  modified_base 23: mod_base = OTHER; note = 2'-O,4'-C-methylene-briged guanosine
  modified_base 24: mod_base = um
  modified_base 1^2: mod_base = OTHER; note = phosphorotioate bond between nucleosides
  modified_base 2^3: mod_base = OTHER; note = phosphorothioate bond between nucleosides
  modified_base 3^4: mod_base = OTHER; note = phosphorothioate bond between nucleosides
  modified_base 4^5: mod_base = OTHER; note = phosphorothioate bond between nucleosides
  modified_base 5^6: mod_base = OTHER; note = phosphorothioate bond between nucleosides
  modified_base 7^8: mod_base = OTHER; note = phosphorothioate bond between nucleosides
  modified_base 6^7: mod_base = OTHER; note = phosphorothioate bond between nucleosides
  modified_base 8^9: mod_base = OTHER; note = phosphorothioate bond between nucleosides
  modified_base 9^10: mod_base = OTHER; note = phosphorothioate bond between nucleosides
  modified_base 10^11: mod_base = OTHER; note = phosphorothioate bond between nucleosides
  modified_base 11^12: mod_base = OTHER; note = cyclobutylphosphate bond between nucleosides
  modified_base 12^13: mod_base = OTHER; note = phosphorothioate bond between nucleosides
  modified_base 13^14: mod_base = OTHER; note = phosphorothioate bond between nucleosides
  modified_base 14^15: mod_base = OTHER; note = phosphorothioate bond between nucleosides
  modified_base 15^16: mod_base = OTHER; note = phosphorothioate bond between nucleosides
  modified_base 16^17: mod_base = OTHER; note = phosphorothioate bond between nucleosides
  modified_base 17^18: mod_base = OTHER; note = phosphorothioate bond between nucleosides
  modified_base 18^19: mod_base = OTHER; note = phosphorothioate bond between nucleosides
  modified_base 19^20: mod_base = OTHER; note = phosphorothioate bond between nucleosides
  modified_base 20^21: mod_base = OTHER; note = phosphorothioate bond between nucleosides
  modified_base 21^22: mod_base = OTHER; note = phosphorothioate bond between nucleosides
  modified_base 22^23: mod_base = OTHER; note = phosphorothioate bond between nucleosides
  modified_base 23^24: mod_base = OTHER; note = phosphorothioate bond between nucleosides
aaagcatgccatcacctcccctgt

SEQ ID NO: 93 - RNA, 24 nt, synthetic construct
  source 1..24: mol_type = other RNA
  modified_base 1: mod_base = OTHER; note = 2'-O-methyladenosine
  modified_base 2: mod_base = OTHER; note = 2'-O,4'-C-ethylene-briged adenosine
  modified_base 3: mod_base = OTHER; note = 2'-O-methyladenosine
  modified_base 4: mod_base = OTHER; note = 2'-O,4'-C-ethylene-briged guanosine
  modified_base 5: mod_base = cm
  modified_base 6: mod_base = OTHER; note = 2'-deoxy-2'-fluoroadenosine
  modified_base 7: mod_base = OTHER; note = 2'-deoxy-2'-fluorouridine
  modified_base 8: mod_base = gm
  modified_base 9: mod_base = cm
  modified_base 10: mod_base = OTHER; note = 2'-deoxycytidine
  modified_base 11: mod_base = OTHER; note = 2'-deoxyadenosine
  modified_base 12: mod_base = um
  modified_base 13: mod_base = OTHER; note = 2'-deoxy-2'-fluorocytidine
  modified_base 14: mod_base = OTHER; note = 2'-O-methyladenosine
  modified_base 15: mod_base = OTHER; note = 2'-deoxy-2'-fluorocytidine
  modified_base 16: mod_base = cm
  modified_base 17: mod_base = OTHER; note = 2'-deoxy-2'-fluorouridine
  modified_base 18: mod_base = cm
  modified_base 19: mod_base = OTHER; note = 2'-deoxy-2'-fluorocytidine
  modified_base 20: mod_base = cm
  modified_base 21: mod_base = OTHER; note = 2'-O,4'-C-ethylene-briged cytidine
  modified_base 22: mod_base = um
  modified_base 23: mod_base = OTHER; note = 2'-O,4'-C-ethylene-briged guanosine
  modified_base 24: mod_base = um
  modified_base 1^2: mod_base = OTHER; note = phosphorotioate bond between nucleosides
  modified_base 2^3: mod_base = OTHER; note = phosphorothioate bond between nucleosides
  modified_base 3^4: mod_base = OTHER; note = phosphorothioate bond between nucleosides
  modified_base 4^5: mod_base = OTHER; note = phosphorothioate bond between nucleosides
  modified_base 5^6: mod_base = OTHER; note = phosphorothioate bond between nucleosides
  modified_base 7^8: mod_base = OTHER; note = phosphorothioate bond between nucleosides
  modified_base 6^7: mod_base = OTHER; note = phosphorothioate bond between nucleosides
  modified_base 8^9: mod_base = OTHER; note = phosphorothioate bond between nucleosides
  modified_base 9^10: mod_base = OTHER; note = phosphorothioate bond between nucleosides
  modified_base 10^11: mod_base = OTHER; note = phosphorothioate bond between nucleosides
  modified_base 11^12: mod_base = OTHER; note = N-methanesulfonylphosphoramidate bond between nucleosides
  modified_base 12^13: mod_base = OTHER; note = phosphorothioate bond between nucleosides
  modified_base 13^14: mod_base = OTHER; note = phosphorothioate bond between nucleosides
  modified_base 14^15: mod_base = OTHER; note = N-methanesulfonylphosphoramidate bond between nucleosides
  modified_base 15^16: mod_base = OTHER; note = phosphorothioate bond between nucleosides
  modified_base 16^17: mod_base = OTHER; note = phosphorothioate bond between nucleosides
  modified_base 17^18: mod_base = OTHER; note = phosphorothioate bond between nucleosides
  modified_base 18^19: mod_base = OTHER; note = phosphorothioate bond between nucleosides
  modified_base 19^20: mod_base = OTHER; note = phosphorothioate bond between nucleosides
  modified_base 20^21: mod_base = OTHER; note = phosphorothioate bond between nucleosides
  modified_base 21^22: mod_base = OTHER; note = phosphorothioate bond between nucleosides
  modified_base 22^23: mod_base = OTHER; note = phosphorothioate bond between nucleosides
  modified_base 23^24: mod_base = OTHER; note = phosphorothioate bond between nucleosides
aaagcatgccatcacctcccctgt

SEQ ID NO: 94 - RNA, 24 nt, synthetic construct
  source 1..24: mol_type = other RNA
  modified_base 1: mod_base = OTHER; note = 2'-O-methyladenosine
  modified_base 2: mod_base = OTHER; note = 2'-O,4'-C-ethylene-briged adenosine
  modified_base 3: mod_base = OTHER; note = 2'-O-methyladenosine
  modified_base 4: mod_base = OTHER; note = 2'-O,4'-C-ethylene-briged guanosine
  modified_base 5: mod_base = cm
  modified_base 6: mod_base = OTHER; note = 2'-deoxy-2'-fluoroadenosine
  modified_base 7: mod_base = OTHER; note = 2'-deoxy-2'-fluorouridine
  modified_base 8: mod_base = gm
  modified_base 9: mod_base = cm
  modified_base 10: mod_base = OTHER; note = 2'-deoxycytidine
  modified_base 11: mod_base = OTHER; note = 2'-deoxyadenosine
  modified_base 12: mod_base = um
  modified_base 13: mod_base = OTHER; note = 2'-deoxy-2'-fluorocytidine
  modified_base 14: mod_base = OTHER; note = 2'-O-methyladenosine
  modified_base 15: mod_base = OTHER; note = 2'-deoxy-2'-fluorocytidine
  modified_base 16: mod_base = cm
  modified_base 17: mod_base = OTHER; note = 2'-deoxy-2'-fluorouridine
  modified_base 18: mod_base = cm
  modified_base 19: mod_base = OTHER; note = 2'-deoxy-2'-fluorocytidine
  modified_base 20: mod_base = cm
  modified_base 21: mod_base = OTHER; note = 2'-O,4'-C-ethylene-briged cytidine
  modified_base 22: mod_base = um
  modified_base 23: mod_base = OTHER; note = 2'-O,4'-C-ethylene-briged guanosine
  modified_base 24: mod_base = um
  modified_base 1^2: mod_base = OTHER; note = phosphorotioate bond between nucleosides
  modified_base 2^3: mod_base = OTHER; note = phosphorothioate bond between nucleosides
  modified_base 3^4: mod_base = OTHER; note = phosphorothioate bond between nucleosides
  modified_base 4^5: mod_base = OTHER; note = phosphorothioate bond between nucleosides
  modified_base 5^6: mod_base = OTHER; note = phosphorothioate bond between nucleosides
  modified_base 7^8: mod_base = OTHER; note = phosphorothioate bond between nucleosides
  modified_base 6^7: mod_base = OTHER; note = phosphorothioate bond between nucleosides
  modified_base 8^9: mod_base = OTHER; note = phosphorothioate bond between nucleosides
  modified_base 9^10: mod_base = OTHER; note = phosphorothioate bond between nucleosides
  modified_base 10^11: mod_base = OTHER; note = phosphorothioate bond between nucleosides
  modified_base 11^12: mod_base = OTHER; note = N-methanesulfonylphosphoramidate bond between nucleosides
  modified_base 12^13: mod_base = OTHER; note = phosphorothioate bond between nucleosides
  modified_base 13^14: mod_base = OTHER; note = phosphorothioate bond between nucleosides
  modified_base 14^15: mod_base = OTHER; note = phosphorothioate bond between nucleosides
  modified_base 15^16: mod_base = OTHER; note = phosphorothioate bond between nucleosides
  modified_base 16^17: mod_base = OTHER; note = phosphorothioate bond between nucleosides
  modified_base 17^18: mod_base = OTHER; note = phosphorothioate bond between nucleosides
  modified_base 18^19: mod_base = OTHER; note = phosphorothioate bond between nucleosides
  modified_base 19^20: mod_base = OTHER; note = phosphorothioate bond between nucleosides
  modified_base 20^21: mod_base = OTHER; note = phosphorothioate bond between nucleosides
  modified_base 21^22: mod_base = OTHER; note = phosphorothioate bond between nucleosides
  modified_base 22^23: mod_base = OTHER; note = phosphorothioate bond between nucleosides
  modified_base 23^24: mod_base = OTHER; note = phosphorothioate bond between nucleosides
aaagcatgccatcacctcccctgt

SEQ ID NO: 95 - RNA, 24 nt, synthetic construct
  source 1..24: mol_type = other RNA
  modified_base 1: mod_base = OTHER; note = 2'-O-methyladenosine
  modified_base 2: mod_base = OTHER; note = 2'-O,4'-C-ethylene-briged adenosine
  modified_base 3: mod_base = OTHER; note = 2'-O-methyladenosine
  modified_base 4: mod_base = OTHER; note = 2'-O,4'-C-ethylene-briged guanosine
  modified_base 5: mod_base = cm
  modified_base 6: mod_base = OTHER; note = 2'-deoxy-2'-fluoroadenosine
  modified_base 7: mod_base = OTHER; note = 2'-deoxy-2'-fluorouridine
  modified_base 8: mod_base = gm
  modified_base 9: mod_base = cm
  modified_base 10: mod_base = OTHER; note = 2'-deoxycytidine
  modified_base 11: mod_base = OTHER; note = 2'-deoxyadenosine
  modified_base 12: mod_base = um
  modified_base 13: mod_base = OTHER; note = 2'-deoxy-2'-fluorocytidine
  modified_base 14: mod_base = OTHER; note = 2'-O-methyladenosine
  modified_base 15: mod_base = OTHER; note = 2'-deoxy-2'-fluorocytidine
  modified_base 16: mod_base = cm
  modified_base 17: mod_base = OTHER; note = 2'-deoxy-2'-fluorouridine
  modified_base 18: mod_base = cm
  modified_base 19: mod_base = OTHER; note = 2'-deoxy-2'-fluorocytidine
  modified_base 20: mod_base = cm
  modified_base 21: mod_base = OTHER; note = 2'-O,4'-C-ethylene-briged cytidine
  modified_base 22: mod_base = um
  modified_base 23: mod_base = OTHER; note = 2'-O,4'-C-ethylene-briged guanosine
  modified_base 24: mod_base = um
  modified_base 1^2: mod_base = OTHER; note = phosphorotioate bond between nucleosides
  modified_base 2^3: mod_base = OTHER; note = phosphorothioate bond between nucleosides
  modified_base 3^4: mod_base = OTHER; note = phosphorothioate bond between nucleosides
  modified_base 4^5: mod_base = OTHER; note = phosphorothioate bond between nucleosides
  modified_base 5^6: mod_base = OTHER; note = phosphorothioate bond between nucleosides
  modified_base 7^8: mod_base = OTHER; note = phosphorothioate bond between nucleosides
  modified_base 6^7: mod_base = OTHER; note = phosphorothioate bond between nucleosides
  modified_base 8^9: mod_base = OTHER; note = phosphorothioate bond between nucleosides
  modified_base 9^10: mod_base = OTHER; note = phosphorothioate bond between nucleosides
  modified_base 10^11: mod_base = OTHER; note = phosphorothioate bond between nucleosides
  modified_base 11^12: mod_base = OTHER; note = phosphorothioate bond between nucleosides
  modified_base 12^13: mod_base = OTHER; note = phosphorothioate bond between nucleosides
  modified_base 13^14: mod_base = OTHER; note = phosphorothioate bond between nucleosides
  modified_base 14^15: mod_base = OTHER; note = N-methanesulfonylphosphoramidate bond between nucleosides
  modified_base 15^16: mod_base = OTHER; note = phosphorothioate bond between nucleosides
  modified_base 16^17: mod_base = OTHER; note = phosphorothioate bond between nucleosides
  modified_base 17^18: mod_base = OTHER; note = phosphorothioate bond between nucleosides
  modified_base 18^19: mod_base = OTHER; note = phosphorothioate bond between nucleosides
  modified_base 19^20: mod_base = OTHER; note = phosphorothioate bond between nucleosides
  modified_base 20^21: mod_base = OTHER; note = phosphorothioate bond between nucleosides
  modified_base 21^22: mod_base = OTHER; note = phosphorothioate bond between nucleosides
  modified_base 22^23: mod_base = OTHER; note = phosphorothioate bond between nucleosides
  modified_base 23^24: mod_base = OTHER; note = phosphorothioate bond between nucleosides
aaagcatgccatcacctcccctgt

SEQ ID NO: 96 - RNA, 24 nt, synthetic construct
  source 1..24: mol_type = other RNA
  modified_base 1: mod_base = OTHER; note = 2'-O-methyladenosine
  modified_base 2: mod_base = OTHER; note = 2'-O,4'-C-ethylene-briged adenosine
  modified_base 3: mod_base = OTHER; note = 2'-O-methyladenosine
  modified_base 4: mod_base = OTHER; note = 2'-O,4'-C-ethylene-briged guanosine
  modified_base 5: mod_base = cm
  modified_base 6: mod_base = OTHER; note = 2'-deoxy-2'-fluoroadenosine
  modified_base 7: mod_base = OTHER; note = 2'-deoxy-2'-fluorouridine
  modified_base 8: mod_base = gm
  modified_base 9: mod_base = cm
  modified_base 10: mod_base = OTHER; note = 2'-deoxycytidine
  modified_base 11: mod_base = OTHER; note = 2'-deoxyadenosine
  modified_base 12: mod_base = um
  modified_base 13: mod_base = OTHER; note = 2'-deoxy-2'-fluorocytidine
  modified_base 14: mod_base = OTHER; note = 2'-O-methyladenosine
  modified_base 15: mod_base = OTHER; note = 2'-deoxy-2'-fluorocytidine
  modified_base 16: mod_base = cm
  modified_base 17: mod_base = OTHER; note = 2'-deoxy-2'-fluorouridine
  modified_base 18: mod_base = cm
  modified_base 19: mod_base = OTHER; note = 2'-deoxy-2'-fluorocytidine
  modified_base 20: mod_base = cm
  modified_base 21: mod_base = OTHER; note = 2'-O,4'-C-ethylene-briged cytidine
  modified_base 22: mod_base = um
  modified_base 23: mod_base = OTHER; note = 2'-O,4'-C-ethylene-briged guanosine
  modified_base 24: mod_base = um
  modified_base 1^2: mod_base = OTHER; note = phosphorotioate bond between nucleosides
  modified_base 2^3: mod_base = OTHER; note = phosphorothioate bond between nucleosides
  modified_base 3^4: mod_base = OTHER; note = phosphorothioate bond between nucleosides
  modified_base 4^5: mod_base = OTHER; note = phosphorothioate bond between nucleosides
  modified_base 5^6: mod_base = OTHER; note = phosphorothioate bond between nucleosides
  modified_base 7^8: mod_base = OTHER; note = phosphorothioate bond between nucleosides
  modified_base 6^7: mod_base = OTHER; note = phosphorothioate bond between nucleosides
  modified_base 8^9: mod_base = OTHER; note = phosphorothioate bond between nucleosides
  modified_base 9^10: mod_base = OTHER; note = phosphorothioate bond between nucleosides
  modified_base 10^11: mod_base = OTHER; note = phosphorothioate bond between nucleosides
  modified_base 11^12: mod_base = OTHER; note = phosphorothioate bond between nucleosides
  modified_base 12^13: mod_base = OTHER; note = N-methanesulfonylphosphoramidate bond between nucleosides
  modified_base 13^14: mod_base = OTHER; note = phosphorothioate bond between nucleosides
  modified_base 14^15: mod_base = OTHER; note = phosphorothioate bond between nucleosides
  modified_base 15^16: mod_base = OTHER; note = phosphorothioate bond between nucleosides
  modified_base 16^17: mod_base = OTHER; note = phosphorothioate bond between nucleosides
  modified_base 17^18: mod_base = OTHER; note = phosphorothioate bond between nucleosides
  modified_base 18^19: mod_base = OTHER; note = phosphorothioate bond between nucleosides
  modified_base 19^20: mod_base = OTHER; note = phosphorothioate bond between nucleosides
  modified_base 20^21: mod_base = OTHER; note = phosphorothioate bond between nucleosides
  modified_base 21^22: mod_base = OTHER; note = phosphorothioate bond between nucleosides
  modified_base 22^23: mod_base = OTHER; note = phosphorothioate bond between nucleosides
  modified_base 23^24: mod_base = OTHER; note = phosphorothioate bond between nucleosides
aaagcatgccatcacctcccctgt

SEQ ID NO: 97 - RNA, 24 nt, synthetic construct
  source 1..24: mol_type = other RNA
  modified_base 1: mod_base = OTHER; note = 2'-O-methyladenosine
  modified_base 2: mod_base = OTHER; note = 2'-O,4'-C-ethylene-briged adenosine
  modified_base 3: mod_base = OTHER; note = 2'-O-methyladenosine
  modified_base 4: mod_base = OTHER; note = 2'-O,4'-C-ethylene-briged guanosine
  modified_base 5: mod_base = cm
  modified_base 6: mod_base = OTHER; note = 2'-deoxy-2'-fluoroadenosine
  modified_base 7: mod_base = OTHER; note = 2'-deoxy-2'-fluorouridine
  modified_base 8: mod_base = gm
  modified_base 9: mod_base = cm
  modified_base 10: mod_base = OTHER; note = 2'-deoxycytidine
  modified_base 11: mod_base = OTHER; note = 2'-deoxyadenosine
  modified_base 12: mod_base = um
  modified_base 13: mod_base = OTHER; note = 2'-deoxy-2'-fluorocytidine
  modified_base 14: mod_base = OTHER; note = 2'-O-methyladenosine
  modified_base 15: mod_base = OTHER; note = 2'-deoxy-2'-fluorocytidine
  modified_base 16: mod_base = cm
  modified_base 17: mod_base = OTHER; note = 2'-deoxy-2'-fluorouridine
  modified_base 18: mod_base = cm
  modified_base 19: mod_base = OTHER; note = 2'-deoxy-2'-fluorocytidine
  modified_base 20: mod_base = cm
  modified_base 21: mod_base = OTHER; note = 2'-O,4'-C-ethylene-briged cytidine
  modified_base 22: mod_base = um
  modified_base 23: mod_base = OTHER; note = 2'-O,4'-C-ethylene-briged guanosine
  modified_base 24: mod_base = um
  modified_base 1^2: mod_base = OTHER; note = phosphorotioate bond between nucleosides
  modified_base 2^3: mod_base = OTHER; note = phosphorothioate bond between nucleosides
  modified_base 3^4: mod_base = OTHER; note = phosphorothioate bond between nucleosides
  modified_base 4^5: mod_base = OTHER; note = phosphorothioate bond between nucleosides
  modified_base 5^6: mod_base = OTHER; note = phosphorothioate bond between nucleosides
  modified_base 7^8: mod_base = OTHER; note = phosphorothioate bond between nucleosides
  modified_base 6^7: mod_base = OTHER; note = phosphorothioate bond between nucleosides
  modified_base 8^9: mod_base = OTHER; note = phosphorothioate bond between nucleosides
  modified_base 9^10: mod_base = OTHER; note = phosphorothioate bond between nucleosides
  modified_base 10^11: mod_base = OTHER; note = phosphorothioate bond between nucleosides
  modified_base 11^12: mod_base = OTHER; note = (1,3-dimethylimidazoridin-2-ylidene)phosphoramidate bond between nucleosides
  modified_base 12^13: mod_base = OTHER; note = phosphorothioate bond between nucleosides
  modified_base 13^14: mod_base = OTHER; note = phosphorothioate bond between nucleosides
  modified_base 14^15: mod_base = OTHER; note = (1,3-dimethylimidazoridin-2-ylidene)phosphoramidate bond between nucleosides
  modified_base 15^16: mod_base = OTHER; note = phosphorothioate bond between nucleosides
  modified_base 16^17: mod_base = OTHER; note = phosphorothioate bond between nucleosides
  modified_base 17^18: mod_base = OTHER; note = phosphorothioate bond between nucleosides
  modified_base 18^19: mod_base = OTHER; note = phosphorothioate bond between nucleosides
  modified_base 19^20: mod_base = OTHER; note = phosphorothioate bond between nucleosides
  modified_base 20^21: mod_base = OTHER; note = phosphorothioate bond between nucleosides
  modified_base 21^22: mod_base = OTHER; note = phosphorothioate bond between nucleosides
  modified_base 22^23: mod_base = OTHER; note = phosphorothioate bond between nucleosides
  modified_base 23^24: mod_base = OTHER; note = phosphorothioate bond between nucleosides
aaagcatgccatcacctcccctgt

SEQ ID NO: 98 - RNA, 24 nt, synthetic construct
  source 1..24: mol_type = other RNA
  modified_base 1: mod_base = OTHER; note = 2'-O-methyladenosine
  modified_base 2: mod_base = OTHER; note = 2'-O,4'-C-methylene-briged adenosine
  modified_base 3: mod_base = OTHER; note = 2'-O-methyladenosine
  modified_base 4: mod_base = OTHER; note = 2'-O,4'-C-methylene-briged guanosine
  modified_base 5: mod_base = cm
  modified_base 6: mod_base = OTHER; note = 2'-deoxy-2'-fluoroadenosine
  modified_base 7: mod_base = OTHER; note = 2'-deoxy-2'-fluorouridine
  modified_base 8: mod_base = gm
  modified_base 9: mod_base = cm
  modified_base 10: mod_base = OTHER; note = 2'-deoxycytidine
  modified_base 11: mod_base = OTHER; note = 2'-deoxyadenosine
  modified_base 12: mod_base = um
  modified_base 13: mod_base = OTHER; note = 2'-deoxy-2'-fluorocytidine
  modified_base 14: mod_base = OTHER; note = 2'-O-methyladenosine
  modified_base 15: mod_base = OTHER; note = 2'-deoxy-2'-fluorocytidine
  modified_base 16: mod_base = cm
  modified_base 17: mod_base = OTHER; note = 2'-deoxy-2'-fluorouridine
  modified_base 18: mod_base = cm
  modified_base 19: mod_base = OTHER; note = 2'-deoxy-2'-fluorocytidine
  modified_base 20: mod_base = cm
  modified_base 21: mod_base = cm
  modified_base 22: mod_base = um
  modified_base 23: mod_base = OTHER; note = 2'-O,4'-C-methylene-briged guanosine
  modified_base 24: mod_base = um
  modified_base 1^2: mod_base = OTHER; note = phosphorotioate bond between nucleosides
  modified_base 2^3: mod_base = OTHER; note = phosphorothioate bond between nucleosides
  modified_base 3^4: mod_base = OTHER; note = phosphorothioate bond between nucleosides
  modified_base 4^5: mod_base = OTHER; note = phosphorothioate bond between nucleosides
  modified_base 5^6: mod_base = OTHER; note = phosphorothioate bond between nucleosides
  modified_base 7^8: mod_base = OTHER; note = phosphorothioate bond between nucleosides
  modified_base 6^7: mod_base = OTHER; note = phosphorothioate bond between nucleosides
  modified_base 8^9: mod_base = OTHER; note = phosphorothioate bond between nucleosides
  modified_base 9^10: mod_base = OTHER; note = phosphorothioate bond between nucleosides
  modified_base 10^11: mod_base = OTHER; note = phosphorothioate bond between nucleosides
  modified_base 11^12: mod_base = OTHER; note = methylphosphonate bond between nucleosides
  modified_base 12^13: mod_base = OTHER; note = phosphorothioate bond between nucleosides
  modified_base 13^14: mod_base = OTHER; note = phosphorothioate bond between nucleosides
  modified_base 14^15: mod_base = OTHER; note = methylphosphonate bond between nucleosides
  modified_base 15^16: mod_base = OTHER; note = phosphorothioate bond between nucleosides
  modified_base 16^17: mod_base = OTHER; note = phosphorothioate bond between nucleosides
  modified_base 17^18: mod_base = OTHER; note = phosphorothioate bond between nucleosides
  modified_base 18^19: mod_base = OTHER; note = phosphorothioate bond between nucleosides
  modified_base 19^20: mod_base = OTHER; note = phosphorothioate bond between nucleosides
  modified_base 20^21: mod_base = OTHER; note = phosphorothioate bond between nucleosides
  modified_base 21^22: mod_base = OTHER; note = phosphorothioate bond between nucleosides
  modified_base 22^23: mod_base = OTHER; note = phosphorothioate bond between nucleosides
  modified_base 23^24: mod_base = OTHER; note = phosphorothioate bond between nucleosides
aaagcatgccatcacctcccctgt

SEQ ID NO: 99 - RNA, 24 nt, synthetic construct
  source 1..24: mol_type = other RNA
  modified_base 1: mod_base = OTHER; note = 2'-O-methyladenosine
  modified_base 2: mod_base = OTHER; note = 2'-O,4'-C-methylene-briged adenosine
  modified_base 3: mod_base = OTHER; note = 2'-O-methyladenosine
  modified_base 4: mod_base = gm
  modified_base 5: mod_base = cm
  modified_base 6: mod_base = OTHER; note = 2'-deoxy-2'-fluoroadenosine
  modified_base 7: mod_base = OTHER; note = 2'-deoxy-2'-fluorouridine
  modified_base 8: mod_base = gm
  modified_base 9: mod_base = cm
  modified_base 10: mod_base = OTHER; note = 2'-deoxycytidine
  modified_base 11: mod_base = OTHER; note = 2'-deoxyadenosine
  modified_base 12: mod_base = um
  modified_base 13: mod_base = OTHER; note = 2'-deoxy-2'-fluorocytidine
  modified_base 14: mod_base = OTHER; note = 2'-O-methyladenosine
  modified_base 15: mod_base = OTHER; note = 2'-deoxy-2'-fluorocytidine
  modified_base 16: mod_base = cm
  modified_base 17: mod_base = OTHER; note = 2'-deoxy-2'-fluorouridine
  modified_base 18: mod_base = cm
  modified_base 19: mod_base = OTHER; note = 2'-deoxy-2'-fluorocytidine
  modified_base 20: mod_base = cm
  modified_base 21: mod_base = OTHER; note = 2'-O,4'-C-methylene-briged cytidine
  modified_base 22: mod_base = um
  modified_base 23: mod_base = OTHER; note = 2'-O,4'-C-methylene-briged guanosine
  modified_base 24: mod_base = um
  modified_base 1^2: mod_base = OTHER; note = phosphorotioate bond between nucleosides
  modified_base 2^3: mod_base = OTHER; note = phosphorothioate bond between nucleosides
  modified_base 3^4: mod_base = OTHER; note = phosphorothioate bond between nucleosides
  modified_base 4^5: mod_base = OTHER; note = phosphorothioate bond between nucleosides
  modified_base 5^6: mod_base = OTHER; note = phosphorothioate bond between nucleosides
  modified_base 7^8: mod_base = OTHER; note = phosphorothioate bond between nucleosides
  modified_base 6^7: mod_base = OTHER; note = phosphorothioate bond between nucleosides
  modified_base 8^9: mod_base = OTHER; note = phosphorothioate bond between nucleosides
  modified_base 9^10: mod_base = OTHER; note = phosphorothioate bond between nucleosides
  modified_base 10^11: mod_base = OTHER; note = phosphorothioate bond between nucleosides
  modified_base 11^12: mod_base = OTHER; note = methylphosphonate bond between nucleosides
  modified_base 12^13: mod_base = OTHER; note = phosphorothioate bond between nucleosides
  modified_base 13^14: mod_base = OTHER; note = phosphorothioate bond between nucleosides
  modified_base 14^15: mod_base = OTHER; note = methylphosphonate bond between nucleosides
  modified_base 15^16: mod_base = OTHER; note = phosphorothioate bond between nucleosides
  modified_base 16^17: mod_base = OTHER; note = phosphorothioate bond between nucleosides
  modified_base 17^18: mod_base = OTHER; note = phosphorothioate bond between nucleosides
  modified_base 18^19: mod_base = OTHER; note = phosphorothioate bond between nucleosides
  modified_base 19^20: mod_base = OTHER; note = phosphorothioate bond between nucleosides
  modified_base 20^21: mod_base = OTHER; note = phosphorothioate bond between nucleosides
  modified_base 21^22: mod_base = OTHER; note = phosphorothioate bond between nucleosides
  modified_base 22^23: mod_base = OTHER; note = phosphorothioate bond between nucleosides
  modified_base 23^24: mod_base = OTHER; note = phosphorothioate bond between nucleosides
aaagcatgccatcacctcccctgt

SEQ ID NO: 100 - RNA, 24 nt, synthetic construct
  source 1..24: mol_type = other RNA
  modified_base 1: mod_base = OTHER; note = 2'-O-methyladenosine
  modified_base 2: mod_base = OTHER; note = 2'-O,4'-C-methylene-briged adenosine
  modified_base 3: mod_base = OTHER; note = 2'-O-methyladenosine
  modified_base 4: mod_base = gm
  modified_base 5: mod_base = cm
  modified_base 6: mod_base = OTHER; note = 2'-deoxy-2'-fluoroadenosine
  modified_base 7: mod_base = OTHER; note = 2'-deoxy-2'-fluorouridine
  modified_base 8: mod_base = gm
  modified_base 9: mod_base = cm
  modified_base 10: mod_base = OTHER; note = 2'-deoxycytidine
  modified_base 11: mod_base = OTHER; note = 2'-deoxyadenosine
  modified_base 12: mod_base = um
  modified_base 13: mod_base = OTHER; note = 2'-deoxy-2'-fluorocytidine
  modified_base 14: mod_base = OTHER; note = 2'-O-methyladenosine
  modified_base 15: mod_base = OTHER; note = 2'-deoxy-2'-fluorocytidine
  modified_base 16: mod_base = cm
  modified_base 17: mod_base = OTHER; note = 2'-deoxy-2'-fluorouridine
  modified_base 18: mod_base = cm
  modified_base 19: mod_base = OTHER; note = 2'-deoxy-2'-fluorocytidine
  modified_base 20: mod_base = cm
  modified_base 21: mod_base = cm
  modified_base 22: mod_base = um
  modified_base 23: mod_base = OTHER; note = 2'-O,4'-C-methylene-briged guanosine
  modified_base 24: mod_base = um
  modified_base 1^2: mod_base = OTHER; note = phosphorotioate bond between nucleosides
  modified_base 2^3: mod_base = OTHER; note = phosphorothioate bond between nucleosides
  modified_base 3^4: mod_base = OTHER; note = phosphorothioate bond between nucleosides
  modified_base 4^5: mod_base = OTHER; note = phosphorothioate bond between nucleosides
  modified_base 5^6: mod_base = OTHER; note = phosphorothioate bond between nucleosides
  modified_base 7^8: mod_base = OTHER; note = phosphorothioate bond between nucleosides
  modified_base 6^7: mod_base = OTHER; note = phosphorothioate bond between nucleosides
  modified_base 8^9: mod_base = OTHER; note = phosphorothioate bond between nucleosides
  modified_base 9^10: mod_base = OTHER; note = phosphorothioate bond between nucleosides
  modified_base 10^11: mod_base = OTHER; note = phosphorothioate bond between nucleosides
  modified_base 11^12: mod_base = OTHER; note = methylphosphonate bond between nucleosides
  modified_base 12^13: mod_base = OTHER; note = phosphorothioate bond between nucleosides
  modified_base 13^14: mod_base = OTHER; note = phosphorothioate bond between nucleosides
  modified_base 14^15: mod_base = OTHER; note = methylphosphonate bond between nucleosides
  modified_base 15^16: mod_base = OTHER; note = phosphorothioate bond between nucleosides
  modified_base 16^17: mod_base = OTHER; note = phosphorothioate bond between nucleosides
  modified_base 17^18: mod_base = OTHER; note = phosphorothioate bond between nucleosides
  modified_base 18^19: mod_base = OTHER; note = phosphorothioate bond between nucleosides
  modified_base 19^20: mod_base = OTHER; note = phosphorothioate bond between nucleosides
  modified_base 20^21: mod_base = OTHER; note = phosphorothioate bond between nucleosides
  modified_base 21^22: mod_base = OTHER; note = phosphorothioate bond between nucleosides
  modified_base 22^23: mod_base = OTHER; note = phosphorothioate bond between nucleosides
  modified_base 23^24: mod_base = OTHER; note = phosphorothioate bond between nucleosides
aaagcatgccatcacctcccctgt

SEQ ID NO: 101 - RNA, 24 nt, synthetic construct
  source 1..24: mol_type = other RNA
  modified_base 1: mod_base = OTHER; note = 2'-O,4'-C-methylene-bridged adenosine
  modified_base 2: mod_base = OTHER; note = 2'-O-methyladenosine
  modified_base 3: mod_base = OTHER; note = 2'-O-methyladenosine
  modified_base 4: mod_base = gm
  modified_base 5: mod_base = cm
  modified_base 6: mod_base = OTHER; note = 2'-deoxy-2'-fluoroadenosine
  modified_base 7: mod_base = OTHER; note = 2'-deoxy-2'-fluorouridine
  modified_base 8: mod_base = gm
  modified_base 9: mod_base = cm
  modified_base 10: mod_base = OTHER; note = 2'-deoxycytidine
  modified_base 11: mod_base = OTHER; note = 2'-deoxyadenosine
  modified_base 12: mod_base = um
  modified_base 13: mod_base = OTHER; note = 2'-deoxy-2'-fluorocytidine
  modified_base 14: mod_base = OTHER; note = 2'-O-methyladenosine
  modified_base 15: mod_base = OTHER; note = 2'-deoxy-2'-fluorocytidine
  modified_base 16: mod_base = cm
  modified_base 17: mod_base = OTHER; note = 2'-deoxy-2'-fluorouridine
  modified_base 18: mod_base = cm
  modified_base 19: mod_base = OTHER; note = 2'-deoxy-2'-fluorocytidine
  modified_base 20: mod_base = cm
  modified_base 21: mod_base = cm
  modified_base 22: mod_base = um
  modified_base 23: mod_base = OTHER; note = 2'-O,4'-C-methylene-briged guanosine
  modified_base 24: mod_base = um
  modified_base 1^2: mod_base = OTHER; note = phosphorotioate bond between nucleosides
  modified_base 2^3: mod_base = OTHER; note = phosphorothioate bond between nucleosides
  modified_base 3^4: mod_base = OTHER; note = phosphorothioate bond between nucleosides
  modified_base 4^5: mod_base = OTHER; note = phosphorothioate bond between nucleosides
  modified_base 5^6: mod_base = OTHER; note = phosphorothioate bond between nucleosides
  modified_base 7^8: mod_base = OTHER; note = phosphorothioate bond between nucleosides
  modified_base 6^7: mod_base = OTHER; note = phosphorothioate bond between nucleosides
  modified_base 8^9: mod_base = OTHER; note = phosphorothioate bond between nucleosides
  modified_base 9^10: mod_base = OTHER; note = phosphorothioate bond between nucleosides
  modified_base 10^11: mod_base = OTHER; note = phosphorothioate bond between nucleosides
  modified_base 11^12: mod_base = OTHER; note = methylphosphonate bond between nucleosides
  modified_base 12^13: mod_base = OTHER; note = phosphorothioate bond between nucleosides
  modified_base 13^14: mod_base = OTHER; note = phosphorothioate bond between nucleosides
  modified_base 14^15: mod_base = OTHER; note = methylphosphonate bond between nucleosides
  modified_base 15^16: mod_base = OTHER; note = phosphorothioate bond between nucleosides
  modified_base 16^17: mod_base = OTHER; note = phosphorothioate bond between nucleosides
  modified_base 17^18: mod_base = OTHER; note = phosphorothioate bond between nucleosides
  modified_base 18^19: mod_base = OTHER; note = phosphorothioate bond between nucleosides
  modified_base 19^20: mod_base = OTHER; note = phosphorothioate bond between nucleosides
  modified_base 20^21: mod_base = OTHER; note = phosphorothioate bond between nucleosides
  modified_base 21^22: mod_base = OTHER; note = phosphorothioate bond between nucleosides
  modified_base 22^23: mod_base = OTHER; note = phosphorothioate bond between nucleosides
  modified_base 23^24: mod_base = OTHER; note = phosphorothioate bond between nucleosides
aaagcatgccatcacctcccctgt

SEQ ID NO: 102 - RNA, 24 nt, synthetic construct
  source 1..24: mol_type = other RNA
  modified_base 1: mod_base = gm
  modified_base 2: mod_base = OTHER; note = 2'-O,4'-C-methylene-briged thymine
  modified_base 3: mod_base = cm
  modified_base 4: mod_base = OTHER; note = 2'-O,4'-C-methylene-briged cytosine
  modified_base 5: mod_base = cm
  modified_base 6: mod_base = OTHER; note = 2'-deoxy-2'-fluorouridine
  modified_base 7: mod_base = OTHER; note = 2'-deoxy-2'-fluorouridine
  modified_base 8: mod_base = cm
  modified_base 9: mod_base = cm
  modified_base 10: mod_base = OTHER; note = 2'-deoxycytidine
  modified_base 11: mod_base = OTHER; note = 2'-deoxyinosine
  modified_base 12: mod_base = um
  modified_base 13: mod_base = OTHER; note = 2'-deoxy-2'-fluorocytidine
  modified_base 14: mod_base = gm
  modified_base 15: mod_base = OTHER; note = 2'-deoxy-2'-fluoroadenosine
  modified_base 16: mod_base = um
  modified_base 17: mod_base = OTHER; note = 2'-deoxy-2'-fluoroguanosine
  modified_base 18: mod_base = gm
  modified_base 19: mod_base = OTHER; note = 2'-deoxy-2'-fluorouridine
  modified_base 20: mod_base = cm
  modified_base 21: mod_base = OTHER; note = 2'-O,4'-C-methylene-briged adenosine
  modified_base 22: mod_base = gm
  modified_base 23: mod_base = OTHER; note = 2'-O,4'-C-methylene-briged cytidine
  modified_base 24: mod_base = OTHER; note = 2'-O-methyladenosine
  modified_base 1^2: mod_base = OTHER; note = phosphorotioate bond between nucleosides
  modified_base 2^3: mod_base = OTHER; note = phosphorothioate bond between nucleosides
  modified_base 3^4: mod_base = OTHER; note = phosphorothioate bond between nucleosides
  modified_base 4^5: mod_base = OTHER; note = phosphorothioate bond between nucleosides
  modified_base 5^6: mod_base = OTHER; note = phosphorothioate bond between nucleosides
  modified_base 7^8: mod_base = OTHER; note = phosphorothioate bond between nucleosides
  modified_base 6^7: mod_base = OTHER; note = phosphorothioate bond between nucleosides
  modified_base 8^9: mod_base = OTHER; note = phosphorothioate bond between nucleosides
  modified_base 9^10: mod_base = OTHER; note = phosphorothioate bond between nucleosides
  modified_base 10^11: mod_base = OTHER; note = phosphorothioate bond between nucleosides
  modified_base 11^12: mod_base = OTHER; note = methylphosphonate bond between nucleosides
  modified_base 12^13: mod_base = OTHER; note = phosphorothioate bond between nucleosides
  modified_base 13^14: mod_base = OTHER; note = phosphorothioate bond between nucleosides
  modified_base 14^15: mod_base = OTHER; note = methylphosphonate bond between nucleosides
  modified_base 15^16: mod_base = OTHER; note = phosphorothioate bond between nucleosides
  modified_base 16^17: mod_base = OTHER; note = phosphorothioate bond between nucleosides
  modified_base 17^18: mod_base = OTHER; note = phosphorothioate bond between nucleosides
  modified_base 18^19: mod_base = OTHER; note = phosphorothioate bond between nucleosides
  modified_base 19^20: mod_base = OTHER; note = phosphorothioate bond between nucleosides
  modified_base 20^21: mod_base = OTHER; note = phosphorothioate bond between nucleosides
  modified_base 21^22: mod_base = OTHER; note = phosphorothioate bond between nucleosides
  modified_base 22^23: mod_base = OTHER; note = phosphorothioate bond between nucleosides
  modified_base 23^24: mod_base = OTHER; note = phosphorothioate bond between nucleosides
gtcccttctcatcgatggtcagca

SEQ ID NO: 103 - RNA, 24 nt, synthetic construct
  source 1..24: mol_type = other RNA
  modified_base 1: mod_base = gm
  modified_base 2: mod_base = OTHER; note = 2'-O,4'-C-methylene-briged thymidine
  modified_base 3: mod_base = cm
  modified_base 4: mod_base = OTHER; note = 2'-O,4'-C-methylene-briged cytidine
  modified_base 5: mod_base = cm
  modified_base 6: mod_base = OTHER; note = 2'-deoxy-2'-fluorouridine
  modified_base 7: mod_base = OTHER; note = 2'-deoxy-2'-fluorouridine
  modified_base 8: mod_base = cm
  modified_base 9: mod_base = OTHER; note = 2'-O-methyluridine
  modified_base 10: mod_base = OTHER; note = 2'-deoxycytidine
  modified_base 11: mod_base = OTHER; note = 2'-deoxyinosine
  modified_base 12: mod_base = um
  modified_base 13: mod_base = OTHER; note = 2'-deoxy-2'-fluorocytidine
  modified_base 14: mod_base = gm
  modified_base 15: mod_base = OTHER; note = 2'-deoxy-2'-fluoroadenosine
  modified_base 16: mod_base = um
  modified_base 17: mod_base = OTHER; note = 2'-deoxy-2'-fluoroguanosine
  modified_base 18: mod_base = gm
  modified_base 19: mod_base = OTHER; note = 2'-deoxy-2'-fluorouridine
  modified_base 20: mod_base = cm
  modified_base 21: mod_base = OTHER; note = 2'-O,4'-C-methylene-briged adenosine
  modified_base 22: mod_base = gm
  modified_base 23: mod_base = OTHER; note = 2'-O,4'-C-methylene-briged cytidine
  modified_base 24: mod_base = OTHER; note = 2'-O-mtheyladenosine
  modified_base 1^2: mod_base = OTHER; note = phosphorotioate bond between nucleosides
  modified_base 2^3: mod_base = OTHER; note = phosphorothioate bond between nucleosides
  modified_base 3^4: mod_base = OTHER; note = phosphorothioate bond between nucleosides
  modified_base 4^5: mod_base = OTHER; note = phosphorothioate bond between nucleosides
  modified_base 5^6: mod_base = OTHER; note = phosphorothioate bond between nucleosides
  modified_base 7^8: mod_base = OTHER; note = phosphorothioate bond between nucleosides
  modified_base 6^7: mod_base = OTHER; note = phosphorothioate bond between nucleosides
  modified_base 8^9: mod_base = OTHER; note = phosphorothioate bond between nucleosides
  modified_base 9^10: mod_base = OTHER; note = phosphorothioate bond between nucleosides
  modified_base 10^11: mod_base = OTHER; note = phosphorothioate bond between nucleosides
  modified_base 11^12: mod_base = OTHER; note = methylphosphonate bond between nucleosides
  modified_base 12^13: mod_base = OTHER; note = phosphorothioate bond between nucleosides
  modified_base 13^14: mod_base = OTHER; note = phosphorothioate bond between nucleosides
  modified_base 14^15: mod_base = OTHER; note = phosphorothioate bond between nucleosides
  modified_base 15^16: mod_base = OTHER; note = phosphorothioate bond between nucleosides
  modified_base 16^17: mod_base = OTHER; note = phosphorothioate bond between nucleosides
  modified_base 17^18: mod_base = OTHER; note = phosphorothioate bond between nucleosides
  modified_base 18^19: mod_base = OTHER; note = phosphorothioate bond between nucleosides
  modified_base 19^20: mod_base = OTHER; note = phosphorothioate bond between nucleosides
  modified_base 20^21: mod_base = OTHER; note = phosphorothioate bond between nucleosides
  modified_base 21^22: mod_base = OTHER; note = phosphorothioate bond between nucleosides
  modified_base 22^23: mod_base = OTHER; note = phosphorothioate bond between nucleosides
  modified_base 23^24: mod_base = OTHER; note = phosphorothioate bond between nucleosides
gtcccttctcatcgatggtcagca

SEQ ID NO: 104 - RNA, 24 nt, synthetic construct
  source 1..24: mol_type = other RNA
  modified_base 1: mod_base = gm
  modified_base 2: mod_base = OTHER; note = 2'-O,4'-C-methylene-briged thymidine
  modified_base 3: mod_base = cm
  modified_base 4: mod_base = OTHER; note = 2'-O,4'-C-methylene-briged cytidine
  modified_base 5: mod_base = cm
  modified_base 6: mod_base = OTHER; note = 2'-deoxy-2'-fluorouridine
  modified_base 7: mod_base = OTHER; note = 2'-deoxy-2'-fluorouridine
  modified_base 8: mod_base = cm
  modified_base 9: mod_base = OTHER; note = 2'-O-methyluridine
  modified_base 10: mod_base = OTHER; note = 2'-deoxycytidine
  modified_base 11: mod_base = OTHER; note = 2'-deoxyinosine
  modified_base 12: mod_base = um
  modified_base 13: mod_base = OTHER; note = 2'-deoxy-2'-fluorocytidine
  modified_base 14: mod_base = gm
  modified_base 15: mod_base = OTHER; note = 2'-deoxy-2'-fluoroadenosine
  modified_base 16: mod_base = OTHER; note = 2'-O-methyluridine
  modified_base 17: mod_base = OTHER; note = 2'-deoxy-2'-fluoroguanosine
  modified_base 18: mod_base = cm
  modified_base 19: mod_base = OTHER; note = 2'-deoxy-2'-fluorouridine
  modified_base 20: mod_base = cm
  modified_base 21: mod_base = OTHER; note = 2'-O,4'-C-methylene-briged adenosine
  modified_base 22: mod_base = gm
  modified_base 23: mod_base = OTHER; note = 2'-O,4'-C-methylene-briged cytidine
  modified_base 24: mod_base = OTHER; note = 2'-O-methyladenosine
  modified_base 1^2: mod_base = OTHER; note = phosphorotioate bond between nucleosides
  modified_base 2^3: mod_base = OTHER; note = phosphorothioate bond between nucleosides
  modified_base 3^4: mod_base = OTHER; note = phosphorothioate bond between nucleosides
  modified_base 4^5: mod_base = OTHER; note = phosphorothioate bond between nucleosides
  modified_base 5^6: mod_base = OTHER; note = phosphorothioate bond between nucleosides
  modified_base 7^8: mod_base = OTHER; note = phosphorothioate bond between nucleosides
  modified_base 6^7: mod_base = OTHER; note = phosphorothioate bond between nucleosides
  modified_base 8^9: mod_base = OTHER; note = phosphorothioate bond between nucleosides
  modified_base 9^10: mod_base = OTHER; note = phosphorothioate bond between nucleosides
  modified_base 10^11: mod_base = OTHER; note = phosphorothioate bond between nucleosides
  modified_base 11^12: mod_base = OTHER; note = phosphorothioate bond between nucleosides
  modified_base 12^13: mod_base = OTHER; note = phosphorothioate bond between nucleosides
  modified_base 13^14: mod_base = OTHER; note = phosphorothioate bond between nucleosides
  modified_base 14^15: mod_base = OTHER; note = methylphosphonate bond between nucleosides
  modified_base 15^16: mod_base = OTHER; note = phosphorothioate bond between nucleosides
  modified_base 16^17: mod_base = OTHER; note = phosphorothioate bond between nucleosides
  modified_base 17^18: mod_base = OTHER; note = phosphorothioate bond between nucleosides
  modified_base 18^19: mod_base = OTHER; note = phosphorothioate bond between nucleosides
  modified_base 19^20: mod_base = OTHER; note = phosphorothioate bond between nucleosides
  modified_base 20^21: mod_base = OTHER; note = phosphorothioate bond between nucleosides
  modified_base 21^22: mod_base = OTHER; note = phosphorothioate bond between nucleosides
  modified_base 22^23: mod_base = OTHER; note = phosphorothioate bond between nucleosides
  modified_base 23^24: mod_base = OTHER; note = phosphorothioate bond between nucleosides
gtcccttctcatcgatggtcagca

SEQ ID NO: 105 - RNA, 24 nt, synthetic construct
  source 1..24: mol_type = other RNA
  modified_base 1: mod_base = gm
  modified_base 2: mod_base = OTHER; note = 2'-O,4'-C-methylene-briged adenosine
  modified_base 3: mod_base = gm
  modified_base 4: mod_base = OTHER; note = 2'-O,4'-C-methylene-briged guanosine
  modified_base 5: mod_base = gm
  modified_base 6: mod_base = OTHER; note = 2'-deoxy-2'-fluorocytidine
  modified_base 7: mod_base = OTHER; note = 2'-deoxy-2'-fluorocytidine
  modified_base 8: mod_base = cm
  modified_base 9: mod_base = cm
  modified_base 10: mod_base = OTHER; note = 2'-deoxycytidine
  modified_base 11: mod_base = OTHER; note = 2'-deoxyadenosine
  modified_base 12: mod_base = gm
  modified_base 13: mod_base = OTHER; note = 2'-deoxy-2'-fluoroguanosine
  modified_base 14: mod_base = cm
  modified_base 15: mod_base = OTHER; note = 2'-deoxy-2'-fluorocytidine
  modified_base 16: mod_base = cm
  modified_base 17: mod_base = OTHER; note = 2'-deoxy-2'-fluorocytidine
  modified_base 18: mod_base = OTHER; note = 2'-O-methyluridine
  modified_base 19: mod_base = OTHER; note = 2'-deoxy-2'-fluorocytidine
  modified_base 20: mod_base = cm
  modified_base 21: mod_base = OTHER; note = 2'-O,4'-C-methylene-briged thymidine
  modified_base 22: mod_base = gm
  modified_base 23: mod_base = OTHER; note = 2'-O,4'-C-methylene-briged guanosine
  modified_base 24: mod_base = um
  modified_base 1^2: mod_base = OTHER; note = phosphorotioate bond between nucleosides
  modified_base 2^3: mod_base = OTHER; note = phosphorothioate bond between nucleosides
  modified_base 3^4: mod_base = OTHER; note = phosphorothioate bond between nucleosides
  modified_base 4^5: mod_base = OTHER; note = phosphorothioate bond between nucleosides
  modified_base 5^6: mod_base = OTHER; note = phosphorothioate bond between nucleosides
  modified_base 7^8: mod_base = OTHER; note = phosphorothioate bond between nucleosides
  modified_base 6^7: mod_base = OTHER; note = phosphorothioate bond between nucleosides
  modified_base 8^9: mod_base = OTHER; note = phosphorothioate bond between nucleosides
  modified_base 9^10: mod_base = OTHER; note = phosphorothioate bond between nucleosides
  modified_base 10^11: mod_base = OTHER; note = phosphorothioate bond between nucleosides
  modified_base 11^12: mod_base = OTHER; note = methylphosphonate bond between nucleosides
  modified_base 12^13: mod_base = OTHER; note = phosphorothioate bond between nucleosides
  modified_base 13^14: mod_base = OTHER; note = phosphorothioate bond between nucleosides
  modified_base 14^15: mod_base = OTHER; note = phosphorothioate bond between nucleosides
  modified_base 15^16: mod_base = OTHER; note = phosphorothioate bond between nucleosides
  modified_base 16^17: mod_base = OTHER; note = phosphorothioate bond between nucleosides
  modified_base 17^18: mod_base = OTHER; note = phosphorothioate bond between nucleosides
  modified_base 18^19: mod_base = OTHER; note = phosphorothioate bond between nucleosides
  modified_base 19^20: mod_base = OTHER; note = phosphorothioate bond between nucleosides
  modified_base 20^21: mod_base = OTHER; note = phosphorothioate bond between nucleosides
  modified_base 21^22: mod_base = OTHER; note = phosphorothioate bond between nucleosides
  modified_base 22^23: mod_base = OTHER; note = phosphorothioate bond between nucleosides
  modified_base 23^24: mod_base = OTHER; note = phosphorothioate bond between nucleosides
gagggcccccaggcccctcctgtt

SEQ ID NO: 106 - RNA, 24 nt, synthetic construct
  source 1..24: mol_type = other RNA
  modified_base 1: mod_base = gm
  modified_base 2: mod_base = OTHER; note = 2'-O,4'-C-methylene-briged adenosine
  modified_base 3: mod_base = gm
  modified_base 4: mod_base = OTHER; note = 2'-O,4'-C-methylene-briged guanosine
  modified_base 5: mod_base = gm
  modified_base 6: mod_base = OTHER; note = 2'-deoxy-2'-fluorocytidine
  modified_base 7: mod_base = OTHER; note = 2'-deoxy-2'-fluorocytidine
  modified_base 8: mod_base = cm
  modified_base 9: mod_base = cm
  modified_base 10: mod_base = OTHER; note = 2'-deoxycytidine
  modified_base 11: mod_base = OTHER; note = 2'-deoxyadenosine
  modified_base 12: mod_base = gm
  modified_base 13: mod_base = OTHER; note = 2'-deoxy-2'-fluoroguanosine
  modified_base 14: mod_base = cm
  modified_base 15: mod_base = OTHER; note = 2'-deoxy-2'-fluorocytidine
  modified_base 16: mod_base = cm
  modified_base 17: mod_base = OTHER; note = 2'-deoxy-2'-fluorocytidine
  modified_base 18: mod_base = um
  modified_base 19: mod_base = OTHER; note = 2'-deoxy-2'-fluorocytidine
  modified_base 20: mod_base = cm
  modified_base 21: mod_base = OTHER; note = 2'-O,4'-C-methylene-briged thymidine
  modified_base 22: mod_base = gm
  modified_base 23: mod_base = OTHER; note = 2'-O,4'-C-methylene-briged thymidine
  modified_base 24: mod_base = um
  modified_base 1^2: mod_base = OTHER; note = phosphorotioate bond between nucleosides
  modified_base 2^3: mod_base = OTHER; note = phosphorothioate bond between nucleosides
  modified_base 3^4: mod_base = OTHER; note = phosphorothioate bond between nucleosides
  modified_base 4^5: mod_base = OTHER; note = phosphorothioate bond between nucleosides
  modified_base 5^6: mod_base = OTHER; note = phosphorothioate bond between nucleosides
  modified_base 7^8: mod_base = OTHER; note = phosphorothioate bond between nucleosides
  modified_base 6^7: mod_base = OTHER; note = phosphorothioate bond between nucleosides
  modified_base 8^9: mod_base = OTHER; note = phosphorothioate bond between nucleosides
  modified_base 9^10: mod_base = OTHER; note = phosphorothioate bond between nucleosides
  modified_base 10^11: mod_base = OTHER; note = phosphorothioate bond between nucleosides
  modified_base 11^12: mod_base = OTHER; note = ethylphosphate bond between nucleosides
  modified_base 12^13: mod_base = OTHER; note = phosphorothioate bond between nucleosides
  modified_base 13^14: mod_base = OTHER; note = phosphorothioate bond between nucleosides
  modified_base 14^15: mod_base = OTHER; note = ethylphosphate bond between nucleosides
  modified_base 15^16: mod_base = OTHER; note = phosphorothioate bond between nucleosides
  modified_base 16^17: mod_base = OTHER; note = phosphorothioate bond between nucleosides
  modified_base 17^18: mod_base = OTHER; note = phosphorothioate bond between nucleosides
  modified_base 18^19: mod_base = OTHER; note = phosphorothioate bond between nucleosides
  modified_base 19^20: mod_base = OTHER; note = phosphorothioate bond between nucleosides
  modified_base 20^21: mod_base = OTHER; note = phosphorothioate bond between nucleosides
  modified_base 21^22: mod_base = OTHER; note = phosphorothioate bond between nucleosides
  modified_base 22^23: mod_base = OTHER; note = phosphorothioate bond between nucleosides
  modified_base 23^24: mod_base = OTHER; note = phosphorothioate bond between nucleosides
gagggcccccaggcccctcctgtt

SEQ ID NO: 107 - RNA, 24 nt, synthetic construct
  source 1..24: mol_type = other RNA
  modified_base 1: mod_base = OTHER; note = 2'-O-methyladenosine
  modified_base 2: mod_base = OTHER; note = 2'-O,4'-C-methylene-briged adenosine
  modified_base 3: mod_base = gm
  modified_base 4: mod_base = OTHER; note = 2'-O,4'-C-methylene-briged guanosine
  modified_base 5: mod_base = gm
  modified_base 6: mod_base = OTHER; note = 2'-deoxy-2'-fluorocytidine
  modified_base 7: mod_base = OTHER; note = 2'-deoxy-2'-fluorocytidine
  modified_base 8: mod_base = cm
  modified_base 9: mod_base = cm
  modified_base 10: mod_base = OTHER; note = 2'-deoxycytidine
  modified_base 11: mod_base = OTHER; note = 2'-deoxyadenosine
  modified_base 12: mod_base = gm
  modified_base 13: mod_base = OTHER; note = 2'-deoxy-2'-fluoroguanosine
  modified_base 14: mod_base = cm
  modified_base 15: mod_base = OTHER; note = 2'-deoxy-2'-fluorocytidine
  modified_base 16: mod_base = cm
  modified_base 17: mod_base = OTHER; note = 2'-deoxy-2'-fluorocytidine
  modified_base 18: mod_base = um
  modified_base 19: mod_base = OTHER; note = 2'-deoxy-2'-fluorocytidine
  modified_base 20: mod_base = cm
  modified_base 21: mod_base = OTHER; note = 2'-O,4'-C-methylene-briged thymidine
  modified_base 22: mod_base = gm
  modified_base 23: mod_base = OTHER; note = 2'-O,4'-C-methylene-briged thymidine
  modified_base 24: mod_base = um
  modified_base 1^2: mod_base = OTHER; note = phosphorotioate bond between nucleosides
  modified_base 2^3: mod_base = OTHER; note = phosphorothioate bond between nucleosides
  modified_base 3^4: mod_base = OTHER; note = phosphorothioate bond between nucleosides
  modified_base 4^5: mod_base = OTHER; note = phosphorothioate bond between nucleosides
  modified_base 5^6: mod_base = OTHER; note = phosphorothioate bond between nucleosides
  modified_base 7^8: mod_base = OTHER; note = phosphorothioate bond between nucleosides
  modified_base 6^7: mod_base = OTHER; note = phosphorothioate bond between nucleosides
  modified_base 8^9: mod_base = OTHER; note = phosphorothioate bond between nucleosides
  modified_base 9^10: mod_base = OTHER; note = phosphorothioate bond between nucleosides
  modified_base 10^11: mod_base = OTHER; note = phosphorothioate bond between nucleosides
  modified_base 11^12: mod_base = OTHER; note = ethylphosphate bond between nucleosides
  modified_base 12^13: mod_base = OTHER; note = phosphorothioate bond between nucleosides
  modified_base 13^14: mod_base = OTHER; note = phosphorothioate bond between nucleosides
  modified_base 14^15: mod_base = OTHER; note = phosphorothioate bond between nucleosides
  modified_base 15^16: mod_base = OTHER; note = phosphorothioate bond between nucleosides
  modified_base 16^17: mod_base = OTHER; note = phosphorothioate bond between nucleosides
  modified_base 17^18: mod_base = OTHER; note = phosphorothioate bond between nucleosides
  modified_base 18^19: mod_base = OTHER; note = phosphorothioate bond between nucleosides
  modified_base 19^20: mod_base = OTHER; note = phosphorothioate bond between nucleosides
  modified_base 20^21: mod_base = OTHER; note = phosphorothioate bond between nucleosides
  modified_base 21^22: mod_base = OTHER; note = phosphorothioate bond between nucleosides
  modified_base 22^23: mod_base = OTHER; note = phosphorothioate bond between nucleosides
  modified_base 23^24: mod_base = OTHER; note = phosphorothioate bond between nucleosides
gagggcccccaggcccctcctgtt

SEQ ID NO: 108 - RNA, 24 nt, synthetic construct
  source 1..24: mol_type = other RNA
  modified_base 1: mod_base = OTHER; note = 2'-O-methyladenosine
  modified_base 2: mod_base = OTHER; note = 2'-O,4'-C-methylene-briged adenosine
  modified_base 3: mod_base = OTHER; note = 2'-O-methyladenosine
  modified_base 4: mod_base = OTHER; note = 2'-O,4'-C-methylene-briged guanosine
  modified_base 5: mod_base = cm
  modified_base 6: mod_base = OTHER; note = 2'-deoxy-2'-fluoroadenosine
  modified_base 7: mod_base = OTHER; note = 2'-deoxy-2'-fluorouridine
  modified_base 8: mod_base = gm
  modified_base 9: mod_base = cm
  modified_base 10: mod_base = OTHER; note = 2'-deoxycytidine
  modified_base 11: mod_base = OTHER; note = 2'-deoxyadenosine
  modified_base 12: mod_base = um
  modified_base 13: mod_base = OTHER; note = 2'-deoxy-2'-fluorocytidine
  modified_base 14: mod_base = OTHER; note = 2'-O-methyladenosine
  modified_base 15: mod_base = OTHER; note = 2'-deoxy-2'-fluorocytidine
  modified_base 16: mod_base = cm
  modified_base 17: mod_base = OTHER; note = 2'-deoxy-2'-fluorouridine
  modified_base 18: mod_base = cm
  modified_base 19: mod_base = OTHER; note = 2'-deoxy-2'-fluorocytidine
  modified_base 20: mod_base = cm
  modified_base 21: mod_base = cm
  modified_base 22: mod_base = um
  modified_base 23: mod_base = OTHER; note = 2'-O,4'-C-methylene-briged guanosine
  modified_base 24: mod_base = um
  modified_base 1^2: mod_base = OTHER; note = phosphorotioate bond between nucleosides
  modified_base 2^3: mod_base = OTHER; note = phosphorothioate bond between nucleosides
  modified_base 3^4: mod_base = OTHER; note = phosphorothioate bond between nucleosides
  modified_base 4^5: mod_base = OTHER; note = phosphorothioate bond between nucleosides
  modified_base 5^6: mod_base = OTHER; note = phosphorothioate bond between nucleosides
  modified_base 7^8: mod_base = OTHER; note = phosphorothioate bond between nucleosides
  modified_base 6^7: mod_base = OTHER; note = phosphorothioate bond between nucleosides
  modified_base 8^9: mod_base = OTHER; note = phosphorothioate bond between nucleosides
  modified_base 9^10: mod_base = OTHER; note = phosphorothioate bond between nucleosides
  modified_base 10^11: mod_base = OTHER; note = phosphorothioate bond between nucleosides
  modified_base 11^12: mod_base = OTHER; note = ethylphosphate bond between nucleosides
  modified_base 12^13: mod_base = OTHER; note = phosphorothioate bond between nucleosides
  modified_base 13^14: mod_base = OTHER; note = phosphorothioate bond between nucleosides
  modified_base 14^15: mod_base = OTHER; note = ethylphosphate bond between nucleosides
  modified_base 15^16: mod_base = OTHER; note = phosphorothioate bond between nucleosides
  modified_base 16^17: mod_base = OTHER; note = phosphorothioate bond between nucleosides
  modified_base 17^18: mod_base = OTHER; note = phosphorothioate bond between nucleosides
  modified_base 18^19: mod_base = OTHER; note = phosphorothioate bond between nucleosides
  modified_base 19^20: mod_base = OTHER; note = phosphorothioate bond between nucleosides
  modified_base 20^21: mod_base = OTHER; note = phosphorothioate bond between nucleosides
  modified_base 21^22: mod_base = OTHER; note = phosphorothioate bond between nucleosides
  modified_base 22^23: mod_base = OTHER; note = phosphorothioate bond between nucleosides
  modified_base 23^24: mod_base = OTHER; note = phosphorothioate bond between nucleosides
aaagcatgccatcacctcccctgt

SEQ ID NO: 109 - RNA, 24 nt, synthetic construct
  source 1..24: mol_type = other RNA
  modified_base 1: mod_base = OTHER; note = 2'-O-methyladenosine
  modified_base 2: mod_base = OTHER; note = 2'-O,4'-C-methylene-briged adenosine
  modified_base 3: mod_base = OTHER; note = 2'-O-methyladenosine
  modified_base 4: mod_base = OTHER; note = 2'-O,4'-C-methylene-briged guanosine
  modified_base 5: mod_base = cm
  modified_base 6: mod_base = OTHER; note = 2'-deoxy-2'-fluoroadenosine
  modified_base 7: mod_base = OTHER; note = 2'-deoxy-2'-fluorouridine
  modified_base 8: mod_base = gm
  modified_base 9: mod_base = cm
  modified_base 10: mod_base = OTHER; note = 2'-deoxycytidine
  modified_base 11: mod_base = OTHER; note = 2'-deoxyadenosine
  modified_base 12: mod_base = um
  modified_base 13: mod_base = OTHER; note = 2'-deoxy-2'-fluorocytidine
  modified_base 14: mod_base = OTHER; note = 2'-O-methyladenosine
  modified_base 15: mod_base = OTHER; note = 2'-deoxy-2'-fluorocytidine
  modified_base 16: mod_base = cm
  modified_base 17: mod_base = OTHER; note = 2'-deoxy-2'-fluorouridine
  modified_base 18: mod_base = cm
  modified_base 19: mod_base = OTHER; note = 2'-deoxy-2'-fluorocytidine
  modified_base 20: mod_base = cm
  modified_base 21: mod_base = cm
  modified_base 22: mod_base = um
  modified_base 23: mod_base = OTHER; note = 2'-O,4'-C-methylene-briged guanosine
  modified_base 24: mod_base = um
  modified_base 1^2: mod_base = OTHER; note = phosphorotioate bond between nucleosides
  modified_base 2^3: mod_base = OTHER; note = phosphorothioate bond between nucleosides
  modified_base 3^4: mod_base = OTHER; note = phosphorothioate bond between nucleosides
  modified_base 4^5: mod_base = OTHER; note = phosphorothioate bond between nucleosides
  modified_base 5^6: mod_base = OTHER; note = phosphorothioate bond between nucleosides
  modified_base 7^8: mod_base = OTHER; note = phosphorothioate bond between nucleosides
  modified_base 6^7: mod_base = OTHER; note = phosphorothioate bond between nucleosides
  modified_base 8^9: mod_base = OTHER; note = phosphorothioate bond between nucleosides
  modified_base 9^10: mod_base = OTHER; note = phosphorothioate bond between nucleosides
  modified_base 10^11: mod_base = OTHER; note = phosphorothioate bond between nucleosides
  modified_base 11^12: mod_base = OTHER; note = ethylphosphate bond between nucleosides
  modified_base 13^14: mod_base = OTHER; note = phosphorothioate bond between nucleosides
  modified_base 14^15: mod_base = OTHER; note = ethylphosphate bond between nucleosides
  modified_base 15^16: mod_base = OTHER; note = phosphorothioate bond between nucleosides
  modified_base 16^17: mod_base = OTHER; note = phosphorothioate bond between nucleosides
  modified_base 17^18: mod_base = OTHER; note = phosphorothioate bond between nucleosides
  modified_base 18^19: mod_base = OTHER; note = phosphorothioate bond between nucleosides
  modified_base 19^20: mod_base = OTHER; note = phosphorothioate bond between nucleosides
  modified_base 20^21: mod_base = OTHER; note = phosphorothioate bond between nucleosides
  modified_base 21^22: mod_base = OTHER; note = phosphorothioate bond between nucleosides
  modified_base 22^23: mod_base = OTHER; note = phosphorothioate bond between nucleosides
  modified_base 23^24: mod_base = OTHER; note = phosphorothioate bond between nucleosides
aaagcatgccatcacctcccctgt

SEQ ID NO: 110 - RNA, 24 nt, synthetic construct
  source 1..24: mol_type = other RNA
  modified_base 1: mod_base = OTHER; note = 2'-O-methyladenosine
  modified_base 2: mod_base = OTHER; note = 2'-O,4'-C-methylene-briged adenosine
  modified_base 3: mod_base = OTHER; note = 2'-O-methyladenosine
  modified_base 4: mod_base = OTHER; note = 2'-O,4'-C-methylene-briged guanosine
  modified_base 5: mod_base = cm
  modified_base 6: mod_base = OTHER; note = 2'-deoxy-2'-fluoroadenosine
  modified_base 7: mod_base = OTHER; note = 2'-deoxy-2'-fluorouridine
  modified_base 8: mod_base = gm
  modified_base 9: mod_base = cm
  modified_base 10: mod_base = OTHER; note = 2'-deoxycytidine
  modified_base 11: mod_base = OTHER; note = 2'-deoxyadenosine
  modified_base 12: mod_base = um
  modified_base 13: mod_base = OTHER; note = 2'-deoxy-2'-fluorocytidine
  modified_base 14: mod_base = OTHER; note = 2'-O-methyladenosine
  modified_base 15: mod_base = OTHER; note = 2'-deoxy-2'-fluorocytidine
  modified_base 16: mod_base = cm
  modified_base 17: mod_base = OTHER; note = 2'-deoxy-2'-fluorouridine
  modified_base 18: mod_base = cm
  modified_base 19: mod_base = OTHER; note = 2'-deoxy-2'-fluorocytidine
  modified_base 20: mod_base = cm
  modified_base 21: mod_base = cm
  modified_base 22: mod_base = um
  modified_base 23: mod_base = OTHER; note = 2'-O,4'-C-methylene-briged guanosine
  modified_base 24: mod_base = um
  modified_base 1^2: mod_base = OTHER; note = phosphorotioate bond between nucleosides
  modified_base 2^3: mod_base = OTHER; note = phosphorothioate bond between nucleosides
  modified_base 3^4: mod_base = OTHER; note = phosphorothioate bond between nucleosides
  modified_base 4^5: mod_base = OTHER; note = phosphorothioate bond between nucleosides
  modified_base 5^6: mod_base = OTHER; note = phosphorothioate bond between nucleosides
  modified_base 7^8: mod_base = OTHER; note = phosphorothioate bond between nucleosides
  modified_base 6^7: mod_base = OTHER; note = phosphorothioate bond between nucleosides
  modified_base 8^9: mod_base = OTHER; note = phosphorothioate bond between nucleosides
  modified_base 9^10: mod_base = OTHER; note = phosphorothioate bond between nucleosides
  modified_base 10^11: mod_base = OTHER; note = phosphorothioate bond between nucleosides
  modified_base 11^12: mod_base = OTHER; note = ethylphosphate bond between nucleosides
  modified_base 13^14: mod_base = OTHER; note = phosphorothioate bond between nucleosides
  modified_base 14^15: mod_base = OTHER; note = ethylphosphate bond between nucleosides
  modified_base 15^16: mod_base = OTHER; note = phosphorothioate bond between nucleosides
  modified_base 17^18: mod_base = OTHER; note = phosphorothioate bond between nucleosides
  modified_base 18^19: mod_base = OTHER; note = phosphorothioate bond between nucleosides
  modified_base 19^20: mod_base = OTHER; note = phosphorothioate bond between nucleosides
  modified_base 20^21: mod_base = OTHER; note = phosphorothioate bond between nucleosides
  modified_base 21^22: mod_base = OTHER; note = phosphorothioate bond between nucleosides
  modified_base 22^23: mod_base = OTHER; note = phosphorothioate bond between nucleosides
  modified_base 23^24: mod_base = OTHER; note = phosphorothioate bond between nucleosides
aaagcatgccatcacctcccctgt

SEQ ID NO: 111 - RNA, 24 nt, synthetic construct
  source 1..24: mol_type = other RNA
  modified_base 1: mod_base = OTHER; note = 2'-O-methyladenosine
  modified_base 2: mod_base = OTHER; note = 2'-O,4'-C-methylene-briged adenosine
  modified_base 3: mod_base = OTHER; note = 2'-O-methyladenosine
  modified_base 4: mod_base = OTHER; note = 2'-O,4'-C-methylene-briged guanosine
  modified_base 5: mod_base = cm
  modified_base 6: mod_base = OTHER; note = 2'-deoxy-2'-fluoroadenosine
  modified_base 7: mod_base = OTHER; note = 2'-deoxy-2'-fluorouridine
  modified_base 8: mod_base = gm
  modified_base 9: mod_base = cm
  modified_base 10: mod_base = OTHER; note = 2'-deoxycytidine
  modified_base 11: mod_base = OTHER; note = 2'-deoxyadenosine
  modified_base 12: mod_base = um
  modified_base 13: mod_base = OTHER; note = 2'-deoxy-2'-fluorocytidine
  modified_base 14: mod_base = OTHER; note = 2'-O-methyladenosine
  modified_base 15: mod_base = OTHER; note = 2'-deoxy-2'-fluorocytidine
  modified_base 16: mod_base = cm
  modified_base 17: mod_base = OTHER; note = 2'-deoxy-2'-fluorouridine
  modified_base 18: mod_base = cm
  modified_base 19: mod_base = OTHER; note = 2'-deoxy-2'-fluorocytidine
  modified_base 20: mod_base = cm
  modified_base 21: mod_base = cm
  modified_base 22: mod_base = um
  modified_base 23: mod_base = OTHER; note = 2'-O,4'-C-methylene-briged guanosine
  modified_base 24: mod_base = um
  modified_base 1^2: mod_base = OTHER; note = phosphorotioate bond between nucleosides
  modified_base 2^3: mod_base = OTHER; note = phosphorothioate bond between nucleosides
  modified_base 3^4: mod_base = OTHER; note = phosphorothioate bond between nucleosides
  modified_base 4^5: mod_base = OTHER; note = phosphorothioate bond between nucleosides
  modified_base 5^6: mod_base = OTHER; note = phosphorothioate bond between nucleosides
  modified_base 7^8: mod_base = OTHER; note = phosphorothioate bond between nucleosides
  modified_base 6^7: mod_base = OTHER; note = phosphorothioate bond between nucleosides
  modified_base 8^9: mod_base = OTHER; note = phosphorothioate bond between nucleosides
  modified_base 9^10: mod_base = OTHER; note = phosphorothioate bond between nucleosides
  modified_base 10^11: mod_base = OTHER; note = phosphorothioate bond between nucleosides
  modified_base 11^12: mod_base = OTHER; note = ethylphosphate bond between nucleosides
  modified_base 13^14: mod_base = OTHER; note = phosphorothioate bond between nucleosides
  modified_base 14^15: mod_base = OTHER; note = ethylphosphate bond between nucleosides
  modified_base 15^16: mod_base = OTHER; note = phosphorothioate bond between nucleosides
  modified_base 16^17: mod_base = OTHER; note = phosphorothioate bond between nucleosides
  modified_base 17^18: mod_base = OTHER; note = phosphorothioate bond between nucleosides
  modified_base 19^20: mod_base = OTHER; note = phosphorothioate bond between nucleosides
  modified_base 20^21: mod_base = OTHER; note = phosphorothioate bond between nucleosides
  modified_base 21^22: mod_base = OTHER; note = phosphorothioate bond between nucleosides
  modified_base 22^23: mod_base = OTHER; note = phosphorothioate bond between nucleosides
  modified_base 23^24: mod_base = OTHER; note = phosphorothioate bond between nucleosides
aaagcatgccatcacctcccctgt

SEQ ID NO: 112 - RNA, 24 nt, synthetic construct
  source 1..24: mol_type = other RNA
  modified_base 1: mod_base = OTHER; note = 2'-O-methyladenosine
  modified_base 2: mod_base = OTHER; note = 2'-O,4'-C-methylene-briged adenosine
  modified_base 3: mod_base = OTHER; note = 2'-O-methyladenosine
  modified_base 4: mod_base = OTHER; note = 2'-O,4'-C-methylene-briged guanosine
  modified_base 5: mod_base = cm
  modified_base 6: mod_base = OTHER; note = 2'-deoxy-2'-fluoroadenosine
  modified_base 7: mod_base = OTHER; note = 2'-deoxy-2'-fluorouridine
  modified_base 8: mod_base = gm
  modified_base 9: mod_base = cm
  modified_base 10: mod_base = OTHER; note = 2'-deoxycytidine
  modified_base 11: mod_base = OTHER; note = 2'-deoxyadenosine
  modified_base 12: mod_base = um
  modified_base 13: mod_base = OTHER; note = 2'-deoxy-2'-fluorocytidine
  modified_base 14: mod_base = OTHER; note = 2'-O-methyladenosine
  modified_base 15: mod_base = OTHER; note = 2'-deoxy-2'-fluorocytidine
  modified_base 16: mod_base = cm
  modified_base 17: mod_base = OTHER; note = 2'-deoxy-2'-fluorouridine
  modified_base 18: mod_base = cm
  modified_base 19: mod_base = OTHER; note = 2'-deoxy-2'-fluorocytidine
  modified_base 20: mod_base = cm
  modified_base 21: mod_base = cm
  modified_base 22: mod_base = um
  modified_base 23: mod_base = OTHER; note = 2'-O,4'-C-methylene-briged guanosine
  modified_base 24: mod_base = um
  modified_base 1^2: mod_base = OTHER; note = phosphorotioate bond between nucleosides
  modified_base 2^3: mod_base = OTHER; note = phosphorothioate bond between nucleosides
  modified_base 3^4: mod_base = OTHER; note = phosphorothioate bond between nucleosides
  modified_base 4^5: mod_base = OTHER; note = phosphorothioate bond between nucleosides
  modified_base 5^6: mod_base = OTHER; note = phosphorothioate bond between nucleosides
  modified_base 7^8: mod_base = OTHER; note = phosphorothioate bond between nucleosides
  modified_base 6^7: mod_base = OTHER; note = phosphorothioate bond between nucleosides
  modified_base 8^9: mod_base = OTHER; note = phosphorothioate bond between nucleosides
  modified_base 9^10: mod_base = OTHER; note = phosphorothioate bond between nucleosides
  modified_base 10^11: mod_base = OTHER; note = phosphorothioate bond between nucleosides
  modified_base 11^12: mod_base = OTHER; note = ethylphosphate bond between nucleosides
  modified_base 13^14: mod_base = OTHER; note = phosphorothioate bond between nucleosides
  modified_base 14^15: mod_base = OTHER; note = ethylphosphate bond between nucleosides
  modified_base 15^16: mod_base = OTHER; note = phosphorothioate bond between nucleosides
  modified_base 16^17: mod_base = OTHER; note = phosphorothioate bond between nucleosides
  modified_base 17^18: mod_base = OTHER; note = phosphorothioate bond between nucleosides
  modified_base 18^19: mod_base = OTHER; note = phosphorothioate bond between nucleosides
  modified_base 19^20: mod_base = OTHER; note = phosphorothioate bond between nucleosides
  modified_base 21^22: mod_base = OTHER; note = phosphorothioate bond between nucleosides
  modified_base 22^23: mod_base = OTHER; note = phosphorothioate bond between nucleosides
  modified_base 23^24: mod_base = OTHER; note = phosphorothioate bond between nucleosides
aaagcatgccatcacctcccctgt

SEQ ID NO: 113 - RNA, 24 nt, synthetic construct
  source 1..24: mol_type = other RNA
  modified_base 1: mod_base = OTHER; note = 2'-O-methyladenosine
  modified_base 2: mod_base = OTHER; note = 2'-O,4'-C-methylene-briged adenosine
  modified_base 3: mod_base = OTHER; note = 2'-O-methyladenosine
  modified_base 4: mod_base = OTHER; note = 2'-O,4'-C-methylene-briged guanosine
  modified_base 5: mod_base = cm
  modified_base 6: mod_base = OTHER; note = 2'-deoxy-2'-fluoroadenosine
  modified_base 7: mod_base = OTHER; note = 2'-deoxy-2'-fluorouridine
  modified_base 8: mod_base = gm
  modified_base 9: mod_base = cm
  modified_base 10: mod_base = OTHER; note = 2'-deoxycytidine
  modified_base 11: mod_base = OTHER; note = 2'-deoxyadenosine
  modified_base 12: mod_base = um
  modified_base 13: mod_base = OTHER; note = 2'-deoxy-2'-fluorocytidine
  modified_base 14: mod_base = OTHER; note = 2'-O-methyladenosine
  modified_base 15: mod_base = OTHER; note = 2'-deoxy-2'-fluorocytidine
  modified_base 16: mod_base = cm
  modified_base 17: mod_base = OTHER; note = 2'-deoxy-2'-fluorouridine
  modified_base 18: mod_base = cm
  modified_base 19: mod_base = OTHER; note = 2'-deoxy-2'-fluorocytidine
  modified_base 20: mod_base = cm
  modified_base 21: mod_base = cm
  modified_base 22: mod_base = um
  modified_base 23: mod_base = OTHER; note = 2'-O,4'-C-methylene-briged guanosine
  modified_base 24: mod_base = um
  modified_base 1^2: mod_base = OTHER; note = phosphorotioate bond between nucleosides
  modified_base 2^3: mod_base = OTHER; note = phosphorothioate bond between nucleosides
  modified_base 3^4: mod_base = OTHER; note = phosphorothioate bond between nucleosides
  modified_base 4^5: mod_base = OTHER; note = phosphorothioate bond between nucleosides
  modified_base 5^6: mod_base = OTHER; note = phosphorothioate bond between nucleosides
  modified_base 7^8: mod_base = OTHER; note = phosphorothioate bond between nucleosides
  modified_base 6^7: mod_base = OTHER; note = phosphorothioate bond between nucleosides
  modified_base 8^9: mod_base = OTHER; note = phosphorothioate bond between nucleosides
  modified_base 9^10: mod_base = OTHER; note = phosphorothioate bond between nucleosides
  modified_base 10^11: mod_base = OTHER; note = phosphorothioate bond between nucleosides
  modified_base 11^12: mod_base = OTHER; note = ethylphosphate bond between nucleosides
  modified_base 13^14: mod_base = OTHER; note = phosphorothioate bond between nucleosides
  modified_base 14^15: mod_base = OTHER; note = ethylphosphate bond between nucleosides
  modified_base 15^16: mod_base = OTHER; note = phosphorothioate bond between nucleosides
  modified_base 17^18: mod_base = OTHER; note = phosphorothioate bond between nucleosides
  modified_base 19^20: mod_base = OTHER; note = phosphorothioate bond between nucleosides
  modified_base 20^21: mod_base = OTHER; note = phosphorothioate bond between nucleosides
  modified_base 21^22: mod_base = OTHER; note = phosphorothioate bond between nucleosides
  modified_base 22^23: mod_base = OTHER; note = phosphorothioate bond between nucleosides
  modified_base 23^24: mod_base = OTHER; note = phosphorothioate bond between nucleosides
aaagcatgccatcacctcccctgt

SEQ ID NO: 114 - RNA, 24 nt, synthetic construct
  source 1..24: mol_type = other RNA
  modified_base 1: mod_base = OTHER; note = 2'-O-methyladenosine
  modified_base 2: mod_base = OTHER; note = 2'-O,4'-C-methylene-briged adenosine
  modified_base 3: mod_base = OTHER; note = 2'-O-methyladenosine
  modified_base 4: mod_base = OTHER; note = 2'-O,4'-C-methylene-briged guanosine
  modified_base 5: mod_base = cm
  modified_base 6: mod_base = OTHER; note = 2'-deoxy-2'-fluoroadenosine
  modified_base 7: mod_base = OTHER; note = 2'-deoxy-2'-fluorouridine
  modified_base 8: mod_base = gm
  modified_base 9: mod_base = cm
  modified_base 10: mod_base = OTHER; note = 2'-deoxycytidine
  modified_base 11: mod_base = OTHER; note = 2'-deoxyadenosine
  modified_base 12: mod_base = um
  modified_base 13: mod_base = OTHER; note = 2'-deoxy-2'-fluorocytidine
  modified_base 14: mod_base = OTHER; note = 2'-O-methyladenosine
  modified_base 15: mod_base = OTHER; note = 2'-deoxy-2'-fluorocytidine
  modified_base 16: mod_base = cm
  modified_base 17: mod_base = OTHER; note = 2'-deoxy-2'-fluorouridine
  modified_base 18: mod_base = cm
  modified_base 19: mod_base = OTHER; note = 2'-deoxy-2'-fluorocytidine
  modified_base 20: mod_base = cm
  modified_base 21: mod_base = cm
  modified_base 22: mod_base = um
  modified_base 23: mod_base = OTHER; note = 2'-O,4'-C-methylene-briged guanosine
  modified_base 24: mod_base = um
  modified_base 1^2: mod_base = OTHER; note = phosphorotioate bond between nucleosides
  modified_base 2^3: mod_base = OTHER; note = phosphorothioate bond between nucleosides
  modified_base 3^4: mod_base = OTHER; note = phosphorothioate bond between nucleosides
  modified_base 4^5: mod_base = OTHER; note = phosphorothioate bond between nucleosides
  modified_base 5^6: mod_base = OTHER; note = phosphorothioate bond between nucleosides
  modified_base 7^8: mod_base = OTHER; note = phosphorothioate bond between nucleosides
  modified_base 6^7: mod_base = OTHER; note = phosphorothioate bond between nucleosides
  modified_base 8^9: mod_base = OTHER; note = phosphorothioate bond between nucleosides
  modified_base 9^10: mod_base = OTHER; note = phosphorothioate bond between nucleosides
  modified_base 10^11: mod_base = OTHER; note = phosphorothioate bond between nucleosides
  modified_base 11^12: mod_base = OTHER; note = ethylphosphate bond between nucleosides
  modified_base 13^14: mod_base = OTHER; note = phosphorothioate bond between nucleosides
  modified_base 14^15: mod_base = OTHER; note = ethylphosphate bond between nucleosides
  modified_base 15^16: mod_base = OTHER; note = phosphorothioate bond between nucleosides
  modified_base 17^18: mod_base = OTHER; note = phosphorothioate bond between nucleosides
  modified_base 18^19: mod_base = OTHER; note = phosphorothioate bond between nucleosides
  modified_base 19^20: mod_base = OTHER; note = phosphorothioate bond between nucleosides
  modified_base 21^22: mod_base = OTHER; note = phosphorothioate bond between nucleosides
  modified_base 22^23: mod_base = OTHER; note = phosphorothioate bond between nucleosides
  modified_base 23^24: mod_base = OTHER; note = phosphorothioate bond between nucleosides
aaagcatgccatcacctcccctgt

SEQ ID NO: 115 - RNA, 24 nt, synthetic construct
  source 1..24: mol_type = other RNA
  modified_base 1: mod_base = OTHER; note = 2'-O-methyladenosine
  modified_base 2: mod_base = OTHER; note = 2'-O,4'-C-methylene-briged adenosine
  modified_base 3: mod_base = OTHER; note = 2'-O-methyladenosine
  modified_base 4: mod_base = OTHER; note = 2'-O,4'-C-methylene-briged guanosine
  modified_base 5: mod_base = cm
  modified_base 6: mod_base = OTHER; note = 2'-deoxy-2'-fluoroadenosine
  modified_base 7: mod_base = OTHER; note = 2'-deoxy-2'-fluorouridine
  modified_base 8: mod_base = gm
  modified_base 9: mod_base = cm
  modified_base 10: mod_base = OTHER; note = 2'-deoxycytidine
  modified_base 11: mod_base = OTHER; note = 2'-deoxyadenosine
  modified_base 12: mod_base = um
  modified_base 13: mod_base = OTHER; note = 2'-deoxy-2'-fluorocytidine
  modified_base 14: mod_base = OTHER; note = 2'-O-methyladenosine
  modified_base 15: mod_base = OTHER; note = 2'-deoxy-2'-fluorocytidine
  modified_base 16: mod_base = cm
  modified_base 17: mod_base = OTHER; note = 2'-deoxy-2'-fluorouridine
  modified_base 18: mod_base = cm
  modified_base 19: mod_base = OTHER; note = 2'-deoxy-2'-fluorocytidine
  modified_base 20: mod_base = cm
  modified_base 21: mod_base = cm
  modified_base 22: mod_base = um
  modified_base 23: mod_base = OTHER; note = 2'-O,4'-C-methylene-briged guanosine
  modified_base 24: mod_base = um
  modified_base 1^2: mod_base = OTHER; note = phosphorotioate bond between nucleosides
  modified_base 2^3: mod_base = OTHER; note = phosphorothioate bond between nucleosides
  modified_base 3^4: mod_base = OTHER; note = phosphorothioate bond between nucleosides
  modified_base 4^5: mod_base = OTHER; note = phosphorothioate bond between nucleosides
  modified_base 5^6: mod_base = OTHER; note = phosphorothioate bond between nucleosides
  modified_base 7^8: mod_base = OTHER; note = phosphorothioate bond between nucleosides
  modified_base 6^7: mod_base = OTHER; note = phosphorothioate bond between nucleosides
  modified_base 8^9: mod_base = OTHER; note = phosphorothioate bond between nucleosides
  modified_base 9^10: mod_base = OTHER; note = phosphorothioate bond between nucleosides
  modified_base 10^11: mod_base = OTHER; note = phosphorothioate bond between nucleosides
  modified_base 11^12: mod_base = OTHER; note = ethylphosphate bond between nucleosides
  modified_base 13^14: mod_base = OTHER; note = phosphorothioate bond between nucleosides
  modified_base 14^15: mod_base = OTHER; note = ethylphosphate bond between nucleosides
  modified_base 15^16: mod_base = OTHER; note = phosphorothioate bond between nucleosides
  modified_base 16^17: mod_base = OTHER; note = phosphorothioate bond between nucleosides
  modified_base 17^18: mod_base = OTHER; note = phosphorothioate bond between nucleosides
  modified_base 19^20: mod_base = OTHER; note = phosphorothioate bond between nucleosides
  modified_base 21^22: mod_base = OTHER; note = phosphorothioate bond between nucleosides
  modified_base 22^23: mod_base = OTHER; note = phosphorothioate bond between nucleosides
  modified_base 23^24: mod_base = OTHER; note = phosphorothioate bond between nucleosides
aaagcatgccatcacctcccctgt

SEQ ID NO: 116 - RNA, 24 nt, synthetic construct
  source 1..24: mol_type = other RNA
  modified_base 1: mod_base = OTHER; note = 2'-O-methyladenosine
  modified_base 2: mod_base = OTHER; note = 2'-O,4'-C-methylene-briged adenosine
  modified_base 3: mod_base = OTHER; note = 2'-O-methyladenosine
  modified_base 4: mod_base = OTHER; note = 2'-O,4'-C-methylene-briged guanosine
  modified_base 5: mod_base = cm
  modified_base 6: mod_base = OTHER; note = 2'-deoxy-2'-fluoroadenosine
  modified_base 7: mod_base = OTHER; note = 2'-deoxy-2'-fluorouridine
  modified_base 8: mod_base = gm
  modified_base 9: mod_base = cm
  modified_base 10: mod_base = OTHER; note = 2'-deoxycytidine
  modified_base 11: mod_base = OTHER; note = 2'-deoxyadenosine
  modified_base 12: mod_base = um
  modified_base 13: mod_base = OTHER; note = 2'-deoxy-2'-fluorocytidine
  modified_base 14: mod_base = OTHER; note = 2'-O-methyladenosine
  modified_base 15: mod_base = OTHER; note = 2'-deoxy-2'-fluorocytidine
  modified_base 16: mod_base = cm
  modified_base 17: mod_base = OTHER; note = 2'-deoxy-2'-fluorouridine
  modified_base 18: mod_base = cm
  modified_base 19: mod_base = OTHER; note = 2'-deoxy-2'-fluorocytidine
  modified_base 20: mod_base = cm
  modified_base 21: mod_base = cm; note = 2'-O,4'-C-methylene-briged cytidine
  modified_base 22: mod_base = um
  modified_base 23: mod_base = OTHER; note = 2'-O,4'-C-methylene-briged guanosine
  modified_base 24: mod_base = um
  modified_base 1^2: mod_base = OTHER; note = phosphorotioate bond between nucleosides
  modified_base 2^3: mod_base = OTHER; note = phosphorothioate bond between nucleosides
  modified_base 3^4: mod_base = OTHER; note = phosphorothioate bond between nucleosides
  modified_base 4^5: mod_base = OTHER; note = phosphorothioate bond between nucleosides
  modified_base 5^6: mod_base = OTHER; note = phosphorothioate bond between nucleosides
  modified_base 7^8: mod_base = OTHER; note = phosphorothioate bond between nucleosides
  modified_base 6^7: mod_base = OTHER; note = phosphorothioate bond between nucleosides
  modified_base 8^9: mod_base = OTHER; note = phosphorothioate bond between nucleosides
  modified_base 9^10: mod_base = OTHER; note = phosphorothioate bond between nucleosides
  modified_base 10^11: mod_base = OTHER; note = phosphorothioate bond between nucleosides
  modified_base 11^12: mod_base = OTHER; note = ethylphosphate bond between nucleosides
  modified_base 13^14: mod_base = OTHER; note = phosphorothioate bond between nucleosides
  modified_base 14^15: mod_base = OTHER; note = ethylphosphate bond between nucleosides
  modified_base 15^16: mod_base = OTHER; note = phosphorothioate bond between nucleosides
  modified_base 17^18: mod_base = OTHER; note = phosphorothioate bond between nucleosides
  modified_base 19^20: mod_base = OTHER; note = phosphorothioate bond between nucleosides
  modified_base 21^22: mod_base = OTHER; note = phosphorothioate bond between nucleosides
  modified_base 22^23: mod_base = OTHER; note = phosphorothioate bond between nucleosides
  modified_base 23^24: mod_base = OTHER; note = phosphorothioate bond between nucleosides
aaagcatgccatcacctcccctgt

SEQ ID NO: 117 - RNA, 24 nt, synthetic construct
  source 1..24: mol_type = other RNA
  modified_base 1: mod_base = OTHER; note = 2'-O-methyladenosine
  modified_base 2: mod_base = OTHER; note = 2'-O,4'-C-methylene-briged adenosine
  modified_base 3: mod_base = OTHER; note = 2'-O-methyladenosine
  modified_base 4: mod_base = OTHER; note = 2'-O,4'-C-methylene-briged guanosine
  modified_base 5: mod_base = cm
  modified_base 6: mod_base = OTHER; note = 2'-deoxy-2'-fluoroadenosine
  modified_base 7: mod_base = OTHER; note = 2'-deoxy-2'-fluorouridine
  modified_base 8: mod_base = gm
  modified_base 9: mod_base = cm
  modified_base 10: mod_base = OTHER; note = 2'-deoxycytidine
  modified_base 11: mod_base = OTHER; note = 2'-deoxyadenosine
  modified_base 12: mod_base = um
  modified_base 13: mod_base = OTHER; note = 2'-deoxy-2'-fluorocytidine
  modified_base 14: mod_base = OTHER; note = 2'-O-methyladenosine
  modified_base 15: mod_base = OTHER; note = 2'-deoxy-2'-fluorocytidine
  modified_base 16: mod_base = cm
  modified_base 17: mod_base = OTHER; note = 2'-deoxy-2'-fluorouridine
  modified_base 18: mod_base = cm
  modified_base 19: mod_base = OTHER; note = 2'-deoxy-2'-fluorocytidine
  modified_base 20: mod_base = cm
  modified_base 21: mod_base = cm
  modified_base 22: mod_base = um
  modified_base 23: mod_base = OTHER; note = 2'-O,4'-C-methylene-briged guanosine
  modified_base 24: mod_base = um
  modified_base 1^2: mod_base = OTHER; note = phosphorotioate bond between nucleosides
  modified_base 2^3: mod_base = OTHER; note = phosphorothioate bond between nucleosides
  modified_base 3^4: mod_base = OTHER; note = phosphorothioate bond between nucleosides
  modified_base 4^5: mod_base = OTHER; note = phosphorothioate bond between nucleosides
  modified_base 5^6: mod_base = OTHER; note = phosphorothioate bond between nucleosides
  modified_base 7^8: mod_base = OTHER; note = phosphorothioate bond between nucleosides
  modified_base 6^7: mod_base = OTHER; note = phosphorothioate bond between nucleosides
  modified_base 8^9: mod_base = OTHER; note = phosphorothioate bond between nucleosides
  modified_base 9^10: mod_base = OTHER; note = phosphorothioate bond between nucleosides
  modified_base 10^11: mod_base = OTHER; note = phosphorothioate bond between nucleosides
  modified_base 11^12: mod_base = OTHER; note = methoxyethylphosphate bond between nucleosides
  modified_base 13^14: mod_base = OTHER; note = phosphorothioate bond between nucleosides
  modified_base 14^15: mod_base = OTHER; note = ethylphosphate bond between nucleosides
  modified_base 15^16: mod_base = OTHER; note = phosphorothioate bond between nucleosides
  modified_base 16^17: mod_base = OTHER; note = phosphorothioate bond between nucleosides
  modified_base 17^18: mod_base = OTHER; note = phosphorothioate bond between nucleosides
  modified_base 18^19: mod_base = OTHER; note = phosphorothioate bond between nucleosides
  modified_base 19^20: mod_base = OTHER; note = phosphorothioate bond between nucleosides
  modified_base 20^21: mod_base = OTHER; note = phosphorothioate bond between nucleosides
  modified_base 21^22: mod_base = OTHER; note = phosphorothioate bond between nucleosides
  modified_base 22^23: mod_base = OTHER; note = phosphorothioate bond between nucleosides
  modified_base 23^24: mod_base = OTHER; note = phosphorothioate bond between nucleosides
aaagcatgccatcacctcccctgt

SEQ ID NO: 118 - RNA, 24 nt, synthetic construct
  source 1..24: mol_type = other RNA
  modified_base 1: mod_base = OTHER; note = 2'-O-methyladenosine
  modified_base 2: mod_base = OTHER; note = 2'-O,4'-C-methylene-briged adenosine
  modified_base 3: mod_base = OTHER; note = 2'-O-methyladenosine
  modified_base 4: mod_base = OTHER; note = 2'-O,4'-C-methylene-briged guanosine
  modified_base 5: mod_base = cm
  modified_base 6: mod_base = OTHER; note = 2'-deoxy-2'-fluoroadenosine
  modified_base 7: mod_base = OTHER; note = 2'-deoxy-2'-fluorouridine
  modified_base 8: mod_base = gm
  modified_base 9: mod_base = cm
  modified_base 10: mod_base = OTHER; note = 2'-deoxycytidine
  modified_base 11: mod_base = OTHER; note = 2'-deoxynebularine
  modified_base 12: mod_base = um
  modified_base 13: mod_base = OTHER; note = 2'-deoxy-2'-fluorocytidine
  modified_base 14: mod_base = OTHER; note = 2'-O-methyladenosine
  modified_base 15: mod_base = OTHER; note = 2'-deoxy-2'-fluorocytidine
  modified_base 16: mod_base = cm
  modified_base 17: mod_base = OTHER; note = 2'-deoxy-2'-fluorouridine
  modified_base 18: mod_base = cm
  modified_base 19: mod_base = OTHER; note = 2'-deoxy-2'-fluorocytidine
  modified_base 20: mod_base = cm
  modified_base 21: mod_base = cm
  modified_base 22: mod_base = um
  modified_base 23: mod_base = OTHER; note = 2'-O,4'-C-methylene-briged guanosine
  modified_base 24: mod_base = um
  modified_base 1^2: mod_base = OTHER; note = phosphorotioate bond between nucleosides
  modified_base 2^3: mod_base = OTHER; note = phosphorothioate bond between nucleosides
  modified_base 3^4: mod_base = OTHER; note = phosphorothioate bond between nucleosides
  modified_base 4^5: mod_base = OTHER; note = phosphorothioate bond between nucleosides
  modified_base 5^6: mod_base = OTHER; note = phosphorothioate bond between nucleosides
  modified_base 7^8: mod_base = OTHER; note = phosphorothioate bond between nucleosides
  modified_base 6^7: mod_base = OTHER; note = phosphorothioate bond between nucleosides
  modified_base 8^9: mod_base = OTHER; note = phosphorothioate bond between nucleosides
  modified_base 9^10: mod_base = OTHER; note = phosphorothioate bond between nucleosides
  modified_base 10^11: mod_base = OTHER; note = phosphorothioate bond between nucleosides
  modified_base 11^12: mod_base = OTHER; note = ethylphosphate bond between nucleosides
  modified_base 13^14: mod_base = OTHER; note = phosphorothioate bond between nucleosides
  modified_base 14^15: mod_base = OTHER; note = ethylphosphate bond between nucleosides
  modified_base 15^16: mod_base = OTHER; note = phosphorothioate bond between nucleosides
  modified_base 16^17: mod_base = OTHER; note = phosphorothioate bond between nucleosides
  modified_base 17^18: mod_base = OTHER; note = phosphorothioate bond between nucleosides
  modified_base 18^19: mod_base = OTHER; note = phosphorothioate bond between nucleosides
  modified_base 19^20: mod_base = OTHER; note = phosphorothioate bond between nucleosides
  modified_base 20^21: mod_base = OTHER; note = phosphorothioate bond between nucleosides
  modified_base 21^22: mod_base = OTHER; note = phosphorothioate bond between nucleosides
  modified_base 22^23: mod_base = OTHER; note = phosphorothioate bond between nucleosides
  modified_base 23^24: mod_base = OTHER; note = phosphorothioate bond between nucleosides
aaagcatgccatcacctcccctgt

SEQ ID NO: 119 - RNA, 24 nt, synthetic construct
  source 1..24: mol_type = other RNA
  modified_base 1: mod_base = OTHER; note = 2'-O-methyladenosine
  modified_base 2: mod_base = OTHER; note = 2'-O,4'-C-methylene-briged adenosine
  modified_base 3: mod_base = OTHER; note = 2'-O-methyladenosine
  modified_base 4: mod_base = OTHER; note = 2'-O,4'-C-methylene-briged guanosine
  modified_base 5: mod_base = cm
  modified_base 6: mod_base = OTHER; note = 2'-deoxy-2'-fluoroadenosine
  modified_base 7: mod_base = OTHER; note = 2'-deoxy-2'-fluorouridine
  modified_base 8: mod_base = gm
  modified_base 9: mod_base = cm
  modified_base 10: mod_base = OTHER; note = 2'-deoxycytidine
  modified_base 11: mod_base = OTHER; note = 2'-deoxyadenosine
  modified_base 12: mod_base = um
  modified_base 13: mod_base = OTHER; note = 2'-deoxy-2'-fluorocytidine
  modified_base 14: mod_base = OTHER; note = 2'-O-methyladenosine
  modified_base 15: mod_base = OTHER; note = 2'-deoxy-2'-fluorocytidine
  modified_base 16: mod_base = cm
  modified_base 17: mod_base = OTHER; note = 2'-deoxy-2'-fluorouridine
  modified_base 18: mod_base = cm
  modified_base 19: mod_base = OTHER; note = 2'-deoxy-2'-fluorocytidine
  modified_base 20: mod_base = cm
  modified_base 21: mod_base = OTHER; note = 2'-O,4'-C-methylene-briged cytidine
  modified_base 22: mod_base = um
  modified_base 23: mod_base = OTHER; note = 2'-O,4'-C-methylene-briged guanosine
  modified_base 24: mod_base = um
  modified_base 1^2: mod_base = OTHER; note = phosphorotioate bond between nucleosides
  modified_base 2^3: mod_base = OTHER; note = phosphorothioate bond between nucleosides
  modified_base 3^4: mod_base = OTHER; note = phosphorothioate bond between nucleosides
  modified_base 4^5: mod_base = OTHER; note = phosphorothioate bond between nucleosides
  modified_base 5^6: mod_base = OTHER; note = phosphorothioate bond between nucleosides
  modified_base 7^8: mod_base = OTHER; note = phosphorothioate bond between nucleosides
  modified_base 6^7: mod_base = OTHER; note = phosphorothioate bond between nucleosides
  modified_base 8^9: mod_base = OTHER; note = phosphorothioate bond between nucleosides
  modified_base 9^10: mod_base = OTHER; note = methylphosphonate bond between nucleosides
  modified_base 10^11: mod_base = OTHER; note = phosphorothioate bond between nucleosides
  modified_base 11^12: mod_base = OTHER; note = phosphorothioate bond between nucleosides
  modified_base 12^13: mod_base = OTHER; note = phosphorothioate bond between nucleosides
  modified_base 13^14: mod_base = OTHER; note = phosphorothioate bond between nucleosides
  modified_base 14^15: mod_base = OTHER; note = phosphorothioate bond between nucleosides
  modified_base 15^16: mod_base = OTHER; note = phosphorothioate bond between nucleosides
  modified_base 16^17: mod_base = OTHER; note = phosphorothioate bond between nucleosides
  modified_base 17^18: mod_base = OTHER; note = phosphorothioate bond between nucleosides
  modified_base 18^19: mod_base = OTHER; note = phosphorothioate bond between nucleosides
  modified_base 19^20: mod_base = OTHER; note = phosphorothioate bond between nucleosides
  modified_base 20^21: mod_base = OTHER; note = phosphorothioate bond between nucleosides
  modified_base 21^22: mod_base = OTHER; note = phosphorothioate bond between nucleosides
  modified_base 22^23: mod_base = OTHER; note = phosphorothioate bond between nucleosides
  modified_base 23^24: mod_base = OTHER; note = phosphorothioate bond between nucleosides
aaagcatgccatcacctcccctgt

SEQ ID NO: 120 - RNA, 24 nt, synthetic construct
  source 1..24: mol_type = other RNA
  modified_base 1: mod_base = OTHER; note = 2'-O-methyladenosine
  modified_base 2: mod_base = OTHER; note = 2'-O,4'-C-methylene-briged adenosine
  modified_base 3: mod_base = OTHER; note = 2'-O-methyladenosine
  modified_base 4: mod_base = OTHER; note = 2'-O,4'-C-methylene-briged guanosine
  modified_base 5: mod_base = cm
  modified_base 6: mod_base = OTHER; note = 2'-deoxy-2'-fluoroadenosine
  modified_base 7: mod_base = OTHER; note = 2'-deoxy-2'-fluorouridine
  modified_base 8: mod_base = gm
  modified_base 9: mod_base = cm
  modified_base 10: mod_base = OTHER; note = 2'-deoxycytidine
  modified_base 11: mod_base = OTHER; note = 2'-deoxyadenosine
  modified_base 12: mod_base = um
  modified_base 13: mod_base = OTHER; note = 2'-deoxy-2'-fluorocytidine
  modified_base 14: mod_base = OTHER; note = 2'-O-methyladenosine
  modified_base 15: mod_base = OTHER; note = 2'-deoxy-2'-fluorocytidine
  modified_base 16: mod_base = cm
  modified_base 17: mod_base = OTHER; note = 2'-deoxy-2'-fluorouridine
  modified_base 18: mod_base = cm
  modified_base 19: mod_base = OTHER; note = 2'-deoxy-2'-fluorocytidine
  modified_base 20: mod_base = cm
  modified_base 21: mod_base = OTHER; note = 2'-O,4'-C-methylene-briged cytidine
  modified_base 22: mod_base = um
  modified_base 23: mod_base = OTHER; note = 2'-O,4'-C-methylene-briged guanosine
  modified_base 24: mod_base = um
  modified_base 1^2: mod_base = OTHER; note = phosphorotioate bond between nucleosides
  modified_base 2^3: mod_base = OTHER; note = phosphorothioate bond between nucleosides
  modified_base 3^4: mod_base = OTHER; note = phosphorothioate bond between nucleosides
  modified_base 4^5: mod_base = OTHER; note = phosphorothioate bond between nucleosides
  modified_base 5^6: mod_base = OTHER; note = phosphorothioate bond between nucleosides
  modified_base 7^8: mod_base = OTHER; note = phosphorothioate bond between nucleosides
  modified_base 6^7: mod_base = OTHER; note = phosphorothioate bond between nucleosides
  modified_base 8^9: mod_base = OTHER; note = phosphorothioate bond between nucleosides
  modified_base 9^10: mod_base = OTHER; note = phosphorothioate bond between nucleosides
  modified_base 10^11: mod_base = OTHER; note = phosphorothioate bond between nucleosides
  modified_base 11^12: mod_base = OTHER; note = phosphorothioate bond between nucleosides
  modified_base 12^13: mod_base = OTHER; note = phosphorothioate bond between nucleosides
  modified_base 13^14: mod_base = OTHER; note = phosphorothioate bond between nucleosides
  modified_base 14^15: mod_base = OTHER; note = phosphorothioate bond between nucleosides
  modified_base 15^16: mod_base = OTHER; note = phosphorothioate bond between nucleosides
  modified_base 16^17: mod_base = OTHER; note = phosphorothioate bond between nucleosides
  modified_base 17^18: mod_base = OTHER; note = phosphorothioate bond between nucleosides
  modified_base 18^19: mod_base = OTHER; note = phosphorothioate bond between nucleosides
  modified_base 19^20: mod_base = OTHER; note = phosphorothioate bond between nucleosides
  modified_base 20^21: mod_base = OTHER; note = phosphorothioate bond between nucleosides
  modified_base 21^22: mod_base = OTHER; note = phosphorothioate bond between nucleosides
  modified_base 22^23: mod_base = OTHER; note = phosphorothioate bond between nucleosides
  modified_base 23^24: mod_base = OTHER; note = phosphorothioate bond between nucleosides
aaagcatgccatcacctcccctgt

SEQ ID NO: 121 - RNA, 24 nt, synthetic construct
  source 1..24: mol_type = other RNA
  modified_base 1: mod_base = OTHER; note = 2'-O-methyladenosine
  modified_base 2: mod_base = OTHER; note = 2'-O,4'-C-ethylene-briged adenosine
  modified_base 3: mod_base = OTHER; note = 2'-O-methyladenosine
  modified_base 4: mod_base = OTHER; note = 2'-O,4'-C-ethylene-briged guanosine
  modified_base 5: mod_base = cm
  modified_base 6: mod_base = OTHER; note = 2'-deoxy-2'-fluoroadenosine
  modified_base 7: mod_base = OTHER; note = 2'-deoxy-2'-fluorouridine
  modified_base 8: mod_base = gm
  modified_base 9: mod_base = cm
  modified_base 10: mod_base = OTHER; note = 2'-deoxycytidine
  modified_base 11: mod_base = OTHER; note = 2'-deoxyadenosine
  modified_base 12: mod_base = um
  modified_base 13: mod_base = OTHER; note = 2'-deoxy-2'-fluorocytidine
  modified_base 14: mod_base = OTHER; note = 2'-O-methyladenosine
  modified_base 15: mod_base = OTHER; note = 2'-deoxy-2'-fluorocytidine
  modified_base 16: mod_base = cm
  modified_base 17: mod_base = OTHER; note = 2'-deoxy-2'-fluorouridine
  modified_base 18: mod_base = cm
  modified_base 19: mod_base = OTHER; note = 2'-deoxy-2'-fluorocytidine
  modified_base 20: mod_base = cm
  modified_base 21: mod_base = OTHER; note = 2'-O,4'-C-ethylene-briged cytidine
  modified_base 22: mod_base = um
  modified_base 23: mod_base = OTHER; note = 2'-O,4'-C-ethylene-briged guanosine
  modified_base 24: mod_base = um
  modified_base 1^2: mod_base = OTHER; note = phosphorotioate bond between nucleosides
  modified_base 2^3: mod_base = OTHER; note = phosphorothioate bond between nucleosides
  modified_base 3^4: mod_base = OTHER; note = phosphorothioate bond between nucleosides
  modified_base 4^5: mod_base = OTHER; note = phosphorothioate bond between nucleosides
  modified_base 5^6: mod_base = OTHER; note = phosphorothioate bond between nucleosides
  modified_base 7^8: mod_base = OTHER; note = phosphorothioate bond between nucleosides
  modified_base 6^7: mod_base = OTHER; note = phosphorothioate bond between nucleosides
  modified_base 8^9: mod_base = OTHER; note = phosphorothioate bond between nucleosides
  modified_base 9^10: mod_base = OTHER; note = phosphorothioate bond between nucleosides
  modified_base 10^11: mod_base = OTHER; note = phosphorothioate bond between nucleosides
  modified_base 11^12: mod_base = OTHER; note = phosphorothioate bond between nucleosides
  modified_base 12^13: mod_base = OTHER; note = phosphorothioate bond between nucleosides
  modified_base 13^14: mod_base = OTHER; note = phosphorothioate bond between nucleosides
  modified_base 14^15: mod_base = OTHER; note = phosphorothioate bond between nucleosides
  modified_base 15^16: mod_base = OTHER; note = phosphorothioate bond between nucleosides
  modified_base 16^17: mod_base = OTHER; note = phosphorothioate bond between nucleosides
  modified_base 17^18: mod_base = OTHER; note = phosphorothioate bond between nucleosides
  modified_base 18^19: mod_base = OTHER; note = phosphorothioate bond between nucleosides
  modified_base 19^20: mod_base = OTHER; note = phosphorothioate bond between nucleosides
  modified_base 20^21: mod_base = OTHER; note = phosphorothioate bond between nucleosides
  modified_base 21^22: mod_base = OTHER; note = phosphorothioate bond between nucleosides
  modified_base 22^23: mod_base = OTHER; note = phosphorothioate bond between nucleosides
  modified_base 23^24: mod_base = OTHER; note = phosphorothioate bond between nucleosides
aaagcatgccatcacctcccctgt

SEQ ID NO: 122 - RNA, 24 nt, synthetic construct
  source 1..24: mol_type = other RNA
  modified_base 1: mod_base = gm
  modified_base 2: mod_base = OTHER; note = 2'-O,4'-C-methylene-briged adenosine
  modified_base 3: mod_base = gm
  modified_base 4: mod_base = OTHER; note = 2'-O,4'-C-methylene-briged guanosine
  modified_base 5: mod_base = gm
  modified_base 6: mod_base = OTHER; note = 2'-deoxy-2'-fluorocytidine
  modified_base 7: mod_base = OTHER; note = 2'-deoxy-2'-fluorocytidine
  modified_base 8: mod_base = cm
  modified_base 9: mod_base = cm
  modified_base 10: mod_base = OTHER; note = 2'-deoxycytidine
  modified_base 11: mod_base = OTHER; note = 2'-deoxyadenosine
  modified_base 12: mod_base = gm
  modified_base 13: mod_base = OTHER; note = 2'-deoxy-2'-fluoroguanosine
  modified_base 14: mod_base = cm
  modified_base 15: mod_base = OTHER; note = 2'-deoxy-2'-fluorocytidine
  modified_base 16: mod_base = cm
  modified_base 17: mod_base = OTHER; note = 2'-deoxy-2'-fluorocytidine
  modified_base 18: mod_base = um
  modified_base 19: mod_base = OTHER; note = 2'-deoxy-2'-fluorocytidine
  modified_base 20: mod_base = cm
  modified_base 21: mod_base = OTHER; note = 2'-O,4'-C-methylene-briged thymidine
  modified_base 22: mod_base = gm
  modified_base 23: mod_base = OTHER; note = 2'-O,4'-C-methylene-briged thymidine
  modified_base 24: mod_base = um
  modified_base 1^2: mod_base = OTHER; note = phosphorotioate bond between nucleosides
  modified_base 2^3: mod_base = OTHER; note = phosphorothioate bond between nucleosides
  modified_base 3^4: mod_base = OTHER; note = phosphorothioate bond between nucleosides
  modified_base 4^5: mod_base = OTHER; note = phosphorothioate bond between nucleosides
  modified_base 5^6: mod_base = OTHER; note = phosphorothioate bond between nucleosides
  modified_base 7^8: mod_base = OTHER; note = phosphorothioate bond between nucleosides
  modified_base 6^7: mod_base = OTHER; note = phosphorothioate bond between nucleosides
  modified_base 8^9: mod_base = OTHER; note = phosphorothioate bond between nucleosides
  modified_base 9^10: mod_base = OTHER; note = phosphorothioate bond between nucleosides
  modified_base 10^11: mod_base = OTHER; note = phosphorothioate bond between nucleosides
  modified_base 11^12: mod_base = OTHER; note = phosphorothioate bond between nucleosides
  modified_base 12^13: mod_base = OTHER; note = phosphorothioate bond between nucleosides
  modified_base 13^14: mod_base = OTHER; note = phosphorothioate bond between nucleosides
  modified_base 14^15: mod_base = OTHER; note = phosphorothioate bond between nucleosides
  modified_base 15^16: mod_base = OTHER; note = phosphorothioate bond between nucleosides
  modified_base 16^17: mod_base = OTHER; note = phosphorothioate bond between nucleosides
  modified_base 17^18: mod_base = OTHER; note = phosphorothioate bond between nucleosides
  modified_base 18^19: mod_base = OTHER; note = phosphorothioate bond between nucleosides
  modified_base 19^20: mod_base = OTHER; note = phosphorothioate bond between nucleosides
  modified_base 20^21: mod_base = OTHER; note = phosphorothioate bond between nucleosides
  modified_base 21^22: mod_base = OTHER; note = phosphorothioate bond between nucleosides
  modified_base 22^23: mod_base = OTHER; note = phosphorothioate bond between nucleosides
  modified_base 23^24: mod_base = OTHER; note = phosphorothioate bond between nucleosides
gagggcccccaggcccctcctgtt

SEQ ID NO: 123 - RNA, 24 nt, synthetic construct
  source 1..24: mol_type = other RNA
  modified_base 1: mod_base = OTHER; note = 2'-O-methyladenosine
  modified_base 2: mod_base = OTHER; note = 2'-O,4'-C-methylene-briged adenosine
  modified_base 3: mod_base = OTHER; note = 2'-O-methyladenosine
  modified_base 4: mod_base = OTHER; note = 2'-O,4'-C-methylene-briged guanosine
  modified_base 5: mod_base = cm
  modified_base 6: mod_base = OTHER; note = 2'-deoxy-2'-fluoroadenosine
  modified_base 7: mod_base = OTHER; note = 2'-deoxy-2'-fluorouridine
  modified_base 8: mod_base = gm
  modified_base 9: mod_base = cm
  modified_base 10: mod_base = OTHER; note = 2'-deoxycytidine
  modified_base 11: mod_base = OTHER; note = 2'-deoxyadenosine
  modified_base 12: mod_base = um
  modified_base 13: mod_base = OTHER; note = 2'-deoxy-2'-fluorocytidine
  modified_base 14: mod_base = OTHER; note = 2'-O-methyladenosine
  modified_base 15: mod_base = OTHER; note = 2'-deoxy-2'-fluorocytidine
  modified_base 16: mod_base = cm
  modified_base 17: mod_base = OTHER; note = 2'-deoxy-2'-fluorouridine
  modified_base 18: mod_base = cm
  modified_base 19: mod_base = OTHER; note = 2'-deoxy-2'-fluorocytidine
  modified_base 20: mod_base = cm
  modified_base 21: mod_base = OTHER; note = 2'-O,4'-C-methylene-briged cytidine
  modified_base 22: mod_base = um
  modified_base 23: mod_base = OTHER; note = 2'-O,4'-C-methylene-briged guanosine
  modified_base 24: mod_base = um
aaagcatgccatcacctcccctgt

SEQ ID NO: 124 - RNA, 24 nt, synthetic construct
  source 1..24: mol_type = other RNA
  modified_base 1: mod_base = gm
  modified_base 2: mod_base = OTHER; note = 2'-O,4'-C-ethylene-briged adenosine
  modified_base 3: mod_base = gm
  modified_base 4: mod_base = OTHER; note = 2'-O,4'-C-ethylene-briged guanosine
  modified_base 5: mod_base = gm
  modified_base 6: mod_base = OTHER; note = 2'-deoxy-2'-fluorocytidine
  modified_base 7: mod_base = OTHER; note = 2'-deoxy-2'-fluorocytidine
  modified_base 8: mod_base = cm
  modified_base 9: mod_base = cm
  modified_base 10: mod_base = OTHER; note = 2'-deoxycytidine
  modified_base 11: mod_base = OTHER; note = 2'-deoxyadenosine
  modified_base 12: mod_base = gm
  modified_base 13: mod_base = OTHER; note = 2'-deoxy-2'-fluoroguanosine
  modified_base 14: mod_base = cm
  modified_base 15: mod_base = OTHER; note = 2'-deoxy-2'-fluorocytidine
  modified_base 16: mod_base = cm
  modified_base 17: mod_base = OTHER; note = 2'-deoxy-2'-fluorocytidine
  modified_base 18: mod_base = um
  modified_base 19: mod_base = OTHER; note = 2'-deoxy-2'-fluorocytidine
  modified_base 20: mod_base = cm
  modified_base 21: mod_base = OTHER; note = 2'-O,4'-C-ethylene-briged thymidine
  modified_base 22: mod_base = gm
  modified_base 23: mod_base = OTHER; note = 2'-O,4'-C-ethylene-briged thymidine
  modified_base 24: mod_base = um
  modified_base 1^2: mod_base = OTHER; note = phosphorotioate bond between nucleosides
  modified_base 2^3: mod_base = OTHER; note = phosphorothioate bond between nucleosides
  modified_base 3^4: mod_base = OTHER; note = phosphorothioate bond between nucleosides
  modified_base 4^5: mod_base = OTHER; note = phosphorothioate bond between nucleosides
  modified_base 5^6: mod_base = OTHER; note = phosphorothioate bond between nucleosides
  modified_base 7^8: mod_base = OTHER; note = phosphorothioate bond between nucleosides
  modified_base 6^7: mod_base = OTHER; note = phosphorothioate bond between nucleosides
  modified_base 8^9: mod_base = OTHER; note = phosphorothioate bond between nucleosides
  modified_base 9^10: mod_base = OTHER; note = phosphorothioate bond between nucleosides
  modified_base 10^11: mod_base = OTHER; note = phosphorothioate bond between nucleosides
  modified_base 11^12: mod_base = OTHER; note = phosphorothioate bond between nucleosides
  modified_base 12^13: mod_base = OTHER; note = phosphorothioate bond between nucleosides
  modified_base 13^14: mod_base = OTHER; note = phosphorothioate bond between nucleosides
  modified_base 14^15: mod_base = OTHER; note = phosphorothioate bond between nucleosides
  modified_base 15^16: mod_base = OTHER; note = phosphorothioate bond between nucleosides
  modified_base 16^17: mod_base = OTHER; note = phosphorothioate bond between nucleosides
  modified_base 17^18: mod_base = OTHER; note = phosphorothioate bond between nucleosides
  modified_base 18^19: mod_base = OTHER; note = phosphorothioate bond between nucleosides
  modified_base 19^20: mod_base = OTHER; note = phosphorothioate bond between nucleosides
  modified_base 20^21: mod_base = OTHER; note = phosphorothioate bond between nucleosides
  modified_base 21^22: mod_base = OTHER; note = phosphorothioate bond between nucleosides
  modified_base 22^23: mod_base = OTHER; note = phosphorothioate bond between nucleosides
  modified_base 23^24: mod_base = OTHER; note = phosphorothioate bond between nucleosides
gagggcccccaggcccctcctgtt

SEQ ID NO: 125 - RNA, 24 nt, synthetic construct
  source 1..24: mol_type = other RNA
  modified_base 1: mod_base = OTHER; note = 2'-O-methyladenosine
  modified_base 2: mod_base = OTHER; note = 2'-O,4'-C-methylene-briged adenosine
  modified_base 3: mod_base = OTHER; note = 2'-O-methyladenosine
  modified_base 4: mod_base = OTHER; note = 2'-O,4'-C-methylene-briged guanosine
  modified_base 5: mod_base = cm
  modified_base 6: mod_base = OTHER; note = 2'-deoxy-2'-fluoroadenosine
  modified_base 7: mod_base = OTHER; note = 2'-deoxy-2'-fluorouridine
  modified_base 8: mod_base = gm
  modified_base 9: mod_base = cm
  modified_base 10: mod_base = OTHER; note = 2'-deoxycytidine
  modified_base 11: mod_base = OTHER; note = 2'-deoxyadenosine
  modified_base 12: mod_base = um
  modified_base 13: mod_base = OTHER; note = 2'-deoxy-2'-fluorocytidine
  modified_base 14: mod_base = OTHER; note = 2'-O-methyladenosine
  modified_base 15: mod_base = OTHER; note = 2'-deoxy-2'-fluorocytidine
  modified_base 16: mod_base = cm
  modified_base 17: mod_base = OTHER; note = 2'-deoxy-2'-fluorouridine
  modified_base 18: mod_base = cm
  modified_base 19: mod_base = OTHER; note = 2'-deoxy-2'-fluorocytidine
  modified_base 20: mod_base = cm
  modified_base 21: mod_base = cm
  modified_base 22: mod_base = um
  modified_base 23: mod_base = OTHER; note = 2'-O,4'-C-methylene-briged guanosine
  modified_base 24: mod_base = um
  modified_base 1^2: mod_base = OTHER; note = phosphorotioate bond between nucleosides
  modified_base 2^3: mod_base = OTHER; note = phosphorothioate bond between nucleosides
  modified_base 3^4: mod_base = OTHER; note = phosphorothioate bond between nucleosides
  modified_base 4^5: mod_base = OTHER; note = phosphorothioate bond between nucleosides
  modified_base 5^6: mod_base = OTHER; note = phosphorothioate bond between nucleosides
  modified_base 7^8: mod_base = OTHER; note = phosphorothioate bond between nucleosides
  modified_base 6^7: mod_base = OTHER; note = phosphorothioate bond between nucleosides
  modified_base 8^9: mod_base = OTHER; note = phosphorothioate bond between nucleosides
  modified_base 9^10: mod_base = OTHER; note = phosphorothioate bond between nucleosides
  modified_base 10^11: mod_base = OTHER; note = phosphorothioate bond between nucleosides
  modified_base 11^12: mod_base = OTHER; note = phosphorothioate bond between nucleosides
  modified_base 12^13: mod_base = OTHER; note = phosphorothioate bond between nucleosides
  modified_base 13^14: mod_base = OTHER; note = phosphorothioate bond between nucleosides
  modified_base 14^15: mod_base = OTHER; note = phosphorothioate bond between nucleosides
  modified_base 15^16: mod_base = OTHER; note = phosphorothioate bond between nucleosides
  modified_base 16^17: mod_base = OTHER; note = phosphorothioate bond between nucleosides
  modified_base 17^18: mod_base = OTHER; note = phosphorothioate bond between nucleosides
  modified_base 18^19: mod_base = OTHER; note = phosphorothioate bond between nucleosides
  modified_base 19^20: mod_base = OTHER; note = phosphorothioate bond between nucleosides
  modified_base 20^21: mod_base = OTHER; note = phosphorothioate bond between nucleosides
  modified_base 21^22: mod_base = OTHER; note = phosphorothioate bond between nucleosides
  modified_base 22^23: mod_base = OTHER; note = phosphorothioate bond between nucleosides
  modified_base 23^24: mod_base = OTHER; note = phosphorothioate bond between nucleosides
aaagcatgccatcacctcccctgt

SEQ ID NO: 126 - RNA, 24 nt, synthetic construct
  source 1..24: mol_type = other RNA
gtcccttctcgtcgatggtcagca

SEQ ID NO: 127 - RNA, 24 nt, synthetic construct
  source 1..24: mol_type = other RNA
gagggcccccaggcccctcctgtt

SEQ ID NO: 128 - RNA, 24 nt, synthetic construct
  source 1..24: mol_type = other RNA
  modified_base 1: mod_base = gm
  modified_base 2: mod_base = OTHER; note = 2'-O,4'-C-ethylene-briged adenosine
  modified_base 3: mod_base = gm
  modified_base 4: mod_base = OTHER; note = 2'-O,4'-C-ethylene-briged guanosine
  modified_base 5: mod_base = gm
  modified_base 6: mod_base = OTHER; note = 2'-deoxy-2'-fluorocytidine
  modified_base 7: mod_base = OTHER; note = 2'-deoxy-2'-fluorocytidine
  modified_base 8: mod_base = cm
  modified_base 9: mod_base = cm
  modified_base 10: mod_base = OTHER; note = 2'-deoxycytidine
  modified_base 11: mod_base = OTHER; note = 2'-deoxyadenosine
  modified_base 12: mod_base = gm
  modified_base 13: mod_base = OTHER; note = 2'-deoxy-2'-fluoroguanosine
  modified_base 14: mod_base = cm
  modified_base 15: mod_base = OTHER; note = 2'-deoxy-2'-fluorocytidine
  modified_base 16: mod_base = cm
  modified_base 17: mod_base = OTHER; note = 2'-deoxy-2'-fluorocytidine
  modified_base 18: mod_base = OTHER; note = 2'-O-methyluridine
  modified_base 19: mod_base = OTHER; note = 2'-deoxy-2'-fluorocytidine
  modified_base 20: mod_base = cm
  modified_base 21: mod_base = OTHER; note = 2'-O,4'-C-ethylene-briged thymidine
  modified_base 22: mod_base = gm
  modified_base 23: mod_base = OTHER; note = 2'-O,4'-C-ethylene-briged guanosine
  modified_base 24: mod_base = um
  modified_base 1^2: mod_base = OTHER; note = phosphorotioate bond between nucleosides
  modified_base 2^3: mod_base = OTHER; note = phosphorothioate bond between nucleosides
  modified_base 3^4: mod_base = OTHER; note = phosphorothioate bond between nucleosides
  modified_base 4^5: mod_base = OTHER; note = phosphorothioate bond between nucleosides
  modified_base 5^6: mod_base = OTHER; note = phosphorothioate bond between nucleosides
  modified_base 7^8: mod_base = OTHER; note = phosphorothioate bond between nucleosides
  modified_base 6^7: mod_base = OTHER; note = phosphorothioate bond between nucleosides
  modified_base 8^9: mod_base = OTHER; note = phosphorothioate bond between nucleosides
  modified_base 9^10: mod_base = OTHER; note = phosphorothioate bond between nucleosides
  modified_base 10^11: mod_base = OTHER; note = phosphorothioate bond between nucleosides
  modified_base 11^12: mod_base = OTHER; note = methoxylethylphosphonate bond between nucleosides
  modified_base 13^14: mod_base = OTHER; note = phosphorothioate bond between nucleosides
  modified_base 14^15: mod_base = OTHER; note = ethylphosphate bond between nucleosides
  modified_base 15^16: mod_base = OTHER; note = phosphorothioate bond between nucleosides
  modified_base 16^17: mod_base = OTHER; note = phosphorothioate bond between nucleosides
  modified_base 17^18: mod_base = OTHER; note = phosphorothioate bond between nucleosides
  modified_base 18^19: mod_base = OTHER; note = phosphorothioate bond between nucleosides
  modified_base 19^20: mod_base = OTHER; note = phosphorothioate bond between nucleosides
  modified_base 20^21: mod_base = OTHER; note = phosphorothioate bond between nucleosides
  modified_base 21^22: mod_base = OTHER; note = phosphorothioate bond between nucleosides
  modified_base 22^23: mod_base = OTHER; note = phosphorothioate bond between nucleosides
  modified_base 23^24: mod_base = OTHER; note = phosphorothioate bond between nucleosides
gagggcccccaggcccctcctgtt

SEQ ID NO: 129 - RNA, 24 nt, synthetic construct
  source 1..24: mol_type = other RNA
  modified_base 1: mod_base = gm
  modified_base 2: mod_base = OTHER; note = 2'-O,4'-C-ethylene-briged adenosine
  modified_base 3: mod_base = gm
  modified_base 4: mod_base = OTHER; note = 2'-O,4'-C-ethylene-briged guanosine
  modified_base 5: mod_base = gm
  modified_base 6: mod_base = OTHER; note = 2'-deoxy-2'-fluorocytidine
  modified_base 7: mod_base = OTHER; note = 2'-deoxy-2'-fluorocytidine
  modified_base 8: mod_base = cm
  modified_base 9: mod_base = cm
  modified_base 10: mod_base = OTHER; note = 2'-deoxycytidine
  modified_base 11: mod_base = OTHER; note = 2'-deoxyadenosine
  modified_base 12: mod_base = gm
  modified_base 13: mod_base = OTHER; note = 2'-deoxy-2'-fluoroguanosine
  modified_base 14: mod_base = cm
  modified_base 15: mod_base = OTHER; note = 2'-deoxy-2'-fluorocytidine
  modified_base 16: mod_base = cm
  modified_base 17: mod_base = OTHER; note = 2'-deoxy-2'-fluorocytidine
  modified_base 18: mod_base = um
  modified_base 19: mod_base = OTHER; note = 2'-deoxy-2'-fluorocytidine
  modified_base 20: mod_base = cm
  modified_base 21: mod_base = OTHER; note = 2'-O,4'-C-ethylene-briged thymidine
  modified_base 22: mod_base = gm
  modified_base 23: mod_base = OTHER; note = 2'-O,4'-C-ethylene-briged thymidine
  modified_base 24: mod_base = um
  modified_base 1^2: mod_base = OTHER; note = phosphorotioate bond between nucleosides
  modified_base 2^3: mod_base = OTHER; note = phosphorothioate bond between nucleosides
  modified_base 3^4: mod_base = OTHER; note = phosphorothioate bond between nucleosides
  modified_base 5^6: mod_base = OTHER; note = phosphorothioate bond between nucleosides
  modified_base 7^8: mod_base = OTHER; note = phosphorothioate bond between nucleosides
  modified_base 6^7: mod_base = OTHER; note = phosphorothioate bond between nucleosides
  modified_base 8^9: mod_base = OTHER; note = phosphorothioate bond between nucleosides
  modified_base 9^10: mod_base = OTHER; note = phosphorothioate bond between nucleosides
  modified_base 10^11: mod_base = OTHER; note = phosphorothioate bond between nucleosides
  modified_base 11^12: mod_base = OTHER; note = methoxyethylphosphate bond between nucleosides
  modified_base 13^14: mod_base = OTHER; note = phosphorothioate bond between nucleosides
  modified_base 14^15: mod_base = OTHER; note = ethylphosphate bond between nucleosides
  modified_base 15^16: mod_base = OTHER; note = phosphorothioate bond between nucleosides
  modified_base 16^17: mod_base = OTHER; note = phosphorothioate bond between nucleosides
  modified_base 17^18: mod_base = OTHER; note = phosphorothioate bond between nucleosides
  modified_base 18^19: mod_base = OTHER; note = phosphorothioate bond between nucleosides
  modified_base 19^20: mod_base = OTHER; note = phosphorothioate bond between nucleosides
  modified_base 20^21: mod_base = OTHER; note = phosphorothioate bond between nucleosides
  modified_base 22^23: mod_base = OTHER; note = phosphorothioate bond between nucleosides
  modified_base 23^24: mod_base = OTHER; note = phosphorothioate bond between nucleosides
gagggcccccaggcccctcctgtt

SEQ ID NO: 130 - RNA, 24 nt, synthetic construct
  source 1..24: mol_type = other RNA
  modified_base 1: mod_base = gm
  modified_base 2: mod_base = OTHER; note = 2'-O,4'-C-ethylene-briged adenosine
  modified_base 3: mod_base = gm
  modified_base 4: mod_base = OTHER; note = 2'-O,4'-C-ethylene-briged guanosine
  modified_base 5: mod_base = gm
  modified_base 6: mod_base = OTHER; note = 2'-deoxy-2'-fluorocytidine
  modified_base 7: mod_base = OTHER; note = 2'-deoxy-2'-fluorocytidine
  modified_base 8: mod_base = cm
  modified_base 9: mod_base = cm
  modified_base 10: mod_base = OTHER; note = 2'-deoxycytidine
  modified_base 11: mod_base = OTHER; note = 2'-deoxyadenosine
  modified_base 12: mod_base = gm
  modified_base 13: mod_base = OTHER; note = 2'-deoxy-2'-fluoroguanosine
  modified_base 14: mod_base = cm
  modified_base 15: mod_base = OTHER; note = 2'-deoxy-2'-fluorocytidine
  modified_base 16: mod_base = cm
  modified_base 17: mod_base = OTHER; note = 2'-deoxy-2'-fluorocytidine
  modified_base 18: mod_base = OTHER; note = 2'-O-methyluridine
  modified_base 19: mod_base = OTHER; note = 2'-deoxy-2'-fluorocytidine
  modified_base 20: mod_base = cm
  modified_base 21: mod_base = um
  modified_base 22: mod_base = gm
  modified_base 23: mod_base = OTHER; note = 2'-O,4'-C-ethylene-briged guanosine
  modified_base 24: mod_base = um
  modified_base 1^2: mod_base = OTHER; note = phosphorotioate bond between nucleosides
  modified_base 2^3: mod_base = OTHER; note = phosphorothioate bond between nucleosides
  modified_base 3^4: mod_base = OTHER; note = phosphorothioate bond between nucleosides
  modified_base 4^5: mod_base = OTHER; note = phosphorothioate bond between nucleosides
  modified_base 5^6: mod_base = OTHER; note = phosphorothioate bond between nucleosides
  modified_base 7^8: mod_base = OTHER; note = phosphorothioate bond between nucleosides
  modified_base 6^7: mod_base = OTHER; note = phosphorothioate bond between nucleosides
  modified_base 8^9: mod_base = OTHER; note = phosphorothioate bond between nucleosides
  modified_base 9^10: mod_base = OTHER; note = phosphorothioate bond between nucleosides
  modified_base 10^11: mod_base = OTHER; note = phosphorothioate bond between nucleosides
  modified_base 11^12: mod_base = OTHER; note = methoxylethylphosphonate bond between nucleosides
  modified_base 13^14: mod_base = OTHER; note = phosphorothioate bond between nucleosides
  modified_base 14^15: mod_base = OTHER; note = ethylphosphate bond between nucleosides
  modified_base 15^16: mod_base = OTHER; note = phosphorothioate bond between nucleosides
  modified_base 16^17: mod_base = OTHER; note = phosphorothioate bond between nucleosides
  modified_base 17^18: mod_base = OTHER; note = phosphorothioate bond between nucleosides
  modified_base 18^19: mod_base = OTHER; note = phosphorothioate bond between nucleosides
  modified_base 19^20: mod_base = OTHER; note = phosphorothioate bond between nucleosides
  modified_base 20^21: mod_base = OTHER; note = phosphorothioate bond between nucleosides
  modified_base 21^22: mod_base = OTHER; note = phosphorothioate bond between nucleosides
  modified_base 22^23: mod_base = OTHER; note = phosphorothioate bond between nucleosides
  modified_base 23^24: mod_base = OTHER; note = phosphorothioate bond between nucleosides
gagggcccccaggcccctcctgtt

SEQ ID NO: 131 - RNA, 24 nt, synthetic construct
  source 1..24: mol_type = other RNA
  modified_base 1: mod_base = gm
  modified_base 2: mod_base = OTHER; note = 2'-O,4'-C-ethylene-briged adenosine
  modified_base 3: mod_base = gm
  modified_base 4: mod_base = OTHER; note = 2'-O,4'-C-ethylene-briged guanosine
  modified_base 5: mod_base = gm
  modified_base 6: mod_base = OTHER; note = 2'-deoxy-2'-fluorocytidine
  modified_base 7: mod_base = OTHER; note = 2'-deoxy-2'-fluorocytidine
  modified_base 8: mod_base = cm
  modified_base 9: mod_base = cm
  modified_base 10: mod_base = OTHER; note = 2'-deoxycytidine
  modified_base 11: mod_base = OTHER; note = 2'-deoxyadenosine
  modified_base 12: mod_base = gm
  modified_base 13: mod_base = OTHER; note = 2'-deoxy-2'-fluoroguanosine
  modified_base 14: mod_base = cm
  modified_base 15: mod_base = OTHER; note = 2'-deoxy-2'-fluorocytidine
  modified_base 16: mod_base = cm
  modified_base 17: mod_base = OTHER; note = 2'-deoxy-2'-fluorocytidine
  modified_base 18: mod_base = um
  modified_base 19: mod_base = OTHER; note = 2'-deoxy-2'-fluorocytidine
  modified_base 20: mod_base = cm
  modified_base 21: mod_base = um
  modified_base 22: mod_base = gm
  modified_base 23: mod_base = OTHER; note = 2'-O,4'-C-ethylene-briged thymidine
  modified_base 24: mod_base = um
  modified_base 1^2: mod_base = OTHER; note = phosphorotioate bond between nucleosides
  modified_base 2^3: mod_base = OTHER; note = phosphorothioate bond between nucleosides
  modified_base 3^4: mod_base = OTHER; note = phosphorothioate bond between nucleosides
  modified_base 4^5: mod_base = OTHER; note = phosphorothioate bond between nucleosides
  modified_base 5^6: mod_base = OTHER; note = phosphorothioate bond between nucleosides
  modified_base 7^8: mod_base = OTHER; note = phosphorothioate bond between nucleosides
  modified_base 6^7: mod_base = OTHER; note = phosphorothioate bond between nucleosides
  modified_base 8^9: mod_base = OTHER; note = phosphorothioate bond between nucleosides
  modified_base 9^10: mod_base = OTHER; note = phosphorothioate bond between nucleosides
  modified_base 10^11: mod_base = OTHER; note = phosphorothioate bond between nucleosides
  modified_base 11^12: mod_base = OTHER; note = methoxyethylphosphate bond between nucleosides
  modified_base 13^14: mod_base = OTHER; note = phosphorothioate bond between nucleosides
  modified_base 14^15: mod_base = OTHER; note = ethylphosphate bond between nucleosides
  modified_base 15^16: mod_base = OTHER; note = phosphorothioate bond between nucleosides
  modified_base 16^17: mod_base = OTHER; note = phosphorothioate bond between nucleosides
  modified_base 17^18: mod_base = OTHER; note = phosphorothioate bond between nucleosides
  modified_base 18^19: mod_base = OTHER; note = phosphorothioate bond between nucleosides
  modified_base 19^20: mod_base = OTHER; note = phosphorothioate bond between nucleosides
  modified_base 21^22: mod_base = OTHER; note = phosphorothioate bond between nucleosides
  modified_base 22^23: mod_base = OTHER; note = phosphorothioate bond between nucleosides
  modified_base 23^24: mod_base = OTHER; note = phosphorothioate bond between nucleosides
gagggcccccaggcccctcctgtt

SEQ ID NO: 132 - RNA, 24 nt, synthetic construct
  source 1..24: mol_type = other RNA
  modified_base 1: mod_base = OTHER; note = 2'-O-methyladenosine
  modified_base 2: mod_base = OTHER; note = 2'-O,4'-C-ethylene-briged adenosine
  modified_base 3: mod_base = OTHER; note = 2'-O-methyladenosine
  modified_base 4: mod_base = OTHER; note = 2'-O,4'-C-ethylene-briged guanosine
  modified_base 5: mod_base = cm
  modified_base 6: mod_base = OTHER; note = 2'-deoxy-2'-fluoroadenosine
  modified_base 7: mod_base = OTHER; note = 2'-deoxy-2'-fluorouridine
  modified_base 8: mod_base = gm
  modified_base 9: mod_base = cm
  modified_base 10: mod_base = OTHER; note = 2'-deoxycytidine
  modified_base 11: mod_base = OTHER; note = 2'-deoxyadenosine
  modified_base 12: mod_base = um
  modified_base 13: mod_base = OTHER; note = 2'-deoxy-2'-fluorocytidine
  modified_base 14: mod_base = OTHER; note = 2'-O-methyladenosine
  modified_base 15: mod_base = OTHER; note = 2'-deoxy-2'-fluorocytidine
  modified_base 16: mod_base = cm
  modified_base 17: mod_base = OTHER; note = 2'-deoxy-2'-fluorouridine
  modified_base 18: mod_base = cm
  modified_base 19: mod_base = OTHER; note = 2'-deoxy-2'-fluorocytidine
  modified_base 20: mod_base = cm
  modified_base 21: mod_base = OTHER; note = 2'-O,4'-C-ethylene-briged cytidine
  modified_base 22: mod_base = um
  modified_base 23: mod_base = OTHER; note = 2'-O,4'-C-ethylene-briged guanosine
  modified_base 24: mod_base = um
  modified_base 1^2: mod_base = OTHER; note = phosphorotioate bond between nucleosides
  modified_base 2^3: mod_base = OTHER; note = phosphorothioate bond between nucleosides
  modified_base 3^4: mod_base = OTHER; note = phosphorothioate bond between nucleosides
  modified_base 4^5: mod_base = OTHER; note = phosphorothioate bond between nucleosides
  modified_base 5^6: mod_base = OTHER; note = phosphorothioate bond between nucleosides
  modified_base 7^8: mod_base = OTHER; note = phosphorothioate bond between nucleosides
  modified_base 6^7: mod_base = OTHER; note = phosphorothioate bond between nucleosides
  modified_base 8^9: mod_base = OTHER; note = phosphorothioate bond between nucleosides
  modified_base 9^10: mod_base = OTHER; note = phosphorothioate bond between nucleosides
  modified_base 10^11: mod_base = OTHER; note = phosphorothioate bond between nucleosides
  modified_base 11^12: mod_base = OTHER; note = ethylphosphate bond between nucleosides
  modified_base 12^13: mod_base = OTHER; note = phosphorothioate bond between nucleosides
  modified_base 14^15: mod_base = OTHER; note = phosphorothioate bond between nucleosides
  modified_base 15^16: mod_base = OTHER; note = phosphorothioate bond between nucleosides
  modified_base 16^17: mod_base = OTHER; note = phosphorothioate bond between nucleosides
  modified_base 17^18: mod_base = OTHER; note = phosphorothioate bond between nucleosides
  modified_base 18^19: mod_base = OTHER; note = phosphorothioate bond between nucleosides
  modified_base 19^20: mod_base = OTHER; note = phosphorothioate bond between nucleosides
  modified_base 20^21: mod_base = OTHER; note = phosphorothioate bond between nucleosides
  modified_base 21^22: mod_base = OTHER; note = phosphorothioate bond between nucleosides
  modified_base 22^23: mod_base = OTHER; note = phosphorothioate bond between nucleosides
  modified_base 23^24: mod_base = OTHER; note = phosphorothioate bond between nucleosides
aaagcatgccatcacctcccctgt